European Patent Specification EP 3 564 380 B1, published June 18, 2025. Title: RECOMBINANT ADENOVIRUSES AND USE THEREOF. Applicant: Beth Israel Deaconess Medical Center, Inc. Washington University. The sequence listing filed with the application follows.

SEQUENCE LISTING (123 sequences)

SEQ ID NO: 1 - DNA, 35079 bp, Simian Adenovirus 4287 (sAd4287) Wild Type
catcatcaataatataccttattctggaaacgtgccaatatgataatgagcggggaggagcgaggcggggccggggtgacgtgcggtgacgcggggtgacgcggggtggcgcgagggcggggcgggagtggggaggcgcttagtttttacgtatgcggaaggaggttttataccggaagttgggtaatttgggcgtatatttgtaagttttgtgtaatttggcgcgaaaaccgggtaatgaggaagttgaggttaatatgtactttttatgactgggcggaatttctgctgatcagcagtgaactttgggcgctgacggggaggtttcgctacgtggcagtaccacgagaaggctcaaaggtcccatttattgtactcctcagcgttttcgctgggtatttaaacgctgtcagatcatcaagaggccactcttgagtgccggcgagtagagttttctcctccgcgctgccgcgatgaggctggttcccgagatgtacggtgttttctgcagcgagacggcccggaactcagatgagctgcttaatacagatctgctggatgttcccaactcgcctgtggcttcgcctccgtcgcttcatgatcttttcgatgtggaagtggatccaccgcaagatcccaacgaggacgcggtaaacagtatgttccctgaatgtctgtttgaggcggctgaggagggttctcacagcagtgaagagagcagacggggagaggaactggacttgaaatgctacgaggaatgtctgccttctagcgattctgaaacggaacagacagggggagacggctgtgagtcggcaatgaaaaatgaacttgtattagactgtccagaacatcctggtcatggctgccgtgcctgtgcttttcatagaaatgccagcggaaatcctgagactctatgtgctctgtgttatctgcgccttaccagcgattttgtatacagtaagtaaagtgttttcattggcgtacggtaggggattcgttgaagtgctttgtgacttattatgtgtcattatttctaggtgacgtgtccgacgtggaaggggaaggagatagatcaggggctgctaattctccttgcactttgggggctgtggttccagctggcattattaaacccgtggcggtcagagtctcaggcagacggtgcgcagttgaaaaaattgaagacttgctgcaggaagaacagacgcaacctttggacctgtccatgaaacgccctaagctgacttaagtgtgtttattgtatgcaataaaagtgttgatctttgaactgtgtttatgtgttgggtgtgtctgtgggtatataagcaggtggatgggaagtgagagcacagctgcttcagatggatctgctaggagacctaagagaatttggcgtggttcggcgcttgttggagttggcctctgacagaacttccaagttttggaggttttgttttggctcaacgcttagcaacgtgctatatagggtcaagaaggagcaggagacgcagtttgctaggctgttggccgatactcctggagtttttgtggctctggatctaggccatcactctcttttccaagagaaaattatcaaaaacctaacttttacgtctcctggccgcacggttgcttccgctgcctttattacctatattttggatcaatggagcaacagcggcagccacctgtcgtgggagtacatgctggattacatgtcgatggcgctgtggagggccatgctgcggaggagggtttgcatttacttgcgggcgcagcctccgcggctgggccgagtggaggaggaggacgagccgggagagatggagaacctgagggccgggctggaccctccaacggaggactaggtgctgaggatgatcctgaagaggggactagtgggggagctaggaaaaagcaaaaaactgagcctgaacctagaaactttttgaatgagttgactgtaagcctgatgaatcggcagcgtcctgagacggtgttttgggctgagttggaggatgagttcaagaagggggaattgaacctcttgtacaagtatgggtttgagcagttgaaaactcactggttggagccgtgggaggacatggaaatggctctagacacctttgctaaagtggctctgcggccggataaagtttacactattcgccgcactgttaatataaaaaagagtgtttatgttatcggtcatggagctctggtgcaggtgcagaccccagaccgggtggctttcaattgcggcatgcagagtttgggccccggggtgataggtttgaatggagttacatttcaaaatgtcaggtttactggtgatgattttaatggctctgtgtttgtgactagcacccagctaaccctccacggtgtttacttttttaactttaacaatacatgtgtggagtcatggggtagggtgtctctgaggggctgcagttttcatggttgctggaaggcggtggtgggaagaattaaaagtgtcatgtctgtgaagaaatgcatatttgaacgctgtgtgatagctctagcagtagaggggtacggacggatcaggaataacgccgcatctgagaatggatgttttcttttgctgaaaggtacggccagcgttaagcataatatgatttgcggcagcggcctgtgcccctcgcagctcttaacttgcgcagatggaaactgtcacaccttgcgcaccgtgcacatagtgtcccactcgcgccgcacctggccaacatttgagcacaatatgctcatgcgttgcgccgttcacctaggtgctagacgcggcgtgtttatgccttatcaatgtaactttagtcatactaagattttgctggaaactgattccttccctcgagtatgtttcaatggggtgtttgacatgtcaatggaactttttaaagtgataagatatgatgaaaccaagtctcgttgtcgctcatgtgaatgcggagctaatcatttgaggttgtatcctgtaaccctgaacgtcaccgaggagctgaggacggaccaccacatgctgtcttgcctgcgtaccgactatgaatccagtgatgaggagtgaggtgaggggcggagccacaaagggtataaaggggcatgaagggtggacgcggtgtttcaaaatgagcgggacgacggacggcaatgcgtttgaggggggagtgttcagcccatatctgacatctcgtcttccttcctgggcaggagtgcgtcagaatgtagtgggctccaccgtggacggacggccggtcgcccctgcaaattccgccaccctcacctatgccaccgtgggatcatcgttggacactgccgcggcagctgccgcttctgctgccgcttctactgctcgcggcatggcggctgattttggactatataaccaactggccactgcagctgtggcgtctcggtctctggttcaagaagatgccctgaatgtgatcttgactcgcctggagatcatgtcacgtcgcctggacgaactggctgcgcagatatcccaagctaaccccgataccgcttcagaatcttaaataaagacaaacaaatttgttgaaaagtaaaatggctttatttgttttttttggctcggtaggctcgggtccacctgtctcggtcgttaaggactttgtgtatgttttccaaaacacggtacagatgggcttggatgttcaagtacatgggcatgaggccatctttggggtggagataggaccactgaagagcgtcatgttccggggtggtattgtaaatcacccagtcgtagcagggtttttgagcgtggaactggaatatgtccttcaggagcaggctaatggccaagggcagccccttagtgtaggtgtttacaaagcggttgagctgggagggatgcatgcggggggagatgatatgcatcttggcttggattttgaggttagctatgttaccacccaggtctctgcgggggttcatgttatgaaggaccaccagcacggtgtagccggtgcacttggggaacttgtcatgcagtttggaggggaaggcgtggaagaatttagatacccccttgtgcccccctaggttttccatgcactcatccataataatggcaatgggacccctggcggccgctttagcaaacacgttttgggggttggaaacatcatagttttgctctagagtgagctcatcataggccatctttacaaagcggggtaggagggtgcccgactgggggatgatagttccatctgggcctggagcgtagttgccctcacagatctgcatctcccaggccttaatttccgagggggggatcatgtccacctggggggcgataaagaacacggtttctggcgggggattgatgagctgggtggaaagcaagttacgcaatagctgggatttgccgcaaccggtggggccgtagatgaccccgatgacgggttgcagctggtagttcagagaggaacagctgccgtcggggcgcaggaggggggccacatcgttcatcatgcttctgacatgtttattttcactcactaagttttgcaagagcctctccccacccagggataagagttcttccaggctgttgaagtgtttcagcggtttcaggccgtcggccatgggcatcttttcaagcgactgacgaagcaagtacagtcggtcccagagctcggtgacgtgctctatggaatctcgatccagcagacttcttggttgcgggggttgggccgactttcgctgtagggcaccagccggtgggcgtccagggccgcgagggttctgtccttccagggtctcagcgttcgggtgagggtggtctcggtgacggtgaagggatgagccccgggctgggcgcttgcgagggtgcgcttcaggctcatcctgctggtgctgaagcgggcgtcgtctccctgtgagtcggccagatagcaacgaagcatgaggtcgtagctgagggactcggccgcgtgtcccttggcgcgcagctttcccttggaaacgtgctgacatttggtgcagtgcagacacttgagggcgtagagttttggggccaggaagaccgactcgggcgagtaggcgtcggctccgcactgagcgcagacggtctcgcactccaccagccacgtgagctcgggtttagcgggatcaaaaaccaagttgcctccattttttttgatgcgtttcttaccttgcgtctccatgagtctgtgtcccgcttccgtgacaaaaaggctgtcggtgtccccgtagaccgacttgagggggcgatcttccaaaggtgttccgaggtcttccgcgtacaggaactgggaccactccgagacaaaggctcgggtccaggctaacacgaaggaggcgatctgcgaggggtatctgtcgttttcaatgagggggtccaccttttccagggtgtgcagacacaggtcgtcctcctccgcgtccacgaaggtgattggcttgtaagtgtaggtcacgtgacccgcacccccccaaggggtataaaagggggcgtgcccactctccccgtcactttcttccgcatcgctgtggaccagagccagctgttcgggtgagtaggccctctcaaaagccggcatgatttcggcgctcaagttgtcagtttctacaaacgaggtggatttgatattcacgtgccccgcggcgatgcttttgatggtggaggggtccatctgatcagaaaacacgatctttttattgtcaagtttggtggcgaaagacccgtagagggcgttggaaagcaacttggcgatggagcgcagggtctgatttttctcccgatcggccctctccttggcagcgatgttgagttgcacgtactcgcgagccacgcaccgccactcggggaacacggcggtgcgctcgtcgggcaggatgcgcacgtgccagccgcggttgtgcagggtgatgaggtccacgctggtggccacctccccgcggaggggctcgttggtccaacacaatcgccccccttttctggagcagaacggaggcaggggatctagcaagttggcgggcggggggtcggcgtcgatggtaaatatgccgggtagcagaattttattaaaataatcgatttcggtgtccgtgtcttgcaacgcgtcttcccacttcttcaccgccagggccctttcgtagggattcaggggcggtccccagggcatggggtgggtcagggccgaggcgtacatgccgcagatgtcgtacacgtacaggggctccctcaacaccccgatgtaagtggggtaacagcgccccccgcggatgctggctcgcacgtagtcgtacatctcgtgagagggagccatgagcccgtctcccaagtgggtcttgtggggtttctcggcccggtagaggatctgcctgaagatggcgtgggagttggaagagatggtggggcgttggaagacattaaagttggctccgggcagtcccacggagtcttggatgaactgggcgtaggattcccggagcttgtccaccagggctgcggttaccagcacgtcgagagcgcagtagtccaacgtctcgcggaccaggttgtaggccgtctcttgttttttctcccacagttcgcgattgaggaggtattcctcgcggtctttccagtactcttcggcgggaaatcctttttcgtccgctcggtaagaacctaacatgtaaaattcgttcacggctttgtatggacaacagcctttttctaccggcagggcgtacgcttgagcggcctttctgagagaggtgtgggtgagggcgaaggtgtcccgcaccatcactttcaggtactgatgtttgaagtccgtgtcgtcgcaggcaccctgttcccacagcgtgaagtcggtgcgctttttctgcctgggattggggagggcgaatgtgacgtcgttaaaaaggattttcccggagcggggcatgaagttgcgagagatcctgaagggtccgggcacgtccgagcggttgttgatgacttgtgccgccaggacgatctcgtcgaagccgttgatgttgtggcccacgatgtaaagttcgataaagcgcggctgtcccttgagggccggcgcttttttcaactcctcgtaggtgagacagtccggcgaggagagacccagctccgcccgggcccagtcggagagctgagggttagccgcgaggaaagagctccataggtcaagggctagcagagtttgcaagcggtcgcggaactcgcgaaactttttccccacggccattttctccggcgtcaccacgtagaaagtgcaggggcggtcgttccagacgtcccatcggagctctagggccagctcgcaggcttggcgaacgagggtctcctcgcccgagacgtgcatgaccagcatgaagggtaccaactgtttcccgaacgagcccatccatgtgtaggtttctacgtcgtaggtgacaaagagccgctgggcgcgcgcgtgggagccgatcgggaagaagctgatctcctgccaccagttggaggaatgggtgttgatgtggtgaaagtagaagtcccgccggcgcacagagcattcgtgctgatgtttgtaaaagcgaccgcagtagtcgcagcgctgcacgctctgtatctcctgaatgagatgcgcttttcgcccgcgcaccagaaaccggagggggaagttgagacggggggcttgtggggcggcatcccattcgccttggcggtgggagtctgcgtctgcgtcctccttctctgggtggacgacggtggggacgacaacgccccgggtgccgcaagtccagatctccgccacggaggggcgcaggcgctgcaggaggggacgcagctgcccgctgtccagggagtcgagggcggccgcgctgaggtcggcgggaagcgtttgcaagttcactttcagaagaccggtaagagcgtgagccaggtgcagatggtacttgatttccaggggggtgttggaagaggcgtccacggcgtagaggaggccgtgtccgcgcggggccaccaccgtgccccgaggaggttttatctcaatcgtcgagggcgagcgccggggggtagaggcggctctgcgccggggggcagcggaggcagcggcacgttttcgtgaggatttggcagcggttgatgacgagcccggagactgctggcgtgggcgacgacgcggcggttgaggtcctggatgtgccgtctctgcgtgaagaccaccggcccccgggtcctgaacctgaaagagagttccacagaatcaatgtctgcatcgttaacggcggcctgcctgaggatctcctgtacgtcgcccgagttgtcttgataggcgatctcggccatgaactgctccacttcttcctcgcggaggtcgccgtggcccgctcgctccacggtggcggccaggtcgttggagatgcgacgcatgagttgagagaaggcgttgaggccgttctcgttccacacgcggctgtacaccacgttgccgaaggagtcgcgcgctcgcatgaccacctgggccacgttgagttccacgtggcgggcgaagacggcgtagtttctgaggcgctggaagaggtagttgagcgtggtggcgatgtgctcgcagacgaagaagtacatgatccagcgccgcagggtcatctcgttgatgtctccgatggcttcgagacgctccatggcctcgtagaagtcgacggcgaagttgaaaaattgggagttgcgggcggccaccgtgagttcttcttgcaggaggcggatgagatcggcgaccgtgtcgcgcacctcctgctcgaaagcgccccgaggcgcctctgcttcttcctccggctcctcctcttccaggggcacgggttcctccggcagctctgcgacggggacggggcggcgacgtcgtcgtctgaccggcaggcggtccacgaagcgctcgatcatttcgccgcgccggcgacgcatggtctcggtgacggcgcgtccgttttcgcgaggtcgcagttcgaagacgccgccgcgcagagcgcccccgtgcagggagggtaagtggttagggccgtcgggcagggacacggcgctgacgatgcattttatcaattgctgcgtaggcactccgtgcagggatctgagaacgtcgaggtcgacgggatccgagaacttctctaagaaagcgtctatccaatcgcagtcgcaaggtaagctgaggacagtgggtcgctggggggcgtccgcgggcagttgggaggtgatgctgctgatgatgtaattaaagtaggcggtcttcaggcggcggatggtggcgaggaggaccacgtctttgggcccggcctgttgaatgcgcaggcgctcggccatgccccaggcctcgctctgacagcgacgcaggtctttgtagtagtcttgcatcagtctctccaccggaacctctgcttctcccctgtctgccatgcgagtcgagccgaacccccgcaggggctgcagcaacgctaggtcggccacgaccctttcggccagcacggcctgttgaatctgcgtgagggtggtctggaagtcgtccaggtccacgaagcggtgataggcccccgtgttgatggtgtaggtgcagttggccatgacggaccagttgacgacttgcataccgggttgggtgatctccgtgtacttgaggcgcgagtaggcgcgggactcgaacacgtagtcgttgcatgtgcgcaccagatactggtagccgaccaggaagtgaggaggcggctctcggtacaggggccagccgacggtggcgggggcgccgggggacaggtcgtccagcatgaggcgatggtagtggtagatgtagcgggagagccaggtgatgccggccgaggtggtcgcggccctggtgaattcccggacgcggttccagatgttgcgcaggggacggaagcgttccatggtgggcacgctctgccccgtgaggcgggcgcagtcctgtacgctctagatggaaaaaagacagggcggtcatcgactcccttccgtagcttggggggtaaagtcgcaagggtgcggcggcggggaaccccggttcgagaccggccggatccgccgctcccgatgcgcctggccccgcatccacgacgtccgcgccgagacccagccgcgacgctctgccccaatacggaggggagtcttttggtgttttttcgtagatgcatccggtgctgcggcagatgcgacctcagacgcccaccaccaccgccgcggcggcagtaaacctgagcggaggcggtgacagggaggtggaggagctggctttagacctggaagagggagaggggctggcccggctgggagcgccgtccccagagagacaccctagggttcagctcgtgagggacgccaggcaggcttttgtgccgaagcagaacctgtttagggaccgcagcggtcaggaggcggaggagatgcgcgattgcaggtttcgggcgggtagagagctgagggcgggcttcgatcgcgagcggctcctgagggcggaggatttcgagcccgacgagcgttctggggtgagcccggcccgcgctcacgtctcggcggccaacctggtgagcgcgtacgagcagacggtgaacgaggagcgcaacttccaaaagagctttaacaatcacgtgaggaccctgatcgcgagggaggaggtgaccatcgggctgatgcatctgtgggacttcgtggaggcctacgtgcagaacccggccagcaaacctctgacggcccagctgttcctgatcgtgcagcacagccgcgacaacgagacgttccgcgacgccatgttgaacatcgcggagcccgagggtcgctggctcttggatctgattaacatcctgcagagcatcgtggtgcaggagaggggtctgagtttagcggacaaggtggcggccattaactattcgatgcagagcctggggaagttctacgctcgcaagatctacaagagcccttacgtgcccatagacaaggaggtgaagatagacagcttttacatgcgcatggcgctaaaggtgctgacgctgagcgacgacctcggcgtgtaccgtaacgacaagatccacaaggcggtgagcgccagccgccggcgggagctgagcgacagggagctgatgcacagcctgcagagggcgctggcgggcgccggggacgaggagcgtgaggcttactttgacatgggagccgatctgcagtggcgtcccagcgcgcgcgccttggaggcggcgggttatcccgacgaggaggatcgggacgatttggaggaggcaggcgagtacgaggacgaagcctgaccgggcaggtgttgttttagatgcagcggccggcggacggggccaccgcggatcccgcacttttggcatccatgcagagtcaaccttcgggcgtgaccgcctccgatgactgggcggcggccatggaccgcatcatggcgctgaccacccgcaaccccgaggcttttaggcagcaaccccaggccaaccgtttttcggccatcttggaagcggtggtgccctcccgcaccaaccccacacacgagaaagtcctgactatcgtgaacgccctggtagacagcaaggccatccgccgcgacgaggcgggcttgatttacaacgctctgctggaacgggtggcgcgctacaacagcactaacgttcagaccaatctggatcgcctcaccaccgacgtgaaggaggcgctggctcagaaggagcggtttctgagggacagcaatctgggctctctggtggcactcaacgccttcctgagcacgcagccggccaacgtgccccgcgggcaggaggactacgtgagcttcatcagcgctctgaggctgctggtgtccgaggtgccccagagcgaggtgtatcagtctgggccggattacttcttccagacgtcccgacagggcttgcaaacggtgaacctgactcaggcctttaaaaacttgcaaggcatgtggggcgttaaggccccggtgggcgatcgagccaccatctccagtctgctgacccccaacactcgcctgctgctgctcttgatcgcgccgttcaccaacagtagcactatcagccgtgactcgtacctgggtcatctcatcactttgtaccgcgaggccatcggtcaggctcagattgacgagcatacatatcaggagatcactaacgtgagccgggccctgggtcaggaagataccggcagcctggaagccacgttgaactttttgctaaccaaccggaggcaaaaaataccctcccagtttacgttaagcgccgaggaggagaggattctgcgatacgtgcagcagtccgtgagtctgtacttgatgcgggagggcgccaccgcttccacggctttagacatgacggctcggaacatggaaccgtccttttactccgcccaccggccgttcattaaccgtctgatggactacttccatcgcgcggccgccatgaacggggagtattttaccaatgccatcctgaatccgcattggatgcccccgtccggcttctacaccggcgagtttgacctgcccgaagccgacgacggctttctttgggacgacgtgtccgacagcattttcacgccgggcaatcgccgattccagaagaaggagggcggagacgagctccccctctccagcgtggaggcggcctctaggggagagagtccctttcccagtctgtcttccgccagcagtggtcgggtaacgcgcccgcggttgccgggggagagcgactacctgaacgaccccttgctgcggccggctaggaagaaaaatttccccaacaacggggtggaaagcttggtggataaaatgaatcgttggaagacctacgcccaggagcagcgggagtgggaggacagtcagccgcgaccgctggttccgccgcactggcgtcgtcagagagaagacccggacgactccgcagacgatagtagcgtgttggacctgggagggagcggagccaacccctttgctcacttgcaacccaaggggcgttcgagccgcctctactaataaaaaagaagcggaaacttaccagagccatggccacagcgtgtgtgctttcttcctctctttcttcctcggcgcggcagaatgagaagagcggtgagagtcacgccggcggcgtatgagggtccgcccccttcttacgaaagcgtgatgggatcagcgaacgtgccggccacgctggaggcgccttacgttcctcccagatacctgggacctacggagggcagaaacagcatccgttactccgagctggcacccctgtacgataccaccaaggtgtacctggtggacaacaagtcggcggacatcgcctccctgaattatcaaaacgatcacagcaactttctgactaccgtggtgcagaacaatgacttcaccccgacggaggcgggcacgcagaccattaactttgacgagcgttcccgctggggcggtcagctgaaaaccatcctgcacaccaacatgcccaacatcaacgagttcatgtccaccaacaagttcagggctaagctgatggtagaaaaaagtaatgcggaaactcggcagccccgatacgagtggttcgagtttaccattccagagggcaactattccgaaactatgactatcgatctcatgaataacgcgatcgtggacaattacctgcaagtggggagacagaacggggtgctggaaagcgatatcggcgtgaaattcgataccagaaacttccgactggggtgggatcccgtgaccaagctggtgatgccaggcgtgtacaccaacgaggcttttcaccccgacatcgtgctgctgccggggtgcggtgtggacttcactcagagccgtttgagtaacctgttaggaattagaaagcgccgccccttccaagagggctttcaaatcatgtatgaggacctggagggaggtaatatacccgccttactggacgtgtcgaagtacgaagctagcatacaacgcgccaaagcggagggtagagagattcggggagacacctttgcggtagctccccaggacctggaaatagtgcctttaactaaagacagcaaagacagaagctacaatattataaacaacacgacggacaccctgtatcggagctggtttctggcttacaactacggagaccccgagaaaggagtgagatcatggaccatactcaccaccacggacgtgacctgtggctcgcagcaagtgtactggtccctgccggatatgatgcaagacccggtcaccttccgcccctccacccaagtcagcaacttcccggtggtgggcaccgagctgctgcccgtccatgccaagagcttctacaacgagcaggccgtctactcgcaacttattcgccagtccaccgcgcttacccacgtgttcaatcgctttcccgagaaccagattctggtgcgccctcccgctcctaccattaccaccgtcagtgaaaacgttcccgccctcacagatcacggaaccctgccgctgcgcagcagtatcagtggagttcagcgcgtgaccatcaccgacgccagacgtcgaacctgcccctacgtttacaaagcgcttggcgtggtggctcctaaagttctttctagtcgcaccttctaaaaacatgtccatcctcatctctcccgataacaacaccggctggggactgggctccggcaagatgtacggcggagccaaaaggcgctccagtcagcacccagttcgagttcggggccacttccgcgctccttggggagcttacaagcgaggactctcgggtcgaacggctgtagacgataccatagatgccgtgattgccgacgcccgccggtacaaccccggaccggtcgctagcgccgcctccaccgtggattccgtgatcgacagcgtggtagccggcgctcgggcctatgctcgccgcaagaggcggctgcatcggagacgtcgccccaccgccgccatgctggcagccagagccgtgctgagacgggcccggagggtaggcaggagggctatgcgccgcgctgccgccaacgccgccgccgggagggcccgccgacaggctgcccgccaggctgctgccgccatcgctagcatggccagacccaggagagggaacgtgtactgggtgcgcgattctgtgacgggagtccgagtgccggtgcgcagccgacctccccgaagttagaagatccaagctgcgaagacggcggtactgagtctccctgttgttatcagcccaacatgagcaagcgcaagtttaaagaagaactgctgcagacgctggtgcctgagatctatggccctccggacgtgaagcctgacattaagccccgcgatatcaagcgtgttaaaaagcgggaaaagaaagaggaactcgcggtggtagacgatggcggagtggaatttattaggagtttcgccccgcggcgcagggttcaatggaaagggcgacgggtacaacgcgttttgaggccgggcaccgcggtagtttttaccccgggagagcggtcggccgttaggggttttaaaaggcagtacgacgaggtgtacggcgacgaggacatattggaacaggcggctcaacagatcggagaatttgcctatggaaagcgctcgcgtcgcgaagacctggccatcgccttagacagcggcaaccccacgcccagcctcaaacccgtgacgctgcagcaggtgcttcccgtgagcgccagcacggacagcaagaggggaataaaaagagaaatggaagatctgcagcctaccatccagctcatggttcctaaacggcagaggctggaagaggtcctggagaagatgaaagtggaccccagcatagagccggacgttaaagtcaggccgatcaaagaagtggcccctggactcggggtgcagacggtggatatccagatccccgtcacgtcagcttcgaccgccgtggaagccatggaaacgcaaaccgaaacccccgccgtggttggtaccaaagaagtggcgttgcaaaccgacccctggtacgaatttgccgccccccggcgtcagaggcgacccgctcgttacggccccgccaacgccatcatgccagaatatgcgctgcatccgtctatcctgcccacccccggctaccggggagtgacgtatcgcccgtcaggaacccgccgccgaacccgtcgccgccgccgctcccgtcgcgctctggcccccgtgtcggtgcgccgcgtaacacgccggggaaagacagtcaccattcccaacccgcgctaccaccctagcatcctttaatgactctgccgttttgcagatggctctgacttgccgcgtgcgccttcccgttccgcactatcgaggaagatctcgtcgtaggagaggcatggcgggcagtggtcgccggcgggctttgcgcaggcgcatgaaaggcggaattttacccgctttgatacccataatcgccgccgccatcggtgccatacccggcgtcgcttcagtggccttgcaagcagctcgtaataaataaacgaaggcttttgcacttatgtcctggtcctgactattttatgcagaaagagcatggaagacatcaattttacgtcgctggctccgcggcacggctcgcggccgctcatgggcacctggaacgacatcggcaccagtcagctcaacgggggcgctttcaattgggggagcctttggagcggcattaaaaactttggctccacgattaaatcctacggcagcaaagcctggaacagtagtgctggtcagatgctccgagataaactgaaggacaccaacttccaagaaaaagtggtcaatggggtggtgaccggcatccacggtgcggtagatctcgccaaccaagcggtgcagaaagagattgacaggcgtttggaaaactcgcgggtgccgccgcagaggggggatgaggtggaggtcgaggaagtagaagtagaggaaaagctgcccccgctggagaaagttcccggtgcacctccgaggccgcagaagcggcccaggccagaactagaagaaactctggtgacggagagcaaggagcctccctcgtacgagcaagccttgaaagagggcgcctctccaccctcctacccgatgactaagccgatcgcacccatggctcgaccggtgtacggcaaggattacaagcccgtcacgctagagctgcccccaccgcccccttcgcgtccgacggtgcctccgctgcctgccccgtcggcgggtcccgagtctgcaccatccgctgtgcctctgccagccgcccgtcccgtggccgtggccactgccaggaaccccagaggccagagaggagccaactggcaaagcacgctgaacagcatcgtgggcctgggggtgaaaagcctgaaacgccgccgttgctattattaaaaagtgtagctaaaaaatttcccgttgtatacgcctcctatgttaccgccagagacgcgtgactgtcgccgcgagcgccgcttccaagatggccaccccatcgatgatgccgcagtggtcttacatgcacatcgccggccaggacgcctcggagtacctgagtcccggcctcgtgcagtttgcccgcgccaccgacacctacttcagcttgggaaacaagtttagaaaccccaccgtggcccccacccacgatgtgaccacggaccgctcgcagaggctgaccctgcgctttgtgcccgtagaccgggaggacaccgcgtactcttacaaagtgcgctacacgctggccgtaggggacaaccgagtgctggacatggccagcacctactttgacatccggggggtgctggatcggggtcccagcttcaagccctactccggcaccgcttacaactccctggctcccaagggcgcccccaatcctgcagaatgggccgataccaacgacagcaacaaactgaaagtgaggggtcaggcgccttttgtcagtacttacggttctgctacggcgcttacaaaagatgggatacaggtgggagtggatacttccgaagcatctcaggctgtttatgccgacagaagttaccagccagaaccccaaattggagagacagagtggaacagcgaagtgggtaatgacgacagagtggcgggaagggtgctaaagaaaacaactcccatgttcccttgttacggttcatatgccaagcccaccaacgaaaaaggcggacaagcaatacagcccaccgccggcaacggcgataatcaggctgtagagttacaattctttgccactactagcactcccactgcgccaaaggcagtattgtacgcggaggacgtggccattgaagctccagatactcacttagtgtttaagccaacagtagtcgcgggaactacaagttcggaagctctgctaacccaacaagccgcacctaaccgcccaaactacattgcctttagagataactttattggtctcatgtactacaattcaaccgggaatatgggagtactggccggacaagcatctcagctcaatgcagtggttgatcttcaggacagaaacaccgaactgtcatatcagctaatgctggatgctctgggagatcgcagtcggtacttttctatgtggaatcaagctgtagatagctatgatccagatgtaagaattgtagaaaaccacggtgtggaagacgaactgcctaattattgcttcccactaggcgggatggtagtaacggacacttacaaagccataaaggtaaatggaagcggatggacggctaatactgacgttttcagcgagagagtagaaataggctcaggtaacctgtttgccatggaaattaacttgcaagctaatctgtggcgcagtttcttgtattccaacataggactgtacctcccggactctttaaaattaacccctgacaacatcacgctccctgagaacaaaaatacctaccagtatatgaacggtcgcgtaacaccacccgggctcgtggacacctacgttaacgtgggtgcgcgctggtcccccgatgttatggacagcattaacccttttaaccaccaccgcaacgccgggctccgctaccgttccatgctcctgggaaacggacgctacgtacccttccacattcaggtgccccagaaattctttgcaattaaaaacctgctgctgctccccggttcctatacctacgagtggaatttccgcaaggacgtgaacatgattttgcaaagctcgctgggtaacgacctgcgagttgacggggccagcatacgcttcgacagcatcaacctgtatgctaactttttccccatggcccacaacacggcctccaccctggaagccatgctgcgcaacgacaccaatgaccagtccttcaacgactacctgtgcgcggccaacatgctgtatcccatccccgccaacgccaccagcgtgcccatctccatcccgtctcgcaactgggccgcctttaggggttggagtttcacccgcctcaaaaccaaggaaaccccctcgctgggctctggcttcgacccctacttcgtctactcaggctccattccctacctggacggcactttctatcttaaccacactttcaaaaaggtgtctatcatgttcgattcctcggtcagctggcccggcaacgaccgcctgctgacgcccaacgagttcgaaatcaagcgttcggtggacggtgaagggtacaacgtggcccagagcaacatgaccaaggactggttcctggttcaaatgctcagccattacaacatcggttaccagggcttctatgtgcccgagaactacaaggaccgcatgtactccttctttaggaacttccaacccatgagtcgccaagtcgtggactcagtggcttacagggactactaccaggacgttaagctcccctaccagcacaacaactcagggttcgtgggctacatgggtcccaccatgcgagaggggcaggcctacccggccaactatccttatcccctaatcggagagactgctgtacccagcctgacgcagaaaaagttcctctgcgaccgggtgatgtggaggatacccttctctagcaacttcatgtctatgggctccctcaccgacctggggcagaacatgctgtacgccaactccgctcacgccttggacatgacctttgaggtggatcccatggatgagcccacgcttctctatgttctgtttgaagtcttcgacgtggtgcgcatccaccagccgcaccgcggcgtcatcgaggccgtctacctgcgcacacctttctctgccggtaacgccaccacctaaagaagccgatgggctccagcgaacaggagctgcaggccattgttcgcgacctgggctgcgggccctactttttgggcaccttcgacaagcggttccccggcttcatgtcccctcacaagccggcctgtgccatcgttaacacggccggacgggaaaccgggggggtccactggctcgccttcgcctggaacccgcgtaaccgcacctgctacctgttcgacccttttggtttctccgacgaaaggctgaagcagatctaccagttcgagtacgaggggctcctccagcgcagcgctctggcctccacgcccgaccactgcgtcaccctggaaaagtccacccagacggtccaggggcccctctcggccgcctgcgggctcttctgttgcatgtttttgcacgccttcgtgcactggcctcacacccccatggatcacaaccccaccatggatctgctcaccggagtgcccaacagcatgcttcacagcccccaggtcgcccccaccctgcgccgtaaccaggaacacctgtatcgctttctggggaaacactctgcctatttccgccgccatcggcagcgcatcgaacaggccacggccttcgaaagcatgagccaaagagtgtaatcaataaaaaccatttttatttgacatgatacgcgcttctggcgtttttattaaaaatcgaagggttcgagggaggggtcctcgtgcccgctggggagggacacgttgcgatactggaatcgggcgctccaacgaaactcggggatcaccagtcgcggcaggggcacgtcttccaggttctgcttccaaaactgtcgcaccagctgcagggctcccatcacgtcgggcgccgatatcttgaagtcgcagttagggccggagctcccgcggctgttccggaacacggggttggcacactggaacaccatcacgctggggttgtgaatactagccagggccgtcggatcggtcacctccgacgcatccagatcctcggcgttgctcagggcgaacggggtcagcttgcacatctgccgcccgatctggggcaccaggtcgggtttgttgaggcaatcgcagcgcagagggatcaggatgcgtcgctgcccgcgttgcatgatagggtaactcgccgccaggaactcctccatctgacggaaggccatctgggccttaacgccctcggtgaaaaacagcccacaggacttgctagaaaatacgttattgccgcagttaatgtcttccgcgcagcagcgtgcatcttcgttcttcagctgaaccacgttacgcccccagcggttctggaccaccttggctttcgtaggatgctccttcagcgcccgctgcccgttctcgctggtcacatccatttccaccacgtgctccttgcagaccatctccactccgtggaagcaaaacaggacgccctcctgccgggtattgcgatgctcccaaacggcacacccggtgggctcccagctcttgtgttttacccccgcgtaggcttccatgtaagccatgaggaatctgcccatcagctcggtgaaggtcttctgattggtgaaggttagcggcaggccgcggtgctcctcgttcaaccaagtttgacagatcttgcggtacaccgttccctggtcgggcagaaacttaaaagccgctctgctgtcgttgtccacgtggaacttctccattaacatcatcatggtttccatacccttctcccacgctgacaccagcggtttgctgtcggggttcttcaccaacacggcggtagaggggccctcgccggccccgacgtccttcatggtcattctttgaaactccacggagccgtccgcgcgacgtactctgcgcaccggagggtagctgaagcccacctccaccacggtgccttcgccctcgctgtcggaaacgatctccggggatggcggcggtgcgggtgtcgccttgcgagccttcttcttgggagggagctgaggcgcctcctgctcgcgctcggggctcatctcccgcaagtagggggttatggagctgcctgcttggttctgacggttggccattgtatcctaggcagaaagacatggagcttatgcgcgaggaaactttaaccgccccgtcccccgtcagcgacgaagatgtcatcgtcgaacaggacccgggctacgttacgccgcccgaggatctggaggggcctgaccggcgcgacgctagtgagcggcaggaaaatgagaaagaggaggcctgctacctcctggaaggcgacgttttgctaaagcatttcgccaggcagagcaccatagttaaggaggccttgcaagaccgctccgaggtgcccttggacgtcgccgcgctctcccaggcctacgaggcgaaccttttctcgcctcgagtgcctccgaagagacagcccaacggcacctgcgagcccaacccgcgactcaacttctaccccgtgttcgccgtaccagaggcgctggccacctatcacatttttttcaaaaaccaacgcatccccctatcgtgccgggccaaccgcaccgcggccgataggaatctcaggcttaaaaacggagccaacatacctgatatcacgtcgctggaggaagtgcccaagattttcgagggtctgggtcgagatgagaagcgggcggcgaacgctctgcagaaagaacagaaagagagtcagaacgtgctggtggagctggagggggacaacgcgcgtctggccgtcctcaaacgctgcatagaagtctcccacttcgcctaccccgccctcaacttgccacccaaagttatgaaatcggtcatggatcagctgctcatcaagagagctgagcccctggatcccgaccaccccgaggcggaaaactcagaggacggaaagcccgtcgtcagcgacgaggagctcgagcggtggctggaaaccagggacccccaacagttgcaagagaggcgcaagatgatgatggcggccgtgctggtcaccgtggagctggaatgcctgcaacggtttttcagcgacgtggagacgctacgcaaaatcggggaatccctgcactacaccttccgccagggctacgtccgccaggcctgcaagatctccaacgtggagctcagcaacctggtctcctacatgggcatcctccacgagaaccggctggggcagagcgtgctgcactgcaccttgcaaggcgaggcgcggcgggactacgtgcgagactgcatctacctcttcctcaccctcacctggcagaccgccatgggcgtctggcagcagtgcttggaagagagaaacctcaaagagctagacaaactcctctgccgccagcggcgcgccctgtggtccggtttcagcgagcgcacggtcgccagcgctctggcggacatcatcttcccggagcgcctgatgaaaaccttgcaaaacggcctgccggatttcatcagtcaaagcattttgcaaaacttccgctcttttgtcctggaacgctccgggatcttgcccgccatgagctgcgcgctaccttctgactttgtccccctctcctaccgcgagtgccctcccccactgtggagccactgctacctcttccaactggccaactttctggcctaccactccgacctcatggaagacgtaagcggagagggtttactggagtgccactgccgctgcaacctgtgcaccccccacagatcgctggcctgcaacaccgagctactcagcgaaacccaggtcataggtaccttcgagatccaggggccccagcagcaagagggtgcttccggcttgaagctcactccggcgctgtggacctcggcttacttacgcaaatttgtagccgaggactaccacgcccacaaaattcagttttacgaagaccaatctcaaccaccgaaagcccccctcacggcctgcgtcatcacccagagcaagatcctggcccaattgcaatccatcaaccaagcgcgccgcgatttccttttgaaaaagggtcggggggtgtatctggacccccagaccggcgaggaactcaacccgtccacactctccgtcgaagcagcccccccgagacatgccgcccaagggaaccgccaagcagctgatcgctcggcagagagcgaagaagcaagagctgctccagcagcaggtggaggacgaggaagagatgtgggacagccaggcagaggaggtgtcagaggacgaggaggagatggaaagctgggacagcctagacgaggaggaggacgagctttcagaggaagaggcgaccgaagaaaaaccacctgcatccagcgcgccttctctgagccgacagccgaagccccggcccccgacgcccccggccggctcactcaaagccagccgtaggtgggacgccaccgaatctccagcggcagcggcaacggcagcgggtaaggccaaacgcgagcggcgggggtattgctcctggcgggcccacaaaagcagtattgtgaactgcttgcaacactgcgggggaaacatctcctttgcccgacgctacctcctcttccatcacggtgtggccttccctcgcaacgttctctattattaccgtcatctctacagcccctacgaaacgctcggagaaaaaagctaaggcctcctccgccgcgaggaaaaactccgccgccgctgccgccgccaaggatccaccggccaccgaggagctgagaaagcgcatctttcccactctgtatgctatctttcagcaaagccgcgggcagcaccctcagcgcgaactgaaaataaaaaaccgctccttccgctcgctcacccgcagctgtctgtaccacaagagagaagaccagctgcagcgcaccctggacgacgccgaagcactgttcagcaaatactgctcagcgtctcttaaagactaaaagacccgcgctttttccccctcggccgccaaaacccacgtcatcgccagcatgagcaaggagattcccaccccctacatgtggagctatcagccccagatgggcctggccgcgggggccgcccaggactactccagcaagatgaactggctcagcgccggcccccacatgatctcacgagttaacggcatccgagcccaccgaaaccagattctcttagaacaggcggcaatcaccgccacaccccggcgccaactcaacccgcctagttggcccgccgcccaggtgtatcaggaaaatccccgcccgaccacagtcctcctgccacgcgacgcggaggccgaagtcctcatgactaactctggggtacaattagcgggcgggtccaggtacgccaggtacagaggtcgggccgctccttactctcccgggagtataaagagggtgatcattcgaggccgaggtatccagctcaacgacgagacggtgagctcctcaaccggtctcagacctgacggagtcttccagctcggaggagcgggccgctcttccttcaccactcgccaggcctacctgaccctgcagagctcttcctcgcagccgcgctccgggggaatcggcactctccagttcgtggaagagttcgttccctccgtctacttcaaccccttctccggctcgcctggacgctacccggacgccttcattcccaactttgacgcagtgagtgaatccgtggacggctacgactgatgacagatggtgcggccgtgagagctcggctgcgacatctgcatcactgccgtcagcctcgctgctacgctcgggaggcgatcgtcttcagctactttgagctgccggacgagcaccctcagggtccggctcacgggttgaaactcgagatcgagaacgcgctcgagtctcgcctcatcgacaccttcaccgcccgacctctcctggtagaaatcgaacgcgggatcactaccatcaccctgttctgcatctgccccacgcccggattacatgaagatctgtgctgtcatctttgcgctcagtttaataaaaactgaactttttgccgcaccttcaacgccacgcgtcgtttctccaaaagttgtcgacagctcttcagtcagaggtatacgagaaactgtttatttttacaactctactacttttctcacccttaactgctcctgcactaacgaactaattcagtggttcgcgaacggctcactctgccaagtcttttttaattctgctgttcttcctgagtttggctcctttgcgtgtggaaattctaccccctccaccttaaccattgcggcgcccttttcggaaatccagtatttttgtattggggcgggaggtaaaccgggttgtattcaccgcttgtttgtaaagccatttgttgcttcaattcccattaacacttcactttcctctaatacatacttacctaccttacattctactcacccctcctggcaacctcttattggcctcacggcttttatttccgttgttttactaaactttataattcttaacaaactttcttaaacatgcttgccattttgcttctgctcgttactttaacgtccgcagattaccacaatgtaattgtacgagaaaacagtttacaaaacccatcacaggtatatgttaaagcaggctctaacttaactttacaatccttctattcgccttaccctgaggacatgccacgtgttacttggtacttagaagtttttgattcgctatttgaaaggcatacgattcctccattttttacaggcgttatactttgtgacatttctggtgacatacagcatgtgtggaaccattggcctttacaatttaattgcataaataaaagcttacatattattaatctcaaaccaagtgatgaaggcctttacaatgtgaaggttttaaaggacagcattcagcataatacatactttcgagtgcatgtagtaagttttccaagacctgaatgtaacatcaccactacatatctttcagatgactactgccttattaacattgattgctctcaattaccataccctgctaaggtctattataatggcaatgaaagtaagctgcattactacttatctgaacgcggtggccagccaaaccttccaaattactttactgttgggtatcgatatagagatctccgacaaaattatacagttgaatatccatttaatgaactatgtacagagataattgctcttgaaacagggtctgattttatgccaatttttatagttaccctagtggtgagcattatagttattgtgatgggcatcacatatcttatttatcactgtaggactttaaagaccaaaaccaaaaccaaaaccaagcctcctgaaatccgtttgctttaattttttccagaatggtagctgctttcttcatttttctctgtataccaatcatctgcgcctccacaacttttgccgctgtttcccacctggaaccagactgtctaccaccttttgttgtatacctgatactgacttttgtggtctgtacagccattaccagcatagcctgcttttttgtaacaattttccaagccgccgattatctctacgtacggtttgcttattttagacatcaccccgagtatcggaatcaaaacgtagcttctttactttgtctagcatgattcgcctatttatactgcacactctgtttaccctcgcaaaatgtcattgcccttttaccaaaccttggtccttttacacctgttacgatgtactgcccgaaacccctattgcctggctttacgtagccacagcggttttagtttttgtagcaacctgcattggcgttaaactgtacttctacttaaaaattggatggcttcatcccccagaagatttaccccgatatcctcttgttaataactttcaacagcctctgccgcctcctgatcctcttccgcgagctccctccgttgttagctactttcaactcaccggtggagatgactgactctcaggacattgatattagtgtggaaagaatagccgctcagcgtcagcgagaaactcgggtgctggagtactttgaactacagcagcttaaagagtcccactggtgtgagaaaggagtgctgtgtcatgttaagcaggcagccctttcttacgatgtcagccttcagggacatgaactgtcttacactttgccttcgcaaaaacaaaccttctgcaccatgatgggctctacctccatcacaatcacccaacaaaccggacctgttgagggagctatcctgtgtcactgtcacgcgcctgattgtatgcccaaactaattagaactctctgtgccttaggtgatatatttaaaatgtaagtcagtatcaataaacttaccttaaatttgacagcagttttttggtaacatcattcagcagcaccactttaccctcttcccaactctcgtatgggacgtgatggtgggcggcaaacttcctccaaaccctaaaacaaatattaatatccacttccttgtccttacccacaattttcatcttttcatagatgaaaagaaccagagttgatgaagacttcaaccccgtctacccttatgactccacatccactcctgcggtcccctttatatcccccccgtttgtaaacagcgatggtcttcaggaaaaccctcctggagtcttaagtttacgaatagctaaacccttgtattttgacatggaaaggaaactagcgctttcacttggaagaggattggcaattacctccaccggacagctagaaagcacacagagcgtgcaaaccacccctccattagttgtcaacaacagcaacacgcttgtcctgcgttattcctccccgttaggcttatcgggtgacaatttaatactaaattgctccgatcctctccgcgtagtaaacaacagcctgacattcagctacctatctccacttcgttttgaaggtggcagtcttacattcaattacacatctccccttaaactgttgaacagcagccttgcgatcggaataaattccaacaaaggtctcggcaatgacagcgatgaactttctgtcaaactaacatcagatctaaagtttaacaacgatggaaaaatagcttttggtatacaaagcctgtgtaccacccccacagccgcctctaactgtaccgtttttaccaacggtgattctttactctgtttatgtttaaccaaatgtggagctcacgtgttaggaagtgtgagtttaaccggaatgcaaggaaccataacagccatgacacagaactacattagtattcaatttctatttgacaacaatggtgcgttgacttcatcaccgctcctcaacaacaacacttggggtatacggcaaaacgacacttcgtccgctaaccccgcctacaatgctcttgcatttatgcctaacagcactgtatatgtaagaggtcaaagtggtgagcccagaaataactattacacccaaacataccttaggggaaacgttaaaaagccaattatccttaccgttacctacaactcggctgcttcaggttattcactaacttttaaatgggatgctgtagtaacagaaaaatttgccactccaacatcttctttttgctatattacagaacaataaattcctattaccccaccaattcgtttttttcagatgaaacgggccagagttgatgaagacttcaacccagtgtacccttatgaccccccatacgctcccgttatgcccttcattactccaccttttacctcctcggatgggttgcaggaaaaaccacttggagtgttaagtttaaactacaaggatcccattactacacaaaatggatctctcacgttgaaaataggaaacggcctcactctagacaaccagggacaattaacatcaactgctggggaagtagagcctccgctcactaatgctaacaacaaacttgcactagcctatagcgaaccattagcagtaaaaagcaaccgcttaactttatcacacaccgccccccttgtcgttgctaataattctttagcgttgcaagtttcagaacctatttttataaatgacgatgacaagctagccctgcagacagccgccccccttgtaactaacgctggcacccttcgcttacagagcgccgcccctttaggattggttgaaaatactcttagactgctgttttctaaacccttgtatttgcaaaatgattttcttgcattaggcattgaacgccccctggctatagcagccgcaggtactctagcactacaactcactcctccattaaagactaacgatgacgggctgacactatccacagtcgagccattaactgtaaaaaacggaaacttaggcttgcaaatatctcgccctttggttgttcaaaacagcagcctttcgcttgctattacccccccgctgcgtctatttaacagcgaccccgttcttggtttgggctttacttttcccctagccgtgacagacaacctactctccttaaacatgggagacggtgttaaactaacctataataaactaacagccaatttgggtagggatttacaatttgaaaacggtgccattgccgtaacgcttactgccgaatcacctttgcaatacactaacaaacttcaactgaatattggagctggccttcgttacaatggagccagcagaaaactagatgtaaacattaaccaaaataagggcttaacttgggacaacgatgcagttattcccaaattaggatcaggtttacaattcgaccctaatggtaacatcgctgttatccctgaaaccgtaaagccgcaaacgttatggacaactgcagatccatcgcctaactgctcagtgtaccaggacttggacgccaggctgtggctcgctcttgttaaaagtggtgacatggttcatggaagcattgctctaaaagccctaaaaggaacgttgctaaatcctacagcaagctacatctccattgtgatatatttttacagcaacggagtcaggcgtaccaactatcccacgtttgacaacgaaggcaccttagctaacagcgctacctggggataccgagaggggcaatctgctaacactaatgtaaccaatgccactgaatttatgcccagctcaaccaggtaccccgtgaataaaggagacaatattcagaatcaatctttttcatacacctgtatcaaaggagatttcgctatgcctgtcccgttccgtgtaacatataatcatgccctggaaggatactcccttaagttcacctggcgcgttgtagccaaccaagcttttgatattccttgctgttccttttcatacatcacagaataaaccactttttaaaatttttctttttattttacacgcacagtaaggcttcctccccccttccatttgacagcatacaccagcctctcccccttcatggcagtaaactgctgcgagccagtccggtatttgggagttaaaatccaaacagtctctttggtgatgaaacgtcgatccgtgatggacacaaatccctggggcaggttttccagcgtttcggtaaaaaactgcacaccgccctacaaaacaaacaggttcaggctctccatgggttatctccccgatcaaactcagacagggtaaaggtgcggtgatgttccactaaaccacgcaggtggcgctgtctgaacctctcggtgcgactcctgtgaggctggtaagaagttagattgtccagtagcctcacagcatggatgatcagtttacgtgtacgtctggcgcaacagcgcatctgaatctcactgagattccggcaagaatcgcacaccatcacaatcaggttgttcatgatcccatagctgaacacgctccagccaaagctcattcgctccaacagcgccaccgcgtgtccgtccaaccttactttaacataaatcaggtgtctgccgcgtacaaacatactacccgcatacagaacttcccggggcaaacccctgttcaccacctgcctgtaccagggaaacctcacatttatcagggagccatagatagccattttaaaccaattagctaacaccgccccaccagctctacactgaagagaaccgggagagttacaatgacagtgaataatccatctctcataacccctgatggtctgatggaaatccagcacaccgccctacaaaacaaacaggttcaggctctccatgggttatctccccgatcaaactcagacagggtaaaggtgcggtgatgttccactaaaccacgcaggtggcgctgtctgaacctctcggtgcgactcctgtgaggctggtaagaagttagattgtccagtagcctcacagcatggatgatcagtttacgtgtacgtctggcgcaacagcgcatctgaatctcactgagattccggcaagaatcgcacaccatcacaatcaggttgttcatgatcccatagctgaacacgctccagccaaagctcattcgctccaacagcgccaccgcgtgtccgtccaaccttactttaacataaatcaggtgtctgccgcgtacaaacatactacccgcatacagaacttcccggggcaaacccctgttcaccacctgcctgtaccagggaaacctcacatttatcagggagccatagatagccattttaaaccaattagctaacaccgccccaccagctctacactgaagagaaccgggagagttacaatgacagtgaataatccatctctcataacccctgatggtctgatggaaatccagatctaacgtggcacagcagatacacactctcatatacattttcatcacatggttttcccaggccgttaaaatacaatcccaatacacgggccactcctgcagtacaataaagctaatacaagatggtatactcctcacctcactaacattgtgcatgttcatattttcacattctaagtaccgagagttctcctctacaacagcactgctgcggtcctcacaaggtggtagctggtgacgatcgtaaggagccagtctgcaacgataccgtctgtcgcgctgcatcgtagaccagagaccgacgcacctcctggtacttgtggtagcagaaccacgtccgctgccaacaggtatccacgtaacgccggtccctgcgtcgcgcgcgctctgttctcaatgcaaaatgcagccactcttgtaatccacacagatccctctcggcctccgggaggatacacacttcaaacctacaaatgtctcggtacagttccaaacacgaagtgagggcgagttccaaccaagacaggcaggctggtctatcccgacacactggaggtggaggaagacacggaagaggcatgttattccaagcgattcaccaacgggtcgaaatgaagatcccgaagatgacaacggtcgcctccggagccctgatggaatttaacagccaaatcaaacattatgcgattttccaggctatcgatcgcggcctccaaaagagcctggacccgcacttccacaaacaccagcaaagcaaaagcgttattatcaaactcttcgatcatcaagctgcaagactgtacaatgcccaagtaattttcatttctccactcgcgaatgatgtcgcggcaaatagtctgaaggttcatgccgtgcatattaaaaagctccgaaagggcgccctctatagccatgcgtagacacaccatcatgactgcaagatatcgggctcctgagacacctgcagcagatttaacagacccaggtcaggttgctctccgcgatcgcgaatctccatccgcaaggtcatttgcaaataattaaatagatctgcgccgactaaatctgttaactccgcgttaggaactaaatcaggtgtggctacgcagcacaaaagttccagggatggcgccaaactcactagaaccgctcccgagtagcaaaactgatgaatgggagtaacacagtgtaaaatgttcagccaaaaatcactaagccgctcctttaaaaagtccagtacttctatattcagttcgtgcaagtactgaagcaactgtgtgggaatatgcacaacaaaaaaaatagggcggctcagatacatgttgacctaaaataaaaagaatcattaaactaaagaagcttggcgaacggtgggataaatgacacgttccagcagcaggcaagcaaccggctgtccccgggaaccgcggtaaaattcatccgaatgattaaaaagaacaacagaaacttcccaccatgtactcggttggatctcctgagcacagagcaatacccccctcacattcatatccgccacagaaaaaaagcgtcccagatacccagcgggaatatccaacgacagctgcaaagacagcaaaacaatccctctgggagcaatcacaaaatcctccggtgaaaaaagcacatacatattagaataaccctgctgctggggcaaaaaggcccgtcgtcccagcaaatgcacataaatatgttcatcagccattgccccgtcttaccgcgtaaacagccacgaaaaattcgagctaaaatccacccaacagcctatagctatatatacactccgcccaatgacgctaataccgcaccacccaccgccaaagttcacccacacccacgaaacccgcgaaaatccagcgccgtcagcacttccgcaatttcagtctcacaacgtcacttccgcgcgccttttcacattcccacacccgcccacaaaccccgcgtcaccgcccgtcaccccggccccgcctcgctcctccccgctcattatcatattggcacgtttccagaataaggtatattattgatgatg

SEQ ID NO: 2 - DNA, 34391 bp, Simian Adenovirus 4310A (sAd4310A) Wild Type
catcatcaataatataccttattctggaaacgtgccaatatgataatgagcggggaggagcgaggcggggccggggtgacgtgcggtgacgcggggtgacgcggggtggcgcgagggcggggcgggtgtgcggaggcgcttagtttttacgtatgcggaaggaggttttataccggaagttgggtaatttgggcgtatacttgtaagttttgtgtagtttggcgcgaaaaccgggtaatgaggaagttgaggttaatatgtactttttatgactgggcggaatttctgctgatcagcagtgaactttgggcgctgacggggaggtttcgctacgtggcagtaccacgagaaggctcaaaggtcccatttattgtactcctcagcgttttcgctgggtatttaaacgctgtcagatcatcaagaggccactcttgagtgccggcgagtagagttttctcctccgcgctgccgcgatgaggctggttcccgagatgtacggtgttttctgcagcgagacggcccggaactcagatgagctgctgaattcagacctgctggaaatttcgaattcgcctgtgcttttgccgccgtcacttcacgacctgtttgatgtggaagtggaccctccggaagatcccaacgaggacgcggtaaatactatgtttccagaatgtctgtttgaggcggctgaggagggttcttacagcggtgaagacggcgggcagggagaggaagtggacctgaagtgctacgaggaatgtctaccttctagcgattctgaaacggaacagacagggggagatggctgtgctgaacctgttgtgaaaaatgaacttgtattagactgtcctgataatcctggtcacggttgccgcgcctgtgattttcatagaaatgccagtggaaatcctgagactctatgtgctctgtgttacctgcgccttaccagccattgtgtatacagtaagtagaaactttttcgctttgtgcatgctggtgggatttttaaagtgcgttgggcttattgttgcgtaatgttttacaggcgacgtgtctgacgcggaaggggatggagatagatcaggctctgctggttctccttgcactttgggggctgtggttccagatggcattattaaacccgtggcggtaagagtttcaggcagacggtgtgcggtcgaaaaaattgaagacttgctgcaggaggaacagatgcaacctttggacctgtccctgaaacgccctaagctgacctaagagtgtttattgtatgcaataaaaagtgttgatctttgaactgtgtttatgtgttgggtgtgtctgtgggtatataagcaggtggatgggaagtgagagcacagctgcttcagatggatctgctaggagacctgagggaatttggcgtggttcggcgcttgctggagttggcctctgacagaacttccaagttttggaggttttgttttggctcaacgcttagcaacgtgctatatagggtcaagaaggagcaggagacgcagtttgctaggctgttggccgatactcctggagtttttgtggctctggatctaggccatcactctcttttccaagagaaaattatcaaaaacttaacttttacgtctcctggtcgcacggttgcttccgctgcctttattacctatattttggatcaatggagcaacagcggcagtcacctgtcgtgggagtacatgctggattacatgtcgatggcgctgtggagggccatgctgcggaggagggtttgcatttacttgcgggcgcagcctccgcggctggaccgagtggaggaggaggacgagccgggggagaccgagaacctgagggccgggctggaccctccaacggaggactaggtgctgaggatgatcccgaagaggggactagtggggctaggaagaagcaaaagactgagtctgaacctcgaaactttttgaatgagttgactgtgagtttgatgaatcgtcagcgtccggagacaattttctggtctgaattggaggaggaattcaggaggggggaactgaacctgctatacaagtatgggtttgaacagttgaaaactcactggttggagccgtgggaggattttgaaaccgccttggacacttttgctaaagtggctctgcgaccggataaggtttacactatccgccgcactgttaacataaagaagagtgtttatgttataggccatggagctctggtgcaggtgcaaaccgccgaccgggtggcctttagttgcggcatgcaaaatctgggccccggggtgataggcttaaatggtgtaacatttcacaatgtaaggtttactggtgaaagttttaacggctctgtgtttgcaaataacacacagctgacgctccacggcgtttacttttttaactttaataacacatgtgtggagtcgtggggcagggtgtctttgaggggctgctgttttcacggctgctggaaggcggtggtgggaagacttaaaagtgtaacatctgtaaaaaaatgcgtgtttgagcgctgtgtgttggctttaaccgtggagggctgtggacgcattaggaataatgcagcgtctgagaatggatgtttccttttgctaaaaggcacggctagcgttaagcataacatgatatgcggcagcggtttgtacccttcgcagctgttaacttgcgcggatggaaactgtcagaccctgcgcaccgtgcacatagcgtcccaccagcgacgcgcctggccaacattcgagcacaatatgcttatgcgctgtgccgttcacctgggccctaggcgaggcgtgtttgtgccttaccagtgtaactttagccataccaagtttttactagaacctgacaccttctctcgagtgtgtttcaacggggtttttgacatgtcaatggaactgtttaaagtgataagatatgatgaatccaagtctcgttgtcgcccatgtgaatgcggagctaatcatttgaggttgtatcctgtaactctgaacgtcaccgaggagctgagaacggaccaccacatgctgtcttgcctgcgcactgactatgaatccagcgacgaggagtgaggtgaggggcggagccaaacgggtataaaggggcgtgaggggtcggtgcggtgtttcaaaatgagcgggacgacggacggcaatgcgtttgaggggggagtgttcagcccatatctgacatctcgtcttccttcctgggcaggagtgcgtcagaatgtagtgggatccaccgtggacggacgaccggtggctcctgcaaattccgccaccctcacctatgccaccgtgggatcatcgttggacactgccgcggcagctgccgcttctgctgccgcttctactgctcgcggcatggcggctgattttggactgtataaccaactggccactgcagctgtggcgtctcggtccctggttcaagaagatgccctgaatgtgattctgactcgcctggagatcatgtcacgccgcctggacgaactggctgcgcagatatcctcaactaaccccgataccacttcagaaccttaaataaagacaaacaaatttgttgaaaagtaaaatggctttatttgtttttttggctcggtaggctcgggtccacctgtcccggtcgttaaggaccttgtgtatgttttccaagacccggtacagatgggcttggatgttcaagtacatgggcatgaggccatctcgggggtggagataggaccattgcagagcgtcatgctccggggtggtgttgtaaataacccagtcgtagcagggtttctgagcgtggaactggaagatgtcctttaggagcaggctgatggccaagggcagccccttagtgtaggtgttaacaaagcggttaagctgggagggatgcatgcggggggagatgatatgcatcttggcttgaattttgaggttagctatgttaccacctaggtccctgcgggggttcatgttatgaaggaccaccagcacggtgtagccggtgcacttggggaacttgtcatgcagtttggaggggaaggcgtggaagaatttagagacccccttgtggcctcctaggttttccatgcactcatccataatgatggcaatgggacccctggcggccgctttggcaaacacgttttgggggttggaaacatcatagttttgctctagagtgagctcatcataggccatcttaacaaagcggggtaggagggtgcccgactgggggatgatagttccatctgggcctggggcgtagttgccctcacaaatctgcatttcccaggccttaatttccgaggggggtatcatgtccacctggggggcgataaagaacacggtttctggcgggggattgatgagctgggtggaaagcaagttacgcaacagttgggatttgccgcaaccggtgggaccgtagatgaccccgatgacgggttgcagctggtagttgagagaggaacagctgccgtcggggcgcaggaggggggctacatcgttcatcatgcttctgacatgtttattttcactcactaagttttgcaagagcctctccccacccagggataagagttcttccaggctgttgaagtgtttcagcggtttcaggccgtctgccatgggcatcttttcaagcgactgacgaagcaagtacagtcggtcccagagctcggtgacgtgctctatggaatctcgatccagcagacttcttggttgcgggggttgggccgactttcgctgtagggcaccagccggtgggcgtccagggccgcgagggttctgtccttccagggtctcagcgttcgggtgagggtggtctcggtgacggtgaagggatgagccccgggctgggcgcttgcgagggtgcgcttcaggctcatcctgctggtgctgaagcgggcgtcgtctccctgtgagtcggccagatagcaacgaagcatgaggtcgtagctgagggactcggccgcgtgtcccttggcgcgcagctttcccttggaaacgtgctgacatttggtgcagtgcagacacttgagggcgtagagtttgggggccaggaagaccgactcggacgagtaggcgtcggctccgcactgagcgcagacggtctcgcactccaccagccacgtgagctcgggtttagcgggatcaaaaaccaagttgcctccattttttttgatgcgtttcttaccttgcgtctccatgagtctgtgtcccgcttccgtgacaaaaaggctgtcggtgtccccgtagaccgacttgagggggcgatcttccaaaggtgttccgagatcttccgcgtacaggaactgggaccactccgagacaaaggctcgggtccaggctaacacgaaggaggcgatctgcgaggggtatctgtcgttttcaatgagggggtccaccttttccagggtgtgcagacacaggtcgtcctcctccgcgtccacgaaggtgattggcttgtaagtgtaggtcacgtgacccgcacccccccaaggggtataaaagggggcgtgcccactctccccgtcactttcttccgcatcgctgtggaccagagccagctgttcgggtgagtaggccctctcaaaagccggcatgatttcggcgctcaagttgtcagtttctacaaacgaggaggatttgatattcacgtgccccgcggcgatgcttttgatggtggaggggtccatctgatcagaaaacacgatctttttattgtcaagtttggtggcgaaagacccgtagagggcgttggaaagcaacttggcgatggagcgcagggtctgatttttctcccgatcggccctctccttggcggcgatgttgagttgcacgtactcgcgagccacgcaccgccactcggggaacacggcggtgcgctcgtcgggcaggatgcgcacgtgccagccgcggttgtgcagggtgatgaggtccacgctggtggccacctccccgcggaggggctcgttggtccaacacaatcgccccccttttctggagcagaacggaggcaggggatctagcaagttggcgggcggggggtcggcgtcgatggtaaatatgccgggtagcagaattttattaaaataatcgatttcggtgtccgtgtcttgcaacgcgtcttcccacttcttcaccgccagggccctttcgtagggatttaggggcggtccccagggcatggggtgggtcagggccgaggcgtacatgccgcagatgtcgtacacgtacaggggctccctcaacaccccgatgtaagtggggtaacagcgccccccgcggatgctggctcgcacgtagtcgtacatctcgtgagagggagccatgagcccgtctcccaagtgggtcttgtggggtttctcggcccggtagaggatctgcctgaagatggcgtgggagttggaagagatggtggggcgttggaagacgttaaagttggctccgggcagtcccacggagtcttggatgaattgggcgtaggattcccggagcttgtccaccagggctgcggttaccagcacgtcgagagcgcagtagtccaacgtctcgcggaccaggttgtaggccgtctcttgttttttctcccacagttcgcggttgaggaggtattcctcgcggtctttccagtactcttcggcgggaaatcctttttcgtccgctcggtaagaacctaacatgtaaaattcgttcacggctttgtatggacaacagcctttttctaccggcagggcgtacgcttgagcggcctttctgagagaggtgtgggtgagggcgaaggtgtcccgcaccatcactttcaggtactgatgtttgaagtccgtgtcgtcgcaggcaccctgttcccacagcgtgaagtcggtgcgctttttctgcctgggattggggagggcgaaggtgacgtcgttaaagaggattttcccggcgcggggcatgaagttgcgagagatcctgaagggtccgggcacgtccgagcggttgttgatgacttgcgccgccaggacgatctcatcgaagccgttgatgttgtggcccacgatgtaaagttcgataaagcgcggctgtcccttgagggccggcgcttttttcaactcctcgtaggtgagacagtccggcgaggacagacccagctcagcccgggcccagtcggagagttgaggattagccgcgaggaaggaactccatagatccaaggccaggagagtttgcaagcggtcgcggaactcgcggaactttttgcccacggccattttctccggcgttaccacgtaaaaggtgtcggggcggttgttccagacgtcccatcggagctctagggccagctcgcaggcttggcgaacgagggtctcctcgcccgagacgtgcatgaccagcatgaagggtaccaactgtttcccgaacgagcccatccatgtgtaggtttctacgtcgtaggtgacaaagagccgctgggtgcgcgcgtgggagccgatcgggaagaagctgatctcctgccaccagctggaggaatgggtgttgatgtggtgaaagtagaagtcccgccggcgcacagagcattcgtgctgatgtttgtaaaagcgaccgcagtagtcgcagcgttgcacgctctgtatctcctgaatgagatgcgcttttcgcccgcgcaccagaaaccggagggggaagttgagactggggcttggtggggcggcatccccttcgccttggcggtgggagtctgcgtctgcgcccttcttctctgggtggacgacggtggggacgacgacgccccgggtgccgcaagtccagatctccgccacggaggggcgcaggcgctgcaggagggggcgcagctgcccgctgtccagggagtcgagggcggccgcgctgaggtcgacgggaagcgtttgcaagttcactttcagaagaccggtaagagcgtgagccaggtgcagatggtacttgatttccaggggggtgttggaagaggcgtccacggcgtagaggaggccgtgtccgcgcggggtcaccaccgtgccccgaggaggttttatctcactcgtcgagggcgagcgccgggtggtagaggcggctctgcgccggggggcagcggaggcagaggcacgttttcgtgaggattcggcagcggttgatgacgagcccggagactgctggcgtgggcgacgacgcggcggttgaggtcctggatgtgctgtctctgcgtgaagaccaccggtccccgggtcctgaacctgaaagagagttccacagaatcaatgtctgcatcgttaacggcggcctgcctgaggatctcctgtacgtcgcccgagttgtcttgataggcgatctcggccatgaactgctccacttcttcctcgcggaggtcgccgtggcccgctcgctccacggtggcggccaggtcgttggagatgcgacgcatgagttgagagaaggcgttgaggccgttctcgttccacacgcggctgtacaccacgtttccgaaggagtcgcgcgctcgcatgaccacctgggccacgttgagttccacgtggcgggcgaagacggcgtagtttctgaggcgctggaagaggtagttgagcgtggtggcgatgtgctcgcagacgaagaagtacatgatccagcgccgcagggtcatctcgttgatgtctccgatggcttcgagacgctccatggcctcgtagaagtcgacggcgaagttgaaaaattgggagttgcgggcggccaccgtgagttcttcttgcaggaggcggatgagatcggcgaccgtgtcgcgcacctcctgctcgaaagcgccccgaggcgcctctgcttcttcctccggctcctcctcttccaggggcacgggttcctccggcagctctgcgacggggacggggcggcgacgtcgtcgtctgaccggcaggcggtccacgaagcgctcgatcatttcgccgcgccggcgacgcatggtctcggtgacggcgcgtccgttttcgcgaggtcgcagttcgaagacgccgccgcgcagagcgcccccgtgcagggagggtaagtggttagggccgtcgggcagggacacggcgctgacgatgcattttatcaattgctgcgtaggcactccgtgcagggatctgagaacgtcgaggtcgacgggatccgagaacttctctaggaaagcgtctatccaatcgcaatcgcaaggtaagctgaggacggtgggccgctggggggcgtccgcgggcagttgggaggtgatgctgctgatgatgtaattaaagtaggcggtcttcaggcggcggatggtggcgaggaggaccacgtctttgggcccggcctgttgaatgcgcaggcgctcggccatgccccaggcctcgctctgacagcgacgcaggtctttgtagtagtcttgcatcagtctctccaccggaacctctgcttctcccctgtctgccatgcgagtcgagccgaagccccgcaggggctgcagcaacgctaggtcggccacgaccctctcggccagcacggcctgttgaatctgcgtgagggtggtctggaagtcgtccaggtccacgaagcggtgataggcccccgtgttgatggtgtaggtgcagttggccataacggaccagttgacgacttgcatgccgggttgggtgatctccgtgtacttgaggcgcgagtaggcgcgggactcgaacacgtagtcgttgcatgtgcgcaccagatactggtagccgaccaggaagtgaggaggcggttctcggtacaggggccagccgacggtggcgggggcgccgggggacaggtcgtccagcatgaggcggtggtagtggtagatgtagcgggagagccaggtgatgccggccgaggtggtcgcggccctggtgaattcgcggacgcggttccagatgttgcgcagggggcgaaagcgctccatggtgggcacgctctgccccgtgaggcgggcgcaatcttgtacgctctagatggaaaaaagacagggcggtcatcgactcccttccgtagctcggggggtaaagtcgcaagggtgcggcggcggggaaccccggttcgagaccggccggatccgccgctcccgatgcgcctggccccgcatccacgacgtccgcgccgagacccagccgcgacgctccgccccaatacggaggggagtcttttggtgttttttcgtagatgcatccggtgctgcggcagatgcgacctcagacgcccaccaccaccgccgcggcggcagtaaacctgagcggaggcggtgacagggaggaggaggagctggctttagacctggaagagggagaggggttggcccggctgggagcgccgtccccagagagacaccctagggttcagctcgtgagggacgccaggcaggcttttgtgccgaagcagaacctgtttagggaccgcagcggtcaggaggcggaggagatgcgcgattgcaggtttcgcgcgggcagagagctgagggcgggcttcgatcgcgagcggctcctgagggcggaggatttcgagcccgacgagcgttctggggtgagcccggcccgcgctcacgtctcggcggccaacctggtgagcgcgtacgagcagacggtgaacgaggagcgcaacttccaaaagagctttaacaatcacgtgaggaccctgatcgcgagggaggaggtgaccatcgggctgatgcatctgtgggacttcgtggaggcctacgtgcagaacccggccagcaaacctctgacggcccagctgttcctgatcgtgcagcacagccgcgacaacgagacgttccgcgacgccatgttgaacatcgcggagcccgagggtcgctggctcttggatctgattaacatcctgcagagcatcgtggtgcaggagagggggctgagtttagcggacaaggtggcggccattaactattcgatgcagagcctggggaagttctacgctcgcaagatctacaagagcccttacgtgcccatagacaaggaggtgaagatagacagcttttacatgcgcatggcgctgaaggtgctgacgctgagcgacgatctcggcgtgtaccgtaacgacaagatccacaaggcggtgagcgccagccgccggcgggagctgagcgacagggagctgatgcacagcctgcagagggcgctggcgggcgccggggacgaggagcgcgaggcttacttcgacatgggagccgatctgcagtggcgtcccagcgcgcgcgccttggaggcggcgggctaccccgacgaggaggaccgggatgatttggaggaggcaggcgagtacgaggacgaagcctgaccgggcaggtgttgttttagatgcagcggccggcggacggggccaccgcggatcccgcacttttggcatccatgcagagtcaaccttcgggcgtgaccgcctccgatgactgggcggcggccatggaccgcatcatggcgctgaccacccgcaaccccgaggcttttaggcagcaaccccaggccaaccgtttttcggccatattggaagcggtggtaccgtcgcgcaccaaccccacacacgagaaagtcctgactatcgtgaacgccctggtagacagcaaagctatccgccgcgacgaggcggggctgatctacaacgctctgttggaacgggtggcgcgctacaacagcactaacttgcagaccaatctggatcgcctcaccacggacgtgaaggaggcgctggctcagaaggagcggtttctgagggatagcaatctgggttctctggtggcactgaacgcctttctgagcacgcagccggccaacgtgccccgcgggcaggaggattacgtgagcttcatcagcgctctgagactgctggtgtccgaggtgccccagagcgaggtgtaccagtctgggccggattacttttttcagacgtcccgacagggcttgcaaacggtgaacctgactcaggcctttaaaaacttgcaaggtatgtggggcgtcaaggccccggtgggcgatcgcgccactatctccagtctgctgacccccaacactcgcctgctgctgctcttgatcgcaccgttcaccaacagtagcactatcagccgtgactcgtacctgggtcatctcatcactctgtaccgcgaggccatcggccaggctcagatcgacgagcatacgtatcaggagatcactaacgtgagccgggccctgggtcaggaagataccggcagcctggaagccacgttgaactttttgctaaccaaccggaggcaaaaaataccctcccagttcacgttaagcgccgaggaggagaggattctgcgatacgtgcagcagtccgtgagcctgtacttgatgcgcgagggcgccaccgcttccacggctttagacatgacggctcggaacatggaaccgtccttttactccgcccaccggccgttcattaaccgtctgatggactacttccatcgtgcggccgccatgaacggggagtacttcaccaatgccatcctgaatccgcattggatgcccccgtccggcttctacaccggggagtttgacctgcccgaagccgacgacggctttctgtgggacgacgtgtccgatagcattttcacgccggggaatcgccgattccagaagaaggagggcggagacgagctccccctctccagcgtggaggctgcctctaggggagagagcccctttcccagtctgtcttccgccagtagcggtcgggtaacgcgcccgcggttgccgggggagagcgactacctgaacgaccccttgctgcgaccggctagaaagaaaaatttccccaacaacggggtggaaagcttggtggataaaatgaatcgttggaagacctacgcccaggagcagcgggagtgggaggacagtcagccgcgaccgctggttccgccgcactggcgtcgccagagagaagacccggacgactccgcagacgatagtagcgtgttggacctgggagggagcggagccaacccctttgctcacttgcaacccaaggggcgttcgagtcgcctctactaataaaaaagacgcggaaacttaccagagccatggccacagcgtgtgtcctttcttcctctctttcttcctcggcgcggcagaatgagaagagcggtgagagtcacgccggcggcgtatgagggtccgcccccttcttacgaaagcgtgatgggatcagcgaacgtgccggccacgctggaggcgccttacgttcctcccagatacctgggacctaccgagggcagaaacagcatccgttactccgagctggcgcccctgtacgataccaccaaggtgtacctggtggacaacaagtcggcggacatcgcctccctgaattaccaaaacgaccacagcaactttctgaccaccgtggtgcagaacaatgacttcaccccgacggaggcgggcacgcagaccattaactttgacgagcgttcccgctggggcggtcagctgaaaaccatcctgcacaccaacatgcccaacatcaacgagttcatgtccaccaacaagttcagggccaggctgatggttaaaaaggtagaaaaccagcctcccgagtacgaatggtttgagttcaccatccccgagggcaactattccgagactatgactatcgatctgatgaacaatgcgatcgtggacaattacctgcaagtggggaggcagaacggggtattggaaagcgatatcggtgtgaaatttgataccagaaacttccgactggggtgggatcccgtgaccaagctggtaatgccaggcgtgtacaccaacgaggcttttcaccccgacatcgtgctgctgccggggtgcggcgtggatttcactcagagccgcttgagtaacctgttaggaatcaggaagcgccgtcccttccaggagggctttcagatcatgtatgaggacctggagggaggtaacattcccgctctactagatgtgacaaagtacgaacaaagtgtacagcgagccaaggcggaagggcgagagattcgcggagacacttttgccgtgtctccccaggatttggttatagagccgttagagcatgacagcaaaaatcgtagttacaatcttttgcccaacaaaaccgacacggcctatcgcagctggtttttggcttacaactacggagaccccgagaaaggagtgagatcatggaccatactcaccaccacggacgtgacctgcggctcgcagcaagtgtactggtccctgccggatatgatgcaagacccggtcaccttccgcccctccacccaagtcagcaacttcccggtggtgggcaccgagctgctgcccgtccatgccaagagcttctacaacgagcaggccgtctactcgcaactcattcgccagtccaccgcgcttacccacgtgttcaatcgttttcccgagaaccagattctggtgcgccctcccgctcctaccattaccaccgtcagtgaaaacgttcccgccctcacagatcacggaaccctaccgctgcgcagcagtatcagtggagttcagcgcgtgaccatcaccgacgccagacgtcgaacctgcccctacgtttacaaagcgctcggcgtggtggcccctaaagttctctctagtcgcaccttttaaacatgtccattctcatctctcccgataacaacaccggctggggattgggctccggcaagatgtacggcggggctaagcgacgctccagtcagcatcccgttcgcgttcggggtcacttccgcgctccctggggagcttacaagcgaggactctctggccgaacggctgtagacgataccatagatgccgtgattgccgacgcccgccggtacaaccccggaccggtcgctagcgccgcctccaccgtggattccgtgatcgacagcgtggtggccagcgccagggcctatgctcgccgcaagaggcggctgcatcggaaacgtcgccccaccgccgccatgctagcagccagggccgtgctgaggcgggcccggagggtaggcaggagggctatgcgccgcgctgccgccaacgccgccgggagggcccgcagacaagccgcccgccaggccgccgctgccatcgctagcatggccagacccaggagagggaacgtgtactgggtgcgcgattctgtaacgggagtccgagtgccggtgcgcagccgacctccccgaagttagaagatccaagctgcgaagacggcggtactgagtctccctgttgttattagcccaacatgagcaagcgcaagtttaaagaagaactgctgcagacgctggtgcctgagatctatggccctccggacgtgaagcctgacattaagccccgcgatatcaagcgtgttaaaaagcgggaaaaaaaagaggaacttgcggcggtagacgatggcggtgtagaatttattaggagtttcgccccacggcgcagggttcaatggaaagggcggcgtgtacaacgcgttctgaggccgggcaccgcggtagtttttaccccgggagagcggtcggccgttaggggtttcaagcggcagtacgatgaggtgtacggcgacgaagacatactggaacaggcggctcagcagattggagaattcgcttatggcaaacgttctcggcgcgaagacctggccatcgccttggacagcggcaatcccacacccagcctcaaacccgtgacgctgcaacaggtgcttcccgtgagcgccagtactgacagcaaaagggggattaaaagagagatggaagagctgcaacccaccatccaacttatggtccctaaacgacagaggttggaagaggtcctggagaagatgaaagtggaccccagcatagagccggatgtgaaagtgaggcctattaaggaagtggcccccggtcttggggtgcaaacggtggacattcaaatccccgtcacgtccgcttcaacagcggtggaagccatggaaacgcaaacggaagcccccgccgtcacggtcggtaccagggaagtggcgttgcaaacggaaccctggtacgaatacgccacccctaggcgtcagaggcggtccgcccgttacggacccgtcaacgccatcatgcccgagtacgcgctacatccgtctatccggcccactcccggctaccggggagtgacgtatcgcccgtcaggaactcgccgccgttaccgtcgccgccgtcgctctcgccgcgctctggccccagtgtcggtgcggcgcgtgacccgccaggggaaaacagtcaccatccccaacccgcgctaccaccctagcattctttaatgactctgccgttttgcagatggctctgacttgccgcgtgcgccttcccgttctgcactatcgaggaagatctcgtcgtaggagaggcatggcgggcagtggtcgccggcgggctttgcgcaggcgcatgaaaggcggaattttacccgccctaatacctataatcgccgccgccataggcgccatacccggcgtcgcttcagtggccttgcaagcagctcgtaataaataaacgaaggcttttgcacttatgtcctggtcctgactattttatgcagaaaaagcatggaagacatcaattttacgtcgctggctccgcggcaaggctcgcggccgctcatgggcacctggaacgacatcggcaccagtcagctcaacgggggcgctttcaattgggggagcctttggagcggcattaaaaactttggctccacgattaaatcctacggcagcaaagcctggaacagtagtgctggtcaaatgctccgagataaactgaaggacaccaacttccaagagaaagtggtcaacggggtggtgaccggcatacacggcgcggtagatcttgccaaccaagcggtgcagaaagagattgacaggcgattggaaaactcgcgggtgccgccgcagagaggggatgaggtggaggtcgaggaagtagaagtagaggaaaagctgccccccttggagaaagttcccggtgcgattccaaggccgcagaagcggccaaggccagaactagaagaaactctggtgacggagagcaaggagcctccctcgtacgagcaagccttaaaagagggcgcttcaccctacccgatgaccaaaccgatcgcgcctatggctcggccggtgtacgggaaggactacaaacctgtcacgctagaacttcctccgccactcccttcgcgtcctacggtgcctcccatgccagcgccgtcggccggtcccgtgtctgcaccttccgcagcgcctctgccagccgcccgcccagtggccgtggccactgccagaaaccccagaggccagagaggagccaactggcaaaacacgctgaacagcatcgtgggcctgggagttaaaagcctgaaacgccgccgttgctattattaaaaaagtgtagctaaaaaatctcccgttgtatacgcctcctatgttaccgccagagacgtgtgactgtcgtcgcgagcagcgctttcaagatggccaccccatcgatgatgccgcagtggtcttacatgcacatcgccgggcaggacgcctcggagtatctgagccccggtcttgtgcagtttgcccgcgccaccgacacctacttcagcttgggaaacaagtttagaaatcccaccgtggcccccacgcacgatgtgaccacggatcgttcgcagaggctgactctgcgctttgtaccggtagaccgtgaggatactgcctattcttacaaagttcggtatacgttagccgtaggagacaacagggtgctggacatggccagtacttactttgacatccgcggtgttcttgaccgcggtccaagctttaaaccgtataccggaacggcatacaatgccttggctccaaagggcgctccaaatgcttgccagtggacaacgaccaacgggggcaataaaacgaacacttttgcccaagcccctttaataggcacggctattgacggaaccaacggactgcagattgggcaagataatggacaagctgtttatgctgacaaaacctttcaacccgaaccacaagtgggagaatctcagtggaatactaatccaaccacaaacgcagcaggacgcgtgttaaaaacaactactcgcatgctgccttgctatggttcttttgcaaggcccaccaatgagaaagggggtcaagcttcaggagacgttaccttccaatttttcgacactgcctcggacaatggcaacaaccctaaggtggtgctatatggagaagacgtcaacattgaatcgcctgacacacacttaatctacaaacccaccgctgacaacacaaactctgaaaaccttttgggtcaacaggccgctccaaacagagccaattacattgcctttcgggacaacttcattggactaatgtactataattcaacaggaaacatgggagtgttggcagggcaggcttcccaactaaatgctgtggtagacttgcaagacagaaacactgagctttcctaccaactcatgttagatgcaataggagaccggagtcgttacttttcaatgtggaaccaagcagtggacagctatgatccagatgtgcgaattattgaaaatcatggcgttgaggacgaactgccaaattactgcttccctcttaacgctcaaggaattgctaacacctataaaggcgttaagaaaaacaacggcaattgggcgaaagacgacgcagtagtagaaactaacgaaattggcataggaaatgtttttgccatggagataaatttaactgctaacttgtggcgaaactttctgtattccaatattgctttgtacctgccagactcctacaagtattcaccgggaaacataaccttacccgaaaacaaaaacagttacaattacattaatggtcgagtaacagctcctggtctggtagacacctttgtaaacattggcgcgcgatggtctcccgaccccatggacaacgtgaatccttttaatcaccatcgcaatgctggtctgcgttatcgctccatgcttctaggcaacggccgctacgtgcccttccacattcaggtgcctcaaaaattctttgccattaagaacctgcttctgctgcctgggtcctacacctacgagtggaacttcagaaaagatgtaaacatgatcttgcagagcacgctgggcaacgacctccgtgtcgacggggccagcgtcagattcgacagcattaacctctacgctaatttcttccccatggcacataacaccgcttccaccctggaggctatgttacgcaacgacaccaacgaccagtcctttaatgactacctctgcgcggccaacatgctataccccattcctgccaatgccaccagtgtgcccatctccatcccctctcgcaactgggcagctttcagagggtggagtttcacccgcctcaaaacaaaagaaaccccctcgctgggttccggatttgatccatactttgtttactcaggctccattccctacctggatggtaccttctacctgaaccacaccttcaaaaaggtgtctattatgttcgactcttctgtgagctggcccggcaacgaccgcctgctgacccctaatgagtttgaaattaagcgctcggtggacggagaaggatacaatgtagcccagagcaacatgaccaaagactggttcttaattcaaatgctcagccactacaacattggttaccaagggttttacgtgcccgaggcttacaaagacagaatgtactccttttttagaaacttccaacctatgagtagacaggtagtggatgcagatcggtatgaacaatacaaaaaagtcaccgttgagtatcaacataataattctggttttgtgggatacatgggacccaccatgagggaagggcaggcttatccagcgaattacccttatcctcttattggagacaccgccgtgcccagcctgacccagaaaaagttcctctgtgaccgcaccatgtggagaatccccttctctagcaacttcatgtctatgggggccctcaccgacctggggcagaacatgctgtacgccaattccgctcacgccttggatatgacctttgaggtggaccccatggatgagcccacgcttctctatgttctgtttgaagtcttcgacgtggtgcgcatccaccagccgcaccgcggcgtcatcgaggccgtctacctgcgcacacctttctctgccggtaacgccaccacataagaagcaaatgggctccagcgaacaggagctgcgggccattattcgcgacctgggctgcggaccctactttttgggcaccttcgacaagcgtttccccggattcatgtccccccagaagccggcctgtgccatagtcaacacggccgggcgggagaccgggggggttcactggctcgccttcgcctggaacccgcgcaaccgcacctgctacctgttcgacccttttggtttttccgacgaaaggctgaagcaaatctaccagttcgaatacgaaggactcctcaagcgcagcgctctggcctccacgcccgaccactgcgtcaccctggaaaaatccacccaaacggtgcaggggcccctctcggccgcctgcgggcttttctgttgcatgtttttgcacgccttcgtgcactggcctcacaaccccatggagcgcaaccccaccatggatctgctcaccggagtgcccaacagcatgcttcacagcccccaggtcgcccccaccctgcgccgtaaccaggaacacctgtatcgctttctggggaaacactctgcctatttccgccgccaccggcagcgcatcgagcaggccacggcctttgaaagcatgagccaaagagtgtaatcaataaaaaccatttttatttaacatgatacgcgcttctggcgtttttattaaaaatcgaacggttcgagggaggggtcctcgtgcccgctgggaagggacacgttgcggtactggaaacgggcgctccaacgaaactcggggatcaccagccgcggcaggggcacgtcttctaggttctgcttccagaactgccgcaccagctgcagggctcccatgacgtcgggcgccgagatcttgaagtcgcagttagggccggagcccccgcggctgttgcggaacacggggttggcacactggaacaccagcacgctggggttgtaaatactggccagggccgttgggtcggtcacctccgacgcatccagatcctcggcattgctcagggcgaacggagtcagcttgcacatctgccgtccgatctggggcaccaggtcgggtttgttgaggcaatcgcagcgcagagggattaggatgcgacgctgcccgcgttgcatgatagggtaactcgccgccaggaactcctccatctgacggaaggccatctgggccttggtaccctcggtgaaaaatagcccacaggacttgctagaaaatacgttattgccgcagttgatgtcttccgcgcagcagcgtgcatcttcgttcttcagctgaaccacgttacgcccccagcggttctggaccaccttggctttcgtaggatgctccttcaacgcccgctgaccgttctcgctggtcacatccatttccaccacgtgctccttgcagaccatctccactccgtggaagcagaacaggacgccctcctgctgggtattgcgatgctcccaaacggcacatccggtgggctcccagctcttgcgtttcacccccgcgtatgcttccatgtaagccatgaggaatctgcccatcagctcggtgaaggtcttctggttggtgaaggttagcggcaggccgcggtgctcctcgttcaaccaagtttgacagattttgcggtacacggctccctggtcgggcagaaacttaaaagccgctctgctctcgttgtccacgtggaacttctccatcaacatcgtcatgacttccatgcccttctcccacgccgtcaccaacggttcggtcccggggttcttcaccaacacggcggtggaggggccctcgccggccccgacgtccttcatggtcattctttggaactccacggtgccgtccgcgcggcgtactctgcgcatcggagggtagctgaagcccacctccaccacggtgccttcgccctcgctgtcggaaacgatctccggggatggcggcggcgcgggtgtcgccttgcgagccttcttcttgggagggagcggaggcacctcctgctcgcgctcggggctcatctcccgcaagtagggggtaatggagcttccgggttggttctgacggttggccattgtatcctaggcagaaagacatggatcttatgcgcgaggaaactttaaccgccccgtcccccgtcagcgacgaagaggtcatcgtcgaacaggacccgggctacgttacgccgcccgaggatctggagtcccccttagacgaccgacgcgacgctagtgagcggcaggaaaatgagaaagaggaggaggagggctgctacctcctggaaggcgacgtcttgctaaagcatttcgccaggcagagcaccatactcaaggaggccttgcaagaccgctccgaggtgcccttggacgtcgccgcgctctcccaggcctacgaggcgaaccttttctcgccccgagtgcctccgaagagacagcccaacggcacctgcgagcccaacccgcgactcaacttctaccccgtgttcgccgtgcccgaggcgctggccacctaccacatctttttcaaaaaccagcgcattcccctttcctgccgggccaaccgcaccgcagccgataggaagctaacactcagaaacggagccagcatacctgatatcacgtcactggaggaagtgcctaagatcttcgagggtctgggtcgagatgagaagcgggcggcgaacgctctgcagaaagaacagaaagagagtcagaacgtgctggtggagctggagggggacaacgcgcgtctggccgtcctcaaacgctgcatagaagtctcccacttcgcctaccccgccctcaacttgccacccaaagttatgaaatcggtcatggatcagctgctcatcaagagagctgagcccctggatcccgaccaccccgaggcggaaaactcagaggacggaaagcccgtcgtcagcgacgaggagctcgagcggtggctggaaaccggggacccccaacagttgcaagagaggcgcaagatgatgatggcggccgtgctggtcaccgtggagctggaatgcctgcaacggtttttcagcgacgtggagacgctacgcaaaatcggggagtccctgcactacaccttccgccagggctacgtccgccaggcctgcaagatctccaacgtggagctcagcaacctggtctcctacatgggcatcctccacgagaaccggctggggcagagcgtgctgcactgcaccttgcaaggcgaggcgcggcgggactacgtccgcgactgcatctacctcttcctcaccctcacctggcagaccgccatgggcgtctggcagcagtgcttggaagagagaaacctcaaagagctagacaaactcctctgccgccagcggcgggccctctggaccggtttcagcgagcgcacggtcgcctgcgccctggcagacattatcttcccggagcgcctgatgaaaaccttgcagaacggcctgccggattttatcagtcaaagtattttgcaaaacttccgctccttcgttctggagcgctccgggatcttgcccgccatgagctgcgcgctgccttctgactttgtccccctttcctaccgcgagtgtcctccccccctgtggagccactgctacctcttccaactggccaactttctggcctaccactccgacctcatggaagacgtgagcggagaggggctgctcgagtgccactgccgctgcaacctctgcaccccccacagatcgctggcctgcaacaccgagctgctcagcgaaacccaggtcataggtaccttcgagatccaggggccccagcagcaagagggtgcttccggcttgaagctcactccggcgctgtggacctcggcttacttacgcaaatttgtagccgaggactaccacgcccacaaaattcagttctatgaagaccaatctcgaccacccaaagcccccctcacggcctgcgtcatcactcagagcaaaatcctggcccaattgcaatccatcaaccaagcgcgccgagatttccttttgaaaaagggtcggggggtgtacctagacccccagaccggcgaggaactcaacccgtccacactctccgtcgaagcagcccccccgagacatgccgcccaagggaaccgccaagcagctgatcgctcggcagagagcgaagaagcaagagctgctccagcagcagcagcaggtggaggacgaggaagagctgtgggacagccaggcagaggaggtgtcagaggacgaggaggagatggaaagctgggacagcctagacgaggaggaggacgagctttcagaggaagaggcgaccgaagaaaaaccacctgcatccagcgcgccttctctgagccgacagccgaagccccggcccccgacgcccccggccggctcactcaaagccagccgtaggtgggacgccaccggatctccagcggcagcggcaacggcagcgggtaaggccaaacgcgagcggcgggggtattgctcctggcgggcccacaaaagcagtatcgtgaactgcttgcaacactgcgggggaaacatctcctttgcccgacgctacctcctcttccatcacggtgtggccttccctcgcaacgttctctattattaccgtcatctctacagcccctacgaaacgctcggagaaaaaagctaaggcctcctctgccgcgaggaaaaactccgccgccgctgccgccgccaaggatccgccggccaccgaggagctgagaaagcgcatctttcccactctgtatgctatctttcagcaaagccgcgggcagcaccctcagcgcgaactgaaaataaaaaaccgctccttccgctcactcacccgcagctgtctgtaccacaagagagaagaccagctgcagcgcaccctggacgacgccgaagcactgttcagcaaatactgctcagcgtctcttaaagactaaaagacccgcgctttttccccctcgggcgccaaaacccacgtcattgccagcatgagcaaggagattcccaccccttacatgtggagctatcagccccagatgggcctggccgcgggggccgcccaggactactccagcaagatgaactggctcagcgccggcccccacatgatctcacgagttaacggcatccgagcccaccgaaaccagatcctcttagaacaggcggcaatcaccgccacaccccggcgccaactcaacccgcccagttggcccgccgcccaggtgtatcaggaaactccccgcccgaccacagtcctcctgccacgcgacgcggaggccgaagtcctcatgactaactctggggtacaattagcgggcgggtccaggtacgccaggtacagaggtcgggccgctccttactctcccgggagtataaagagggtgatcattcgaggccgaggtatccagctcaacgacgaggcggtgagctcctcaaccggtctcagacctgacggagtcttccagctcggaggagcgggccgctcttccttcaccactcgccaggcctacctgaccctgcagagctcttcctcgcagccgcgctccgggggaatcggcactctccagttcgtggaagagttcgtcccctccgtctacttcaacccgttttccggctcacctggacgctacccggacgccttcattcccaactttgacgcagtgagtgaatccgtggacggctacgactgatgacagatggtgcggccgtgagagctcggctgcgacatctgcatcactgccgccagcctcgctgctacgctcgggaggcgatcgtgttcagctactttgagctgccggacgagcaccctcaggggccggctcacgggttgaaactcgagatcgagaacgcgctcgagtctcgcctcatcgacgccttcaccgcccggcctctcctggtagaaaccgaacgcgggatcactaccatcaccctgttctgcatctgccccacgcccggattacatgaagatctgtgttgtcatctttgcgctcagtttaataaaaactgaactgtttgccgcaccttcaacgccatctgtgatttctacaacaaaaagttcttctggcaaaggtacacaaactgtattttattctaattctacctcatctattgtgctgaactgcgcctgcactaacgaacttatccagtggattgcaaacggtagtgtgtgcaagtacttttgggggaacgagatagttagtagaaataacagcctttgcaagcactgcaactcctccacactaatcctttatcccccatttgttactggatggtatatgtgcgttggctccggtttaaatcctagttgctttcataagtggtttctacaaaaagagacccttcccaacaattctgtttcttttttcaccctgtcctactgctgttctccctctggttactctttcaaacctctaattggtattttagctttgatactgataatctttattaactttataataattaacaacttacagtaaacatgcttgttatcctcctgctcgccacatttttcgctctctctcacgccagaacaagtattgttggcgcaggttacaatgcaactcttcaatctgcttacatgccagattccgaccagataccccatattacgtggtacttacaaacctccaaacctaattcttcattttatgaaggaaacaaactctgcgatgactccgacaacaggacgcacacatttccccacccttcactacaattcgaatgcgtaaacaaaagcttgaagctttacaacttaaagccttcagattctggcttgtatcatgctgtagttgaaaaaagtaatttagaagtccacagtgattacattgaattgatggttgtggacctgccacctccaaaatgtgaggtttcctcctcttaccttgaagttcaaggcgtggatgcctactgcctcatacacattaactgcagcaactctaaatatccagctagaatttactataatggacaggaaagtaatcttttttattatttaacaacaagcgctggtaacggtaaacagttacctgattattttactgctgttgttgaattttccacctacagagaaacgtatgccaagcggccttacaatttctcatacccgtttaacgacctttgcaatgaaatacaagcgctcgaaactggaactgattttactccaattttcattgctgccattgttgtgagcttaattaccattattgtcagcctagcattttactgcttttgcaagcccaaaaaacctaagtttgaaaaacttaaactaaaacctgtcattcaacaagtgtgattttgttttccagcatggtagctgcatttctacttctcctctgtctacccatcattttcgtctcttcaactttcgccgcagtttcccacctggaaccagagtgcctaccgccttttgacgtgtatctgattctcacctttgtttgttgtatatccatttgcagtatagcctgcttttttataacaatctttcaagccgccgactatctttacgtgcgaattgcttactttagacaccatcctgaatacagaaatcaaaacgttgcctccttactttgtttggcatgattaagctattgctaatacttaattatttacccctaatcaactgtaattgtccattcaccaaaccctggtcattctacacctgttatgataaaatccccgacactcctgttgcttggctttacgcagccaccgccgctttggtatttgtatctacttgccttggagtaaaattgtattttattctacacactgggtggctacatcccagagaagatttacctagacatcctcttgtaaacgcttttcaattacagcctctgcctcctcctgatcttcttcctcgagctccctctattgtgagctactttcaactcaccggtggagatgactgactctcaggacattaatattagtgtggaaagaatagctgctcagcgtcagcgagaaacgcgagtgttggaatacctggaactacaacagcttaaggagtcccactggtgtgagaaaggagtgctgtgtcatgttaagcaggcagccctttcctacgatgtcagcgttcagggacatgaactgtcttacactttgcctttgcagaaacaaaccttctgcaccatgatgggctctacctccatcacaatcacccaacaagccgggcctgtagagggggctatcctctgtcactgtcacgcacctgattgcatgtccaaactaatcaaaactctctgtgctttaggtgatatttttaaaatgtaaatcataataaacttaccttaaatttgacaacaattttctggtgacatcattcagcagcaccactttaccctcttcccagctctcgtatgggatgcgatagtgggtggcaaacttcctccaaaccctaaaagaaatattggtatccacttccttgtcctcacccacaattttcatcttttcatagatgaaaagaaccagagttgatgaagacttcaaccccgtctacccctatgacaccacaaccactcctgcagttccctttatatcacccccctttgtaaacagcgatggtcttcaggaaaaccccccaggtgttttaagtctgcgaatagctaaacccctatatttcgacatggagagaaaactagccctttcacttggaagagggttgacaattaccgccgccggacaattagaaagtacgcagagcgtacaaaccaacccaccgttgataattaccaacaacaacacactgaccctacgtcattctccccccttaaacctaactgacaatagcttagtgctaggctactcgagtccgctccgcgtcacagacaacaaacttacatttaacttcacatcaccactccgttatgaaaatgaaaaccttacttttaactatacagagcctcttaaacttataaataacagccttgccattgacatcaattcctcaaaaggccttagtagcgtcggaggctcactagctgtaaacctgagttcagacttaaagtttgacagcaacggatccatagcttttggcatacaaaccctgtggaccgctccgacctcgactggcaactgcaccgtctacagcgagggcgattccctacttagtctctgtttaaccaaatgcggagctcacgtcttaggaagtgtaagtttaaccggtttaacaggaaccataacccaaatgactgatatttctgtcaccattcaatttacatttgacaacaatggtaagctactaagctctccgcttataaacaacgcctttagtattcgacagaatgacagtacggcctcaaaccctacctacaacgccctggcgtttatgcctaacagtaccatatatgcaagagggggaggtggtgaaccacgaaacaactactacgtccaaacgtatcttaggggaaatgttcaaaaaccaatcattcttactgtaacctacaactcagccgccacaggatattccttatcttttaagtggactgctcttgcacgtgaaaagtttgcaaccccaacaacttcgttttgctacattacagaacaataaaaccgtgtaccccaccgtttcgtttttttcagatgaaacgggcgagagttgatgaagacttcaacccagtgtacccttatgaccccccacatgctcccgttatgcccttcattactccaccttttacctcctcggatgggttgcaggaaaaaccacttggagtgttaagtttaaactacagagatcccattactacgcaaaatgggtctcttacagttaaactaggaaacggcctcactctagacaaccagggacaactaacatcaaccgctggggaagtagaacctccactcactaacgctaacaacaaacttgcactggtctatagcgatcctttagcagtaaagcgcaacagcctaaccttatcgcacaccgctccccttgttattgctgataactctttagcattgcaagtttcagagcctatttttataaatgacaaggacaaactagccctgcaaacagccgcgccccttgtaactaacgctggcacccttcgcttacaaagcgccgcccctttaggcattgcagaccaaaccctaaaactcctgtttaccaaccctttgtacttgcagaataactttctcacgttagccattgaacgaccccttgccattaccaatagtggaaagctggctctacagctctccccaccgctacaaacagcagacacaggcttgactttgcaaaccaacgtgccattaactgtaagcaacgggaccctaggcttagccataaagcgcccacttattgttcaggacaacaacttgtttttggacttcagagctcccctgcgtcttttcaacagcgaccccgtactagggcttaacttttacacccctcttgcagtgcgcgatgaggcgctcactgttaacacaggccgcggcctcacagtgagttacgatggtttaattttaaatcttggtaaggatcttcgctttgacaacaacaccgtttctgtcgctcttagtgctgctttgcctttacaatacactgatcagcttcgccttaacgtgggcgctgggctgcgttacaatccagtgagtaaaaaattggacgtgaaccccaatcaaaacaagggtttaacctgggaaaatgactacctcattgtaaagctaggaaatggattaggttttgatggcaatggaaacatagctgtttctcctcaagttacatcgcctgacaccttatggaccactgccgatccatcccccaattgttccatctacactgatttagatgccaaaatgtggctctcgttggtaaaacaagggggtgtggttcacggttctgttgctttaaaagcattgaaaggaaccctattgagtcctacggaaagtgccattgttattatactacattttgacaattatggagtgcgaattctcaattatcccactttgggcactcaaggcacgttgggaaataatgcaacttggggttataggcagggagaatctgcagacactaatgtactcaatgcactagcatttatgcccagttcaaaaaggtacccaagagggcgtggaagcgaagttcagaatcaaactgtgggctacacttgtatacagggtgacctttctatgcccgtaccgtaccaaatacagtacaactatggaccaactggctactcctttaaatttatttggagaactgtttcaagacaaccatttgacatcccatgctgttttttctcttacattacggaagaataaaacaacttttcctttttattttctttttattttacacgcacagtaaggcttcctccacccttccatttgacagcatacaccagcctctcccccttcatggcagtaaactgctgcgagccagtccggtatttgggagttaagatccaaacagtctctttggtaatcagatgtcgatccgtgatggacacaaatccctggggcaggttctccaacgtttcggtgaaaaactgcatgccgccctacaaaacaaacaggttcaggctctccacgggttatctccccgatcaaactcagacagggtaaaggtgcgatgatgttccactaaaccacgcaggtggcgctgtctgaacctctcggtgcgactcctgtgaggctggtaagaagttagattgtccagcagcctcacagcatggatcatcagtctacgagtgcgtctggcgcagcagcgcatctgaatctcactgagattccggcaagaatcgcacaccatcacaatcaggttgttcatgatcccatagctgaacacgctccagccaaagctcattcgctccaacagcgccaccgcgtgtccgtccaaccttactttaacataaatcaggtgtctgccgcgtacaaacatgctacccgcatacagaacctcccggggcagtcccctgttcaccacctgcctgtaccagggaaacctcacatttatcagggagccatagatagccatcttaaaccaattagctaacaccgccccaccagctctacactgaagagaaccgggagagttacaatgacagtgaataatccatctctcataacccctaatggtctgatggaaatccagatctaacgtggcacagcagatacacactttcatatacattttcatcacatgtttttcccaggccgttaaaatacaatcccaatacacgggccactcctgcagtacaataaagctaatacaagatggtatactcctcacctcactaacattgtgcatgttcatattttcacattctaagtaccgagagctctcctctacaacagcactgccgcggtcctcacaaggtggtagctggtgacaattgtagggagccagtctgcagcgataccgtctgtcgcgttgcatcgtagaccagggaccgacgcacttcctcgtacttgtagtagcagaaccacgtccgctgccagcacgtctccaagtaacgccggtccctgcgtcgctcacgctccctcctcaacgcaaagtgcaaccactcttgtaatccacacagatccctctcggcctccggggcgatgcacacctcaaacctacagatgtctcggtacagttccaaacacgtagtgagggcgagttccaaccaagacagacagcctgatctatcccgacacactggaggtggaggaagacacggaagaggcatgttattccaagcgattcaccaacgggtcgaaatgaagatcccgaagatgacaacggtcgcctccggagccctgatggaatttaacagccagatcaaacattatgcgattttccaggctatcaatcgcggcctccaaaagagcctggacccgcacttccacaaacaccagcaaagcaaaagcgttattatcaaactcttcgatcatcaagctgcaggactgtacaatgcccaagtaattttcatttctccactcgcgaatgatgtcgcggcaaatagtctgaaggttcatgccgtgcatattaaaaagctccgaaagggcgccctctatagccatgcgtagacacaccatcatgactgcaagatatcgggctcctgagacacctgcagcagatttaacagacccaggtcaggttgctctccgcgatcgcgaatctccatccgcaaggtcatttgcaaataattaaatagatctgcgccgactaaatctgttaactccgcgctaggaactaaatcaggtgtggctatgcagcacaaaagttccagggatggcgccaaactcactagaaccgctcccgagtagcaaaactgatgaatgggagtaacacagtgtaaaatgttcagccaaaaatcactaagctgctcctttaaaaagtccagtacttctatattcagtccgtgcaagtactgaagcaactgtgcgggaatatgcacagcaaaaaaaatagggcggctcagatacatgttgacctaaaataaaaataaacattaaactaaagaagcttggcgaacggtgggatatatgacacgctccagcagcaggcaagcaaccggctgtccccgggaaccgcggtaaaattcatccgaatgattaaaaagaacaacagaaacttcccaccatgtactcggttggatctcctgagcacacagcaatacccccctcacattcatatccgccacagaaaaaaaacgtcccagatacccagtgggaatatccaacgacagctgcaaagacagcaaaataatccctctgggagcaagcacaaaatcctccggtgaaaaaagaacatacatattagaataaccctgttgctggggcaaaaaggcccgacgtcccagcaaatgcacatatatgtgttgatcagccattgccccgtcttaccgcgtataaagccacgaaaaagtcgagctaaaatccacccaacagcctatagctatatatacactccgcccaatgacgctaacaccgtaccacccacgaccaaagttcacccacacccacaaaacccgcgaaaatccagcgccgtcagcacttccgcaatttcagtctcacaacgtcacttccgcgcgccttttttcactattcccacacccgccctcgcgccaccccgcgtcaccccgcgtcaccgcacgtcaccccggccccgcctcgctcctccccgctcattatcatattggcacgtttccagaataaggtatattattgatgatg

SEQ ID NO: 3 - DNA, 34475 bp, Simian Adenovirus 4312 (sAd4312) Wild Type
catcatcaataatataccttattctggaaacgtgccaatatgataatgagtggggaggagcgaggcggggccggggtggggtgaggcggggccggggtggggtgagggtgacgtcggggcgggcggggcggccgacgtgtgtggggaggcgcgtagtgtttacgtatgcggaaggaggttttataccggaagatgggtaatttgggcgtatacttgtaagttttgtgtaatttggcgcgaaaactgggtaatgaggaagttgaggttaatatgtactttttatgactgggcggaatttctgctgttcagcagtgaactttgggcgctgacggggaggtttcgctacgtggcagtaccacgagaaggctcaaaggtcccatttattgtactcctcagcgttttcgccgggtatttaaacgctgtcagatcatcaagaggccactcttgagtgctggcgagtagagttttctcctccgcgctgccacaatgaggctggtccccgagatgtttggtgttttttgcgacgaggcggcgcggaactcagatgacctgctgaattcagatttgctggaaattcccaattcgcctgtggcttcgcctccgtcacttcacgaccttttcgatgtggaagtggatcctccggcagatcccaacgaggacgcggtaaatagtatgtttcccgaatgtctgttcgaggcggctgacgagggtagcgacagcggtggagagagtggacagggtgaggaactggacttaaaatgctacgaggaatgcataccgtctagcgattctgaaacggaacaaacagggggagatggctgcgctgagccaactgagaaaaatgaacttatattagactgtcctgaacatcctggtcatggctgccgtgcctgtgcttttcatagagatgccagtggaaatcctgaaactctatgtgctctgtgttacctgcgtcttaccggcaattttgtatacagtaagtaggttttttactttgtgtacggtagggaagtttttgtaaagtgtgttatgacttattgcttgtgtaatgttttacaggtgacgtgtctgatgtggaggagggagataagtcagtccatactagttctccttgcactttgggggctgtggttccagataatgttattaaacccgtggcggtcagagtatcaggcaggcggtgtgcagtcgaaaaaattgaagacttgctgcaggaagagcagatgcaacctttggacctgtccctcaaacgccctaagatgacctaagcctgtttattgagtgcaataaaactgttgatctttgaactgtgtttatgtgttgggtgtgtctgtggatatataagcaggtggatgggaagtgagagcacatctgccttgatggatctgttggggaacttgcgggaatttgacgtggttcgtcgcttgctggagttggcctccgacaaaacttccaggctttggaggttttggtttggctcaacgcttagcagcgtagtgtacagggtcaagaaggagcaggaggggcaattttctaggctgttggctgatattcctggagtttttgtggctctggatttaggccatcacagtctttttcaagagaaaattgtcaaaagcttaactttctcgtctcctggccgcacggttgtttcagcagcctttattacctatattttggatcaatggagcagcagcggcagccacctgtcgtgggattacatgctggattacctggcaatggccctgtggagggccatgctgcggaggagggtttgcatttactcgcgggcgcagcctccgcggctggatcgagtggtggaggaggacgagccggacgagaccgagaacctgagagccggcctggaccctccaatggaagactaggtgcagaggataatcctgaagagggaactagtgggggtgctagaaaaaagcaaaaaaccgagactgagcctagaaactttttgaatgagctgactgtgagtttgatgaatcgccatcgtcccgagacaattttctggtctgagttggaggaagagtttaggaagggggatttgaacctgctgtacaagtatgggttcgaacagttgaagactcactggttggagccgtgggaggattttgaaaccgctctggacacttttgctaaagtggctttgcggccggataaagtttatactatccgctgcactgttaatataaggaaaagtgtttatgttataggccatggagcactggtgcaggtggagaccgccgatcgggtggctttcaactgcggcatgcagaatctgggccctggggtgataggtgttaatggtgtcacgtttcagaacgtgaggttcgcgggtgaaagctttagcggctccgtgtttgcaaataacacacagctcactctccacggcgtttacttttttaactttaacaatacatgtgtggagtcgtggggcagggcgtccttgaggggctgcacttttcacggttgctggaaggcggtggtgggaagactgaaaagtgtaacgtctgtgaaaaaatgcatattcgagcggtgtgtgctagctgtaaccgtggaagggcatggacgcattagaaacaacgcagcgtctgagaatgggtgttttcttttactgaaaggcacggccagcgttaagcataacatgatctgtggcagtgggctgtacccgtcgcagttgttaacctgcgcggatggaaactgccagacattgcgcaccgtgcacatagtgtctcacccgcgtcgccactggccaacgtttgagcacaacttgcttatgcgttgtacggtccatctggggcctagacggggcatgtttgtgccttttcagtgtaactttagccacactaagatcttactagaagcagatgccttcactcgagtgtgtttcaatggggtgtttgacatgtcggtggaaatttttaaagtgataagatatgatgaatccaagtctcgttgtcgcccctgtgaatgcggagctaatcatttgaggttgtatcccgcgaccctgaacgtaaccgaggagctgagggccgaccaccacatgttgtcctgcttgcgcaccgactatgagtccagcgacgaagagtgaggtgaggggcggagccacaaagggtataaagggtcaggatgggtgggcacaggtattcaaaatgagcgggacgacggacggcaacgcgtttgaggggggagtgttcagcccatatctgacatctcgtcttccttcctgggcaggagtgcgtcagaatgtagtgggctccaccgtggacggacggccggtcgcccctgcgaattccgccacccttacctatgccaccgtgggatcaccgttggacactgccgcggcagccgcagcttctgctgccgcttctactgctcgcggtatggcggctgactttggactttataaccaactggctaccgcggctgtggcatctcgcactctggttcaagaagatgccctgagcgtggttctgcttcgactggaagatctgtctcgtcgcttggatcagctggctgcgcagatatccccacctaaccccgatactactcaagaatcttaaataaagacaaacagatttgttgaaaataaatggctttatttgttttttttggctcgataggctcgggtccacctgtcccggtcgttaaggactttgtgtatgctttccaagacccggtacagatgggcttggatgtttagatacatgggcatgaggccatcccgggggtggagataggaccattgcagagcgtcatgctccggggtggtgttgtagatgacccagtcgtagcagggtttttgggcgtggaactgaaaaatgtccttgagaagcaggctgatggccaggggcagacccttagtgtaggtgttcacaaagcggttgagctgggagggatgcatgcggggagagatgatatgcatcttagcctggattttcaggttagctatgttgccccccaggtcccttcgagggttcatattgtggaggaccaccagaacggtgtagccggtacacttgggaaacttatcgtgcagtttggaggggaaggcgtgaaagaatttggaaacccctttgtgaccacctaagttttccatgcactcgtccatgataatggcgatgggccccttggcggcagctttagcgaacacgttgtgggggttggaaacatcatagttttgctctagagttagctcgtcataggccatttttacgaagcggggtaggagggtgccagactgagggacgatagttccatctggccccggtgcgtaattaccctcgcagatctgcatctcccaagctttaatttccgagggagggatcatgtccacctggggggcgataaagaacacggtttctggcgggggattaatgagctgggtggaaagcaggttgcgcaagagctgagacttgccgcaaccggtgggaccgtagatgaccccgatgacgggctgcagctggtagttgagagaggagcagctgccgtcggggcgtaggaggggagccacctcgttcatcatgcttcttacatgtttattttcactgactaagctttgcaagagcctctccccacccagggacaagagttcttccaggctgttgaagtgtttcagcggtttcaggccgtcggccatgggcatcttttcaagcgactgacgaagcaagtacagccggtcccagagctcggtgacgtgctctatggaatctcgatccagcagacttcttggttgcgggggttgggccgactttcgctgtagggtacgagccggtgggcgtccagggccgcgagggttttgtccttccagggtctcagcgtccgggtgagggtggtctcggtgacggtgaacggatgagccccgggctgggcgcttgccagggtgcgcttcaggctcatccggctggtgctgaagcgggcgtcgtctccctgggaatcggccagatagcaacggagcatgaggtcgtagctaagggattcggccgcgtgtcccttggcgcgcagttttcccttggaaacatgctggcatctggtgcagtgtaaacacttgagggcgtacagcttgggggcgaggaagacggactcgggcgagtaggcgtcggccccgcactcggcgcagacggtttcacactccaccagccacgtgagctcgggtttgtcggggtcaaaaaccaggttgcctccattttttttgatgcgtttcttaccttgcgtctccatgagcctgtgacccgcttcggtgacaaaaaggctgtctgtgtctccgtagaccgacttgagggggcgttcttccaagggcgtgccgcggtcttctgcgtacaaaaactgggaccactccgaaacgaaggccctggtccacgctaacacgaaggatgcgatctgcgaggggtatctgtcgttctcaatgaggggatccaccttttccagggtatgcagacacaggtcgtcctcctccgcgtccacaaaggtgattggcttgtaagtgtaggtcacgtgaccggcgccccccggaggggtataaaagggggcgtgcccaccctccccgtcactttcttccgcatcgctgtggaccagagccagctgttcgggtgagtaggccctctcaaaggccggcatgacttcggcactcaagttgtcagtttctacaaacgaggaggatttgatgttcacgtgccccgcggcgatgcttttgatggtggagtggtccatctggtcagaaaacacgatctttttgttgtcaagtttggtggcaaaagacccatagagggcgttggaaagcaacttggcgatggagcgcagggtctgatttttttcccgatcggccctttccttcgcggcgatgtttaattgcacgtactcgcgggccacgcatcgccattccgggaacacggcggtgcgctcgtcgggcaggatgcgcacgcgccagccgcgattgtgcagggtgatcatgtccacgctggtggccacctccccccggaggggctcgttggtccaacacaatctccctccttttctggagcagaacggagggaggggatctaggaggttggcgtgcggggggtcggcgtcgatggtgaagatgccaggcaggagaactttattaaagtaatcgatctcggtttccacgtcttgcaacgcctcctcccatctctttaccgccagggccctctcgtaggggttcaggggcgccccccagggcatggggtgggtgagagccgaggcgtacatgccacagatgtcatagacgtagaggggctcccgtaggaccccgatgtaagtgggataacagcgccccccgcggatgctggcccgcacgtagtcgtacatctcgtgagatggggccaggagaccctctcccaagtgggtcttgtggggcttctccgcccggtagaggatctgcctgaagatggcgtgggagttggaagagatggtgggccgttggaagacgttaaagttggcccgcggcagccccaccgagtcttcgatgaactgggcgtaggattcctggagtttgttcacgagggcggcggtgaccagcacgtccagggcgcagtaatccagggtctcgcggaccaggttgtaggagctctcttgttttttctcccacagttcgcggttgaggaggtattcctcgcggtctttccagtactcttcggcgggaaatcctttttcgtccgctcggtaagaacctaacatgtaaaactcgttcaccgctttgtatggacaacagcctttctctaccggcagggcgtacgcctgagcggcctttctgagagaagtgtgggtgagggcgaaggtgtcccgcaccatgactttcaggtactgatgtttgaagtccgtgtcgtcgcagcttccttgttcccacaggctgaagtcggtgcgctttttctgcctcgggttggggagggcgaaagtgacatcgttaaacaagattttcccggcgcggggcataaagttgcgagagattctgaagggccctggcacgtccgagcggttgttgatgacctgcgccgccaggacgatctcgtcgaagccgttgatgttatgccccacgatgtacagttctatgaagcgcggctgtcccttgagggcgggcgcttttttcagttcctcgtaggtgagggactcgggagaggcgagccccagctccgcgcgggcccagtcggccagttgagggttagccgcgaggaaggaattccagagctccgaggccagaagagtttgcaagcgatcgcgaaactcgcggaactttttccccacggccattttttctggcgtgaccacgtagaaagtggcggagcgatcgttccagacgtcccacttgagctcccgggccagctcgcaggcctgacgcacgagagtttcctcgcccgagacgtgcatgaccaacatgaaaggcactaactgttttccgaacgcgcccatccacgtgtaggtctctacatcgtaggtgacaaagagccgttgggtgcgtgcgtgggagccgatcggaaagaagctgatctcctgccaccagctggaggaatgggtgttgatgtggtgaaagtagaagtcccgccggcgcacagagcattcgtgctggtgtttgtaaaagcgaccgcagtagtcgcagcgctgcacgctctgtatttcttgaatgagatgcacttttcgcccgcgaaccagaaatcggaggggaaagttgagcccgggggatggtggagtcgcgtccccttcgccttggcggtgggcgtctgcgtctgcgtcctgtttttctgggtggacgacggtggggacgacgacgccccgggttccgcaagtccagatttcagcgacggaggggcgcagacgcagaaggagggggcgcagttgcccgctgtccagagagtcgaggaaagcgacgctgaggtcagcggggagcgtttgcaaattcactttcaagagaccggtaagagcgtgagccaggtggagatgatacttgatttccaggggggtgttggaagaggcgtccacgccgtacaagaggccgtgtccgcgcggagccaccacggttccccgcggaggttttatctcactcgccgagggcgagcgccggggggtagaggcggctctgcgccgggtggtagcggaggcagaggcacgttttcgtgaggattcggcagcggctgatgacgcgctcggagactgctggcgtgggcgacgacgcggcggttgaggtcctggatgtgctgcctctgcgtgaagaccaccggtcccctggtcctgaacctgaaagagagttccacagagtcaatgtctgcatcgttaacggccgcctgcctgaggatctcctgcacgtcgcccgagttgtcttggtaggcgatctcggccatgaactgttcgacttcttcttcgcggaggtcgccgtggcccgcgcgttctacggtggcggccaggtcgttagagatgcgacgcatgagctgggagaaggcgttgaggccgttctcgttccacacgcggctgtacaccacgttaccgaaggagtcgcgcgctcgcatgaccacctgcgccacgttgagttccacgtggcgggcgaagacggcgtagtttctgaggcgctggaagaggtagttgagcgtggtggcgatgtgctcgcagacgaagaagtacatgatccagcgcctcagagtctgctcgttgatgtctccgatggcttcgaggcgttccatggcctcgtagaagtcgacggcgaagttgaaaaattgggagttgcgggcggccaccgtgagttcttcttgcaggaggcggatgagatcggcgacggtgtcgcgcacctcctgttcgaaagcgccccgaggcgcctctgcttcttcctccagctcctcctcttccaggggcacaggttcctccggcacctctgcggcggggacggggcggcgacgtcgtcgtctgaccggcagtcggtccacgaagcgttcgatcatttcaccgcgccggcgacgcatggtctcggtgacggcgcgtccgttttcgcggggacgcagttcgaagacgccgccgcgcagagcgcccccgtgcagggagggtaagtggttagggccgtcgggcagagacacggcgctgacgatgcattttatcaattgttgcgtaggcactccgtgcagggatctgagaacgtcgaggtcgacgggatccgaaaacttctctaggaaagcgtctatccaatcgcaatcgcaaggtaagctgaggacggtgggccgctggggggcgtccgcgggtagttgggaggtgatgctgctgatgatgtaattaaagtaggcggttttcaggcggcggatggtggcgaggaggaccacgtctttgggcccggcctgttgaatgcgcaggcgctcggccatcccccaggcctcgctctgacagcgacgcaggtctttgtagtagtcttgcatcagtctctccaccggaatctctgcttctcccctgtctgccatgcgagtcgagccgtacccccgcaagggctgcagcaacgctaggtctgccactactctttcggccagcacggcctgttgaatctgcgtgagggtggcctggaagtcgtccaggtccacgaagcggtggtaggctcccgtgttgatggtgtaggtgcagttggccatgacggaccagttgacgacttggatgccgggttgggtgatctccgtgtacttgaggcgcgagtaggccctggactcgaacacgtagtcgttgcatgcgcgcaccagatactggtagccgacgagaaagtgcggaggcggttcccgatacaggggccagcccacggtggcgggggctccgggggccaggtcttccagcatgaggcggtggtagtggtacacgtatcgagagagccaggtgatgccggctgaggtggtggcggccctggtgaactcgcggacgcggttccagatgttgcgcagggggcggaagcgttccatggtgggcacgctctgtcccgtcaggcgcgcgcaatcctgtacgctctagatggagaaaagacagggcggtcatcgactcccgtccgtagctgggaggtaaagtcgcaagggtgcggcggcggggaaccccggttcgagaccggctggatccgccgttcccgatgcgcctggccccgcatccacgacgttcgcgccgagacccagccgcggcacaccgccccaatacggaggggagtcttttggtgttttttcatagatgcatccggtgctgcgacagatgcgaccccagacgcccactgctactaccgccgcggcggcagtaaacctgagcggaggcggtgacagggaggacgaagagctggctttagacctggaagagggagagggtctggcgcgactgggcgccccctcccccgagagacaccccagggtccagctcgtgagggatgcgagacaggcttttgtaccgcggcagaacctgtttagggaccgcagcggccaggaggcggaggagatgcgcgattgtcggtttcgggcgggcagagagctgagggcggggttcgaccgggagcggttgctgcgggcggaggatttcgaacccgacgagcggtcgggggtgagtccggcccgagcccacgtgtcggccgccaacctggtgagtgcgtatgagcagacggtgaacgaggagcgtaactttcaaaagagctttaataatcacgttcggaccctcatcgcgagggaggaggtggccatcgggctgatgcatctgtgggacttcgtggaggcctacgtgcagaacccggcgagcaagcccctgacggctcagctgttcctgatcgtgcagcacagccgcgacaacgagacgtttcgcgacgccatgctcaacatcgccgagcccgagggccgctggctcttggatcttatcaacatcttgcagagcatcgtggttcaggagaggggtctcagcttagcggacaaggtggcggccattaactactccatgcagagtctgggaaaattctacgctcgcaagatctacaagagcccctacgtgcccatagacaaggaggtgaagatagacagcttttacatgcgcatggcgctgaaggtgctgacgctgagcgacgatctcggcgtgtaccgtaacgacaagatccacaaggcggtgagcgccagccgccggcgggagctgagcgatagggagctgatgcacagcctgcagagggcgctggcgggtgccggggacgaggagcgcgagacttacttcgatatgggagcggacttacagtggaaacccagcgcccgagcgttggaggcggcgggctaccgtggcgacgaggatcgggatgactttgaggaggcaggcgagtacgaggacgaagcctgaccgggcaggtgttgttttagatgcagcgtccggcggacggggccaccgtggatcccgcgcttttggcatccatgcagagtcaacctacgggcgtgaccgcctccgatgactgggcggcggccatggaccgcatcatggcactgaccacccgcaaccccgaggcttttaggcagcaaccccaggccaaccgtttttcggccatcttggaagcggtagtgccgtctcgcactaatccgacccacgaaaaggttttaactatcgtgaacgcgctggtagacagcaaggccatccgccgcgacgaggcggggctgatttacaacgctctgctggaacgcgtggcgcgctacaacagcactaacgtgcagaccaatctggaccgcctcaccacggacgtgaaggaagcgttggctcagaaggagcggttcttaagggacagcaatctgggttctctggtggcgctgaacgcttttctgagcacgcagccggcgaacgtaccccgcgggcaggaggactacgtgagcttcatcagcgctctgagactgctcgtttccgaggtgccgcagagcgaggtgtaccagtcgggacctgactacttcttccagacgtcccgacagggcttgcaaacggtgaacctgactcaggcttttaaaaacttgcaaggcatgtggggcgtgaaggcgccggttggcgatcgcgcgaccatttccagcctgctgacccccaacacgagactgctgttgcttttaatcgccccgttcaccaacagcagcaccatcagccgcgactcgtacctgggccatctcatcactctgtaccgagaggccataggtcaggctcagattgacgagcatacgtatcaagagatcaccaatgtgagccgagccctgggtcaggaagacaccggcagtttggaagccacgctaaactttctgctgaccaatcggagacaaaagattccctcgcagtacacgttaagcgccgaggaggagaggattctgcgctacgtgcagcagtccgtgagcctgtacttgatgcgggagggtgctaccgcttccacggccttggacatgacggctcgaaacatggaaccgtctttttactcagcccaccgtccgttcatcaatcgcctgatggactacttccatcgcgcggccgccatgaacggggagtatttcaccaatgccatcttgaatccgcattggatgcctccgtccggtttctacaccggggagttcgacctgcccgaggccgacgacggctttctgtgggacgatgtgtccgacagcatttttacgccaggtaacagtcgtttccataaaaaggaagggggagacgaacttcccctttcgagtgtggaggcggcctccaggggggagagccccttttccagcttgtcttccgtgagtagcggtcgggtgacgcgcccacgcttgccgggggagagcgactacctaaacgaccctttgctgcgaccggctaaaaagaaaaattttcccaacaacggggtggaaagcttggtggataaaatgaatcgttggaagacctacgctcaggagcagcgggagtgggaggacagtcagccccgaccgctggtcccgccgcactggcgccgccagagagaagacccggacgactccgcagacgatagtagcgtgttggacttgggagggagcggagccaacccctttgctcacttgcaacccaaggggcgcttgagtcgcctgtactaataaaaagaaagcggaaacgtaccagagccatggccacagcgtgtgtcctttcttcctctctttcctcctcggcgcggcagaatgagaagagcggtgagagtcacgccggcggtgtatgccgagggtccgcccccttcttacgaaagcgtgatgggatcagcgaacgtgccggccacgctggaggcgccttacgttcctcccagatacctgggacctaccgagggcagaaacagcatccgttactccgagctggcccccctgtacgataccaccaaggtgtacctggtggacaacaagtcggcggacatcgcctccctgaattaccaaaacgaccacagcaacttcctgaccaccgtggtgcagaacaatgacttcaccccgacggaggcgggcacgcaaaccattaactttgacgagcgttcccgctggggcggtcagctgaaaaccatcctgcacaccaacatgcccaacatcaacgagtttatgtccaccaacaagtttagggccaggttgatggtagagaagactagcggccagccgcccaaatacgagtggttcgagttcaccattcccgagggtaactactccgagaccatgactatcgatctcatgaataacgcgatcgtggacaattacctgcaagttggaaggcaaaacggggtattggagagcgacataggagtaaaatttgataccaggaacttccgactggggtgggatccggtgaccaagctggtgatgcctggcgtgtacaccaacgaggcttttcaccccgatatcgtgctgcttccggggtgcggagtggactttacgcagagccgcttgagtaacctgttaggaatcaggaagcgccgtccctttcaggagggctttcagattatgtatgaggacttggagggaggtaatattccaggcctgctagacgtgccggcctatgaacaaagcttacaacaggcccaagaggagggaagagtcactcgcggagacacctttgccacggctcccaacgaggtagtgattaagcccttattgaaagacagtaaggatagaagttataatattataaccgacaccacggacactttgtaccggagttggtttctggcttacaactacggggaccccgaaaacggagtgagatcatggaccatactcaccaccacggacgtgacctgcggctcgcagcaagtgtactggtccctgccggatatgatgcaagacccagtcaccttccgcccctccacccaagtcagcaactttccggtggtgggcactgagctgttgcccgttcacgccaagagcttctacaacgagcaggctgtttattcgcaactcattcgccagtctaccgcgcttacccacgtattcaaccgtttccccgagaaccagattctcgtgcgccctcccgctcctaccattaccaccgtgagtgaaaacgttcccgccctcacagatcacggaaccctgccgctgcgcagcagtatcagtggagttcagcgcgtgaccatcaccgacgccagacgtcgaacctgcccttacgtttacaaagcgctcggcgtagtggccccaaaagtgctctctagtcgcaccttctaaaacatgtccattctcatctctcccgataacaacaccggctggggactgggctccggcaagatgtatggcggggcgaagcggcgctccagtcagcaccctgttcgcgttcggggtcatttccgcgctccctggggagcttacaaacgaggactctcgggccgaacggcggtagacgacaccattgacgccgtcattgccgatgcccgccggtataaccccggaacggtcgctagcgccgcctccaccgtggattccgtgatcgacagcgtggtggccggcgccagggcctacgctcgccgcaaaaggcggctgcaccgcaggcgtcgacccacggccgccatgctggccgccagggccgtgctgagacgggcccgcagggtaggcaggagggccatgcgccgcgcggccgccaacgctgccgccgggagggcccgcaggcaagccgccagccgggccgccgccgccatcgctaacatggccagacccaggagagggaacgtttactgggtgcgcgattctgtgacgggagtcagagtgccggtgcgcagccgacctccccgaagttagaagaccaaaggtgcgaagacggcgtactgagtctccctgttgttatcagcccaacatgagcaagcgcaagtttaaagaagaactcctgcagaccctggctcctgaaatctatggccctccggacgtgaagcccgacattaagccccgcgatatcaagcgtgttaaaaagcgggaaaaaaaagaggaactcgcggtggtagacgatggcggggtagaatttattagaagtttcgccccgcgacgcagggtgcagtggaaagggcggcgcgtgcaacgcgttctcaggccaggcaccgcggtagtttttactccgggagagcggtcggctgtcaggggtttcaagcggcaatatgacgaggtgtacggcgacgaagacatcctggaacaggcggctcagcagattggagaattcgcctacggaaagcggtctcgccgcgaagacctggccattgccttggacagtggcaaccccacccccagcctcaaacccgtcacgctgcagcaggtgctccccgtgagcgcgagcacggagagcaaaaggggaatcaagagagagatggaagatctgaagcccaccatccaacttatggtccctaaacgacagaagctggaggaggttctggaaaacatgaaagtggaccccagcatagagccggatgtaaaagtgaggcctattaaggaagtggctccgggtctcggggtgcaaacggtggacattcagatcccagtcagatccgcttcgaccgccgtggaagccatggaaacgcaaaccgaaactccggtcgcggccggtaccagagaagtggctttgcaaacggagccctggtacgaatacaccgctcctcggcgccagaggcggcgttacggcccggcaaatgccatcatgccagagtatgcgctgcacccgtctatccgacccacccccggctaccggggggtaacgtatcgcccgtcgccaacccgacgccgttatcgtcgccgccgccgttctcgtcgcgctctggcgcccgtgtccgtgcgacgcgtaacgcgccggggaagaacagtcaccatccctaacccgcgctaccaccctagcattctttaatgactctgccgttttgcagatggctctgacttgccgcgtgcgccttcccgttctgcactatcgaggaagatctcgtcgtaggagaggcatggcggggagcggccgccgtcgggctttacgcaggcgcatgaaaggcggaattttgcccgcactgattcccataattgccgccgccattggggcgatacccggcgttgcttcagtggccttgcaagcagctcgtaataaataaacgaaggcttttcaacttatgacctggtcctgactattttatgcagaaaaagcatggaagacatcaattttacgtcgctggctccgcggcaaggctcacgcccgctcatgggcacctggaacgacatcggcagcagccagctcaacgggggcgctttcaattgggggagcctttggagcggcattaaaaactttggctccgcgattaaatcctacggcagcaaagcctggaacagtagtactggtcagatgctccgggataaactgaaggacacaaactttcaagagaaagtggtcaacggggtggtgaccggcatccacggcgcggtggatctcgctaatcaagcggtgcaaaaagagatagacagacgatgggaaaactcgcgggtgcctccgcagagaggggacgaagtggaggtggaggaagtagaagtcgaggagaaactgcccccgctagagaaagttcccggggcgccgcccaggccacagaagcgtccccggccggatctggaagaaactttagtgacggaaaccatcgaacctccctcgtacgaacaagctttaaaggagggcgcctctccttaccccatgactaagcccatcgcgcccatggcgcgtccggtgtacggaaaagatcacaagccagtaacgttagagctacccccaccacccccttcccgtcctacggtgcctccgttacccgccccgtcggcaggtcccagctctgcaccatccgcagctcctgcaccaaccgctcgcccggtggccgtggcaaccgccagagcccccagaggatccaactggcaaagcacgctgaacagcatcgtgggcttgggagtgaaaaccctaaaacgccgccgctgctattattaaagagtgtagctaaaaatttcccgttgtatacgcctcctatgttaccgccagagacgcgtgactggtcgccgctccgccgctttcaagatggccaccccatcgatgatgccgcagtggtcttacatgcacatcgccggccaggacgcctcggagtacctgagtcccggcctggtgcagtttgcccgcgccaccgaaagctacttcagcttgggaaacaagtttagaaaccccaccgtggcccccacgcacgatgtaaccacggaccgctcgcagaggctgacactgcgcttcgtgcccgtagaccgggaggacaccgcgtactcctacaaagtgcgcttcaccctcgccgtaggggacaacagggtgctggacatggccagcacgtactttgacatccggggaatgctggaccgagggcccagctttaaaccctactcgggaactgcctacaattcgctggcacctaagggcgctcccaaccctagtcaatggactactaccaacggagggaataaaacaaattcatttgcccaagcatcctacataggtcaaagcctgtcgaaagacggggtgcaagtagcagtagatacagccgctgggggggctgcagtatatgctgacaaaacgtttcaaccagaaccccaagtaggaatatcacaatggaatgaaaatcctactacaaatgctgcaggaagaattttaaagcctactaccgcaatgcgtccatgctacggttcatacgcttaccccaccaacgaaaaaggtgggcaggtaaaaatcactgaccctaacaatgacaaaaccggcgctaataacgttagcttaaattttttcaacactgccgctgacaatgggaataacaatccaaaagtagtactctacagcgaagatgtaaatttagaagggccagatacccaccttgtttttaagccagatgtaactggcgacgcaaccagtgcagaaaccctgttaggtcaacaagcagctcccaatcgtccaaactacattgggttcagggacaactttattggcctgatgtactacaattcaactggaaacatgggagtgctagcaggtcaggcttctcagctaaacgccgtagtggatcttcaagacagaaataccgaattgtcatatcagctaatgcttgacgctttgggtgacagaagtcggtacttttctatgtggaatcaagcagtggacagctacgatcctgacgttagaatcatagaaaatcatggagtagaagacgaacttccaaattattgttttccgttaaatggacaggggatttcgaatacatacaaaggtgtgaaatataacacaaacacttggacgcaagacactgatgtagtcacaaccaatgaaatttccattggcaacatttttgccatggaaataaacctggcggctaacttgtggcgcagctttctgtactccaatgtcgccctgtacttgccagattcctacaaatacactcccgacaatattgaacttcctacaaacaagaacagctacggctacattaacggaagggtaaccgcccccactgccatcgacacttacgttaacatcggcgcccggtggtctccggaccccatggacaacgttaaccctttcaaccaccaccgcaacgccggcttgcgataccgctccatgctgctgggcaacggtcgctacgtacccttccacattcaggtgccccagaaattttttgccattaaaaacctgcttctgcttcccgggtcctacacctacgagtggaacttcaggaaagatgtaaacatgatcttgcagagcaccttgggcaacgacctccgcgttgacggagctagcgtgaggtttgacagcattaacctctacgctaacttcttccccatggcccacaacacggcctccaccttggaagccatgctgcgcaacgacaccaacgaccagtcctttaatgattacctgtgcgcggccaacatgctgtaccccatccccgccaatgccaccagcgtgccgatctccattccctcacgcaactgggccgccttcagaggttggagtttcactcgcctgaaaaccaaggagaccccctcgctgggctccggtttcgacccatactttgtttactccgggagcattccctacctggacggaactttctacctgaaccacaccttcaaaaaggtgtctattatgtttgactcctccgtgagctggcccggtaacgaccgcttgctaacccccaacgagttcgaaatcaaacgctcggtggacggagagggttacaatgtagcccagagcaacatgaccaaagactggtttttaattcaaatgctaagccactataacattggctaccaaggattctacgtgcctgaagcctacaaggacagaatgtactccttctttagaaacttccaacccatgagccgccaggtagtagacacggtaaactatgctaactacaaggaagtaacaatgccattccagcacaacaactcaggcttcgtggggtacatgggacctaccatgagagaggggcaggcctacccggctaattatccctaccccctaatcggagccactgccgtgcccagcctgacacagaaaaagtttctctgcgatcgaacaatgtggaggattcccttctctagcaacttcatgtccatgggggctctcaccgacctggggcagaacatgctgtacgctaactccgctcacgccttggacatgacctttgaggtggaccccatggatgagcccacgcttctctatgttctgtttgaagtcttcgacgtggtgcgcattcaccagccgcaccgcggcgtcatcgaggccgtctacctgcgcacacctttctctgccggtaacgccaccacctaagaagctgatgggctccagcgaacaggagctgcgggccattgttcgcgacctgggctgcgggccctactttttgggcaccttcgacaagcgcttccccggcttcatgtccccccacaagccggcctgcgccatcgtcaacacggccggacgcgagaccgggggggttcactggctcgcctttgcctggaacccgcgtaaccacacctgctacctgttcgacccttttggtttttctgacgaaaggcttaaacagatttaccagttcgagtacgaggggctccttaaacgcagcgctctggcctccacgcccgaccactgcgtcaccctggagaagtccacccaaacggttcagggtcccctctcggcggcctgcggactcttttgttgcatgtttttgcatgctttcgtccactggccgaacacccccatggaccgcaaccccactatggatctgctcacgggagtgcctaacagcatgcttcacagccctcaggtcgcacccaccctgcgtcgcaatcaggaacagctgtatgcttttctgggaaaacattctgcctactttcgccgccaccggcagcgcatagaacaggccacggcctttgaaagcatgagtcaaagagtgtaatcaataaaatcaacttttattttacatcacacgcgcttctggcgttttcttaaaaatcaaagggttcgggggaggggtcgtcgtgcccgctgggcagggacacgttgcgatactggaagcgggggctccagcggaactcggggatcgccagccggggcagaggcacttcttccaggttctgcttccaaaactgccgcaccagctggagggctcccattacgtcgggcgccgagatcttgaagtcgcagttggggcccgagcttccgcggctgttgcgaaacacggggttggcacactggaacaccagcacgctcgggtagttgatactggccagggccgttgcgtcggtcaccgccgttacatccagatcctccgcgttggtcagggcgaagggagtcagcttgcacatctgccgcccgatgtggggcacgccgtcatgcttgttgaggcagtcgcaacgcaggggaatcagaatgcgatgctggccgcgttgcatctgagggtagttggcccgcaagaacgcttccatctgacggaaggccgtctgggctttcattccctcggtgtagaaaagaccgcaggacttgctagaaaatacattattgccgcaggtgacgtcttccgcgcagcagcgggcgtcttcgttctttagctgcaccacgttgcgaccccaccggttctgtaccaccttggccctcgtgggctgctccttcagcgcccgctggccgttttcgctggtcacatccatttccaacacgtgctccttacacaccatttccactccgtggaagcagaacaggacgccctcctgctgggtattgcgatgctcccacacggcgcagcctgtggcctcccagctcttatgcttcacccccgcgtagttttccatgtaagccatcaggaatctgcccatcatctcggtaaaggttttctgactggtgaaggtcaaaggcaagccgcggtgctcttcgttcagccacgtttgacagatcttgcggtacgtggcgccctgatccggcagaaacttaaacgcccccttgctctcgttgtccacgtggaacttttccatcagcattagcataacttccatacccttctcccacgccgtcaccagcggtgtgctgtcggggttcttcaccaacatggtagaagggccctcgccggccctgaagtcgctcatactcattttttgaaactccacagtgccgtccgcacgacggacccggcgcatcggagggtagctgaagccaacctccaccagggtgccttcgctctcgctgtcggagacgatctccggggagggcggcggcgcgggtgtcgacttgcgagccttcttcttgggaggaagcggtggcgcctcttggtcgcgctcgggactcatctccctcaagtagggggtgatggagcttcctgcttggttctgacggttggccattgtatcctaggcagaaacacatggagcttatgcgcgaggaaactttaaccgccccgtcccccgtcaacgacgaagaggtcatcatcgaacaggacccgggctacgttactccgcccgaggatctggaggggcctttagacgaccggcgcgacgctagtgagcagcaggaaaatgagaaagaggaagcctgctacctcctggaaggcgacgtgttgctaaaacatttcgccaggcagagcaccatagtgaaggaggctttgcaagaccgctcggaggtgcccttggacgtcgccgcgctctcccaggcctacgaggcgaacctcttctcgccccgagtgcctccgaagagacagcccaacggcacctgcgagcccaacccgcgccttaacttctaccccgtgttcgccgtgcccgaggcgctggccacctaccacatttttttcaagaaccagcgcatcccgctctcgtgccgggccaaccgcaccgcggccgatagaaagctgagactcaaaaacggagctagcatacctgatatcacgtccctggaggaagtgcctaagatcttcgaaggtctgggtcgagacgagaaacgggcggcaaacgctctgcagaaagaacagaaggacagtcagaacgtgctggtggaactggagggggacaatgcgcgtctggccgttctcaagcgctgcatagaagtttcccacttcgcctaccctgccctgaacctgccgcccaaagtcatgcgctcggtcatggaccagctgctcatcaagagagctgagcccctgaaccccgagcaccccgaggcggagaactcggaggacggaaagcccgtcgtcagcgacgaggagctcgagcggtggctggacagcacggaccccgagcagttgcaagagcggcgcaaaatgatgatggcggccgtcctggtcaccgttgagctggagtgcctgcagcggttttttagcgacgtggaaacgctgcgtaaaatcggagagtccctgcactacaccttccgccagggctacgtccgccaggcctgcaagatctccaacgtggagctcagcaacctggtctcctacatgggcatcctccacgagaaccggctgggacagagcgtgctgcactgcaccttgcaaggcgaggcgcggcgggactacgtgcgagactgcgtctacctcttcctcactctcacctggcagaccgccatgggagtgtggcagcagtgcttggaagacagaaacctcaaagagctagacaaactcctctgccgccagcggcgcgccctgtggtccggtttcagcgagcgcacggtcgccagcgctctggcggacatcatcttcccggagcgcctgatgaaaaccttgcaaaacggcctgccggatttcatcagtcaaagcattttgcaaaacttccgctcttttgtcctggaacgctccgggatattgcccgccatgagctgcgcgctaccttctgactttgtccccctctcctaccgcgagtgccctcccccactgtggagccactgctacctcttccaactggccaactttctggcctaccactccgacctcatggaagacgtaagcggagagggtttactggagtgccactgccgctgcaacctgtgcaccccccacagatcgctggcctgcaacaccgagctactcagcgaaacccaggtcataggtaccttcgagatccaggggccccagcagcaagagggtgcttccggcttgaagctcactccggcgctgtggacctcggcttacttacgcaaatttgtagccgaggactaccacgcccacaaaattcagttttacgaagaccaatctcgaccaccgaaagcccccctcacggcctgcgtcatcacccagagcaagatcctggcccaattgcaatccatcaaccaagcgcgccgcgatttccttttgaaaaagggtcggggggtgtacctggacccccagaccggcgaggaactcaacccgtccacactctccgtcgaagcagcccccccgagacatgccgcccaagggaaccgccaagcagctgatcgctcggcagagagcgaagaagcaagagctgctccagcagcaggtggaggacgaggaagagatgtgggacagccaggcagaggaggtgtcagaggacgaggaggagatggaaagctgggacagcctagacgaggaggaggacgagctttcagaggaagaggcgaccgaagaaaaaccacctgcatccagcgcgccttctctgagccgacagccgaagccccggcccccgacgcccccggccggctcactcaaagccagccgtaggtgggacgccaccgaatctccagcggcagcggcaacggcagcgggtaaggccaaacgcgagcggcgggggtattgctcctggcgggcccacaaaagcagtattgtgaactgcttgcaacactgcgggggaaacatctcctttgcccgacgctacctcctcttccatcacggtgtggccttccctcgcaacgttctctattattaccgtcatctctacagcccctacgaaacgctcggagaaaaaagctaaggcctcctccgccgcgaggaaaaactccgccgccgctgccgccgccaaggatccaccggccaccgaagagctgagaaagcgcatctttcccactctgtatgctatctttcagcaaagccgcgggcagcaccctcagcgcgaactgaaaataaaaaaccgctccttccgctcgctcacccgcagctgtctgtaccacaagagagaagaccagctgcagcgcaccctggacgacgccgaagcactgttcagcaaatactgctcagcgtctcttaaagactaaaagacccgcgctttttccccctcggccgccaaaacccacgtcatcgccagcatgagcaaggagattcccaccccctacatgtggagctatcagccccagatgggcctggccgcgggggccgcccaggactactccagcaagatgaactggctcagcgccggcccccacatgatctcacgagttaacggcatccgagcccaccgaaaccagattctcttagaacaggcggcaatcaccgccacaccccggcgccaactcaacccgcctagttggcccgccgcccaggtgtatcaggaaaatccccgcccgaccacagtcctcctgccacgcgacgcggaggccgaagtcctcatgactaactctggggtacaattagcgggcgggtccaggtacgccaggtacagaggtcgggccgctccttactctcccgggagtataaagagggtgatcattcgaggccgaggtatccagctcaacgacgagacggtgagctcctcaaccggtctcagacctgacggagtcttccagctcggaggagcaggccgctcttccttcaccactcgccaggcctacctgaccctgcagagctcttcctcgcagccgcgctccgggggaatcggcactctccagttcgtggaagagttcgttccctccgtctacttcaaccccttctccggctcgcctggacgctacccggacgccttcattcccaactttgacgcagtgagtgaatccgtggacggctacgactgatgacagatggtgcggccgtgagagctcggctgcgacatctgcatcactgccgtcagcctcgctgctacgctcgggaggcgatcgtgttcagctactttgagctgccggacgagcaccctcagggtccggctcacgggttgaaactcgagatcgagaacgcgctcgagtctcgcctcatcgacaccttcaccgcccgacctctcctggtagaaatccaacgggggatcactaccatcaccctgttctgcatctgccccacgcccggattacatgaagatctgtgttgtcatctttgcgctcagtttaataaaaactgaactttttgccgcaccttcaacgccacgcgttgtttctccaacagtcgacgatagctcttcaattaaaggtacccgagaaactgtttattttgacaattctactacttctcttatccttaactgttcttgcactaacgaactaattcagtggttcgccaacggttcactctgcaaagttttccttgactctgcgatacttcccggatttagcagctctgcgtgtgataattctaccccctccaccttaaccatcacaaagccattttcagaagtccagtatttttgtattggagcggggggtaaaccgggctgtattcaccgcttctttctggagacatttgttgcttcgattcccattaacacttcactttcctctaatacatacttaactaccttacattctactcacccctcctggaaacctcttattggcctcacagcttttatttccgttgttttactaaactttataattcttaacaaactttcttaaacatgcttgccattttgcttctgctcgttactttaacctccgcagattaccacaatgcaattgtacgagaaaacagtttacaaaacccatcacaggtatatgttaaagcaggttctaacttaactctacaatccttctattcgccttaccctgaggacatgccacgtgtcacctggtacttagaagtttttgattcgctatttgaaagacatacaattcctccattttttacaggcgttatactttgtgacatttctggtgacatacagcatgtgtggaaccattggcctttacaatttaattgcataaataaaagcttacatattatcaatctcaaaccaagtgatgaaggcctttacaatgtgaaggttttaaagggcagcattcagcataatacatactttcgtgtgcatgtagtaagttttccaaaacctgaatgtaacatcaccactacatatctttcagatgactactgccttattaacattgattgctctcaattaccataccctgctaaggtctattataatggcaatgaaagtaagctgcattactacttatctgaacgcggtggccaaccaaaccttccaaattactttactgttgggtatcgatatagagatctccgacagaattatacagttgaatatccatttaatgaactctgtacagatataattgctcttgaaacagggtctgattttacgccaatttttatagttaccctagtggtgagcattatagttattgtgatgggcatcacatatcttatttatcactgtaggactttaaaaaccaaaaccaaaaccaagcctcctgaaatccgtctgctttaattttttccagaatggtagctgctttcttcattctcctctgtataccaatcatctgcgcctccacaacttttgccgctgtttcccacctggaaccagactgtctaccaccttttgttgtatacctaatactgacttttgtggtctgtacagccattaccagtatagcctgcttttttgtaacaattttccaagccgccgattacctctacgtacggtttgcttactttagacatcaccccgagtatcggaatcaaaacgtagcctctctgctttgtttagcatgattcgcatttttatactttgtaagctctttaccaccacaatatgtcaatgcccttttaccaaaccctggtccttttacacttgttataatgtattacccgaaacccccattgcctggctttacgtagccacagcggctttagtttttgtagcaacctgcattggcgttaaactgtacttttacttaaaaattggatggcttcatcccccagaagatttaccccgatatcctcttgttaataactttcaacagcctctaccgcctcctgatcttccgcgagctccctccgttgttagctactttcaactcaccggtggagatgactgacactcaggacattaacattactgtggaaagaatagctgctcagcgtcagcgagagacgcgggtgatggagtacgtggaactacagcagcttaaagagtcccactggtgtgaaaaaggagtgctttgccatgttaagcaagcagccctttcttacgatgtcagcactcagggacatgaactgtcctacactttgcctttacagaaacaaaccttctgcaccatgatgggctctacctccattacaatcagccaacaaaccggacctgtcgagggggctatcctgtgtcactgtcacgcgcctgattgtatgcccaaactaatcagaactctttgtgctttaggtgatatatttaaaatatagatagtatcaataaacttaccttaaatttgacagcaattttttggtatcatcattcagcagcaccactttaccctcttcccaactctcatatgggatatgatggtgggcggcaaacttcctccaaaccctgaaagaaatatcggtatccacttccttgtcctcacccacaattttcatcttttcatagatgaaaagaacccgagttgatgaagacttcaaccccgtctacccttatgacaccacaaccactccagccgttcctttcatatcacccccgtttgtaaacagtgacggtcttcaggaaaacccccccggagttttaagcctgcgaatagctaaacccctgtattttgacatggagagaaaactagccctttcacttggaagagggttaacaattaccgcgaacggacaattagaaagcacccagagcgtgcagactaacccgccgttaactgtcaccaataacaacacacttatcctacgccactcctcccctttaatcctaactgacaataatttaaccgtaggcttctcaagtcctctccgtgttatagacaacaaactgacattcacttttacctcacctctccgttatgaaaacgaaacccttaccttcaattacacagagccccttacacttatgaacagcaaccttgcgcttaacgtaaactcctctaaaggccttagggttgacgggggctcactaggtacaaacttaagtccggacttaaggtttaacagcagtggagccatagcttttggtatacaaaccctatggacacccccgacctcaaatcctaactgcaccgtttacaccgaaagcgattccttacttagtctctgcttaactaaatgcggagctcacgttttaggaagtgtaagcttaaccggggtagcaggtaccatgataaacatggctgaaacttcgcttgctattgaatttacgtttgacgacactggaaaactacttcactcaccacttgttaacaccacttttagcattcgtcagggcgacagccccgcctcaaatcctacctacaatgctctagcatttatgccaaacagtaccctctacgctagaggaggaagtggtgaaccccgaaacaattactacgtccaaacatacctcaggggaaatgttcagagaccgattaccctcactgttactttcaactcagccgccacgggatattccttatcttttaagtggactgctgttgcacgtgaaaaatttgcagctcctgcaacttcattttgctacattaccgaacaataaaaccctgtgttcccaccgtttcgttttttccagatgaaacgggccagagttgatgaagacttcaatcccgtgtacccttacgatcccccttacgcccccattatgccgtttattaccccgccgtttacatcttcagatgggttacaggaaaaaccacttggtgttttaagtttaaaatacaaggatcctatcactacacaaaatggttctctaacccttaaattaggaaacgggctgaacattaacaaccagggccaacttacatcatctgctggggaagtcgagcctcccctcaccaatgctgacaacaagctggccttagcctacagcgaccctctgacattaaaaaacagccgtctaacactgtctcacaatgccccacttgcaattaacaataattctctaagtttggaagtatcagagcctatatttataaataacgacaacaaactgtctctgaaagctgacgcccccctgacaaccagcgctggaaccctccgcctgcaaagcgctgctccattaggacttgctgaacagacactaaagctgctgttttctaaccctttgtacttgcgaggtgacttccttacattagccattgaacgcccattggctgtaacagcagacgggctattatcacttgccctcaaccctccgctcacaacaactaacacaggcttagctctctctaccgcggttccattaactgttaccaacgggaaccttagcctaaacgtaaaacggccgtttattatacaggacggcagcctttacatggattttagacccccactatatctgtttaacagcgagccacaacttggtgttaattttaatgcccctctaactgttagagataacggcctagctataaacaccggagacgggctaacagtaacgtataataaactaacattaaacctcggtagagacttgcaatatgaaaatggagctgcagctgttaagctaagtaccgcccctcctctacagtatactactcaactgcagctgaatttgggagcgggcttacgtctaggtcctactaggaacttagacgtggccattaaccacaataaagggttagcgtgggaaaacaatgaagtggttactaaattaggacaaggcctttactttgattcctccggaagcatagctttatcgcctacaaaccccagaccagatactttatggaccacggccgatccttcgccaaactgcactgtatatgaatcacttgactctagactgtggctagcgcttgttaaatgtgggggaatggtacacggcagcatagccctacaagctgaaaaaggccaattgctgcgtcctactgctagttttatctccatcgtaatttacttctacagtgatggggtccgtcgcaccaactaccctacaattggcaatgatgagggtactctggccaacagcgctacttggggctacagacaagggcaatctgcagacaccaacgtcaccaatgctgttgaattcatgcctagtttacacagatatcctataaatcagggagacaatattaaaaaccaaatgataacttacacttgcatacaaggcaacgtgaacatgccagtacccttgaaaatcacgttcaatcatgctcttgaaggctactccttaaagtttacatggcgtgtggtggctaatgaaaagtttgatattccttgctgttcgttttcttacattacagaacaataaaacaacttttttatttttcatttcttttattttacacgcacagtaagacttcctccccccttccatttaacagcgtacaccagcctttcccccttcatggcggtaaacttctgtgagttagtccggtatttgggagttaaaatccaaacaggctctttggtgattaaacgttgatccgtgatggacacaaatccctgagacaggtcctccaacgttgcggtaaaaaactgaacgccgccctacaaaacaaacagttcaggctctccacgggttatcaccccgatcaaactcagacagagtaaaggtgcggtgatgttccacaagaccgcgcaagtggcgctgtctaaagctctcagtgcgacttctatgcggctggtaggatgttacattatccaacagcctcacagcgcggattattagtctacgagtgcgcctggcgcagcagcgcatctgaatttcagtcaagtcttgacaagaagcgcataccataacaatcaggttgttcatgatcccatagctaaacgcgctccagccaaaactcattcgctccaacagcaccaccgcgtgtccgtcaagtcttacttttacataaacaaggtgtctgccacgtacatacatgctacccgcatacaaaacttcccggggcaaacctctattcaccacctgtctgtaccagggaaacctgatgtttatcagggaaccatagatggccattttaaaccagttagccagcaccaccccgccagctctacactgaagggaaccgggagagttacaatgacagtggatcatccacctctcgtaacccctaattacctgattaaaatccaaatctaacgtggcacaacagatacacactctcataaacattttcatgacatgtttttcccaggatgttaaaatacaatcccaatacacgggccactcctgtaatacaataaagctaatgcatgatggaacgctcctcacctcactaacattgtgcatgtttacattttcacactctaagtaccgagtcctctcctcaacagccgcagtgtcgcgctcctcacacggtggtagctgatgacaattgtaaggggccagtctgcagcgatatcgtctgtcgcgctgcatcgtaaaacagggaccgtctcacttcctcgtacttccaatagcagaaccacgtccgctgccagcaggtttccacgaaccgccgatcccttcgtcgttcacgctccctcctcaacgcaaaatgcagccactcctgcaatccacacaaatccctctcggcctccggagtcatgcacacctcatacctatatatgtctcggtacagttccaaacacgaagtaagggcgagctccaaccaacacaaacaggctgatttatcccgacacactggaggtggaggaagacacggaagaggcatgttattccaagcgatccggcaaaggatcaaagtgcagatcccgaagatggcaacgctcgcctccggagccctggtgaaatttaacggccaaatcaaacattatgcggttttccaaactatcaatcgccgcctccaaaagggcctgaacccgcacttccacaatcaccagcaaagcaaaagcgtgattatcaaagtcttcaatcatcagatggcatgactgtacaatgcccaaataattctcatttctccactcgcgaatagtgtcgcggcagatcgtctgaaggtccatgccatgcatgttaaaaagctcccagagggcgccctctaccgacatgcgtagacacaccatcatgactgcaaaatatcaggctcctgagacacctgcagcagatttaacagatcaaagtcaggttgctgtccgcggtcacgaatctccatgcgcaaagccatttgcaaaaaattatataggtctgtgccaactagctctgttaattccgcgttaggaagcaaatcaggtgaggctatgcagcacaaaagttgcagggaaggcgccaaactcagtaaaaccgctccagaataacaaaattgatgaagcggagtcacacagtgtaaaatgtgcaaccaaaaatcattcagctgctcttttaaatagtccagtacttctatattcaatccgtgcaagtactgaagcaactgcgcgggaacagtcacattaaaaaaaatggggcggctcaaatacatgtcgacctaaaataaaaataatcattaaaccagagaagcttgacgaatggaaggataaaatacacgctccagcaaaaggcaggcaaccggctgtccccgagaaccgtaaaaaaattcatccgaatgattaaaaagaaccacagaaatttcccaccatgtactcggttgtaactcctgagcacacagcaacacccccctaacgttcatgtccgccactgaaaaaagacgtcccaaatacccaggtggaatgtcaagagacaactgcagagacagcaaaacaacccctctgggagcgatcataaactcctccggtgagaaaagcgcatacaaattagaataaccctgttgctggggcaaaatagcccggcggcccagcaaatggacataaatatgttcagcagccatcgccccgtcttaccgcgtaaaaagccagaaaaatccagctaactacactctacagcctattactatatatactctcctcccactgacgctataccaccccgcccacgtccaaagttcacccacgcccaaaaaacccgcgaaaatccagcgccgtcagcacttccgcaattgtagtctctcaacgtcacttccgcgcgccttttccctattcccacacacgcccgcggacttcgccccgcccgccctcgcgccaccccgcgtcaccccgcgtcaccgcacgtcaccccggccccgcctcgctcctccccactcattatcatattggcacgtttccagaataaggtatattattgatgatg

SEQ ID NO: 4 - DNA, 1092 bp, Artificial Sequence
  Synthetic oligonucleotide sAd4287 Fiber-1
atgaaaagaaccagagttgatgaagacttcaaccccgtctacccttatgactccacatccactcctgcggtcccctttatatcccccccgtttgtaaacagcgatggtcttcaggaaaaccctcctggagtcttaagtttacgaatagctaaacccttgtattttgacatggaaaggaaactagcgctttcacttggaagaggattggcaattacctccaccggacagctagaaagcacacagagcgtgcaaaccacccctccattagttgtcaacaacagcaacacgcttgtcctgcgttattcctccccgttaggcttatcgggtgacaatttaatactaaattgctccgatcctctccgcgtagtaaacaacagcctgacattcagctacctatctccacttcgttttgaaggtggcagtcttacattcaattacacatctccccttaaactgttgaacagcagccttgcgatcggaataaattccaacaaaggtctcggcaatgacagcgatgaactttctgtcaaactaacatcagatctaaagtttaacaacgatggaaaaatagcttttggtatacaaagcctgtgtaccacccccacagccgcctctaactgtaccgtttttaccaacggtgattctttactctgtttatgtttaaccaaatgtggagctcacgtgttaggaagtgtgagtttaaccggaatgcaaggaaccataacagccatgacacagaactacattagtattcaatttctatttgacaacaatggtgcgttgacttcatcaccgctcctcaacaacaacacttggggtatacggcaaaacgacacttcgtccgctaaccccgcctacaatgctcttgcatttatgcctaacagcactgtatatgtaagaggtcaaagtggtgagcccagaaataactattacacccaaacataccttaggggaaacgttaaaaagccaattatccttaccgttacctacaactcggctgcttcaggttattcactaacttttaaatgggatgctgtagtaacagaaaaatttgccactccaacatcttctttttgctatattacagaacaa

SEQ ID NO: 5 - DNA, 1089 bp, Artificial Sequence
  Synthetic oligonucleotide sAd4310A Fiber-1
atgaaaagaaccagagttgatgaagacttcaaccccgtctacccctatgacaccacaaccactcctgcagttccctttatatcacccccctttgtaaacagcgatggtcttcaggaaaaccccccaggtgttttaagtctgcgaatagctaaacccctatatttcgacatggagagaaaactagccctttcacttggaagagggttgacaattaccgccgccggacaattagaaagtacgcagagcgtacaaaccaacccaccgttgataattaccaacaacaacacactgaccctacgtcattctccccccttaaacctaactgacaatagcttagtgctaggctactcgagtccgctccgcgtcacagacaacaaacttacatttaacttcacatcaccactccgttatgaaaatgaaaaccttacttttaactatacagagcctcttaaacttataaataacagccttgccattgacatcaattcctcaaaaggccttagtagcgtcggaggctcactagctgtaaacctgagttcagacttaaagtttgacagcaacggatccatagcttttggcatacaaaccctgtggaccgctccgacctcgactggcaactgcaccgtctacagcgagggcgattccctacttagtctctgtttaaccaaatgcggagctcacgtcttaggaagtgtaagtttaaccggtttaacaggaaccataacccaaatgactgatatttctgtcaccattcaatttacatttgacaacaatggtaagctactaagctctccgcttataaacaacgcctttagtattcgacagaatgacagtacggcctcaaaccctacctacaacgccctggcgtttatgcctaacagtaccatatatgcaagagggggaggtggtgaaccacgaaacaactactacgtccaaacgtatcttaggggaaatgttcaaaaaccaatcattcttactgtaacctacaactcagccgccacaggatattccttatcttttaagtggactgctcttgcacgtgaaaagtttgcaaccccaacaacttcgttttgctacattacagaacaa

SEQ ID NO: 6 - DNA, 1089 bp, Artificial Sequence
  Synthetic oligonucleotide sAd4312 Fiber-1
atgaaaagaacccgagttgatgaagacttcaaccccgtctacccttatgacaccacaaccactccagccgttcctttcatatcacccccgtttgtaaacagtgacggtcttcaggaaaacccccccggagttttaagcctgcgaatagctaaacccctgtattttgacatggagagaaaactagccctttcacttggaagagggttaacaattaccgcgaacggacaattagaaagcacccagagcgtgcagactaacccgccgttaactgtcaccaataacaacacacttatcctacgccactcctcccctttaatcctaactgacaataatttaaccgtaggcttctcaagtcctctccgtgttatagacaacaaactgacattcacttttacctcacctctccgttatgaaaacgaaacccttaccttcaattacacagagccccttacacttatgaacagcaaccttgcgcttaacgtaaactcctctaaaggccttagggttgacgggggctcactaggtacaaacttaagtccggacttaaggtttaacagcagtggagccatagcttttggtatacaaaccctatggacacccccgacctcaaatcctaactgcaccgtttacaccgaaagcgattccttacttagtctctgcttaactaaatgcggagctcacgttttaggaagtgtaagcttaaccggggtagcaggtaccatgataaacatggctgaaacttcgcttgctattgaatttacgtttgacgacactggaaaactacttcactcaccacttgttaacaccacttttagcattcgtcagggcgacagccccgcctcaaatcctacctacaatgctctagcatttatgccaaacagtaccctctacgctagaggaggaagtggtgaaccccgaaacaattactacgtccaaacatacctcaggggaaatgttcagagaccgattaccctcactgttactttcaactcagccgccacgggatattccttatcttttaagtggactgctgttgcacgtgaaaaatttgcagctcctgcaacttcattttgctacattaccgaacaa

SEQ ID NO: 7 - DNA, 1677 bp, Artificial Sequence
  Synthetic oligonucleotide sAd4287 Fiber-2
atgaaacgggccagagttgatgaagacttcaacccagtgtacccttatgaccccccatacgctcccgttatgcccttcattactccaccttttacctcctcggatgggttgcaggaaaaaccacttggagtgttaagtttaaactacaaggatcccattactacacaaaatggatctctcacgttgaaaataggaaacggcctcactctagacaaccagggacaattaacatcaactgctggggaagtagagcctccgctcactaatgctaacaacaaacttgcactagcctatagcgaaccattagcagtaaaaagcaaccgcttaactttatcacacaccgccccccttgtcgttgctaataattctttagcgttgcaagtttcagaacctatttttataaatgacgatgacaagctagccctgcagacagccgccccccttgtaactaacgctggcacccttcgcttacagagcgccgcccctttaggattggttgaaaatactcttagactgctgttttctaaacccttgtatttgcaaaatgattttcttgcattaggcattgaacgccccctggctatagcagccgcaggtactctagcactacaactcactcctccattaaagactaacgatgacgggctgacactatccacagtcgagccattaactgtaaaaaacggaaacttaggcttgcaaatatctcgccctttggttgttcaaaacagcagcctttcgcttgctattacccccccgctgcgtctatttaacagcgaccccgttcttggtttgggctttacttttcccctagccgtgacagacaacctactctccttaaacatgggagacggtgttaaactaacctataataaactaacagccaatttgggtagggatttacaatttgaaaacggtgccattgccgtaacgcttactgccgaatcacctttgcaatacactaacaaacttcaactgaatattggagctggccttcgttacaatggagccagcagaaaactagatgtaaacattaaccaaaataagggcttaacttgggacaacgatgcagttattcccaaattaggatcaggtttacaattcgaccctaatggtaacatcgctgttatccctgaaaccgtaaagccgcaaacgttatggacaactgcagatccatcgcctaactgctcagtgtaccaggacttggacgccaggctgtggctcgctcttgttaaaagtggtgacatggttcatggaagcattgctctaaaagccctaaaaggaacgttgctaaatcctacagcaagctacatctccattgtgatatatttttacagcaacggagtcaggcgtaccaactatcccacgtttgacaacgaaggcaccttagctaacagcgctacctggggataccgagaggggcaatctgctaacactaatgtaaccaatgccactgaatttatgcccagctcaaccaggtaccccgtgaataaaggagacaatattcagaatcaatctttttcatacacctgtatcaaaggagatttcgctatgcctgtcccgttccgtgtaacatataatcatgccctggaaggatactcccttaagttcacctggcgcgttgtagccaaccaagcttttgatattccttgctgttccttttcatacatcacagaa

SEQ ID NO: 8 - DNA, 1680 bp, Artificial Sequence
  Synthetic oligonucleotide sAd4310A Fiber-2
atgaaacgggcgagagttgatgaagacttcaacccagtgtacccttatgaccccccacatgctcccgttatgcccttcattactccaccttttacctcctcggatgggttgcaggaaaaaccacttggagtgttaagtttaaactacagagatcccattactacgcaaaatgggtctcttacagttaaactaggaaacggcctcactctagacaaccagggacaactaacatcaaccgctggggaagtagaacctccactcactaacgctaacaacaaacttgcactggtctatagcgatcctttagcagtaaagcgcaacagcctaaccttatcgcacaccgctccccttgttattgctgataactctttagcattgcaagtttcagagcctatttttataaatgacaaggacaaactagccctgcaaacagccgcgccccttgtaactaacgctggcacccttcgcttacaaagcgccgcccctttaggcattgcagaccaaaccctaaaactcctgtttaccaaccctttgtacttgcagaataactttctcacgttagccattgaacgaccccttgccattaccaatagtggaaagctggctctacagctctccccaccgctacaaacagcagacacaggcttgactttgcaaaccaacgtgccattaactgtaagcaacgggaccctaggcttagccataaagcgcccacttattgttcaggacaacaacttgtttttggacttcagagctcccctgcgtcttttcaacagcgaccccgtactagggcttaacttttacacccctcttgcagtgcgcgatgaggcgctcactgttaacacaggccgcggcctcacagtgagttacgatggtttaattttaaatcttggtaaggatcttcgctttgacaacaacaccgtttctgtcgctcttagtgctgctttgcctttacaatacactgatcagcttcgccttaacgtgggcgctgggctgcgttacaatccagtgagtaaaaaattggacgtgaaccccaatcaaaacaagggtttaacctgggaaaatgactacctcattgtaaagctaggaaatggattaggttttgatggcaatggaaacatagctgtttctcctcaagttacatcgcctgacaccttatggaccactgccgatccatcccccaattgttccatctacactgatttagatgccaaaatgtggctctcgttggtaaaacaagggggtgtggttcacggttctgttgctttaaaagcattgaaaggaaccctattgagtcctacggaaagtgccattgttattatactacattttgacaattatggagtgcgaattctcaattatcccactttgggcactcaaggcacgttgggaaataatgcaacttggggttataggcagggagaatctgcagacactaatgtactcaatgcactagcatttatgcccagttcaaaaaggtacccaagagggcgtggaagcgaagttcagaatcaaactgtgggctacacttgtatacagggtgacctttctatgcccgtaccgtaccaaatacagtacaactatggaccaactggctactcctttaaatttatttggagaactgtttcaagacaaccatttgacatcccatgctgttttttctcttacattacggaagaa

SEQ ID NO: 9 - DNA, 1680 bp, Artificial Sequence
  Synthetic oligonucleotide sAd4312 Fiber-2
atgaaacgggccagagttgatgaagacttcaatcccgtgtacccttacgatcccccttacgcccccattatgccgtttattaccccgccgtttacatcttcagatgggttacaggaaaaaccacttggtgttttaagtttaaaatacaaggatcctatcactacacaaaatggttctctaacccttaaattaggaaacgggctgaacattaacaaccagggccaacttacatcatctgctggggaagtcgagcctcccctcaccaatgctgacaacaagctggccttagcctacagcgaccctctgacattaaaaaacagccgtctaacactgtctcacaatgccccacttgcaattaacaataattctctaagtttggaagtatcagagcctatatttataaataacgacaacaaactgtctctgaaagctgacgcccccctgacaaccagcgctggaaccctccgcctgcaaagcgctgctccattaggacttgctgaacagacactaaagctgctgttttctaaccctttgtacttgcgaggtgacttccttacattagccattgaacgcccattggctgtaacagcagacgggctattatcacttgccctcaaccctccgctcacaacaactaacacaggcttagctctctctaccgcggttccattaactgttaccaacgggaaccttagcctaaacgtaaaacggccgtttattatacaggacggcagcctttacatggattttagacccccactatatctgtttaacagcgagccacaacttggtgttaattttaatgcccctctaactgttagagataacggcctagctataaacaccggagacgggctaacagtaacgtataataaactaacattaaacctcggtagagacttgcaatatgaaaatggagctgcagctgttaagctaagtaccgcccctcctctacagtatactactcaactgcagctgaatttgggagcgggcttacgtctaggtcctactaggaacttagacgtggccattaaccacaataaagggttagcgtgggaaaacaatgaagtggttactaaattaggacaaggcctttactttgattcctccggaagcatagctttatcgcctacaaaccccagaccagatactttatggaccacggccgatccttcgccaaactgcactgtatatgaatcacttgactctagactgtggctagcgcttgttaaatgtgggggaatggtacacggcagcatagccctacaagctgaaaaaggccaattgctgcgtcctactgctagttttatctccatcgtaatttacttctacagtgatggggtccgtcgcaccaactaccctacaattggcaatgatgagggtactctggccaacagcgctacttggggctacagacaagggcaatctgcagacaccaacgtcaccaatgctgttgaattcatgcctagtttacacagatatcctataaatcagggagacaatattaaaaaccaaatgataacttacacttgcatacaaggcaacgtgaacatgccagtacccttgaaaatcacgttcaatcatgctcttgaaggctactccttaaagtttacatggcgtgtggtggctaatgaaaagtttgatattccttgctgttcgttttcttacattacagaacaa

SEQ ID NO: 10 - DNA, 2799 bp, Artificial Sequence
  Synthetic oligonucleotide sAd4287 Hexon
atggccaccccatcgatgatgccgcagtggtcttacatgcacatcgccggccaggacgcctcggagtacctgagtcccggcctcgtgcagtttgcccgcgccaccgacacctacttcagcttgggaaacaagtttagaaaccccaccgtggcccccacccacgatgtgaccacggaccgctcgcagaggctgaccctgcgctttgtgcccgtagaccgggaggacaccgcgtactcttacaaagtgcgctacacgctggccgtaggggacaaccgagtgctggacatggccagcacctactttgacatccggggggtgctggatcggggtcccagcttcaagccctactccggcaccgcttacaactccctggctcccaagggcgcccccaatcctgcagaatgggccgataccaacgacagcaacaaactgaaagtgaggggtcaggcgccttttgtcagtacttacggttctgctacggcgcttacaaaagatgggatacaggtgggagtggatacttccgaagcatctcaggctgtttatgccgacagaagttaccagccagaaccccaaattggagagacagagtggaacagcgaagtgggtaatgacgacagagtggcgggaagggtgctaaagaaaacaactcccatgttcccttgttacggttcatatgccaagcccaccaacgaaaaaggcggacaagcaatacagcccaccgccggcaacggcgataatcaggctgtagagttacaattctttgccactactagcactcccactgcgccaaaggcagtattgtacgcggaggacgtggccattgaagctccagatactcacttagtgtttaagccaacagtagtcgcgggaactacaagttcggaagctctgctaacccaacaagccgcacctaaccgcccaaactacattgcctttagagataactttattggtctcatgtactacaattcaaccgggaatatgggagtactggccggacaagcatctcagctcaatgcagtggttgatcttcaggacagaaacaccgaactgtcatatcagctaatgctggatgctctgggagatcgcagtcggtacttttctatgtggaatcaagctgtagatagctatgatccagatgtaagaattgtagaaaaccacggtgtggaagacgaactgcctaattattgcttcccactaggcgggatggtagtaacggacacttacaaagccataaaggtaaatggaagcggatggacggctaatactgacgttttcagcgagagagtagaaataggctcaggtaacctgtttgccatggaaattaacttgcaagctaatctgtggcgcagtttcttgtattccaacataggactgtacctcccggactctttaaaattaacccctgacaacatcacgctccctgagaacaaaaatacctaccagtatatgaacggtcgcgtaacaccacccgggctcgtggacacctacgttaacgtgggtgcgcgctggtcccccgatgttatggacagcattaacccttttaaccaccaccgcaacgccgggctccgctaccgttccatgctcctgggaaacggacgctacgtacccttccacattcaggtgccccagaaattctttgcaattaaaaacctgctgctgctccccggttcctatacctacgagtggaatttccgcaaggacgtgaacatgattttgcaaagctcgctgggtaacgacctgcgagttgacggggccagcatacgcttcgacagcatcaacctgtatgctaactttttccccatggcccacaacacggcctccaccctggaagccatgctgcgcaacgacaccaatgaccagtccttcaacgactacctgtgcgcggccaacatgctgtatcccatccccgccaacgccaccagcgtgcccatctccatcccgtctcgcaactgggccgcctttaggggttggagtttcacccgcctcaaaaccaaggaaaccccctcgctgggctctggcttcgacccctacttcgtctactcaggctccattccctacctggacggcactttctatcttaaccacactttcaaaaaggtgtctatcatgttcgattcctcggtcagctggcccggcaacgaccgcctgctgacgcccaacgagttcgaaatcaagcgttcggtggacggtgaagggtacaacgtggcccagagcaacatgaccaaggactggttcctggttcaaatgctcagccattacaacatcggttaccagggcttctatgtgcccgagaactacaaggaccgcatgtactccttctttaggaacttccaacccatgagtcgccaagtcgtggactcagtggcttacagggactactaccaggacgttaagctcccctaccagcacaacaactcagggttcgtgggctacatgggtcccaccatgcgagaggggcaggcctacccggccaactatccttatcccctaatcggagagactgctgtacccagcctgacgcagaaaaagttcctctgcgaccgggtgatgtggaggatacccttctctagcaacttcatgtctatgggctccctcaccgacctggggcagaacatgctgtacgccaactccgctcacgccttggacatgacctttgaggtggatcccatggatgagcccacgcttctctatgttctgtttgaagtcttcgacgtggtgcgcatccaccagccgcaccgcggcgtcatcgaggccgtctacctgcgcacacctttctctgccggtaacgccaccacc

SEQ ID NO: 11 - DNA, 2736 bp, Artificial Sequence
  Synthetic oligonucleotide sAd4310A Hexon
atggccaccccatcgatgatgccgcagtggtcttacatgcacatcgccgggcaggacgcctcggagtatctgagccccggtcttgtgcagtttgcccgcgccaccgacacctacttcagcttgggaaacaagtttagaaatcccaccgtggcccccacgcacgatgtgaccacggatcgttcgcagaggctgactctgcgctttgtaccggtagaccgtgaggatactgcctattcttacaaagttcggtatacgttagccgtaggagacaacagggtgctggacatggccagtacttactttgacatccgcggtgttcttgaccgcggtccaagctttaaaccgtataccggaacggcatacaatgccttggctccaaagggcgctccaaatgcttgccagtggacaacgaccaacgggggcaataaaacgaacacttttgcccaagcccctttaataggcacggctattgacggaaccaacggactgcagattgggcaagataatggacaagctgtttatgctgacaaaacctttcaacccgaaccacaagtgggagaatctcagtggaatactaatccaaccacaaacgcagcaggacgcgtgttaaaaacaactactcgcatgctgccttgctatggttcttttgcaaggcccaccaatgagaaagggggtcaagcttcaggagacgttaccttccaatttttcgacactgcctcggacaatggcaacaaccctaaggtggtgctatatggagaagacgtcaacattgaatcgcctgacacacacttaatctacaaacccaccgctgacaacacaaactctgaaaaccttttgggtcaacaggccgctccaaacagagccaattacattgcctttcgggacaacttcattggactaatgtactataattcaacaggaaacatgggagtgttggcagggcaggcttcccaactaaatgctgtggtagacttgcaagacagaaacactgagctttcctaccaactcatgttagatgcaataggagaccggagtcgttacttttcaatgtggaaccaagcagtggacagctatgatccagatgtgcgaattattgaaaatcatggcgttgaggacgaactgccaaattactgcttccctcttaacgctcaaggaattgctaacacctataaaggcgttaagaaaaacaacggcaattgggcgaaagacgacgcagtagtagaaactaacgaaattggcataggaaatgtttttgccatggagataaatttaactgctaacttgtggcgaaactttctgtattccaatattgctttgtacctgccagactcctacaagtattcaccgggaaacataaccttacccgaaaacaaaaacagttacaattacattaatggtcgagtaacagctcctggtctggtagacacctttgtaaacattggcgcgcgatggtctcccgaccccatggacaacgtgaatccttttaatcaccatcgcaatgctggtctgcgttatcgctccatgcttctaggcaacggccgctacgtgcccttccacattcaggtgcctcaaaaattctttgccattaagaacctgcttctgctgcctgggtcctacacctacgagtggaacttcagaaaagatgtaaacatgatcttgcagagcacgctgggcaacgacctccgtgtcgacggggccagcgtcagattcgacagcattaacctctacgctaatttcttccccatggcacataacaccgcttccaccctggaggctatgttacgcaacgacaccaacgaccagtcctttaatgactacctctgcgcggccaacatgctataccccattcctgccaatgccaccagtgtgcccatctccatcccctctcgcaactgggcagctttcagagggtggagtttcacccgcctcaaaacaaaagaaaccccctcgctgggttccggatttgatccatactttgtttactcaggctccattccctacctggatggtaccttctacctgaaccacaccttcaaaaaggtgtctattatgttcgactcttctgtgagctggcccggcaacgaccgcctgctgacccctaatgagtttgaaattaagcgctcggtggacggagaaggatacaatgtagcccagagcaacatgaccaaagactggttcttaattcaaatgctcagccactacaacattggttaccaagggttttacgtgcccgaggcttacaaagacagaatgtactccttttttagaaacttccaacctatgagtagacaggtagtggatgcagatcggtatgaacaatacaaaaaagtcaccgttgagtatcaacataataattctggttttgtgggatacatgggacccaccatgagggaagggcaggcttatccagcgaattacccttatcctcttattggagacaccgccgtgcccagcctgacccagaaaaagttcctctgtgaccgcaccatgtggagaatccccttctctagcaacttcatgtctatgggggccctcaccgacctggggcagaacatgctgtacgccaattccgctcacgccttggatatgacctttgaggtggaccccatggatgagcccacgcttctctatgttctgtttgaagtcttcgacgtggtgcgcatccaccagccgcaccgcggcgtcatcgaggccgtctacctgcgcacacctttctctgccggtaacgccaccaca

SEQ ID NO: 12 - DNA, 2784 bp, Artificial Sequence
  Synthetic oligonucleotide sAd4312 Hexon
atggccaccccatcgatgatgccgcagtggtcttacatgcacatcgccggccaggacgcctcggagtacctgagtcccggcctggtgcagtttgcccgcgccaccgaaagctacttcagcttgggaaacaagtttagaaaccccaccgtggcccccacgcacgatgtaaccacggaccgctcgcagaggctgacactgcgcttcgtgcccgtagaccgggaggacaccgcgtactcctacaaagtgcgcttcaccctcgccgtaggggacaacagggtgctggacatggccagcacgtactttgacatccggggaatgctggaccgagggcccagctttaaaccctactcgggaactgcctacaattcgctggcacctaagggcgctcccaaccctagtcaatggactactaccaacggagggaataaaacaaattcatttgcccaagcatcctacataggtcaaagcctgtcgaaagacggggtgcaagtagcagtagatacagccgctgggggggctgcagtatatgctgacaaaacgtttcaaccagaaccccaagtaggaatatcacaatggaatgaaaatcctactacaaatgctgcaggaagaattttaaagcctactaccgcaatgcgtccatgctacggttcatacgcttaccccaccaacgaaaaaggtgggcaggtaaaaatcactgaccctaacaatgacaaaaccggcgctaataacgttagcttaaattttttcaacactgccgctgacaatgggaataacaatccaaaagtagtactctacagcgaagatgtaaatttagaagggccagatacccaccttgtttttaagccagatgtaactggcgacgcaaccagtgcagaaaccctgttaggtcaacaagcagctcccaatcgtccaaactacattgggttcagggacaactttattggcctgatgtactacaattcaactggaaacatgggagtgctagcaggtcaggcttctcagctaaacgccgtagtggatcttcaagacagaaataccgaattgtcatatcagctaatgcttgacgctttgggtgacagaagtcggtacttttctatgtggaatcaagcagtggacagctacgatcctgacgttagaatcatagaaaatcatggagtagaagacgaacttccaaattattgttttccgttaaatggacaggggatttcgaatacatacaaaggtgtgaaatataacacaaacacttggacgcaagacactgatgtagtcacaaccaatgaaatttccattggcaacatttttgccatggaaataaacctggcggctaacttgtggcgcagctttctgtactccaatgtcgccctgtacttgccagattcctacaaatacactcccgacaatattgaacttcctacaaacaagaacagctacggctacattaacggaagggtaaccgcccccactgccatcgacacttacgttaacatcggcgcccggtggtctccggaccccatggacaacgttaaccctttcaaccaccaccgcaacgccggcttgcgataccgctccatgctgctgggcaacggtcgctacgtacccttccacattcaggtgccccagaaattttttgccattaaaaacctgcttctgcttcccgggtcctacacctacgagtggaacttcaggaaagatgtaaacatgatcttgcagagcaccttgggcaacgacctccgcgttgacggagctagcgtgaggtttgacagcattaacctctacgctaacttcttccccatggcccacaacacggcctccaccttggaagccatgctgcgcaacgacaccaacgaccagtcctttaatgattacctgtgcgcggccaacatgctgtaccccatccccgccaatgccaccagcgtgccgatctccattccctcacgcaactgggccgccttcagaggttggagtttcactcgcctgaaaaccaaggagaccccctcgctgggctccggtttcgacccatactttgtttactccgggagcattccctacctggacggaactttctacctgaaccacaccttcaaaaaggtgtctattatgtttgactcctccgtgagctggcccggtaacgaccgcttgctaacccccaacgagttcgaaatcaaacgctcggtggacggagagggttacaatgtagcccagagcaacatgaccaaagactggtttttaattcaaatgctaagccactataacattggctaccaaggattctacgtgcctgaagcctacaaggacagaatgtactccttctttagaaacttccaacccatgagccgccaggtagtagacacggtaaactatgctaactacaaggaagtaacaatgccattccagcacaacaactcaggcttcgtggggtacatgggacctaccatgagagaggggcaggcctacccggctaattatccctaccccctaatcggagccactgccgtgcccagcctgacacagaaaaagtttctctgcgatcgaacaatgtggaggattcccttctctagcaacttcatgtccatgggggctctcaccgacctggggcagaacatgctgtacgctaactccgctcacgccttggacatgacctttgaggtggaccccatggatgagcccacgcttctctatgttctgtttgaagtcttcgacgtggtgcgcattcaccagccgcaccgcggcgtcatcgaggccgtctacctgcgcacacctttctctgccggtaacgccaccacc

SEQ ID NO: 13 - DNA, 492 bp, Artificial Sequence
  Synthetic oligonucleotide sAd4287 Fiber-1 Knob
ctgtgtaccacccccacagccgcctctaactgtaccgtttttaccaacggtgattctttactctgtttatgtttaaccaaatgtggagctcacgtgttaggaagtgtgagtttaaccggaatgcaaggaaccataacagccatgacacagaactacattagtattcaatttctatttgacaacaatggtgcgttgacttcatcaccgctcctcaacaacaacacttggggtatacggcaaaacgacacttcgtccgctaaccccgcctacaatgctcttgcatttatgcctaacagcactgtatatgtaagaggtcaaagtggtgagcccagaaataactattacacccaaacataccttaggggaaacgttaaaaagccaattatccttaccgttacctacaactcggctgcttcaggttattcactaacttttaaatgggatgctgtagtaacagaaaaatttgccactccaacatcttctttttgctat

SEQ ID NO: 14 - DNA, 489 bp, Artificial Sequence
  Synthetic oligonucleotide sAd4310A Fiber-1 Knob
ctgtggaccgctccgacctcgactggcaactgcaccgtctacagcgagggcgattccctacttagtctctgtttaaccaaatgcggagctcacgtcttaggaagtgtaagtttaaccggtttaacaggaaccataacccaaatgactgatatttctgtcaccattcaatttacatttgacaacaatggtaagctactaagctctccgcttataaacaacgcctttagtattcgacagaatgacagtacggcctcaaaccctacctacaacgccctggcgtttatgcctaacagtaccatatatgcaagagggggaggtggtgaaccacgaaacaactactacgtccaaacgtatcttaggggaaatgttcaaaaaccaatcattcttactgtaacctacaactcagccgccacaggatattccttatcttttaagtggactgctcttgcacgtgaaaagtttgcaaccccaacaacttcgttttgctac

SEQ ID NO: 15 - DNA, 489 bp, Artificial Sequence
  Synthetic oligonucleotide sAd4312 Fiber-1 Knob
ctatggacacccccgacctcaaatcctaactgcaccgtttacaccgaaagcgattccttacttagtctctgcttaactaaatgcggagctcacgttttaggaagtgtaagcttaaccggggtagcaggtaccatgataaacatggctgaaacttcgcttgctattgaatttacgtttgacgacactggaaaactacttcactcaccacttgttaacaccacttttagcattcgtcagggcgacagccccgcctcaaatcctacctacaatgctctagcatttatgccaaacagtaccctctacgctagaggaggaagtggtgaaccccgaaacaattactacgtccaaacatacctcaggggaaatgttcagagaccgattaccctcactgttactttcaactcagccgccacgggatattccttatcttttaagtggactgctgttgcacgtgaaaaatttgcagctcctgcaacttcattttgctac

SEQ ID NO: 16 - DNA, 510 bp, Artificial Sequence
  Synthetic oligonucleotide sAd4287 Fiber-2 Knob
tggacaactgcagatccatcgcctaactgctcagtgtaccaggacttggacgccaggctgtggctcgctcttgttaaaagtggtgacatggttcatggaagcattgctctaaaagccctaaaaggaacgttgctaaatcctacagcaagctacatctccattgtgatatatttttacagcaacggagtcaggcgtaccaactatcccacgtttgacaacgaaggcaccttagctaacagcgctacctggggataccgagaggggcaatctgctaacactaatgtaaccaatgccactgaatttatgcccagctcaaccaggtaccccgtgaataaaggagacaatattcagaatcaatctttttcatacacctgtatcaaaggagatttcgctatgcctgtcccgttccgtgtaacatataatcatgccctggaaggatactcccttaagttcacctggcgcgttgtagccaaccaagcttttgatattccttgctgttccttttcatac

SEQ ID NO: 17 - DNA, 513 bp, Artificial Sequence
  Synthetic oligonucleotide sAd4310A Fiber-2 Knob
ttatggaccactgccgatccatcccccaattgttccatctacactgatttagatgccaaaatgtggctctcgttggtaaaacaagggggtgtggttcacggttctgttgctttaaaagcattgaaaggaaccctattgagtcctacggaaagtgccattgttattatactacattttgacaattatggagtgcgaattctcaattatcccactttgggcactcaaggcacgttgggaaataatgcaacttggggttataggcagggagaatctgcagacactaatgtactcaatgcactagcatttatgcccagttcaaaaaggtacccaagagggcgtggaagcgaagttcagaatcaaactgtgggctacacttgtatacagggtgacctttctatgcccgtaccgtaccaaatacagtacaactatggaccaactggctactcctttaaatttatttggagaactgtttcaagacaaccatttgacatcccatgctgttttttctcttac

SEQ ID NO: 18 - DNA, 516 bp, Artificial Sequence
  Synthetic oligonucleotide sAd4312 Fiber-2 Knob
ttatggaccacggccgatccttcgccaaactgcactgtatatgaatcacttgactctagactgtggctagcgcttgttaaatgtgggggaatggtacacggcagcatagccctacaagctgaaaaaggccaattgctgcgtcctactgctagttttatctccatcgtaatttacttctacagtgatggggtccgtcgcaccaactaccctacaattggcaatgatgagggtactctggccaacagcgctacttggggctacagacaagggcaatctgcagacaccaacgtcaccaatgctgttgaattcatgcctagtttacacagatatcctataaatcagggagacaatattaaaaaccaaatgataacttacacttgcatacaaggcaacgtgaacatgccagtacccttgaaaatcacgttcaatcatgctcttgaaggctactccttaaagtttacatggcgtgtggtggctaatgaaaagtttgatattccttgctgttcgttttcttac

SEQ ID NO: 19 - protein, 364 aa, Artificial Sequence
  Synthetic polypeptide sAd4287 Fiber-1
MKRTRVDEDFNPVYPYDSTSTPAVPFISPPFVNSDGLQENPPGVLSLRIAKPLYFDMERKLALSLGRGLAITSTGQLESTQSVQTTPPLVVNNSNTLVLRYSSPLGLSGDNLILNCSDPLRVVNNSLTFSYLSPLRFEGGSLTFNYTSPLKLLNSSLAIGINSNKGLGNDSDELSVKLTSDLKFNNDGKIAFGIQSLCTTPTAASNCTVFTNGDSLLCLCLTKCGAHVLGSVSLTGMQGTITAMTQNYISIQFLFDNNGALTSSPLLNNNTWGIRQNDTSSANPAYNALAFMPNSTVYVRGQSGEPRNNYYTQTYLRGNVKKPIILTVTYNSAASGYSLTFKWDAVVTEKFATPTSSFCYITEQ

SEQ ID NO: 20 - protein, 363 aa, Artificial Sequence
  Synthetic polypeptide sAd4310A Fiber-1
MKRTRVDEDFNPVYPYDTTTTPAVPFISPPFVNSDGLQENPPGVLSLRIAKPLYFDMERKLALSLGRGLTITAAGQLESTQSVQTNPPLIITNNNTLTLRHSPPLNLTDNSLVLGYSSPLRVTDNKLTFNFTSPLRYENENLTFNYTEPLKLINNSLAIDINSSKGLSSVGGSLAVNLSSDLKFDSNGSIAFGIQTLWTAPTSTGNCTVYSEGDSLLSLCLTKCGAHVLGSVSLTGLTGTITQMTDISVTIQFTFDNNGKLLSSPLINNAFSIRQNDSTASNPTYNALAFMPNSTIYARGGGGEPRNNYYVQTYLRGNVQKPIILTVTYNSAATGYSLSFKWTALAREKFATPTTSFCYITEQ

SEQ ID NO: 21 - protein, 360 aa, Artificial Sequence
  Synthetic polypeptide sAd4312 Fiber-1
MKRTRVDEDFNPVYPYDTTTTPAVPFISPPFVNSDGLQENPPGVLSLRIAKPLYFDMERKLALSLGRGLTITANGQLESTQSVQTNPPLTVTNNNTLILRHSSPLILTDNNLTVGFSSPLRVIDNKLTFTFTSPLRYENETLTFNYTEPLTLMNSNLALNVNSSKGLRVDGGSLGTNLSPDLRFNSSGAIAFGIQTLWTPPTSNPNCTVYTESDSLLSLCLTKCGAHVLGSVSLTGVAGTMINMAETSLAIEFTFDDTGKLLHSPLVNTTFSIRQGDSPASNPTYNALAFMPNSTLYARGGSGEPRNNYYVQTYLRGNVQRPITLTVTFNSAATGYSLSFKWTAVAREKFAAPATSFCYI

SEQ ID NO: 22 - protein, 559 aa, Artificial Sequence
  Synthetic polypeptide sAd4287 Fiber-2
MKRARVDEDFNPVYPYDPPYAPVMPFITPPFTSSDGLQEKPLGVLSLNYKDPITTQNGSLTLKIGNGLTLDNQGQLTSTAGEVEPPLTNANNKLALAYSEPLAVKSNRLTLSHTAPLVVANNSLALQVSEPIFINDDDKLALQTAAPLVTNAGTLRLQSAAPLGLVENTLRLLFSKPLYLQNDFLALGIERPLAIAAAGTLALQLTPPLKTNDDGLTLSTVEPLTVKNGNLGLQISRPLVVQNSSLSLAITPPLRLFNSDPVLGLGFTFPLAVTDNLLSLNMGDGVKLTYNKLTANLGRDLQFENGAIAVTLTAESPLQYTNKLQLNIGAGLRYNGASRKLDVNINQNKGLTWDNDAVIPKLGSGLQFDPNGNIAVIPETVKPQTLWTTADPSPNCSVYQDLDARLWLALVKSGDMVHGSIALKALKGTLLNPTASYISIVIYFYSNGVRRTNYPTFDNEGTLANSATWGYREGQSANTNVTNATEFMPSSTRYPVNKGDNIQNQSFSYTCIKGDFAMPVPFRVTYNHALEGYSLKFTWRVVANQAFDIPCCSFSYITE

SEQ ID NO: 23 - protein, 560 aa, Artificial Sequence
  Synthetic polypeptide sAd4310A Fiber-2
MKRARVDEDFNPVYPYDPPHAPVMPFITPPFTSSDGLQEKPLGVLSLNYRDPITTQNGSLTVKLGNGLTLDNQGQLTSTAGEVEPPLTNANNKLALVYSDPLAVKRNSLTLSHTAPLVIADNSLALQVSEPIFINDKDKLALQTAAPLVTNAGTLRLQSAAPLGIADQTLKLLFTNPLYLQNNFLTLAIERPLAITNSGKLALQLSPPLQTADTGLTLQTNVPLTVSNGTLGLAIKRPLIVQDNNLFLDFRAPLRLFNSDPVLGLNFYTPLAVRDEALTVNTGRGLTVSYDGLILNLGKDLRFDNNTVSVALSAALPLQYTDQLRLNVGAGLRYNPVSKKLDVNPNQNKGLTWENDYLIVKLGNGLGFDGNGNIAVSPQVTSPDTLWTTADPSPNCSIYTDLDAKMWLSLVKQGGVVHGSVALKALKGTLLSPTESAIVIILHFDNYGVRILNYPTLGTQGTLGNNATWGYRQGESADTNVLNALAFMPSSKRYPRGRGSEVQNQTVGYTCIQGDLSMPVPYQIQYNYGPTGYSFKFIWRTVSRQPFDIPCCFFSYITEE

SEQ ID NO: 24 - protein, 560 aa, Artificial Sequence
  Synthetic polypeptide sAd4312 Fiber-2
MKRARVDEDFNPVYPYDPPYAPIMPFITPPFTSSDGLQEKPLGVLSLKYKDPITTQNGSLTLKLGNGLNINNQGQLTSSAGEVEPPLTNADNKLALAYSDPLTLKNSRLTLSHNAPLAINNNSLSLEVSEPIFINNDNKLSLKADAPLTTSAGTLRLQSAAPLGLAEQTLKLLFSNPLYLRGDFLTLAIERPLAVTADGLLSLALNPPLTTTNTGLALSTAVPLTVTNGNLSLNVKRPFIIQDGSLYMDFRPPLYLFNSEPQLGVNFNAPLTVRDNGLAINTGDGLTVTYNKLTLNLGRDLQYENGAAAVKLSTAPPLQYTTQLQLNLGAGLRLGPTRNLDVAINHNKGLAWENNEVVTKLGQGLYFDSSGSIALSPTNPRPDTLWTTADPSPNCTVYESLDSRLWLALVKCGGMVHGSIALQAEKGQLLRPTASFISIVIYFYSDGVRRTNYPTIGNDEGTLANSATWGYRQGQSADTNVTNAVEFMPSLHRYPINQGDNIKNQMITYTCIQGNVNMPVPLKITFNHALEGYSLKFTWRVVANEKFDIPCCSFSYITEQ

SEQ ID NO: 25 - protein, 933 aa, Artificial Sequence
  Synthetic polypeptide sAd4287 Hexon
MATPSMMPQWSYMHIAGQDASEYLSPGLVQFARATDTYFSLGNKFRNPTVAPTHDVTTDRSQRLTLRFVPVDREDTAYSYKVRYTLAVGDNRVLDMASTYFDIRGVLDRGPSFKPYSGTAYNSLAPKGAPNPAEWADTNDSNKLKVRGQAPFVSTYGSATALTKDGIQVGVDTSEASQAVYADRSYQPEPQIGETEWNSEVGNDDRVAGRVLKKTTPMFPCYGSYAKPTNEKGGQAIQPTAGNGDNQAVELQFFATTSTPTAPKAVLYAEDVAIEAPDTHLVFKPTVVAGTTSSEALLTQQAAPNRPNYIAFRDNFIGLMYYNSTGNMGVLAGQASQLNAVVDLQDRNTELSYQLMLDALGDRSRYFSMWNQAVDSYDPDVRIVENHGVEDELPNYCFPLGGMVVTDTYKAIKVNGSGWTANTDVFSERVEIGSGNLFAMEINLQANLWRSFLYSNIGLYLPDSLKLTPDNITLPENKNTYQYMNGRVTPPGLVDTYVNVGARWSPDVMDSINPFNHHRNAGLRYRSMLLGNGRYVPFHIQVPQKFFAIKNLLLLPGSYTYEWNFRKDVNMILQSSLGNDLRVDGASIRFDSINLYANFFPMAHNTASTLEAMLRNDTNDQSFNDYLCAANMLYPIPANATSVPISIPSRNWAAFRGWSFTRLKTKETPSLGSGFDPYFVYSGSIPYLDGTFYLNHTFKKVSIMFDSSVSWPGNDRLLTPNEFEIKRSVDGEGYNVAQSNMTKDWFLVQMLSHYNIGYQGFYVPENYKDRMYSFFRNFQPMSRQVVDSVAYRDYYQDVKLPYQHNNSGFVGYMGPTMREGQAYPANYPYPLIGETAVPSLTQKKFLCDRVMWRIPFSSNFMSMGSLTDLGQNMLYANSAHALDMTFEVDPMDEPTLLYVLFEVFDVVRIHQPHRGVIEAVYLRTPFSAGNATT

SEQ ID NO: 26 - protein, 912 aa, Artificial Sequence
  Synthetic polypeptide sAd4310A Hexon
MATPSMMPQWSYMHIAGQDASEYLSPGLVQFARATDTYFSLGNKFRNPTVAPTHDVTTDRSQRLTLRFVPVDREDTAYSYKVRYTLAVGDNRVLDMASTYFDIRGVLDRGPSFKPYTGTAYNALAPKGAPNACQWTTTNGGNKTNTFAQAPLIGTAIDGTNGLQIGQDNGQAVYADKTFQPEPQVGESQWNTNPTTNAAGRVLKTTTRMLPCYGSFARPTNEKGGQASGDVTFQFFDTASDNGNNPKVVLYGEDVNIESPDTHLIYKPTADNTNSENLLGQQAAPNRANYIAFRDNFIGLMYYNSTGNMGVLAGQASQLNAVVDLQDRNTELSYQLMLDAIGDRSRYFSMWNQAVDSYDPDVRIIENHGVEDELPNYCFPLNAQGIANTYKGVKKNNGNWAKDDAVVETNEIGIGNVFAMEINLTANLWRNFLYSNIALYLPDSYKYSPGNITLPENKNSYNYINGRVTAPGLVDTFVNIGARWSPDPMDNVNPFNHHRNAGLRYRSMLLGNGRYVPFHIQVPQKFFAIKNLLLLPGSYTYEWNFRKDVNMILQSTLGNDLRVDGASVRFDSINLYANFFPMAHNTASTLEAMLRNDTNDQSFNDYLCAANMLYPIPANATSVPISIPSRNWAAFRGWSFTRLKTKETPSLGSGFDPYFVYSGSIPYLDGTFYLNHTFKKVSIMFDSSVSWPGNDRLLTPNEFEIKRSVDGEGYNVAQSNMTKDWFLIQMLSHYNIGYQGFYVPEAYKDRMYSFFRNFQPMSRQVVDADRYEQYKKVTVEYQHNNSGFVGYMGPTMREGQAYPANYPYPLIGDTAVPSLTQKKFLCDRTMWRIPFSSNFMSMGALTDLGQNMLYANSAHALDMTFEVDPMDEPTLLYVLFEVFDVVRIHQPHRGVIEAVYLRTPFSAGNATT

SEQ ID NO: 27 - protein, 928 aa, Artificial Sequence
  Synthetic polypeptide sAd4312 Hexon
MATPSMMPQWSYMHIAGQDASEYLSPGLVQFARATESYFSLGNKFRNPTVAPTHDVTTDRSQRLTLRFVPVDREDTAYSYKVRFTLAVGDNRVLDMASTYFDIRGMLDRGPSFKPYSGTAYNSLAPKGAPNPSQWTTTNGGNKTNSFAQASYIGQSLSKDGVQVAVDTAAGGAAVYADKTFQPEPQVGISQWNENPTTNAAGRILKPTTAMRPCYGSYAYPTNEKGGQVKITDPNNDKTGANNVSLNFFNTAADNGNNNPKVVLYSEDVNLEGPDTHLVFKPDVTGDATSAETLLGQQAAPNRPNYIGFRDNFIGLMYYNSTGNMGVLAGQASQLNAVVDLQDRNTELSYQLMLDALGDRSRYFSMWNQAVDSYDPDVRIIENHGVEDELPNYCFPLNGQGISNTYKGVKYNTNTWTQDTDVVTTNEISIGNIFAMEINLAANLWRSFLYSNVALYLPDSYKYTPDNIELPTNKNSYGYINGRVTAPTAIDTYVNIGARWSPDPMDNVNPFNHHRNAGLRYRSMLLGNGRYVPFHIQVPQKFFAIKNLLLLPGSYTYEWNFRKDVNMILQSTLGNDLRVDGASVRFDSINLYANFFPMAHNTASTLEAMLRNDTNDQSFNDYLCAANMLYPIPANATSVPISIPSRNWAAFRGWSFTRLKTKETPSLGSGFDPYFVYSGSIPYLDGTFYLNHTFKKVSIMFDSSVSWPGNDRLLTPNEFEIKRSVDGEGYNVAQSNMTKDWFLIQMLSHYNIGYQGFYVPEAYKDRMYSFFRNFQPMSRQVVDTVNYANYKEVTMPFQHNNSGFVGYMGPTMREGQAYPANYPYPLIGATAVPSLTQKKFLCDRTMWRIPFSSNFMSMGALTDLGQNMLYANSAHALDMTFEVDPMDEPTLLYVLFEVFDVVRIHQPHRGVIEAVYLRTPFSAGNATT

SEQ ID NO: 28 - protein, 168 aa, Artificial Sequence
  Synthetic polypeptide sAd4287 Fiber-1 Knob
LCTTPTAASNCTVFTNGDSLLCLCLTKCGAHVLGSVSLTGMQGTITAMTQNYISIQFLFDNNGALTSSPLLNNNTWGIRQNDTSSANPAYNALAFMPNSTVYVRGQSGEPRNNYYTQTYLRGNVKKPIILTVTYNSAASGYSLTFKWDAVVTEKFATPTSSFCYITEQ

SEQ ID NO: 29 - protein, 163 aa, Artificial Sequence
  Synthetic polypeptide sAd4310A Fiber-1 Knob
LWTAPTSTGNCTVYSEGDSLLSLCLTKCGAHVLGSVSLTGLTGTITQMTDISVTIQFTFDNNGKLLSSPLINNAFSIRQNDSTASNPTYNALAFMPNSTIYARGGGGEPRNNYYVQTYLRGNVQKPIILTVTYNSAATGYSLSFKWTALAREKFATPTTSFCY

SEQ ID NO: 30 - protein, 163 aa, Artificial Sequence
  Synthetic polypeptide sAd4312 Fiber-1 Knob
LWTPPTSNPNCTVYTESDSLLSLCLTKCGAHVLGSVSLTGVAGTMINMAETSLAIEFTFDDTGKLLHSPLVNTTFSIRQGDSPASNPTYNALAFMPNSTLYARGGSGEPRNNYYVQTYLRGNVQRPITLTVTFNSAATGYSLSFKWTAVAREKFAAPATSFCY

SEQ ID NO: 31 - protein, 171 aa, Artificial Sequence
  Synthetic polypeptide sAd4287 Fiber-2 Knob
LWTTADPSPNCSVYQDLDARLWLALVKSGDMVHGSIALKALKGTLLNPTASYISIVIYFYSNGVRRTNYPTFDNEGTLANSATWGYREGQSANTNVTNATEFMPSSTRYPVNKGDNIQNQSFSYTCIKGDFAMPVPFRVTYNHALEGYSLKFTWRVVANQAFDIPCCSFSY

SEQ ID NO: 32 - protein, 171 aa, Artificial Sequence
  Synthetic polypeptide sAd4310A Fiber-2 Knob
LWTTADPSPNCSIYTDLDAKMWLSLVKQGGVVHGSVALKALKGTLLSPTESAIVIILHFDNYGVRILNYPTLGTQGTLGNNATWGYRQGESADTNVLNALAFMPSSKRYPRGRGSEVQNQTVGYTCIQGDLSMPVPYQIQYNYGPTGYSFKFIWRTVSRQPFDIPCCFFSY

SEQ ID NO: 33 - protein, 172 aa, Artificial Sequence
  Synthetic polypeptide sAd4312 Fiber-2 Knob
LWTTADPSPNCTVYESLDSRLWLALVKCGGMVHGSIALQAEKGQLLRPTASFISIVIYFYSDGVRRTNYPTIGNDEGTLANSATWGYRQGQSADTNVTNAVEFMPSLHRYPINQGDNIKNQMITYTCIQGNVNMPVPLKITFNHALEGYSLKFTWRVVANEKFDIPCCSFSY

SEQ ID NO: 34 - DNA, 6109 bp, Artificial Sequence
  Synthetic oligonucleotide sAdApt4287.Empty
attaacatcatcaataatataccttattctggaaacgtgccaatatgataatgagcggggaggagcgaggcggggccggggtgacgtgcggtgacgcggggtgacgcggggtggcgcgagggcggggcgggagtggggaggcgcttagtttttacgtatgcggaaggaggttttataccggaagttgggtaatttgggcgtatatttgtaagttttgtgtaatttggcgcgaaaaccgggtaatgaggaagttgaggttaatatgtactttttatgactgggcggaatttctgctgatcagcagtgaactttgggcgctgacggggaggtttcgctacgtggcagtaccacgagaaggctcaaaggtcccatttattgtactcctcagcgttttcgctgggtatttaaacgctgtcagatcatcaagaggccactcttgagtgccggcgagtagagttttctcctgtcgactggtcaatattggccattagccatattattcattggttatatagcataaatcaatattggctattggccattgcatacgttgtatccatatcataatatgtacatttatattggctcatgtccaacattaccgccatgttgacattgattattgactagttattaatagtaatcaattacggggtcattagttcatagcccatatatggagttccgcgttacataacttacggtaaatggcccgcctggctgaccgcccaacgacccccgcccattgacgtcaataatgacgtatgttcccatagtaacgccaatagggactttccattgacgtcaatgggtggagtatttacggtaaactgcccacttggcagtacatcaagtgtatcatatgccaagtacgccccctattgacgtcaatgacggtaaatggcccgcctggcattatgcccagtacatgaccttatgggactttcctacttggcagtacatctacgtattagtcatcgctattaccatggtgatgcggttttggcagtacatcaatgggcgtggatagcggtttgactcacggggatttccaagtctccaccccattgacgtcaatgggagtttgttttggcaccaaaatcaacgggactttccaaaatgtcgtaacaactccgccccattgacgcaaatgggcggtaggcgtgtacggtgggaggtctatataagcagagctcgtttagtgaaccgtcagatcgcctggagacgccatccacgctgttttgacctccatagaagacaccgggaccgatccagcctccgcggccgggaacggtgcattggaagcttggtaccggtgaattcgctagcgttaacggatcctctagacgagatccgaacttgtttattgcagcttataatggttacaaataaagcaatagcatcacaaatttcacaaataaagcatttttttcactgcattctagttgtggtttgtccaaactcatcaatgtatcttatcatgtctagatccttaaggaatgcggagctaatcatttgaggttgtatcctgtaaccctgaacgtcaccgaggagctgaggacggaccaccacatgctgtcttgcctgcgtaccgactatgaatccagtgatgaggagtgaggtgaggggcggagccacaaagggtataaaggggcatgaagggtggacgcggtgtttcaaaatgagcgggacgacggacggcaatgcgtttgaggggggagtgttcagcccatatctgacatctcgtcttccttcctgggcaggagtgcgtcagaatgtagtgggctccaccgtggacggacggccggtcgcccctgcaaattccgccaccctcacctatgccaccgtgggatcatcgttggacactgccgcggcagctgccgcttctgctgccgcttctactgctcgcggcatggcggctgattttggactatataaccaactggccactgcagctgtggcgtctcggtctctggttcaagaagatgccctgaatgtgatcttgactcgcctggagatcatgtcacgtcgcctggacgaactggctgcgcagatatcccaagctaaccccgataccgcttcagaatcttaaataaagacaaacaaatttgttgaaaagtaaaatggctttatttgttttttttggctcggtaggctcgggtccacctgtctcggtcgttaaggactttgtgtatgttttccaaaacacggtacagatgggcttggatgttcaagtacatgggcatgaggccatctttggggtggagataggaccactgaagagcgtcatgttccggggtggtattgtaaatcacccagtcgtagcagggtttttgagcgtggaactggaatatgtccttcaggagcaggctaatggccaagggcagccccttagtgtaggtgtttacaaagcggttgagctgggagggatgcatgcggggggagatgatatgcatcttggcttggattttgaggttagctatgttaccacccaggtctctgcgggggttcatgttatgaaggaccaccagcacggtgtagccggtgcacttggggaacttgtcatgcagtttggaggggaaggcgtggaagaatttagatacccccttgtgcccccctaggttttccatgcactcatccataataatggcaatgggacccctggcggccgctttagcaaacacgttttgggggttggaaacatcatagttttgctctagagtgagctcatcataggccatctttacaaagcggggtaggagggtgcccgactgggggatgatagttccatctgggcctggagcgtagttgccctcacagatctgcatctcccaggccttaatttccgagggggggatcatgtccacctggggggcgataaagaacacggtttctggcgggggattgatgagctgggtggaaagcaagttacgcaatagctgggatttgccgcaaccggtggggccgtagatgaccccgatgacgggttgcagctggtagttcagagaggaacagctgccgtcggggcgcaggaggggggccacatcgttcatcatgcttctgacatgtttattttcactcactaagttttgcaagagcctctccccacccagggataagagttcttccaggctgttgaagtgtttcagcggtttcaggccgtcggccatgggcatcttttcaagcgactgacgaagcaagtacagtcggtcccagagctcggtgacgtgctctatggaatctcgatccagcagacttcttggttgcgggggttgggccgactttcgctgtagggcaccagccggtgggcgtccagggccgcgagggttctgtccttccagggtctcagcgttcgggtgagggtggtctcggtgacggtgaagggatgagccccgggctgggcgcttgcgagggtgcgcttcaggctcatcctgctggtgctgaagcgggcgtcgtctccctgtgagtcggccagatagcaacgaagcatgaggtcgtagctgagggactcggccgcgtgtcccttggcgcgcagctttcccttggaaacgtgctgacatttggtgcagtgcagacacttgagggcgtagagttttggggccaggaagaccgactcgggcgagtaggcgtcggctccgcactgagcgcagacggtctcgcactccaccagccacgtgagctcgggtttagcgggatcaaaaaccaagttgcctccattttttttgatgcgtttcttaccttgcgtctccatgagtctgtgtcccgcttccgtgacaaaaaggctgtcggtgtccccgtagaccgacttgagggggcgatcttccaaaggtgttccgaggtcttccgcgtacaggaactgggaccactccgagacaaaggctcgggtccaggctaacacgaaggaggcgatctgcgaggggtatctgtcgttttcaatgagggggtccaccttttccagggtgtgcagacacaggtcgtcctcctccgcgtccacgaagttaattaattcgaacccataatacccataatagctgtttgccatcgacgcgaggctggatggccttccccattatgattcttctcgcttccggcggcatcgggatgcccgcgttgcaggccatgctgtccaggcaggtagatgacgaccatcagggacagcttcaaggatcgctcgcggctcttaccagcccagcaaaaggccaggaaccgtaaaaaggccgcgttgctggcgtttttccataggctccgcccccctgacgagcatcacaaaaatcgacgctcaagtcagaggtggcgaaacccgacaggactataaagataccaggcgtttccccctggaagctccctcgtgcgctctcctgttccgaccctgccgcttaccggatacctgtccgcctttctcccttcgggaagcgtggcgctttctcatagctcacgctgtaggtatctcagttcggtgtaggtcgttcgctccaagctgggctgtgtgcacgaaccccccgttcagcccgaccgctgcgccttatccggtaactatcgtcttgagtccaacccggtaagacacgacttatcgccactggcagcagccactggtaacaggattagcagagcgaggtatgtaggcggtgctacagagttcttgaagtggtggcctaactacggctacactagaaggacagtatttggtatctgcgctctgctgaagccagttaccttcggaaaaagagttggtagctcttgatccggcaaacaaaccaccgctggtagcggtggtttttttgtttgcaagcagcagattacgcgcagaaaaaaaggatctcaagaagatcctttgatcttttctacggggtctgacgctcagtggaacgaaaactcacgttaagggattttggtcatgagattatcaaaaaggatcttcacctagatccttttaaattaaaaatgaagttttaaatcaatctaaagtatatatgagtaaacttggtctgacagttaccaatgcttaatcagtgaggcacctatctcagcgatctgtctatttcgttcatccatagttgcctgactccccgtcgtgtagataactacgatacgggagggcttaccatctggccccagtgctgcaatgataccgcgagacccacgctcaccggctccagatttatcagcaataaaccagccagccggaagggccgagcgcagaagtggtcctgcaactttatccgcctccatccagtctattaattgttgccgggaagctagagtaagtagttcgccagttaatagtttgcgcaacgttgttgccattgctgcaggcatcgtggtgtcacgctcgtcgtttggtatggcttcattcagctccggttcccaacgatcaaggcgagttacatgatcccccatgttgtgcaaaaaagcggttagctccttcggtcctccgatcgttgtcagaagtaagttggccgcagtgttatcactcatggttatggcagcactgcataattctcttactgtcatgccatccgtaagatgcttttctgtgactggtgagtactcaaccaagtcattctgagaatagtgtatgcggcgaccgagttgctcttgcccggcgtcaacacgggataataccgcgccacatagcagaactttaaaagtgctcatcattggaaaacgttcttcggggcgaaaactctcaaggatcttaccgctgttgagatccagttcgatgtaacccactcgtgcacccaactgatcttcagcatcttttactttcaccagcgtttctgggtgagcaaaaacaggaaggcaaaatgccgcaaaaaagggaataagggcgacacggaaatgttgaatactcatactcttcctttttcaatattattgaagcatttatcagggttattgtctcatgagcggatacatatttgaatgtatttagaaaaataaacaaataggggttccgcgcacatttccccgaaaagtgccacctgacgtctaagaaaccattattatcatgacattaacctataaaaataggcgtatcacgaggccctttcgtcttcaagaattggtcgatggcaaacagctattatgggtattatgggttcgaattaat

SEQ ID NO: 35 - DNA, 15808 bp, Artificial Sequence
  Synthetic oligonucleotide pBr/sAd4287.pIX-pV
attaagaatgcggagctaatcatttgaggttgtatcctgtaaccctgaacgtcaccgaggagctgaggacggaccaccacatgctgtcttgcctgcgtaccgactatgaatccagtgatgaggagtgaggtgaggggcggagccacaaagggtataaaggggcatgaagggtggacgcggtgtttcaaaatgagcgggacgacggacggcaatgcgtttgaggggggagtgttcagcccatatctgacatctcgtcttccttcctgggcaggagtgcgtcagaatgtagtgggctccaccgtggacggacggccggtcgcccctgcaaattccgccaccctcacctatgccaccgtgggatcatcgttggacactgccgcggcagctgccgcttctgctgccgcttctactgctcgcggcatggcggctgattttggactatataaccaactggccactgcagctgtggcgtctcggtctctggttcaagaagatgccctgaatgtgatcttgactcgcctggagatcatgtcacgtcgcctggacgaactggctgcgcagatatcccaagctaaccccgataccgcttcagaatcttaaataaagacaaacaaatttgttgaaaagtaaaatggctttatttgttttttttggctcggtaggctcgggtccacctgtctcggtcgttaaggactttgtgtatgttttccaaaacacggtacagatgggcttggatgttcaagtacatgggcatgaggccatctttggggtggagataggaccactgaagagcgtcatgttccggggtggtattgtaaatcacccagtcgtagcagggtttttgagcgtggaactggaatatgtccttcaggagcaggctaatggccaagggcagccccttagtgtaggtgtttacaaagcggttgagctgggagggatgcatgcggggggagatgatatgcatcttggcttggattttgaggttagctatgttaccacccaggtctctgcgggggttcatgttatgaaggaccaccagcacggtgtagccggtgcacttggggaacttgtcatgcagtttggaggggaaggcgtggaagaatttagatacccccttgtgcccccctaggttttccatgcactcatccataataatggcaatgggacccctggcggccgctttagcaaacacgttttgggggttggaaacatcatagttttgctctagagtgagctcatcataggccatctttacaaagcggggtaggagggtgcccgactgggggatgatagttccatctgggcctggagcgtagttgccctcacagatctgcatctcccaggccttaatttccgagggggggatcatgtccacctggggggcgataaagaacacggtttctggcgggggattgatgagctgggtggaaagcaagttacgcaatagctgggatttgccgcaaccggtggggccgtagatgaccccgatgacgggttgcagctggtagttcagagaggaacagctgccgtcggggcgcaggaggggggccacatcgttcatcatgcttctgacatgtttattttcactcactaagttttgcaagagcctctccccacccagggataagagttcttccaggctgttgaagtgtttcagcggtttcaggccgtcggccatgggcatcttttcaagcgactgacgaagcaagtacagtcggtcccagagctcggtgacgtgctctatggaatctcgatccagcagacttcttggttgcgggggttgggccgactttcgctgtagggcaccagccggtgggcgtccagggccgcgagggttctgtccttccagggtctcagcgttcgggtgagggtggtctcggtgacggtgaagggatgagccccgggctgggcgcttgcgagggtgcgcttcaggctcatcctgctggtgctgaagcgggcgtcgtctccctgtgagtcggccagatagcaacgaagcatgaggtcgtagctgagggactcggccgcgtgtcccttggcgcgcagctttcccttggaaacgtgctgacatttggtgcagtgcagacacttgagggcgtagagttttggggccaggaagaccgactcgggcgagtaggcgtcggctccgcactgagcgcagacggtctcgcactccaccagccacgtgagctcgggtttagcgggatcaaaaaccaagttgcctccattttttttgatgcgtttcttaccttgcgtctccatgagtctgtgtcccgcttccgtgacaaaaaggctgtcggtgtccccgtagaccgacttgagggggcgatcttccaaaggtgttccgaggtcttccgcgtacaggaactgggaccactccgagacaaaggctcgggtccaggctaacacgaaggaggcgatctgcgaggggtatctgtcgttttcaatgagggggtccaccttttccagggtgtgcagacacaggtcgtcctcctccgcgtccacgaaggtgattggcttgtaagtgtaggtcacgtgacccgcacccccccaaggggtataaaagggggcgtgcccactctccccgtcactttcttccgcatcgctgtggaccagagccagctgttcgggtgagtaggccctctcaaaagccggcatgatttcggcgctcaagttgtcagtttctacaaacgaggtggatttgatattcacgtgccccgcggcgatgcttttgatggtggaggggtccatctgatcagaaaacacgatctttttattgtcaagtttggtggcgaaagacccgtagagggcgttggaaagcaacttggcgatggagcgcagggtctgatttttctcccgatcggccctctccttggcagcgatgttgagttgcacgtactcgcgagccacgcaccgccactcggggaacacggcggtgcgctcgtcgggcaggatgcgcacgtgccagccgcggttgtgcagggtgatgaggtccacgctggtggccacctccccgcggaggggctcgttggtccaacacaatcgccccccttttctggagcagaacggaggcaggggatctagcaagttggcgggcggggggtcggcgtcgatggtaaatatgccgggtagcagaattttattaaaataatcgatttcggtgtccgtgtcttgcaacgcgtcttcccacttcttcaccgccagggccctttcgtagggattcaggggcggtccccagggcatggggtgggtcagggccgaggcgtacatgccgcagatgtcgtacacgtacaggggctccctcaacaccccgatgtaagtggggtaacagcgccccccgcggatgctggctcgcacgtagtcgtacatctcgtgagagggagccatgagcccgtctcccaagtgggtcttgtggggtttctcggcccggtagaggatctgcctgaagatggcgtgggagttggaagagatggtggggcgttggaagacattaaagttggctccgggcagtcccacggagtcttggatgaactgggcgtaggattcccggagcttgtccaccagggctgcggttaccagcacgtcgagagcgcagtagtccaacgtctcgcggaccaggttgtaggccgtctcttgttttttctcccacagttcgcgattgaggaggtattcctcgcggtctttccagtactcttcggcgggaaatcctttttcgtccgctcggtaagaacctaacatgtaaaattcgttcacggctttgtatggacaacagcctttttctaccggcagggcgtacgcttgagcggcctttctgagagaggtgtgggtgagggcgaaggtgtcccgcaccatcactttcaggtactgatgtttgaagtccgtgtcgtcgcaggcaccctgttcccacagcgtgaagtcggtgcgctttttctgcctgggattggggagggcgaatgtgacgtcgttaaaaaggattttcccggagcggggcatgaagttgcgagagatcctgaagggtccgggcacgtccgagcggttgttgatgacttgtgccgccaggacgatctcgtcgaagccgttgatgttgtggcccacgatgtaaagttcgataaagcgcggctgtcccttgagggccggcgcttttttcaactcctcgtaggtgagacagtccggcgaggagagacccagctccgcccgggcccagtcggagagctgagggttagccgcgaggaaagagctccataggtcaagggctagcagagtttgcaagcggtcgcggaactcgcgaaactttttccccacggccattttctccggcgtcaccacgtagaaagtgcaggggcggtcgttccagacgtcccatcggagctctagggccagctcgcaggcttggcgaacgagggtctcctcgcccgagacgtgcatgaccagcatgaagggtaccaactgtttcccgaacgagcccatccatgtgtaggtttctacgtcgtaggtgacaaagagccgctgggcgcgcgcgtgggagccgatcgggaagaagctgatctcctgccaccagttggaggaatgggtgttgatgtggtgaaagtagaagtcccgccggcgcacagagcattcgtgctgatgtttgtaaaagcgaccgcagtagtcgcagcgctgcacgctctgtatctcctgaatgagatgcgcttttcgcccgcgcaccagaaaccggagggggaagttgagacggggggcttgtggggcggcatcccattcgccttggcggtgggagtctgcgtctgcgtcctccttctctgggtggacgacggtggggacgacaacgccccgggtgccgcaagtccagatctccgccacggaggggcgcaggcgctgcaggaggggacgcagctgcccgctgtccagggagtcgagggcggccgcgctgaggtcggcgggaagcgtttgcaagttcactttcagaagaccggtaagagcgtgagccaggtgcagatggtacttgatttccaggggggtgttggaagaggcgtccacggcgtagaggaggccgtgtccgcgcggggccaccaccgtgccccgaggaggttttatctcaatcgtcgagggcgagcgccggggggtagaggcggctctgcgccggggggcagcggaggcagcggcacgttttcgtgaggatttggcagcggttgatgacgagcccggagactgctggcgtgggcgacgacgcggcggttgaggtcctggatgtgccgtctctgcgtgaagaccaccggcccccgggtcctgaacctgaaagagagttccacagaatcaatgtctgcatcgttaacggcggcctgcctgaggatctcctgtacgtcgcccgagttgtcttgataggcgatctcggccatgaactgctccacttcttcctcgcggaggtcgccgtggcccgctcgctccacggtggcggccaggtcgttggagatgcgacgcatgagttgagagaaggcgttgaggccgttctcgttccacacgcggctgtacaccacgttgccgaaggagtcgcgcgctcgcatgaccacctgggccacgttgagttccacgtggcgggcgaagacggcgtagtttctgaggcgctggaagaggtagttgagcgtggtggcgatgtgctcgcagacgaagaagtacatgatccagcgccgcagggtcatctcgttgatgtctccgatggcttcgagacgctccatggcctcgtagaagtcgacggcgaagttgaaaaattgggagttgcgggcggccaccgtgagttcttcttgcaggaggcggatgagatcggcgaccgtgtcgcgcacctcctgctcgaaagcgccccgaggcgcctctgcttcttcctccggctcctcctcttccaggggcacgggttcctccggcagctctgcgacggggacggggcggcgacgtcgtcgtctgaccggcaggcggtccacgaagcgctcgatcatttcgccgcgccggcgacgcatggtctcggtgacggcgcgtccgttttcgcgaggtcgcagttcgaagacgccgccgcgcagagcgcccccgtgcagggagggtaagtggttagggccgtcgggcagggacacggcgctgacgatgcattttatcaattgctgcgtaggcactccgtgcagggatctgagaacgtcgaggtcgacgggatccgagaacttctctaagaaagcgtctatccaatcgcagtcgcaaggtaagctgaggacagtgggtcgctggggggcgtccgcgggcagttgggaggtgatgctgctgatgatgtaattaaagtaggcggtcttcaggcggcggatggtggcgaggaggaccacgtctttgggcccggcctgttgaatgcgcaggcgctcggccatgccccaggcctcgctctgacagcgacgcaggtctttgtagtagtcttgcatcagtctctccaccggaacctctgcttctcccctgtctgccatgcgagtcgagccgaacccccgcaggggctgcagcaacgctaggtcggccacgaccctttcggccagcacggcctgttgaatctgcgtgagggtggtctggaagtcgtccaggtccacgaagcggtgataggcccccgtgttgatggtgtaggtgcagttggccatgacggaccagttgacgacttgcataccgggttgggtgatctccgtgtacttgaggcgcgagtaggcgcgggactcgaacacgtagtcgttgcatgtgcgcaccagatactggtagccgaccaggaagtgaggaggcggctctcggtacaggggccagccgacggtggcgggggcgccgggggacaggtcgtccagcatgaggcgatggtagtggtagatgtagcgggagagccaggtgatgccggccgaggtggtcgcggccctggtgaattcccggacgcggttccagatgttgcgcaggggacggaagcgttccatggtgggcacgctctgccccgtgaggcgggcgcagtcctgtacgctctagatggaaaaaagacagggcggtcatcgactcccttccgtagcttggggggtaaagtcgcaagggtgcggcggcggggaaccccggttcgagaccggccggatccgccgctcccgatgcgcctggccccgcatccacgacgtccgcgccgagacccagccgcgacgctctgccccaatacggaggggagtcttttggtgttttttcgtagatgcatccggtgctgcggcagatgcgacctcagacgcccaccaccaccgccgcggcggcagtaaacctgagcggaggcggtgacagggaggtggaggagctggctttagacctggaagagggagaggggctggcccggctgggagcgccgtccccagagagacaccctagggttcagctcgtgagggacgccaggcaggcttttgtgccgaagcagaacctgtttagggaccgcagcggtcaggaggcggaggagatgcgcgattgcaggtttcgggcgggtagagagctgagggcgggcttcgatcgcgagcggctcctgagggcggaggatttcgagcccgacgagcgttctggggtgagcccggcccgcgctcacgtctcggcggccaacctggtgagcgcgtacgagcagacggtgaacgaggagcgcaacttccaaaagagctttaacaatcacgtgaggaccctgatcgcgagggaggaggtgaccatcgggctgatgcatctgtgggacttcgtggaggcctacgtgcagaacccggccagcaaacctctgacggcccagctgttcctgatcgtgcagcacagccgcgacaacgagacgttccgcgacgccatgttgaacatcgcggagcccgagggtcgctggctcttggatctgattaacatcctgcagagcatcgtggtgcaggagaggggtctgagtttagcggacaaggtggcggccattaactattcgatgcagagcctggggaagttctacgctcgcaagatctacaagagcccttacgtgcccatagacaaggaggtgaagatagacagcttttacatgcgcatggcgctaaaggtgctgacgctgagcgacgacctcggcgtgtaccgtaacgacaagatccacaaggcggtgagcgccagccgccggcgggagctgagcgacagggagctgatgcacagcctgcagagggcgctggcgggcgccggggacgaggagcgtgaggcttactttgacatgggagccgatctgcagtggcgtcccagcgcgcgcgccttggaggcggcgggttatcccgacgaggaggatcgggacgatttggaggaggcaggcgagtacgaggacgaagcctgaccgggcaggtgttgttttagatgcagcggccggcggacggggccaccgcggatcccgcacttttggcatccatgcagagtcaaccttcgggcgtgaccgcctccgatgactgggcggcggccatggaccgcatcatggcgctgaccacccgcaaccccgaggcttttaggcagcaaccccaggccaaccgtttttcggccatcttggaagcggtggtgccctcccgcaccaaccccacacacgagaaagtcctgactatcgtgaacgccctggtagacagcaaggccatccgccgcgacgaggcgggcttgatttacaacgctctgctggaacgggtggcgcgctacaacagcactaacgttcagaccaatctggatcgcctcaccaccgacgtgaaggaggcgctggctcagaaggagcggtttctgagggacagcaatctgggctctctggtggcactcaacgccttcctgagcacgcagccggccaacgtgccccgcgggcaggaggactacgtgagcttcatcagcgctctgaggctgctggtgtccgaggtgccccagagcgaggtgtatcagtctgggccggattacttcttccagacgtcccgacagggcttgcaaacggtgaacctgactcaggcctttaaaaacttgcaaggcatgtggggcgttaaggccccggtgggcgatcgagccaccatctccagtctgctgacccccaacactcgcctgctgctgctcttgatcgcgccgttcaccaacagtagcactatcagccgtgactcgtacctgggtcatctcatcactttgtaccgcgaggccatcggtcaggctcagattgacgagcatacatatcaggagatcactaacgtgagccgggccctgggtcaggaagataccggcagcctggaagccacgttgaactttttgctaaccaaccggaggcaaaaaataccctcccagtttacgttaagcgccgaggaggagaggattctgcgatacgtgcagcagtccgtgagtctgtacttgatgcgggagggcgccaccgcttccacggctttagacatgacggctcggaacatggaaccgtccttttactccgcccaccggccgttcattaaccgtctgatggactacttccatcgcgcggccgccatgaacggggagtattttaccaatgccatcctgaatccgcattggatgcccccgtccggcttctacaccggcgagtttgacctgcccgaagccgacgacggctttctttgggacgacgtgtccgacagcattttcacgccgggcaatcgccgattccagaagaaggagggcggagacgagctccccctctccagcgtggaggcggcctctaggggagagagtccctttcccagtctgtcttccgccagcagtggtcgggtaacgcgcccgcggttgccgggggagagcgactacctgaacgaccccttgctgcggccggctaggaagaaaaatttccccaacaacggggtggaaagcttggtggataaaatgaatcgttggaagacctacgcccaggagcagcgggagtgggaggacagtcagccgcgaccgctggttccgccgcactggcgtcgtcagagagaagacccggacgactccgcagacgatagtagcgtgttggacctgggagggagcggagccaacccctttgctcacttgcaacccaaggggcgttcgagccgcctctactaataaaaaagaagcggaaacttaccagagccatggccacagcgtgtgtgctttcttcctctctttcttcctcggcgcggcagaatgagaagagcggtgagagtcacgccggcggcgtatgagggtccgcccccttcttacgaaagcgtgatgggatcagcgaacgtgccggccacgctggaggcgccttacgttcctcccagatacctgggacctacggagggcagaaacagcatccgttactccgagctggcacccctgtacgataccaccaaggtgtacctggtggacaacaagtcggcggacatcgcctccctgaattatcaaaacgatcacagcaactttctgactaccgtggtgcagaacaatgacttcaccccgacggaggcgggcacgcagaccattaactttgacgagcgttcccgctggggcggtcagctgaaaaccatcctgcacaccaacatgcccaacatcaacgagttcatgtccaccaacaagttcagggctaagctgatggtagaaaaaagtaatgcggaaactcggcagccccgatacgagtggttcgagtttaccattccagagggcaactattccgaaactatgactatcgatctcatgaataacgcgatcgtggacaattacctgcaagtggggagacagaacggggtgctggaaagcgatatcggcgtgaaattcgataccagaaacttccgactggggtgggatcccgtgaccaagctggtgatgccaggcgtgtacaccaacgaggcttttcaccccgacatcgtgctgctgccggggtgcggtgtggacttcactcagagccgtttgagtaacctgttaggaattagaaagcgccgccccttccaagagggctttcaaatcatgtatgaggacctggagggaggtaatatacccgccttactggacgtgtcgaagtacgaagctagcatacaacgcgccaaagcggagggtagagagattcggggagacacctttgcggtagctccccaggacctggaaatagtgcctttaactaaagacagcaaagacagaagctacaatattataaacaacacgacggacaccctgtatcggagctggtttctggcttacaactacggagaccccgagaaaggagtgagatcatggaccatactcaccaccacggacgtgacctgtggctcgcagcaagtgtactggtccctgccggatatgatgcaagacccggtcaccttccgcccctccacccaagtcagcaacttcccggtggtgggcaccgagctgctgcccgtccatgccaagagcttctacaacgagcaggccgtctactcgcaacttattcgccagtccaccgcgcttacccacgtgttcaatcgctttcccgagaaccagattctggtgcgccctcccgctcctaccattaccaccgtcagtgaaaacgttcccgccctcacagatcacggaaccctgccgctgcgcagcagtatcagtggagttcagcgcgtgaccatcaccgacgccagacgtcgaacctgcccctacgtttacaaagcgcttggcgtggtggctcctaaagttctttctagtcgcaccttctaaaaacatgtccatcctcatctctcccgataacaacaccggctggggactgggctccggcaagatgtacggcggagccaaaaggcgctccagtcagcacccagttcgagttcggggccacttccgcgctccttggggagcttacaagcgaggactctcgggtcgaacggctgtagacgataccatagatgccgtgattgccgacgcccgccggtacaaccccggaccggtcgctagcgccgcctccaccgtggattccgtgatcgacagcgtggtagccggcgctcgggcctatgctcgccgcaagaggcggctgcatcggagacgtcgccccaccgccgccatgctggcagccagagccgtgctgagacgggcccggagggtaggcaggagggctatgcgccgcgctgccgccaacgccgccgccgggagggcccgccgacaggctgcccgccaggctgctgccgccatcgctagcatggccagacccaggagagggaacgtgtactgggtgcgcgattctgtgacgggagtccgagtgccggtgcgcagccgacctccccgaagttagaagatccaagctgcgaagacggcggtactgagtctccctgttgttatcagcccaacatgagcaagcgcaagtttaaagaagaactgctgcagacgctggtgcctgagatctatggccctccggacgtgaagcctgacattaagccccgcgatatcaagcgtgttaaaaagcgggaaaagaaagaggaactcgcggtggtagacgatggcggagtggaatttattaggagtttcgccccgcggcgcagggttcaatggaaagggcgacgggtacaacgcgttttgaggccgggcaccgcggtagtttttaccccgggagagcggtcggccgttaggggttttaaaaggcagtacgacgaggtgtacggcgacgaggacatattggaacaggcggctcaacagatcggagaatttgcctatggaaagcgctcgcgtcgcgaagacctggccatcgccttagacagcggcaaccccacgcccagcctcaaacccgtgacgctgcagcaggtgcttcccgtgagcgccagcacggacagcaagaggggaataaaaagagaaatggaagatctgcagcctaccatccagctcatggttcctaaacggcagaggctggaagaggtcctggagaagatgaaagtggaccccagcatagagccggacgttaaagtcaggccgatcaaagaagtggcccctggactcggggtgcagacggtggatatccagatccccgtcacgtcagcttcgaccgccgtggaagccatggaaacgcaaaccgaaacccccgccgtggttggtaccaaagaagtggcgttgcaaaccgacccctggtacgaatttgccgccccccggcgtcagaggcgacccgctcgttacggccccgccaacgccatcatgccagaatatgcgctgcatccgtctatcctgcccacccccggctaccggggagtgacgtatcgcccgtcaggaacccgccgccgaacccgtcgccgccgccgctcccgtcgcgctctggcccccgtgtcggtgcgccgcgtaacacgccggggaaagacagtcaccattcccaacccgcgctaccaccctagcatcctttaatgactctgccgttttgcagatggctctgacttgccgcgtgcgccttcccgttccgcactatcgaggaagatctcgtcgtaggagaggcatggcgggcagtggtcgccggcgggctttgcgcaggcgcatgaaaggcggaattttacccgctttgatacccataatcgccgccgccatcggtgccatacccggcgtcgcttcagtggccttgcaagcagctcgtaataaataaacgaaggcttttgcacttatgtcctggtcctgactattttatgcagaaagagcatggaagacatcaattttacgtcgctggctccgcggcacggctcgcggccgctcatgggcacctggaacgacatcggcaccagtcagttaattaattcgaacccataatacccataatagctgtttgccatcgacgcgaggctggatggccttccccattatgattcttctcgcttccggcggcatcgggatgcccgcgttgcaggccatgctgtccaggcaggtagatgacgaccatcagggacagcttcaaggccagcaaaaggccaggaaccgtaaaaaggccgcgttgctggcgtttttccataggctccgcccccctgacgagcatcacaaaaatcgacgctcaagtcagaggtggcgaaacccgacaggactataaagataccaggcgtttccccctggaagctccctcgtgcgctctcctgttccgaccctgccgcttaccggatacctgtccgcctttctcccttcgggaagcgtggcgctttctcatagctcacgctgtaggtatctcagttcggtgtaggtcgttcgctccaagctgggctgtgtgcacgaaccccccgttcagcccgaccgctgcgccttatccggtaactatcgtcttgagtccaacccggtaagacacgacttatcgccactggcagcagccactggtaacaggattagcagagcgaggtatgtaggcggtgctacagagttcttgaagtggtggcctaactacggctacactagaaggacagtatttggtatctgcgctctgctgaagccagttaccttcggaaaaagagttggtagctcttgatccggcaaacaaaccaccgctggtagcggtggtttttttgtttgcaagcagcagattacgcgcagaaaaaaaggatctcaagaagatcctttgatcttttctacggggtctgacgctcagtggaacgaaaactcacgttaagggattttggtcatgagattatcaaaaaggatcttcacctagatccttttaaattaaaaatgaagttttaaatcaatctaaagtatatatgagtaaacttggtctgacagttaccaatgcttaatcagtgaggcacctatctcagcgatctgtctatttcgttcatccatagttgcctgactccccgtcgtgtagataactacgatacgggagggcttaccatctggccccagtgctgcaatgataccgcgagacccacgctcaccggctccagatttatcagcaataaaccagccagccggaagggccgagcgcagaagtggtcctgcaactttatccgcctccatccagtctattaattgttgccgggaagctagagtaagtagttcgccagttaatagtttgcgcaacgttgttgccattgctgcaggcatcgtggtgtcacgctcgtcgtttggtatggcttcattcagctccggttcccaacgatcaaggcgagttacatgatcccccatgttgtgcaaaaaagcggttagctccttcggtcctccgatcgttgtcagaagtaagttggccgcagtgttatcactcatggttatggcagcactgcataattctcttactgtcatgccatccgtaagatgcttttctgtgactggtgagtactcaaccaagtcattctgagaatagtgtatgcggcgaccgagttgctcttgcccggcgtcaacacgggataataccgcgccacatagcagaactttaaaagtgctcatcattggaaaacgttcttcggggcgaaaactctcaaggatcttaccgctgttgagatccagttcgatgtaacccactcgtgcacccaactgatcttcagcatcttttactttcaccagcgtttctgggtgagcaaaaacaggaaggcaaaatgccgcaaaaaagggaataagggcgacacggaaatgttgaatactcatactcttcctttttcaatattattgaagcatttatcagggttattgtctcatgagcggatacatatttgaatgtatttagaaaaataaacaaataggggttccgcgcacatttccccgaaaagtgccacctgacgtctaagaaaccattattatcatgacattaacctataaaaataggcgtatcacgaggccctttcgtcttcaagaattggtcgatggcaaacagctattatgggtattatgggttcgaattaat

SEQ ID NO: 36 - DNA, 23168 bp, Artificial Sequence
  Synthetic oligonucleotide pBr/sAd4287.PsiI-rITR
attaacccaggacctggaaatagtgcctttaactaaagacagcaaagacagaagctacaatattataaacaacacgacggacaccctgtatcggagctggtttctggcttacaactacggagaccccgagaaaggagtgagatcatggaccatactcaccaccacggacgtgacctgtggctcgcagcaagtgtactggtccctgccggatatgatgcaagacccggtcaccttccgcccctccacccaagtcagcaacttcccggtggtgggcaccgagctgctgcccgtccatgccaagagcttctacaacgagcaggccgtctactcgcaacttattcgccagtccaccgcgcttacccacgtgttcaatcgctttcccgagaaccagattctggtgcgccctcccgctcctaccattaccaccgtcagtgaaaacgttcccgccctcacagatcacggaaccctgccgctgcgcagcagtatcagtggagttcagcgcgtgaccatcaccgacgccagacgtcgaacctgcccctacgtttacaaagcgcttggcgtggtggctcctaaagttctttctagtcgcaccttctaaaaacatgtccatcctcatctctcccgataacaacaccggctggggactgggctccggcaagatgtacggcggagccaaaaggcgctccagtcagcacccagttcgagttcggggccacttccgcgctccttggggagcttacaagcgaggactctcgggtcgaacggctgtagacgataccatagatgccgtgattgccgacgcccgccggtacaaccccggaccggtcgctagcgccgcctccaccgtggattccgtgatcgacagcgtggtagccggcgctcgggcctatgctcgccgcaagaggcggctgcatcggagacgtcgccccaccgccgccatgctggcagccagagccgtgctgagacgggcccggagggtaggcaggagggctatgcgccgcgctgccgccaacgccgccgccgggagggcccgccgacaggctgcccgccaggctgctgccgccatcgctagcatggccagacccaggagagggaacgtgtactgggtgcgcgattctgtgacgggagtccgagtgccggtgcgcagccgacctccccgaagttagaagatccaagctgcgaagacggcggtactgagtctccctgttgttatcagcccaacatgagcaagcgcaagtttaaagaagaactgctgcagacgctggtgcctgagatctatggccctccggacgtgaagcctgacattaagccccgcgatatcaagcgtgttaaaaagcgggaaaagaaagaggaactcgcggtggtagacgatggcggagtggaatttattaggagtttcgccccgcggcgcagggttcaatggaaagggcgacgggtacaacgcgttttgaggccgggcaccgcggtagtttttaccccgggagagcggtcggccgttaggggttttaaaaggcagtacgacgaggtgtacggcgacgaggacatattggaacaggcggctcaacagatcggagaatttgcctatggaaagcgctcgcgtcgcgaagacctggccatcgccttagacagcggcaaccccacgcccagcctcaaacccgtgacgctgcagcaggtgcttcccgtgagcgccagcacggacagcaagaggggaataaaaagagaaatggaagatctgcagcctaccatccagctcatggttcctaaacggcagaggctggaagaggtcctggagaagatgaaagtggaccccagcatagagccggacgttaaagtcaggccgatcaaagaagtggcccctggactcggggtgcagacggtggatatccagatccccgtcacgtcagcttcgaccgccgtggaagccatggaaacgcaaaccgaaacccccgccgtggttggtaccaaagaagtggcgttgcaaaccgacccctggtacgaatttgccgccccccggcgtcagaggcgacccgctcgttacggccccgccaacgccatcatgccagaatatgcgctgcatccgtctatcctgcccacccccggctaccggggagtgacgtatcgcccgtcaggaacccgccgccgaacccgtcgccgccgccgctcccgtcgcgctctggcccccgtgtcggtgcgccgcgtaacacgccggggaaagacagtcaccattcccaacccgcgctaccaccctagcatcctttaatgactctgccgttttgcagatggctctgacttgccgcgtgcgccttcccgttccgcactatcgaggaagatctcgtcgtaggagaggcatggcgggcagtggtcgccggcgggctttgcgcaggcgcatgaaaggcggaattttacccgctttgatacccataatcgccgccgccatcggtgccatacccggcgtcgcttcagtggccttgcaagcagctcgtaataaataaacgaaggcttttgcacttatgtcctggtcctgactattttatgcagaaagagcatggaagacatcaattttacgtcgctggctccgcggcacggctcgcggccgctcatgggcacctggaacgacatcggcaccagtcagctcaacgggggcgctttcaattgggggagcctttggagcggcattaaaaactttggctccacgattaaatcctacggcagcaaagcctggaacagtagtgctggtcagatgctccgagataaactgaaggacaccaacttccaagaaaaagtggtcaatggggtggtgaccggcatccacggtgcggtagatctcgccaaccaagcggtgcagaaagagattgacaggcgtttggaaaactcgcgggtgccgccgcagaggggggatgaggtggaggtcgaggaagtagaagtagaggaaaagctgcccccgctggagaaagttcccggtgcacctccgaggccgcagaagcggcccaggccagaactagaagaaactctggtgacggagagcaaggagcctccctcgtacgagcaagccttgaaagagggcgcctctccaccctcctacccgatgactaagccgatcgcacccatggctcgaccggtgtacggcaaggattacaagcccgtcacgctagagctgcccccaccgcccccttcgcgtccgacggtgcctccgctgcctgccccgtcggcgggtcccgagtctgcaccatccgctgtgcctctgccagccgcccgtcccgtggccgtggccactgccaggaaccccagaggccagagaggagccaactggcaaagcacgctgaacagcatcgtgggcctgggggtgaaaagcctgaaacgccgccgttgctattattaaaaagtgtagctaaaaaatttcccgttgtatacgcctcctatgttaccgccagagacgcgtgactgtcgccgcgagcgccgcttccaagatggccaccccatcgatgatgccgcagtggtcttacatgcacatcgccggccaggacgcctcggagtacctgagtcccggcctcgtgcagtttgcccgcgccaccgacacctacttcagcttgggaaacaagtttagaaaccccaccgtggcccccacccacgatgtgaccacggaccgctcgcagaggctgaccctgcgctttgtgcccgtagaccgggaggacaccgcgtactcttacaaagtgcgctacacgctggccgtaggggacaaccgagtgctggacatggccagcacctactttgacatccggggggtgctggatcggggtcccagcttcaagccctactccggcaccgcttacaactccctggctcccaagggcgcccccaatcctgcagaatgggccgataccaacgacagcaacaaactgaaagtgaggggtcaggcgccttttgtcagtacttacggttctgctacggcgcttacaaaagatgggatacaggtgggagtggatacttccgaagcatctcaggctgtttatgccgacagaagttaccagccagaaccccaaattggagagacagagtggaacagcgaagtgggtaatgacgacagagtggcgggaagggtgctaaagaaaacaactcccatgttcccttgttacggttcatatgccaagcccaccaacgaaaaaggcggacaagcaatacagcccaccgccggcaacggcgataatcaggctgtagagttacaattctttgccactactagcactcccactgcgccaaaggcagtattgtacgcggaggacgtggccattgaagctccagatactcacttagtgtttaagccaacagtagtcgcgggaactacaagttcggaagctctgctaacccaacaagccgcacctaaccgcccaaactacattgcctttagagataactttattggtctcatgtactacaattcaaccgggaatatgggagtactggccggacaagcatctcagctcaatgcagtggttgatcttcaggacagaaacaccgaactgtcatatcagctaatgctggatgctctgggagatcgcagtcggtacttttctatgtggaatcaagctgtagatagctatgatccagatgtaagaattgtagaaaaccacggtgtggaagacgaactgcctaattattgcttcccactaggcgggatggtagtaacggacacttacaaagccataaaggtaaatggaagcggatggacggctaatactgacgttttcagcgagagagtagaaataggctcaggtaacctgtttgccatggaaattaacttgcaagctaatctgtggcgcagtttcttgtattccaacataggactgtacctcccggactctttaaaattaacccctgacaacatcacgctccctgagaacaaaaatacctaccagtatatgaacggtcgcgtaacaccacccgggctcgtggacacctacgttaacgtgggtgcgcgctggtcccccgatgttatggacagcattaacccttttaaccaccaccgcaacgccgggctccgctaccgttccatgctcctgggaaacggacgctacgtacccttccacattcaggtgccccagaaattctttgcaattaaaaacctgctgctgctccccggttcctatacctacgagtggaatttccgcaaggacgtgaacatgattttgcaaagctcgctgggtaacgacctgcgagttgacggggccagcatacgcttcgacagcatcaacctgtatgctaactttttccccatggcccacaacacggcctccaccctggaagccatgctgcgcaacgacaccaatgaccagtccttcaacgactacctgtgcgcggccaacatgctgtatcccatccccgccaacgccaccagcgtgcccatctccatcccgtctcgcaactgggccgcctttaggggttggagtttcacccgcctcaaaaccaaggaaaccccctcgctgggctctggcttcgacccctacttcgtctactcaggctccattccctacctggacggcactttctatcttaaccacactttcaaaaaggtgtctatcatgttcgattcctcggtcagctggcccggcaacgaccgcctgctgacgcccaacgagttcgaaatcaagcgttcggtggacggtgaagggtacaacgtggcccagagcaacatgaccaaggactggttcctggttcaaatgctcagccattacaacatcggttaccagggcttctatgtgcccgagaactacaaggaccgcatgtactccttctttaggaacttccaacccatgagtcgccaagtcgtggactcagtggcttacagggactactaccaggacgttaagctcccctaccagcacaacaactcagggttcgtgggctacatgggtcccaccatgcgagaggggcaggcctacccggccaactatccttatcccctaatcggagagactgctgtacccagcctgacgcagaaaaagttcctctgcgaccgggtgatgtggaggatacccttctctagcaacttcatgtctatgggctccctcaccgacctggggcagaacatgctgtacgccaactccgctcacgccttggacatgacctttgaggtggatcccatggatgagcccacgcttctctatgttctgtttgaagtcttcgacgtggtgcgcatccaccagccgcaccgcggcgtcatcgaggccgtctacctgcgcacacctttctctgccggtaacgccaccacctaaagaagccgatgggctccagcgaacaggagctgcaggccattgttcgcgacctgggctgcgggccctactttttgggcaccttcgacaagcggttccccggcttcatgtcccctcacaagccggcctgtgccatcgttaacacggccggacgggaaaccgggggggtccactggctcgccttcgcctggaacccgcgtaaccgcacctgctacctgttcgacccttttggtttctccgacgaaaggctgaagcagatctaccagttcgagtacgaggggctcctccagcgcagcgctctggcctccacgcccgaccactgcgtcaccctggaaaagtccacccagacggtccaggggcccctctcggccgcctgcgggctcttctgttgcatgtttttgcacgccttcgtgcactggcctcacacccccatggatcacaaccccaccatggatctgctcaccggagtgcccaacagcatgcttcacagcccccaggtcgcccccaccctgcgccgtaaccaggaacacctgtatcgctttctggggaaacactctgcctatttccgccgccatcggcagcgcatcgaacaggccacggccttcgaaagcatgagccaaagagtgtaatcaataaaaaccatttttatttgacatgatacgcgcttctggcgtttttattaaaaatcgaagggttcgagggaggggtcctcgtgcccgctggggagggacacgttgcgatactggaatcgggcgctccaacgaaactcggggatcaccagtcgcggcaggggcacgtcttccaggttctgcttccaaaactgtcgcaccagctgcagggctcccatcacgtcgggcgccgatatcttgaagtcgcagttagggccggagctcccgcggctgttccggaacacggggttggcacactggaacaccatcacgctggggttgtgaatactagccagggccgtcggatcggtcacctccgacgcatccagatcctcggcgttgctcagggcgaacggggtcagcttgcacatctgccgcccgatctggggcaccaggtcgggtttgttgaggcaatcgcagcgcagagggatcaggatgcgtcgctgcccgcgttgcatgatagggtaactcgccgccaggaactcctccatctgacggaaggccatctgggccttaacgccctcggtgaaaaacagcccacaggacttgctagaaaatacgttattgccgcagttaatgtcttccgcgcagcagcgtgcatcttcgttcttcagctgaaccacgttacgcccccagcggttctggaccaccttggctttcgtaggatgctccttcagcgcccgctgcccgttctcgctggtcacatccatttccaccacgtgctccttgcagaccatctccactccgtggaagcaaaacaggacgccctcctgccgggtattgcgatgctcccaaacggcacacccggtgggctcccagctcttgtgttttacccccgcgtaggcttccatgtaagccatgaggaatctgcccatcagctcggtgaaggtcttctgattggtgaaggttagcggcaggccgcggtgctcctcgttcaaccaagtttgacagatcttgcggtacaccgttccctggtcgggcagaaacttaaaagccgctctgctgtcgttgtccacgtggaacttctccattaacatcatcatggtttccatacccttctcccacgctgacaccagcggtttgctgtcggggttcttcaccaacacggcggtagaggggccctcgccggccccgacgtccttcatggtcattctttgaaactccacggagccgtccgcgcgacgtactctgcgcaccggagggtagctgaagcccacctccaccacggtgccttcgccctcgctgtcggaaacgatctccggggatggcggcggtgcgggtgtcgccttgcgagccttcttcttgggagggagctgaggcgcctcctgctcgcgctcggggctcatctcccgcaagtagggggttatggagctgcctgcttggttctgacggttggccattgtatcctaggcagaaagacatggagcttatgcgcgaggaaactttaaccgccccgtcccccgtcagcgacgaagatgtcatcgtcgaacaggacccgggctacgttacgccgcccgaggatctggaggggcctgaccggcgcgacgctagtgagcggcaggaaaatgagaaagaggaggcctgctacctcctggaaggcgacgttttgctaaagcatttcgccaggcagagcaccatagttaaggaggccttgcaagaccgctccgaggtgcccttggacgtcgccgcgctctcccaggcctacgaggcgaaccttttctcgcctcgagtgcctccgaagagacagcccaacggcacctgcgagcccaacccgcgactcaacttctaccccgtgttcgccgtaccagaggcgctggccacctatcacatttttttcaaaaaccaacgcatccccctatcgtgccgggccaaccgcaccgcggccgataggaatctcaggcttaaaaacggagccaacatacctgatatcacgtcgctggaggaagtgcccaagattttcgagggtctgggtcgagatgagaagcgggcggcgaacgctctgcagaaagaacagaaagagagtcagaacgtgctggtggagctggagggggacaacgcgcgtctggccgtcctcaaacgctgcatagaagtctcccacttcgcctaccccgccctcaacttgccacccaaagttatgaaatcggtcatggatcagctgctcatcaagagagctgagcccctggatcccgaccaccccgaggcggaaaactcagaggacggaaagcccgtcgtcagcgacgaggagctcgagcggtggctggaaaccagggacccccaacagttgcaagagaggcgcaagatgatgatggcggccgtgctggtcaccgtggagctggaatgcctgcaacggtttttcagcgacgtggagacgctacgcaaaatcggggaatccctgcactacaccttccgccagggctacgtccgccaggcctgcaagatctccaacgtggagctcagcaacctggtctcctacatgggcatcctccacgagaaccggctggggcagagcgtgctgcactgcaccttgcaaggcgaggcgcggcgggactacgtgcgagactgcatctacctcttcctcaccctcacctggcagaccgccatgggcgtctggcagcagtgcttggaagagagaaacctcaaagagctagacaaactcctctgccgccagcggcgcgccctgtggtccggtttcagcgagcgcacggtcgccagcgctctggcggacatcatcttcccggagcgcctgatgaaaaccttgcaaaacggcctgccggatttcatcagtcaaagcattttgcaaaacttccgctcttttgtcctggaacgctccgggatcttgcccgccatgagctgcgcgctaccttctgactttgtccccctctcctaccgcgagtgccctcccccactgtggagccactgctacctcttccaactggccaactttctggcctaccactccgacctcatggaagacgtaagcggagagggtttactggagtgccactgccgctgcaacctgtgcaccccccacagatcgctggcctgcaacaccgagctactcagcgaaacccaggtcataggtaccttcgagatccaggggccccagcagcaagagggtgcttccggcttgaagctcactccggcgctgtggacctcggcttacttacgcaaatttgtagccgaggactaccacgcccacaaaattcagttttacgaagaccaatctcaaccaccgaaagcccccctcacggcctgcgtcatcacccagagcaagatcctggcccaattgcaatccatcaaccaagcgcgccgcgatttccttttgaaaaagggtcggggggtgtatctggacccccagaccggcgaggaactcaacccgtccacactctccgtcgaagcagcccccccgagacatgccgcccaagggaaccgccaagcagctgatcgctcggcagagagcgaagaagcaagagctgctccagcagcaggtggaggacgaggaagagatgtgggacagccaggcagaggaggtgtcagaggacgaggaggagatggaaagctgggacagcctagacgaggaggaggacgagctttcagaggaagaggcgaccgaagaaaaaccacctgcatccagcgcgccttctctgagccgacagccgaagccccggcccccgacgcccccggccggctcactcaaagccagccgtaggtgggacgccaccgaatctccagcggcagcggcaacggcagcgggtaaggccaaacgcgagcggcgggggtattgctcctggcgggcccacaaaagcagtattgtgaactgcttgcaacactgcgggggaaacatctcctttgcccgacgctacctcctcttccatcacggtgtggccttccctcgcaacgttctctattattaccgtcatctctacagcccctacgaaacgctcggagaaaaaagctaaggcctcctccgccgcgaggaaaaactccgccgccgctgccgccgccaaggatccaccggccaccgaggagctgagaaagcgcatctttcccactctgtatgctatctttcagcaaagccgcgggcagcaccctcagcgcgaactgaaaataaaaaaccgctccttccgctcgctcacccgcagctgtctgtaccacaagagagaagaccagctgcagcgcaccctggacgacgccgaagcactgttcagcaaatactgctcagcgtctcttaaagactaaaagacccgcgctttttccccctcggccgccaaaacccacgtcatcgccagcatgagcaaggagattcccaccccctacatgtggagctatcagccccagatgggcctggccgcgggggccgcccaggactactccagcaagatgaactggctcagcgccggcccccacatgatctcacgagttaacggcatccgagcccaccgaaaccagattctcttagaacaggcggcaatcaccgccacaccccggcgccaactcaacccgcctagttggcccgccgcccaggtgtatcaggaaaatccccgcccgaccacagtcctcctgccacgcgacgcggaggccgaagtcctcatgactaactctggggtacaattagcgggcgggtccaggtacgccaggtacagaggtcgggccgctccttactctcccgggagtataaagagggtgatcattcgaggccgaggtatccagctcaacgacgagacggtgagctcctcaaccggtctcagacctgacggagtcttccagctcggaggagcgggccgctcttccttcaccactcgccaggcctacctgaccctgcagagctcttcctcgcagccgcgctccgggggaatcggcactctccagttcgtggaagagttcgttccctccgtctacttcaaccccttctccggctcgcctggacgctacccggacgccttcattcccaactttgacgcagtgagtgaatccgtggacggctacgactgatgacagatggtgcggccgtgagagctcggctgcgacatctgcatcactgccgtcagcctcgctgctacgctcgggaggcgatcgtcttcagctactttgagctgccggacgagcaccctcagggtccggctcacgggttgaaactcgagatcgagaacgcgctcgagtctcgcctcatcgacaccttcaccgcccgacctctcctggtagaaatcgaacgcgggatcactaccatcaccctgttctgcatctgccccacgcccggattacatgaagatctgtgctgtcatctttgcgctcagtttaataaaaactgaactttttgccgcaccttcaacgccacgcgtcgtttctccaaaagttgtcgacagctcttcagtcagaggtatacgagaaactgtttatttttacaactctactacttttctcacccttaactgctcctgcactaacgaactaattcagtggttcgcgaacggctcactctgccaagtcttttttaattctgctgttcttcctgagtttggctcctttgcgtgtggaaattctaccccctccaccttaaccattgcggcgcccttttcggaaatccagtatttttgtattggggcgggaggtaaaccgggttgtattcaccgcttgtttgtaaagccatttgttgcttcaattcccattaacacttcactttcctctaatacatacttacctaccttacattctactcacccctcctggcaacctcttattggcctcacggcttttatttccgttgttttactaaactttataattcttaacaaactttcttaaacatgcttgccattttgcttctgctcgttactttaacgtccgcagattaccacaatgtaattgtacgagaaaacagtttacaaaacccatcacaggtatatgttaaagcaggctctaacttaactttacaatccttctattcgccttaccctgaggacatgccacgtgttacttggtacttagaagtttttgattcgctatttgaaaggcatacgattcctccattttttacaggcgttatactttgtgacatttctggtgacatacagcatgtgtggaaccattggcctttacaatttaattgcataaataaaagcttacatattattaatctcaaaccaagtgatgaaggcctttacaatgtgaaggttttaaaggacagcattcagcataatacatactttcgagtgcatgtagtaagttttccaagacctgaatgtaacatcaccactacatatctttcagatgactactgccttattaacattgattgctctcaattaccataccctgctaaggtctattataatggcaatgaaagtaagctgcattactacttatctgaacgcggtggccagccaaaccttccaaattactttactgttgggtatcgatatagagatctccgacaaaattatacagttgaatatccatttaatgaactatgtacagagataattgctcttgaaacagggtctgattttatgccaatttttatagttaccctagtggtgagcattatagttattgtgatgggcatcacatatcttatttatcactgtaggactttaaagaccaaaaccaaaaccaaaaccaagcctcctgaaatccgtttgctttaattttttccagaatggtagctgctttcttcatttttctctgtataccaatcatctgcgcctccacaacttttgccgctgtttcccacctggaaccagactgtctaccaccttttgttgtatacctgatactgacttttgtggtctgtacagccattaccagcatagcctgcttttttgtaacaattttccaagccgccgattatctctacgtacggtttgcttattttagacatcaccccgagtatcggaatcaaaacgtagcttctttactttgtctagcatgattcgcctatttatactgcacactctgtttaccctcgcaaaatgtcattgcccttttaccaaaccttggtccttttacacctgttacgatgtactgcccgaaacccctattgcctggctttacgtagccacagcggttttagtttttgtagcaacctgcattggcgttaaactgtacttctacttaaaaattggatggcttcatcccccagaagatttaccccgatatcctcttgttaataactttcaacagcctctgccgcctcctgatcctcttccgcgagctccctccgttgttagctactttcaactcaccggtggagatgactgactctcaggacattgatattagtgtggaaagaatagccgctcagcgtcagcgagaaactcgggtgctggagtactttgaactacagcagcttaaagagtcccactggtgtgagaaaggagtgctgtgtcatgttaagcaggcagccctttcttacgatgtcagccttcagggacatgaactgtcttacactttgccttcgcaaaaacaaaccttctgcaccatgatgggctctacctccatcacaatcacccaacaaaccggacctgttgagggagctatcctgtgtcactgtcacgcgcctgattgtatgcccaaactaattagaactctctgtgccttaggtgatatatttaaaatgtaagtcagtatcaataaacttaccttaaatttgacagcagttttttggtaacatcattcagcagcaccactttaccctcttcccaactctcgtatgggacgtgatggtgggcggcaaacttcctccaaaccctaaaacaaatattaatatccacttccttgtccttacccacaattttcatcttttcatagatgaaaagaaccagagttgatgaagacttcaaccccgtctacccttatgactccacatccactcctgcggtcccctttatatcccccccgtttgtaaacagcgatggtcttcaggaaaaccctcctggagtcttaagtttacgaatagctaaacccttgtattttgacatggaaaggaaactagcgctttcacttggaagaggattggcaattacctccaccggacagctagaaagcacacagagcgtgcaaaccacccctccattagttgtcaacaacagcaacacgcttgtcctgcgttattcctccccgttaggcttatcgggtgacaatttaatactaaattgctccgatcctctccgcgtagtaaacaacagcctgacattcagctacctatctccacttcgttttgaaggtggcagtcttacattcaattacacatctccccttaaactgttgaacagcagccttgcgatcggaataaattccaacaaaggtctcggcaatgacagcgatgaactttctgtcaaactaacatcagatctaaagtttaacaacgatggaaaaatagcttttggtatacaaagcctgtgtaccacccccacagccgcctctaactgtaccgtttttaccaacggtgattctttactctgtttatgtttaaccaaatgtggagctcacgtgttaggaagtgtgagtttaaccggaatgcaaggaaccataacagccatgacacagaactacattagtattcaatttctatttgacaacaatggtgcgttgacttcatcaccgctcctcaacaacaacacttggggtatacggcaaaacgacacttcgtccgctaaccccgcctacaatgctcttgcatttatgcctaacagcactgtatatgtaagaggtcaaagtggtgagcccagaaataactattacacccaaacataccttaggggaaacgttaaaaagccaattatccttaccgttacctacaactcggctgcttcaggttattcactaacttttaaatgggatgctgtagtaacagaaaaatttgccactccaacatcttctttttgctatattacagaacaataaattcctattaccccaccaattcgtttttttcagatgaaacgggccagagttgatgaagacttcaacccagtgtacccttatgaccccccatacgctcccgttatgcccttcattactccaccttttacctcctcggatgggttgcaggaaaaaccacttggagtgttaagtttaaactacaaggatcccattactacacaaaatggatctctcacgttgaaaataggaaacggcctcactctagacaaccagggacaattaacatcaactgctggggaagtagagcctccgctcactaatgctaacaacaaacttgcactagcctatagcgaaccattagcagtaaaaagcaaccgcttaactttatcacacaccgccccccttgtcgttgctaataattctttagcgttgcaagtttcagaacctatttttataaatgacgatgacaagctagccctgcagacagccgccccccttgtaactaacgctggcacccttcgcttacagagcgccgcccctttaggattggttgaaaatactcttagactgctgttttctaaacccttgtatttgcaaaatgattttcttgcattaggcattgaacgccccctggctatagcagccgcaggtactctagcactacaactcactcctccattaaagactaacgatgacgggctgacactatccacagtcgagccattaactgtaaaaaacggaaacttaggcttgcaaatatctcgccctttggttgttcaaaacagcagcctttcgcttgctattacccccccgctgcgtctatttaacagcgaccccgttcttggtttgggctttacttttcccctagccgtgacagacaacctactctccttaaacatgggagacggtgttaaactaacctataataaactaacagccaatttgggtagggatttacaatttgaaaacggtgccattgccgtaacgcttactgccgaatcacctttgcaatacactaacaaacttcaactgaatattggagctggccttcgttacaatggagccagcagaaaactagatgtaaacattaaccaaaataagggcttaacttgggacaacgatgcagttattcccaaattaggatcaggtttacaattcgaccctaatggtaacatcgctgttatccctgaaaccgtaaagccgcaaacgttatggacaactgcagatccatcgcctaactgctcagtgtaccaggacttggacgccaggctgtggctcgctcttgttaaaagtggtgacatggttcatggaagcattgctctaaaagccctaaaaggaacgttgctaaatcctacagcaagctacatctccattgtgatatatttttacagcaacggagtcaggcgtaccaactatcccacgtttgacaacgaaggcaccttagctaacagcgctacctggggataccgagaggggcaatctgctaacactaatgtaaccaatgccactgaatttatgcccagctcaaccaggtaccccgtgaataaaggagacaatattcagaatcaatctttttcatacacctgtatcaaaggagatttcgctatgcctgtcccgttccgtgtaacatataatcatgccctggaaggatactcccttaagttcacctggcgcgttgtagccaaccaagcttttgatattccttgctgttccttttcatacatcacagaataaaccactttttaaaatttttctttttattttacacgcacagtaaggcttcctccccccttccatttgacagcatacaccagcctctcccccttcatggcagtaaactgctgcgagccagtccggtatttgggagttaaaatccaaacagtctctttggtgatgaaacgtcgatccgtgatggacacaaatccctggggcaggttttccagcgtttcggtaaaaaactgcacaccgccctacaaaacaaacaggttcaggctctccatgggttatctccccgatcaaactcagacagggtaaaggtgcggtgatgttccactaaaccacgcaggtggcgctgtctgaacctctcggtgcgactcctgtgaggctggtaagaagttagattgtccagtagcctcacagcatggatgatcagtttacgtgtacgtctggcgcaacagcgcatctgaatctcactgagattccggcaagaatcgcacaccatcacaatcaggttgttcatgatcccatagctgaacacgctccagccaaagctcattcgctccaacagcgccaccgcgtgtccgtccaaccttactttaacataaatcaggtgtctgccgcgtacaaacatactacccgcatacagaacttcccggggcaaacccctgttcaccacctgcctgtaccagggaaacctcacatttatcagggagccatagatagccattttaaaccaattagctaacaccgccccaccagctctacactgaagagaaccgggagagttacaatgacagtgaataatccatctctcataacccctgatggtctgatggaaatccagcacaccgccctacaaaacaaacaggttcaggctctccatgggttatctccccgatcaaactcagacagggtaaaggtgcggtgatgttccactaaaccacgcaggtggcgctgtctgaacctctcggtgcgactcctgtgaggctggtaagaagttagattgtccagtagcctcacagcatggatgatcagtttacgtgtacgtctggcgcaacagcgcatctgaatctcactgagattccggcaagaatcgcacaccatcacaatcaggttgttcatgatcccatagctgaacacgctccagccaaagctcattcgctccaacagcgccaccgcgtgtccgtccaaccttactttaacataaatcaggtgtctgccgcgtacaaacatactacccgcatacagaacttcccggggcaaacccctgttcaccacctgcctgtaccagggaaacctcacatttatcagggagccatagatagccattttaaaccaattagctaacaccgccccaccagctctacactgaagagaaccgggagagttacaatgacagtgaataatccatctctcataacccctgatggtctgatggaaatccagatctaacgtggcacagcagatacacactctcatatacattttcatcacatggttttcccaggccgttaaaatacaatcccaatacacgggccactcctgcagtacaataaagctaatacaagatggtatactcctcacctcactaacattgtgcatgttcatattttcacattctaagtaccgagagttctcctctacaacagcactgctgcggtcctcacaaggtggtagctggtgacgatcgtaaggagccagtctgcaacgataccgtctgtcgcgctgcatcgtagaccagagaccgacgcacctcctggtacttgtggtagcagaaccacgtccgctgccaacaggtatccacgtaacgccggtccctgcgtcgcgcgcgctctgttctcaatgcaaaatgcagccactcttgtaatccacacagatccctctcggcctccgggaggatacacacttcaaacctacaaatgtctcggtacagttccaaacacgaagtgagggcgagttccaaccaagacaggcaggctggtctatcccgacacactggaggtggaggaagacacggaagaggcatgttattccaagcgattcaccaacgggtcgaaatgaagatcccgaagatgacaacggtcgcctccggagccctgatggaatttaacagccaaatcaaacattatgcgattttccaggctatcgatcgcggcctccaaaagagcctggacccgcacttccacaaacaccagcaaagcaaaagcgttattatcaaactcttcgatcatcaagctgcaagactgtacaatgcccaagtaattttcatttctccactcgcgaatgatgtcgcggcaaatagtctgaaggttcatgccgtgcatattaaaaagctccgaaagggcgccctctatagccatgcgtagacacaccatcatgactgcaagatatcgggctcctgagacacctgcagcagatttaacagacccaggtcaggttgctctccgcgatcgcgaatctccatccgcaaggtcatttgcaaataattaaatagatctgcgccgactaaatctgttaactccgcgttaggaactaaatcaggtgtggctacgcagcacaaaagttccagggatggcgccaaactcactagaaccgctcccgagtagcaaaactgatgaatgggagtaacacagtgtaaaatgttcagccaaaaatcactaagccgctcctttaaaaagtccagtacttctatattcagttcgtgcaagtactgaagcaactgtgtgggaatatgcacaacaaaaaaaatagggcggctcagatacatgttgacctaaaataaaaagaatcattaaactaaagaagcttggcgaacggtgggataaatgacacgttccagcagcaggcaagcaaccggctgtccccgggaaccgcggtaaaattcatccgaatgattaaaaagaacaacagaaacttcccaccatgtactcggttggatctcctgagcacagagcaatacccccctcacattcatatccgccacagaaaaaaagcgtcccagatacccagcgggaatatccaacgacagctgcaaagacagcaaaacaatccctctgggagcaatcacaaaatcctccggtgaaaaaagcacatacatattagaataaccctgctgctggggcaaaaaggcccgtcgtcccagcaaatgcacataaatatgttcatcagccattgccccgtcttaccgcgtaaacagccacgaaaaattcgagctaaaatccacccaacagcctatagctatatatacactccgcccaatgacgctaataccgcaccacccaccgccaaagttcacccacacccacgaaacccgcgaaaatccagcgccgtcagcacttccgcaatttcagtctcacaacgtcacttccgcgcgccttttcacattcccacacccgcccacaaaccccgcgtcaccgcccgtcaccccggccccgcctcgctcctccccgctcattatcatattggcacgtttccagaataaggtatattattgatgatgttaattaattcgaacccataatacccataatagctgtttgccatcgaccaattctcccatattcccggttgaattgtagtacatgagaccaataaagttatttgaagacgaaagggcctcgtgatacgcctatttttataggttaatgtcatgataataatggtttcttagacgtcaggtggcacttttcggggaaatgtgcgcggaacccctatttgtttatttttctaaatacattcaaatatgtatccgctcatgagacaataaccctgataaatgcttcaataatattgaaaaaggaagagtatgagtattcaacatttccgtgtcgcccttattcccttttttgcggcattttgccttcctgtttttgctcacccagaaacgctggtgaaagtaaaagatgctgaagatcagttgggtgcacgagtgggttacatcgaactggatctcaacagcggtaagatccttgagagttttcgccccgaagaacgttttccaatgatgagcacttttaaagttctgctatgtggcgcggtattatcccgtgttgacgccgggcaagagcaactcggtcgccgcatacactattctcagaatgacttggttgagtactcaccagtcacagaaaagcatcttacggatggcatgacagtaagagaattatgcagtgctgccataaccatgagtgataacactgcggccaacttacttctgacaacgatcggaggaccgaaggagctaaccgcttttttgcacaacatgggggatcatgtaactcgccttgatcgttgggaaccggagctgaatgaagccataccaaacgacgagcgtgacaccacgatgcctgcagcaatggcaacaacgttgcgcaaactattaactggcgaactacttactctagcttcccggcaacaattaatagactggatggaggcggataaagttgcaggaccacttctgcgctcggcccttccggctggctggtttattgctgataaatctggagccggtgagcgtgggtctcgcggtatcattgcagcactggggccagatggtaagccctcccgtatcgtagttatctacacgacggggagtcaggcaactatggatgaacgaaatagacagatcgctgagataggtgcctcactgattaagcattggtaactgtcagaccaagtttactcatatatactttagattgatttaaaacttcatttttaatttaaaaggatctaggtgaagatcctttttgataatctcatgaccaaaatcccttaacgtgagttttcgttccactgagcgtcagaccccgtagaaaagatcaaaggatcttcttgagatcctttttttctgcgcgtaatctgctgcttgcaaacaaaaaaaccaccgctaccagcggtggtttgtttgccggatcaagagctaccaactctttttccgaaggtaactggcttcagcagagcgcagataccaaatactgtccttctagtgtagccgtagttaggccaccacttcaagaactctgtagcaccgcctacatacctcgctctgctaatcctgttaccagtggctgctgccagtggcgataagtcgtgtcttaccgggttggactcaagacgatagttaccggataaggcgcagcggtcgggctgaacggggggttcgtgcacacagcccagcttggagcgaacgacctacaccgaactgagatacctacagcgtgagctatgagaaagcgccacgcttcccgaagggagaaaggcggacaggtatccggtaagcggcagggtcggaacaggagagcgcacgagggagcttccagggggaaacgcctggtatctttatagtcctgtcgggtttcgccacctctgacttgagcgtcgatttttgtgatgctcgtcaggggggcggagcctatggaaaaacgccagcaacgcggcctttttacggttcctggccttttgctggccttgaagctgtccctgatggtcgtcatctacctgcctggacagcatggcctgcaacgcgggcatcccgatgccgccggaagcgagaagaatcataatggggaaggccatccagcctcgcgtcgatggcaaacagctattatgggtattatgggttcgaattaat

SEQ ID NO: 37 - DNA, 21190 bp, Artificial Sequence
  Synthetic oligonucleotide pBr/sAd4287.PsiI-rITR.dE3
attaacccaggacctggaaatagtgcctttaactaaagacagcaaagacagaagctacaatattataaacaacacgacggacaccctgtatcggagctggtttctggcttacaactacggagaccccgagaaaggagtgagatcatggaccatactcaccaccacggacgtgacctgtggctcgcagcaagtgtactggtccctgccggatatgatgcaagacccggtcaccttccgcccctccacccaagtcagcaacttcccggtggtgggcaccgagctgctgcccgtccatgccaagagcttctacaacgagcaggccgtctactcgcaacttattcgccagtccaccgcgcttacccacgtgttcaatcgctttcccgagaaccagattctggtgcgccctcccgctcctaccattaccaccgtcagtgaaaacgttcccgccctcacagatcacggaaccctgccgctgcgcagcagtatcagtggagttcagcgcgtgaccatcaccgacgccagacgtcgaacctgcccctacgtttacaaagcgcttggcgtggtggctcctaaagttctttctagtcgcaccttctaaaaacatgtccatcctcatctctcccgataacaacaccggctggggactgggctccggcaagatgtacggcggagccaaaaggcgctccagtcagcacccagttcgagttcggggccacttccgcgctccttggggagcttacaagcgaggactctcgggtcgaacggctgtagacgataccatagatgccgtgattgccgacgcccgccggtacaaccccggaccggtcgctagcgccgcctccaccgtggattccgtgatcgacagcgtggtagccggcgctcgggcctatgctcgccgcaagaggcggctgcatcggagacgtcgccccaccgccgccatgctggcagccagagccgtgctgagacgggcccggagggtaggcaggagggctatgcgccgcgctgccgccaacgccgccgccgggagggcccgccgacaggctgcccgccaggctgctgccgccatcgctagcatggccagacccaggagagggaacgtgtactgggtgcgcgattctgtgacgggagtccgagtgccggtgcgcagccgacctccccgaagttagaagatccaagctgcgaagacggcggtactgagtctccctgttgttatcagcccaacatgagcaagcgcaagtttaaagaagaactgctgcagacgctggtgcctgagatctatggccctccggacgtgaagcctgacattaagccccgcgatatcaagcgtgttaaaaagcgggaaaagaaagaggaactcgcggtggtagacgatggcggagtggaatttattaggagtttcgccccgcggcgcagggttcaatggaaagggcgacgggtacaacgcgttttgaggccgggcaccgcggtagtttttaccccgggagagcggtcggccgttaggggttttaaaaggcagtacgacgaggtgtacggcgacgaggacatattggaacaggcggctcaacagatcggagaatttgcctatggaaagcgctcgcgtcgcgaagacctggccatcgccttagacagcggcaaccccacgcccagcctcaaacccgtgacgctgcagcaggtgcttcccgtgagcgccagcacggacagcaagaggggaataaaaagagaaatggaagatctgcagcctaccatccagctcatggttcctaaacggcagaggctggaagaggtcctggagaagatgaaagtggaccccagcatagagccggacgttaaagtcaggccgatcaaagaagtggcccctggactcggggtgcagacggtggatatccagatccccgtcacgtcagcttcgaccgccgtggaagccatggaaacgcaaaccgaaacccccgccgtggttggtaccaaagaagtggcgttgcaaaccgacccctggtacgaatttgccgccccccggcgtcagaggcgacccgctcgttacggccccgccaacgccatcatgccagaatatgcgctgcatccgtctatcctgcccacccccggctaccggggagtgacgtatcgcccgtcaggaacccgccgccgaacccgtcgccgccgccgctcccgtcgcgctctggcccccgtgtcggtgcgccgcgtaacacgccggggaaagacagtcaccattcccaacccgcgctaccaccctagcatcctttaatgactctgccgttttgcagatggctctgacttgccgcgtgcgccttcccgttccgcactatcgaggaagatctcgtcgtaggagaggcatggcgggcagtggtcgccggcgggctttgcgcaggcgcatgaaaggcggaattttacccgctttgatacccataatcgccgccgccatcggtgccatacccggcgtcgcttcagtggccttgcaagcagctcgtaataaataaacgaaggcttttgcacttatgtcctggtcctgactattttatgcagaaagagcatggaagacatcaattttacgtcgctggctccgcggcacggctcgcggccgctcatgggcacctggaacgacatcggcaccagtcagctcaacgggggcgctttcaattgggggagcctttggagcggcattaaaaactttggctccacgattaaatcctacggcagcaaagcctggaacagtagtgctggtcagatgctccgagataaactgaaggacaccaacttccaagaaaaagtggtcaatggggtggtgaccggcatccacggtgcggtagatctcgccaaccaagcggtgcagaaagagattgacaggcgtttggaaaactcgcgggtgccgccgcagaggggggatgaggtggaggtcgaggaagtagaagtagaggaaaagctgcccccgctggagaaagttcccggtgcacctccgaggccgcagaagcggcccaggccagaactagaagaaactctggtgacggagagcaaggagcctccctcgtacgagcaagccttgaaagagggcgcctctccaccctcctacccgatgactaagccgatcgcacccatggctcgaccggtgtacggcaaggattacaagcccgtcacgctagagctgcccccaccgcccccttcgcgtccgacggtgcctccgctgcctgccccgtcggcgggtcccgagtctgcaccatccgctgtgcctctgccagccgcccgtcccgtggccgtggccactgccaggaaccccagaggccagagaggagccaactggcaaagcacgctgaacagcatcgtgggcctgggggtgaaaagcctgaaacgccgccgttgctattattaaaaagtgtagctaaaaaatttcccgttgtatacgcctcctatgttaccgccagagacgcgtgactgtcgccgcgagcgccgcttccaagatggccaccccatcgatgatgccgcagtggtcttacatgcacatcgccggccaggacgcctcggagtacctgagtcccggcctcgtgcagtttgcccgcgccaccgacacctacttcagcttgggaaacaagtttagaaaccccaccgtggcccccacccacgatgtgaccacggaccgctcgcagaggctgaccctgcgctttgtgcccgtagaccgggaggacaccgcgtactcttacaaagtgcgctacacgctggccgtaggggacaaccgagtgctggacatggccagcacctactttgacatccggggggtgctggatcggggtcccagcttcaagccctactccggcaccgcttacaactccctggctcccaagggcgcccccaatcctgcagaatgggccgataccaacgacagcaacaaactgaaagtgaggggtcaggcgccttttgtcagtacttacggttctgctacggcgcttacaaaagatgggatacaggtgggagtggatacttccgaagcatctcaggctgtttatgccgacagaagttaccagccagaaccccaaattggagagacagagtggaacagcgaagtgggtaatgacgacagagtggcgggaagggtgctaaagaaaacaactcccatgttcccttgttacggttcatatgccaagcccaccaacgaaaaaggcggacaagcaatacagcccaccgccggcaacggcgataatcaggctgtagagttacaattctttgccactactagcactcccactgcgccaaaggcagtattgtacgcggaggacgtggccattgaagctccagatactcacttagtgtttaagccaacagtagtcgcgggaactacaagttcggaagctctgctaacccaacaagccgcacctaaccgcccaaactacattgcctttagagataactttattggtctcatgtactacaattcaaccgggaatatgggagtactggccggacaagcatctcagctcaatgcagtggttgatcttcaggacagaaacaccgaactgtcatatcagctaatgctggatgctctgggagatcgcagtcggtacttttctatgtggaatcaagctgtagatagctatgatccagatgtaagaattgtagaaaaccacggtgtggaagacgaactgcctaattattgcttcccactaggcgggatggtagtaacggacacttacaaagccataaaggtaaatggaagcggatggacggctaatactgacgttttcagcgagagagtagaaataggctcaggtaacctgtttgccatggaaattaacttgcaagctaatctgtggcgcagtttcttgtattccaacataggactgtacctcccggactctttaaaattaacccctgacaacatcacgctccctgagaacaaaaatacctaccagtatatgaacggtcgcgtaacaccacccgggctcgtggacacctacgttaacgtgggtgcgcgctggtcccccgatgttatggacagcattaacccttttaaccaccaccgcaacgccgggctccgctaccgttccatgctcctgggaaacggacgctacgtacccttccacattcaggtgccccagaaattctttgcaattaaaaacctgctgctgctccccggttcctatacctacgagtggaatttccgcaaggacgtgaacatgattttgcaaagctcgctgggtaacgacctgcgagttgacggggccagcatacgcttcgacagcatcaacctgtatgctaactttttccccatggcccacaacacggcctccaccctggaagccatgctgcgcaacgacaccaatgaccagtccttcaacgactacctgtgcgcggccaacatgctgtatcccatccccgccaacgccaccagcgtgcccatctccatcccgtctcgcaactgggccgcctttaggggttggagtttcacccgcctcaaaaccaaggaaaccccctcgctgggctctggcttcgacccctacttcgtctactcaggctccattccctacctggacggcactttctatcttaaccacactttcaaaaaggtgtctatcatgttcgattcctcggtcagctggcccggcaacgaccgcctgctgacgcccaacgagttcgaaatcaagcgttcggtggacggtgaagggtacaacgtggcccagagcaacatgaccaaggactggttcctggttcaaatgctcagccattacaacatcggttaccagggcttctatgtgcccgagaactacaaggaccgcatgtactccttctttaggaacttccaacccatgagtcgccaagtcgtggactcagtggcttacagggactactaccaggacgttaagctcccctaccagcacaacaactcagggttcgtgggctacatgggtcccaccatgcgagaggggcaggcctacccggccaactatccttatcccctaatcggagagactgctgtacccagcctgacgcagaaaaagttcctctgcgaccgggtgatgtggaggatacccttctctagcaacttcatgtctatgggctccctcaccgacctggggcagaacatgctgtacgccaactccgctcacgccttggacatgacctttgaggtggatcccatggatgagcccacgcttctctatgttctgtttgaagtcttcgacgtggtgcgcatccaccagccgcaccgcggcgtcatcgaggccgtctacctgcgcacacctttctctgccggtaacgccaccacctaaagaagccgatgggctccagcgaacaggagctgcaggccattgttcgcgacctgggctgcgggccctactttttgggcaccttcgacaagcggttccccggcttcatgtcccctcacaagccggcctgtgccatcgttaacacggccggacgggaaaccgggggggtccactggctcgccttcgcctggaacccgcgtaaccgcacctgctacctgttcgacccttttggtttctccgacgaaaggctgaagcagatctaccagttcgagtacgaggggctcctccagcgcagcgctctggcctccacgcccgaccactgcgtcaccctggaaaagtccacccagacggtccaggggcccctctcggccgcctgcgggctcttctgttgcatgtttttgcacgccttcgtgcactggcctcacacccccatggatcacaaccccaccatggatctgctcaccggagtgcccaacagcatgcttcacagcccccaggtcgcccccaccctgcgccgtaaccaggaacacctgtatcgctttctggggaaacactctgcctatttccgccgccatcggcagcgcatcgaacaggccacggccttcgaaagcatgagccaaagagtgtaatcaataaaaaccatttttatttgacatgatacgcgcttctggcgtttttattaaaaatcgaagggttcgagggaggggtcctcgtgcccgctggggagggacacgttgcgatactggaatcgggcgctccaacgaaactcggggatcaccagtcgcggcaggggcacgtcttccaggttctgcttccaaaactgtcgcaccagctgcagggctcccatcacgtcgggcgccgatatcttgaagtcgcagttagggccggagctcccgcggctgttccggaacacggggttggcacactggaacaccatcacgctggggttgtgaatactagccagggccgtcggatcggtcacctccgacgcatccagatcctcggcgttgctcagggcgaacggggtcagcttgcacatctgccgcccgatctggggcaccaggtcgggtttgttgaggcaatcgcagcgcagagggatcaggatgcgtcgctgcccgcgttgcatgatagggtaactcgccgccaggaactcctccatctgacggaaggccatctgggccttaacgccctcggtgaaaaacagcccacaggacttgctagaaaatacgttattgccgcagttaatgtcttccgcgcagcagcgtgcatcttcgttcttcagctgaaccacgttacgcccccagcggttctggaccaccttggctttcgtaggatgctccttcagcgcccgctgcccgttctcgctggtcacatccatttccaccacgtgctccttgcagaccatctccactccgtggaagcaaaacaggacgccctcctgccgggtattgcgatgctcccaaacggcacacccggtgggctcccagctcttgtgttttacccccgcgtaggcttccatgtaagccatgaggaatctgcccatcagctcggtgaaggtcttctgattggtgaaggttagcggcaggccgcggtgctcctcgttcaaccaagtttgacagatcttgcggtacaccgttccctggtcgggcagaaacttaaaagccgctctgctgtcgttgtccacgtggaacttctccattaacatcatcatggtttccatacccttctcccacgctgacaccagcggtttgctgtcggggttcttcaccaacacggcggtagaggggccctcgccggccccgacgtccttcatggtcattctttgaaactccacggagccgtccgcgcgacgtactctgcgcaccggagggtagctgaagcccacctccaccacggtgccttcgccctcgctgtcggaaacgatctccggggatggcggcggtgcgggtgtcgccttgcgagccttcttcttgggagggagctgaggcgcctcctgctcgcgctcggggctcatctcccgcaagtagggggttatggagctgcctgcttggttctgacggttggccattgtatcctaggcagaaagacatggagcttatgcgcgaggaaactttaaccgccccgtcccccgtcagcgacgaagatgtcatcgtcgaacaggacccgggctacgttacgccgcccgaggatctggaggggcctgaccggcgcgacgctagtgagcggcaggaaaatgagaaagaggaggcctgctacctcctggaaggcgacgttttgctaaagcatttcgccaggcagagcaccatagttaaggaggccttgcaagaccgctccgaggtgcccttggacgtcgccgcgctctcccaggcctacgaggcgaaccttttctcgcctcgagtgcctccgaagagacagcccaacggcacctgcgagcccaacccgcgactcaacttctaccccgtgttcgccgtaccagaggcgctggccacctatcacatttttttcaaaaaccaacgcatccccctatcgtgccgggccaaccgcaccgcggccgataggaatctcaggcttaaaaacggagccaacatacctgatatcacgtcgctggaggaagtgcccaagattttcgagggtctgggtcgagatgagaagcgggcggcgaacgctctgcagaaagaacagaaagagagtcagaacgtgctggtggagctggagggggacaacgcgcgtctggccgtcctcaaacgctgcatagaagtctcccacttcgcctaccccgccctcaacttgccacccaaagttatgaaatcggtcatggatcagctgctcatcaagagagctgagcccctggatcccgaccaccccgaggcggaaaactcagaggacggaaagcccgtcgtcagcgacgaggagctcgagcggtggctggaaaccagggacccccaacagttgcaagagaggcgcaagatgatgatggcggccgtgctggtcaccgtggagctggaatgcctgcaacggtttttcagcgacgtggagacgctacgcaaaatcggggaatccctgcactacaccttccgccagggctacgtccgccaggcctgcaagatctccaacgtggagctcagcaacctggtctcctacatgggcatcctccacgagaaccggctggggcagagcgtgctgcactgcaccttgcaaggcgaggcgcggcgggactacgtgcgagactgcatctacctcttcctcaccctcacctggcagaccgccatgggcgtctggcagcagtgcttggaagagagaaacctcaaagagctagacaaactcctctgccgccagcggcgcgccctgtggtccggtttcagcgagcgcacggtcgccagcgctctggcggacatcatcttcccggagcgcctgatgaaaaccttgcaaaacggcctgccggatttcatcagtcaaagcattttgcaaaacttccgctcttttgtcctggaacgctccgggatcttgcccgccatgagctgcgcgctaccttctgactttgtccccctctcctaccgcgagtgccctcccccactgtggagccactgctacctcttccaactggccaactttctggcctaccactccgacctcatggaagacgtaagcggagagggtttactggagtgccactgccgctgcaacctgtgcaccccccacagatcgctggcctgcaacaccgagctactcagcgaaacccaggtcataggtaccttcgagatccaggggccccagcagcaagagggtgcttccggcttgaagctcactccggcgctgtggacctcggcttacttacgcaaatttgtagccgaggactaccacgcccacaaaattcagttttacgaagaccaatctcaaccaccgaaagcccccctcacggcctgcgtcatcacccagagcaagatcctggcccaattgcaatccatcaaccaagcgcgccgcgatttccttttgaaaaagggtcggggggtgtatctggacccccagaccggcgaggaactcaacccgtccacactctccgtcgaagcagcccccccgagacatgccgcccaagggaaccgccaagcagctgatcgctcggcagagagcgaagaagcaagagctgctccagcagcaggtggaggacgaggaagagatgtgggacagccaggcagaggaggtgtcagaggacgaggaggagatggaaagctgggacagcctagacgaggaggaggacgagctttcagaggaagaggcgaccgaagaaaaaccacctgcatccagcgcgccttctctgagccgacagccgaagccccggcccccgacgcccccggccggctcactcaaagccagccgtaggtgggacgccaccgaatctccagcggcagcggcaacggcagcgggtaaggccaaacgcgagcggcgggggtattgctcctggcgggcccacaaaagcagtattgtgaactgcttgcaacactgcgggggaaacatctcctttgcccgacgctacctcctcttccatcacggtgtggccttccctcgcaacgttctctattattaccgtcatctctacagcccctacgaaacgctcggagaaaaaagctaaggcctcctccgccgcgaggaaaaactccgccgccgctgccgccgccaaggatccaccggccaccgaggagctgagaaagcgcatctttcccactctgtatgctatctttcagcaaagccgcgggcagcaccctcagcgcgaactgaaaataaaaaaccgctccttccgctcgctcacccgcagctgtctgtaccacaagagagaagaccagctgcagcgcaccctggacgacgccgaagcactgttcagcaaatactgctcagcgtctcttaaagactaaaagacccgcgctttttccccctcggccgccaaaacccacgtcatcgccagcatgagcaaggagattcccaccccctacatgtggagctatcagccccagatgggcctggccgcgggggccgcccaggactactccagcaagatgaactggctcagcgccggcccccacatgatctcacgagttaacggcatccgagcccaccgaaaccagattctcttagaacaggcggcaatcaccgccacaccccggcgccaactcaacccgcctagttggcccgccgcccaggtgtatcaggaaaatccccgcccgaccacagtcctcctgccacgcgacgcggaggccgaagtcctcatgactaactctggggtacaattagcgggcgggtccaggtacgccaggtacagaggtcgggccgctccttactctcccgggagtataaagagggtgatcattcgaggccgaggtatccagctcaacgacgagacggtgagctcctcaaccggtctcagacctgacggagtcttccagctcggaggagcgggccgctcttccttcaccactcgccaggcctacctgaccctgcagagctcttcctcgcagccgcgctccgggggaatcggcactctccagttcgtggaagagttcgttccctccgtctacttcaaccccttctccggctcgcctggacgctacccggacgccttcattcccaactttgacgcagtgagtgaatccgtggacggctacgactgatgacagatggtgcggccgtgagagctcggctgcgacatctgcatcactgccgtcagcctcgctgctacgctcgggaggcgatcgtcttcagctactttgagctgccggacgagcaccctcagggtccggctcacgggttgaaactcgagatcgagaacgcgctcgagtctcgcctcatcgacaccttcaccgcccgacctctcctggtagaaatcgaacgcgggatcactaccatcaccctgttctgcatctgccccacgcccggattacatgaagatctgtgctgtcatctttgcgctcagtttaataaaaactgaactttttgccgcaccttcaacgccacgcgtcgtttctccaaaagttgtcgacagctcttcagtcagaggtatacgagaaactgtttatttttacaactctactacttttctcacccttaactgctcctgcactaacgaactaattcagtggttcgcgaacggctcactctgccaagtcttttttaattctgctgttcttcctgagtttggctcctttgcgtgtggaaattctacactagtgggagctatcctgtgtcactgtcacgcgcctgattgtatgcccaaactaattagaactctctgtgccttaggtgatatatttaaaatgtaagtcagtatcaataaacttaccttaaatttgacagcagttttttggtaacatcattcagcagcaccactttaccctcttcccaactctcgtatgggacgtgatggtgggcggcaaacttcctccaaaccctaaaacaaatattaatatccacttccttgtccttacccacaattttcatcttttcatagatgaaaagaaccagagttgatgaagacttcaaccccgtctacccttatgactccacatccactcctgcggtcccctttatatcccccccgtttgtaaacagcgatggtcttcaggaaaaccctcctggagtcttaagtttacgaatagctaaacccttgtattttgacatggaaaggaaactagcgctttcacttggaagaggattggcaattacctccaccggacagctagaaagcacacagagcgtgcaaaccacccctccattagttgtcaacaacagcaacacgcttgtcctgcgttattcctccccgttaggcttatcgggtgacaatttaatactaaattgctccgatcctctccgcgtagtaaacaacagcctgacattcagctacctatctccacttcgttttgaaggtggcagtcttacattcaattacacatctccccttaaactgttgaacagcagccttgcgatcggaataaattccaacaaaggtctcggcaatgacagcgatgaactttctgtcaaactaacatcagatctaaagtttaacaacgatggaaaaatagcttttggtatacaaagcctgtgtaccacccccacagccgcctctaactgtaccgtttttaccaacggtgattctttactctgtttatgtttaaccaaatgtggagctcacgtgttaggaagtgtgagtttaaccggaatgcaaggaaccataacagccatgacacagaactacattagtattcaatttctatttgacaacaatggtgcgttgacttcatcaccgctcctcaacaacaacacttggggtatacggcaaaacgacacttcgtccgctaaccccgcctacaatgctcttgcatttatgcctaacagcactgtatatgtaagaggtcaaagtggtgagcccagaaataactattacacccaaacataccttaggggaaacgttaaaaagccaattatccttaccgttacctacaactcggctgcttcaggttattcactaacttttaaatgggatgctgtagtaacagaaaaatttgccactccaacatcttctttttgctatattacagaacaataaattcctattaccccaccaattcgtttttttcagatgaaacgggccagagttgatgaagacttcaacccagtgtacccttatgaccccccatacgctcccgttatgcccttcattactccaccttttacctcctcggatgggttgcaggaaaaaccacttggagtgttaagtttaaactacaaggatcccattactacacaaaatggatctctcacgttgaaaataggaaacggcctcactctagacaaccagggacaattaacatcaactgctggggaagtagagcctccgctcactaatgctaacaacaaacttgcactagcctatagcgaaccattagcagtaaaaagcaaccgcttaactttatcacacaccgccccccttgtcgttgctaataattctttagcgttgcaagtttcagaacctatttttataaatgacgatgacaagctagccctgcagacagccgccccccttgtaactaacgctggcacccttcgcttacagagcgccgcccctttaggattggttgaaaatactcttagactgctgttttctaaacccttgtatttgcaaaatgattttcttgcattaggcattgaacgccccctggctatagcagccgcaggtactctagcactacaactcactcctccattaaagactaacgatgacgggctgacactatccacagtcgagccattaactgtaaaaaacggaaacttaggcttgcaaatatctcgccctttggttgttcaaaacagcagcctttcgcttgctattacccccccgctgcgtctatttaacagcgaccccgttcttggtttgggctttacttttcccctagccgtgacagacaacctactctccttaaacatgggagacggtgttaaactaacctataataaactaacagccaatttgggtagggatttacaatttgaaaacggtgccattgccgtaacgcttactgccgaatcacctttgcaatacactaacaaacttcaactgaatattggagctggccttcgttacaatggagccagcagaaaactagatgtaaacattaaccaaaataagggcttaacttgggacaacgatgcagttattcccaaattaggatcaggtttacaattcgaccctaatggtaacatcgctgttatccctgaaaccgtaaagccgcaaacgttatggacaactgcagatccatcgcctaactgctcagtgtaccaggacttggacgccaggctgtggctcgctcttgttaaaagtggtgacatggttcatggaagcattgctctaaaagccctaaaaggaacgttgctaaatcctacagcaagctacatctccattgtgatatatttttacagcaacggagtcaggcgtaccaactatcccacgtttgacaacgaaggcaccttagctaacagcgctacctggggataccgagaggggcaatctgctaacactaatgtaaccaatgccactgaatttatgcccagctcaaccaggtaccccgtgaataaaggagacaatattcagaatcaatctttttcatacacctgtatcaaaggagatttcgctatgcctgtcccgttccgtgtaacatataatcatgccctggaaggatactcccttaagttcacctggcgcgttgtagccaaccaagcttttgatattccttgctgttccttttcatacatcacagaataaaccactttttaaaatttttctttttattttacacgcacagtaaggcttcctccccccttccatttgacagcatacaccagcctctcccccttcatggcagtaaactgctgcgagccagtccggtatttgggagttaaaatccaaacagtctctttggtgatgaaacgtcgatccgtgatggacacaaatccctggggcaggttttccagcgtttcggtaaaaaactgcacaccgccctacaaaacaaacaggttcaggctctccatgggttatctccccgatcaaactcagacagggtaaaggtgcggtgatgttccactaaaccacgcaggtggcgctgtctgaacctctcggtgcgactcctgtgaggctggtaagaagttagattgtccagtagcctcacagcatggatgatcagtttacgtgtacgtctggcgcaacagcgcatctgaatctcactgagattccggcaagaatcgcacaccatcacaatcaggttgttcatgatcccatagctgaacacgctccagccaaagctcattcgctccaacagcgccaccgcgtgtccgtccaaccttactttaacataaatcaggtgtctgccgcgtacaaacatactacccgcatacagaacttcccggggcaaacccctgttcaccacctgcctgtaccagggaaacctcacatttatcagggagccatagatagccattttaaaccaattagctaacaccgccccaccagctctacactgaagagaaccgggagagttacaatgacagtgaataatccatctctcataacccctgatggtctgatggaaatccagcacaccgccctacaaaacaaacaggttcaggctctccatgggttatctccccgatcaaactcagacagggtaaaggtgcggtgatgttccactaaaccacgcaggtggcgctgtctgaacctctcggtgcgactcctgtgaggctggtaagaagttagattgtccagtagcctcacagcatggatgatcagtttacgtgtacgtctggcgcaacagcgcatctgaatctcactgagattccggcaagaatcgcacaccatcacaatcaggttgttcatgatcccatagctgaacacgctccagccaaagctcattcgctccaacagcgccaccgcgtgtccgtccaaccttactttaacataaatcaggtgtctgccgcgtacaaacatactacccgcatacagaacttcccggggcaaacccctgttcaccacctgcctgtaccagggaaacctcacatttatcagggagccatagatagccattttaaaccaattagctaacaccgccccaccagctctacactgaagagaaccgggagagttacaatgacagtgaataatccatctctcataacccctgatggtctgatggaaatccagatctaacgtggcacagcagatacacactctcatatacattttcatcacatggttttcccaggccgttaaaatacaatcccaatacacgggccactcctgcagtacaataaagctaatacaagatggtatactcctcacctcactaacattgtgcatgttcatattttcacattctaagtaccgagagttctcctctacaacagcactgctgcggtcctcacaaggtggtagctggtgacgatcgtaaggagccagtctgcaacgataccgtctgtcgcgctgcatcgtagaccagagaccgacgcacctcctggtacttgtggtagcagaaccacgtccgctgccaacaggtatccacgtaacgccggtccctgcgtcgcgcgcgctctgttctcaatgcaaaatgcagccactcttgtaatccacacagatccctctcggcctccgggaggatacacacttcaaacctacaaatgtctcggtacagttccaaacacgaagtgagggcgagttccaaccaagacaggcaggctggtctatcccgacacactggaggtggaggaagacacggaagaggcatgttattccaagcgattcaccaacgggtcgaaatgaagatcccgaagatgacaacggtcgcctccggagccctgatggaatttaacagccaaatcaaacattatgcgattttccaggctatcgatcgcggcctccaaaagagcctggacccgcacttccacaaacaccagcaaagcaaaagcgttattatcaaactcttcgatcatcaagctgcaagactgtacaatgcccaagtaattttcatttctccactcgcgaatgatgtcgcggcaaatagtctgaaggttcatgccgtgcatattaaaaagctccgaaagggcgccctctatagccatgcgtagacacaccatcatgactgcaagatatcgggctcctgagacacctgcagcagatttaacagacccaggtcaggttgctctccgcgatcgcgaatctccatccgcaaggtcatttgcaaataattaaatagatctgcgccgactaaatctgttaactccgcgttaggaactaaatcaggtgtggctacgcagcacaaaagttccagggatggcgccaaactcactagaaccgctcccgagtagcaaaactgatgaatgggagtaacacagtgtaaaatgttcagccaaaaatcactaagccgctcctttaaaaagtccagtacttctatattcagttcgtgcaagtactgaagcaactgtgtgggaatatgcacaacaaaaaaaatagggcggctcagatacatgttgacctaaaataaaaagaatcattaaactaaagaagcttggcgaacggtgggataaatgacacgttccagcagcaggcaagcaaccggctgtccccgggaaccgcggtaaaattcatccgaatgattaaaaagaacaacagaaacttcccaccatgtactcggttggatctcctgagcacagagcaatacccccctcacattcatatccgccacagaaaaaaagcgtcccagatacccagcgggaatatccaacgacagctgcaaagacagcaaaacaatccctctgggagcaatcacaaaatcctccggtgaaaaaagcacatacatattagaataaccctgctgctggggcaaaaaggcccgtcgtcccagcaaatgcacataaatatgttcatcagccattgccccgtcttaccgcgtaaacagccacgaaaaattcgagctaaaatccacccaacagcctatagctatatatacactccgcccaatgacgctaataccgcaccacccaccgccaaagttcacccacacccacgaaacccgcgaaaatccagcgccgtcagcacttccgcaatttcagtctcacaacgtcacttccgcgcgccttttcacattcccacacccgcccacaaaccccgcgtcaccgcccgtcaccccggccccgcctcgctcctccccgctcattatcatattggcacgtttccagaataaggtatattattgatgatgttaattaattcgaacccataatacccataatagctgtttgccatcgaccaattctcccatattcccggttgaattgtagtacatgagaccaataaagttatttgaagacgaaagggcctcgtgatacgcctatttttataggttaatgtcatgataataatggtttcttagacgtcaggtggcacttttcggggaaatgtgcgcggaacccctatttgtttatttttctaaatacattcaaatatgtatccgctcatgagacaataaccctgataaatgcttcaataatattgaaaaaggaagagtatgagtattcaacatttccgtgtcgcccttattcccttttttgcggcattttgccttcctgtttttgctcacccagaaacgctggtgaaagtaaaagatgctgaagatcagttgggtgcacgagtgggttacatcgaactggatctcaacagcggtaagatccttgagagttttcgccccgaagaacgttttccaatgatgagcacttttaaagttctgctatgtggcgcggtattatcccgtgttgacgccgggcaagagcaactcggtcgccgcatacactattctcagaatgacttggttgagtactcaccagtcacagaaaagcatcttacggatggcatgacagtaagagaattatgcagtgctgccataaccatgagtgataacactgcggccaacttacttctgacaacgatcggaggaccgaaggagctaaccgcttttttgcacaacatgggggatcatgtaactcgccttgatcgttgggaaccggagctgaatgaagccataccaaacgacgagcgtgacaccacgatgcctgcagcaatggcaacaacgttgcgcaaactattaactggcgaactacttactctagcttcccggcaacaattaatagactggatggaggcggataaagttgcaggaccacttctgcgctcggcccttccggctggctggtttattgctgataaatctggagccggtgagcgtgggtctcgcggtatcattgcagcactggggccagatggtaagccctcccgtatcgtagttatctacacgacggggagtcaggcaactatggatgaacgaaatagacagatcgctgagataggtgcctcactgattaagcattggtaactgtcagaccaagtttactcatatatactttagattgatttaaaacttcatttttaatttaaaaggatctaggtgaagatcctttttgataatctcatgaccaaaatcccttaacgtgagttttcgttccactgagcgtcagaccccgtagaaaagatcaaaggatcttcttgagatcctttttttctgcgcgtaatctgctgcttgcaaacaaaaaaaccaccgctaccagcggtggtttgtttgccggatcaagagctaccaactctttttccgaaggtaactggcttcagcagagcgcagataccaaatactgtccttctagtgtagccgtagttaggccaccacttcaagaactctgtagcaccgcctacatacctcgctctgctaatcctgttaccagtggctgctgccagtggcgataagtcgtgtcttaccgggttggactcaagacgatagttaccggataaggcgcagcggtcgggctgaacggggggttcgtgcacacagcccagcttggagcgaacgacctacaccgaactgagatacctacagcgtgagctatgagaaagcgccacgcttcccgaagggagaaaggcggacaggtatccggtaagcggcagggtcggaacaggagagcgcacgagggagcttccagggggaaacgcctggtatctttatagtcctgtcgggtttcgccacctctgacttgagcgtcgatttttgtgatgctcgtcaggggggcggagcctatggaaaaacgccagcaacgcggcctttttacggttcctggccttttgctggccttgaagctgtccctgatggtcgtcatctacctgcctggacagcatggcctgcaacgcgggcatcccgatgccgccggaagcgagaagaatcataatggggaaggccatccagcctcgcgtcgatggcaaacagctattatgggtattatgggttcgaattaat

SEQ ID NO: 38 - DNA, 19781 bp, Artificial Sequence
  Synthetic oligonucleotide pBr/sAd4287.PsiI-rITR.dE3.dE4
attaacccaggacctggaaatagtgcctttaactaaagacagcaaagacagaagctacaatattataaacaacacgacggacaccctgtatcggagctggtttctggcttacaactacggagaccccgagaaaggagtgagatcatggaccatactcaccaccacggacgtgacctgtggctcgcagcaagtgtactggtccctgccggatatgatgcaagacccggtcaccttccgcccctccacccaagtcagcaacttcccggtggtgggcaccgagctgctgcccgtccatgccaagagcttctacaacgagcaggccgtctactcgcaacttattcgccagtccaccgcgcttacccacgtgttcaatcgctttcccgagaaccagattctggtgcgccctcccgctcctaccattaccaccgtcagtgaaaacgttcccgccctcacagatcacggaaccctgccgctgcgcagcagtatcagtggagttcagcgcgtgaccatcaccgacgccagacgtcgaacctgcccctacgtttacaaagcgcttggcgtggtggctcctaaagttctttctagtcgcaccttctaaaaacatgtccatcctcatctctcccgataacaacaccggctggggactgggctccggcaagatgtacggcggagccaaaaggcgctccagtcagcacccagttcgagttcggggccacttccgcgctccttggggagcttacaagcgaggactctcgggtcgaacggctgtagacgataccatagatgccgtgattgccgacgcccgccggtacaaccccggaccggtcgctagcgccgcctccaccgtggattccgtgatcgacagcgtggtagccggcgctcgggcctatgctcgccgcaagaggcggctgcatcggagacgtcgccccaccgccgccatgctggcagccagagccgtgctgagacgggcccggagggtaggcaggagggctatgcgccgcgctgccgccaacgccgccgccgggagggcccgccgacaggctgcccgccaggctgctgccgccatcgctagcatggccagacccaggagagggaacgtgtactgggtgcgcgattctgtgacgggagtccgagtgccggtgcgcagccgacctccccgaagttagaagatccaagctgcgaagacggcggtactgagtctccctgttgttatcagcccaacatgagcaagcgcaagtttaaagaagaactgctgcagacgctggtgcctgagatctatggccctccggacgtgaagcctgacattaagccccgcgatatcaagcgtgttaaaaagcgggaaaagaaagaggaactcgcggtggtagacgatggcggagtggaatttattaggagtttcgccccgcggcgcagggttcaatggaaagggcgacgggtacaacgcgttttgaggccgggcaccgcggtagtttttaccccgggagagcggtcggccgttaggggttttaaaaggcagtacgacgaggtgtacggcgacgaggacatattggaacaggcggctcaacagatcggagaatttgcctatggaaagcgctcgcgtcgcgaagacctggccatcgccttagacagcggcaaccccacgcccagcctcaaacccgtgacgctgcagcaggtgcttcccgtgagcgccagcacggacagcaagaggggaataaaaagagaaatggaagatctgcagcctaccatccagctcatggttcctaaacggcagaggctggaagaggtcctggagaagatgaaagtggaccccagcatagagccggacgttaaagtcaggccgatcaaagaagtggcccctggactcggggtgcagacggtggatatccagatccccgtcacgtcagcttcgaccgccgtggaagccatggaaacgcaaaccgaaacccccgccgtggttggtaccaaagaagtggcgttgcaaaccgacccctggtacgaatttgccgccccccggcgtcagaggcgacccgctcgttacggccccgccaacgccatcatgccagaatatgcgctgcatccgtctatcctgcccacccccggctaccggggagtgacgtatcgcccgtcaggaacccgccgccgaacccgtcgccgccgccgctcccgtcgcgctctggcccccgtgtcggtgcgccgcgtaacacgccggggaaagacagtcaccattcccaacccgcgctaccaccctagcatcctttaatgactctgccgttttgcagatggctctgacttgccgcgtgcgccttcccgttccgcactatcgaggaagatctcgtcgtaggagaggcatggcgggcagtggtcgccggcgggctttgcgcaggcgcatgaaaggcggaattttacccgctttgatacccataatcgccgccgccatcggtgccatacccggcgtcgcttcagtggccttgcaagcagctcgtaataaataaacgaaggcttttgcacttatgtcctggtcctgactattttatgcagaaagagcatggaagacatcaattttacgtcgctggctccgcggcacggctcgcggccgctcatgggcacctggaacgacatcggcaccagtcagctcaacgggggcgctttcaattgggggagcctttggagcggcattaaaaactttggctccacgattaaatcctacggcagcaaagcctggaacagtagtgctggtcagatgctccgagataaactgaaggacaccaacttccaagaaaaagtggtcaatggggtggtgaccggcatccacggtgcggtagatctcgccaaccaagcggtgcagaaagagattgacaggcgtttggaaaactcgcgggtgccgccgcagaggggggatgaggtggaggtcgaggaagtagaagtagaggaaaagctgcccccgctggagaaagttcccggtgcacctccgaggccgcagaagcggcccaggccagaactagaagaaactctggtgacggagagcaaggagcctccctcgtacgagcaagccttgaaagagggcgcctctccaccctcctacccgatgactaagccgatcgcacccatggctcgaccggtgtacggcaaggattacaagcccgtcacgctagagctgcccccaccgcccccttcgcgtccgacggtgcctccgctgcctgccccgtcggcgggtcccgagtctgcaccatccgctgtgcctctgccagccgcccgtcccgtggccgtggccactgccaggaaccccagaggccagagaggagccaactggcaaagcacgctgaacagcatcgtgggcctgggggtgaaaagcctgaaacgccgccgttgctattattaaaaagtgtagctaaaaaatttcccgttgtatacgcctcctatgttaccgccagagacgcgtgactgtcgccgcgagcgccgcttccaagatggccaccccatcgatgatgccgcagtggtcttacatgcacatcgccggccaggacgcctcggagtacctgagtcccggcctcgtgcagtttgcccgcgccaccgacacctacttcagcttgggaaacaagtttagaaaccccaccgtggcccccacccacgatgtgaccacggaccgctcgcagaggctgaccctgcgctttgtgcccgtagaccgggaggacaccgcgtactcttacaaagtgcgctacacgctggccgtaggggacaaccgagtgctggacatggccagcacctactttgacatccggggggtgctggatcggggtcccagcttcaagccctactccggcaccgcttacaactccctggctcccaagggcgcccccaatcctgcagaatgggccgataccaacgacagcaacaaactgaaagtgaggggtcaggcgccttttgtcagtacttacggttctgctacggcgcttacaaaagatgggatacaggtgggagtggatacttccgaagcatctcaggctgtttatgccgacagaagttaccagccagaaccccaaattggagagacagagtggaacagcgaagtgggtaatgacgacagagtggcgggaagggtgctaaagaaaacaactcccatgttcccttgttacggttcatatgccaagcccaccaacgaaaaaggcggacaagcaatacagcccaccgccggcaacggcgataatcaggctgtagagttacaattctttgccactactagcactcccactgcgccaaaggcagtattgtacgcggaggacgtggccattgaagctccagatactcacttagtgtttaagccaacagtagtcgcgggaactacaagttcggaagctctgctaacccaacaagccgcacctaaccgcccaaactacattgcctttagagataactttattggtctcatgtactacaattcaaccgggaatatgggagtactggccggacaagcatctcagctcaatgcagtggttgatcttcaggacagaaacaccgaactgtcatatcagctaatgctggatgctctgggagatcgcagtcggtacttttctatgtggaatcaagctgtagatagctatgatccagatgtaagaattgtagaaaaccacggtgtggaagacgaactgcctaattattgcttcccactaggcgggatggtagtaacggacacttacaaagccataaaggtaaatggaagcggatggacggctaatactgacgttttcagcgagagagtagaaataggctcaggtaacctgtttgccatggaaattaacttgcaagctaatctgtggcgcagtttcttgtattccaacataggactgtacctcccggactctttaaaattaacccctgacaacatcacgctccctgagaacaaaaatacctaccagtatatgaacggtcgcgtaacaccacccgggctcgtggacacctacgttaacgtgggtgcgcgctggtcccccgatgttatggacagcattaacccttttaaccaccaccgcaacgccgggctccgctaccgttccatgctcctgggaaacggacgctacgtacccttccacattcaggtgccccagaaattctttgcaattaaaaacctgctgctgctccccggttcctatacctacgagtggaatttccgcaaggacgtgaacatgattttgcaaagctcgctgggtaacgacctgcgagttgacggggccagcatacgcttcgacagcatcaacctgtatgctaactttttccccatggcccacaacacggcctccaccctggaagccatgctgcgcaacgacaccaatgaccagtccttcaacgactacctgtgcgcggccaacatgctgtatcccatccccgccaacgccaccagcgtgcccatctccatcccgtctcgcaactgggccgcctttaggggttggagtttcacccgcctcaaaaccaaggaaaccccctcgctgggctctggcttcgacccctacttcgtctactcaggctccattccctacctggacggcactttctatcttaaccacactttcaaaaaggtgtctatcatgttcgattcctcggtcagctggcccggcaacgaccgcctgctgacgcccaacgagttcgaaatcaagcgttcggtggacggtgaagggtacaacgtggcccagagcaacatgaccaaggactggttcctggttcaaatgctcagccattacaacatcggttaccagggcttctatgtgcccgagaactacaaggaccgcatgtactccttctttaggaacttccaacccatgagtcgccaagtcgtggactcagtggcttacagggactactaccaggacgttaagctcccctaccagcacaacaactcagggttcgtgggctacatgggtcccaccatgcgagaggggcaggcctacccggccaactatccttatcccctaatcggagagactgctgtacccagcctgacgcagaaaaagttcctctgcgaccgggtgatgtggaggatacccttctctagcaacttcatgtctatgggctccctcaccgacctggggcagaacatgctgtacgccaactccgctcacgccttggacatgacctttgaggtggatcccatggatgagcccacgcttctctatgttctgtttgaagtcttcgacgtggtgcgcatccaccagccgcaccgcggcgtcatcgaggccgtctacctgcgcacacctttctctgccggtaacgccaccacctaaagaagccgatgggctccagcgaacaggagctgcaggccattgttcgcgacctgggctgcgggccctactttttgggcaccttcgacaagcggttccccggcttcatgtcccctcacaagccggcctgtgccatcgttaacacggccggacgggaaaccgggggggtccactggctcgccttcgcctggaacccgcgtaaccgcacctgctacctgttcgacccttttggtttctccgacgaaaggctgaagcagatctaccagttcgagtacgaggggctcctccagcgcagcgctctggcctccacgcccgaccactgcgtcaccctggaaaagtccacccagacggtccaggggcccctctcggccgcctgcgggctcttctgttgcatgtttttgcacgccttcgtgcactggcctcacacccccatggatcacaaccccaccatggatctgctcaccggagtgcccaacagcatgcttcacagcccccaggtcgcccccaccctgcgccgtaaccaggaacacctgtatcgctttctggggaaacactctgcctatttccgccgccatcggcagcgcatcgaacaggccacggccttcgaaagcatgagccaaagagtgtaatcaataaaaaccatttttatttgacatgatacgcgcttctggcgtttttattaaaaatcgaagggttcgagggaggggtcctcgtgcccgctggggagggacacgttgcgatactggaatcgggcgctccaacgaaactcggggatcaccagtcgcggcaggggcacgtcttccaggttctgcttccaaaactgtcgcaccagctgcagggctcccatcacgtcgggcgccgatatcttgaagtcgcagttagggccggagctcccgcggctgttccggaacacggggttggcacactggaacaccatcacgctggggttgtgaatactagccagggccgtcggatcggtcacctccgacgcatccagatcctcggcgttgctcagggcgaacggggtcagcttgcacatctgccgcccgatctggggcaccaggtcgggtttgttgaggcaatcgcagcgcagagggatcaggatgcgtcgctgcccgcgttgcatgatagggtaactcgccgccaggaactcctccatctgacggaaggccatctgggccttaacgccctcggtgaaaaacagcccacaggacttgctagaaaatacgttattgccgcagttaatgtcttccgcgcagcagcgtgcatcttcgttcttcagctgaaccacgttacgcccccagcggttctggaccaccttggctttcgtaggatgctccttcagcgcccgctgcccgttctcgctggtcacatccatttccaccacgtgctccttgcagaccatctccactccgtggaagcaaaacaggacgccctcctgccgggtattgcgatgctcccaaacggcacacccggtgggctcccagctcttgtgttttacccccgcgtaggcttccatgtaagccatgaggaatctgcccatcagctcggtgaaggtcttctgattggtgaaggttagcggcaggccgcggtgctcctcgttcaaccaagtttgacagatcttgcggtacaccgttccctggtcgggcagaaacttaaaagccgctctgctgtcgttgtccacgtggaacttctccattaacatcatcatggtttccatacccttctcccacgctgacaccagcggtttgctgtcggggttcttcaccaacacggcggtagaggggccctcgccggccccgacgtccttcatggtcattctttgaaactccacggagccgtccgcgcgacgtactctgcgcaccggagggtagctgaagcccacctccaccacggtgccttcgccctcgctgtcggaaacgatctccggggatggcggcggtgcgggtgtcgccttgcgagccttcttcttgggagggagctgaggcgcctcctgctcgcgctcggggctcatctcccgcaagtagggggttatggagctgcctgcttggttctgacggttggccattgtatcctaggcagaaagacatggagcttatgcgcgaggaaactttaaccgccccgtcccccgtcagcgacgaagatgtcatcgtcgaacaggacccgggctacgttacgccgcccgaggatctggaggggcctgaccggcgcgacgctagtgagcggcaggaaaatgagaaagaggaggcctgctacctcctggaaggcgacgttttgctaaagcatttcgccaggcagagcaccatagttaaggaggccttgcaagaccgctccgaggtgcccttggacgtcgccgcgctctcccaggcctacgaggcgaaccttttctcgcctcgagtgcctccgaagagacagcccaacggcacctgcgagcccaacccgcgactcaacttctaccccgtgttcgccgtaccagaggcgctggccacctatcacatttttttcaaaaaccaacgcatccccctatcgtgccgggccaaccgcaccgcggccgataggaatctcaggcttaaaaacggagccaacatacctgatatcacgtcgctggaggaagtgcccaagattttcgagggtctgggtcgagatgagaagcgggcggcgaacgctctgcagaaagaacagaaagagagtcagaacgtgctggtggagctggagggggacaacgcgcgtctggccgtcctcaaacgctgcatagaagtctcccacttcgcctaccccgccctcaacttgccacccaaagttatgaaatcggtcatggatcagctgctcatcaagagagctgagcccctggatcccgaccaccccgaggcggaaaactcagaggacggaaagcccgtcgtcagcgacgaggagctcgagcggtggctggaaaccagggacccccaacagttgcaagagaggcgcaagatgatgatggcggccgtgctggtcaccgtggagctggaatgcctgcaacggtttttcagcgacgtggagacgctacgcaaaatcggggaatccctgcactacaccttccgccagggctacgtccgccaggcctgcaagatctccaacgtggagctcagcaacctggtctcctacatgggcatcctccacgagaaccggctggggcagagcgtgctgcactgcaccttgcaaggcgaggcgcggcgggactacgtgcgagactgcatctacctcttcctcaccctcacctggcagaccgccatgggcgtctggcagcagtgcttggaagagagaaacctcaaagagctagacaaactcctctgccgccagcggcgcgccctgtggtccggtttcagcgagcgcacggtcgccagcgctctggcggacatcatcttcccggagcgcctgatgaaaaccttgcaaaacggcctgccggatttcatcagtcaaagcattttgcaaaacttccgctcttttgtcctggaacgctccgggatcttgcccgccatgagctgcgcgctaccttctgactttgtccccctctcctaccgcgagtgccctcccccactgtggagccactgctacctcttccaactggccaactttctggcctaccactccgacctcatggaagacgtaagcggagagggtttactggagtgccactgccgctgcaacctgtgcaccccccacagatcgctggcctgcaacaccgagctactcagcgaaacccaggtcataggtaccttcgagatccaggggccccagcagcaagagggtgcttccggcttgaagctcactccggcgctgtggacctcggcttacttacgcaaatttgtagccgaggactaccacgcccacaaaattcagttttacgaagaccaatctcaaccaccgaaagcccccctcacggcctgcgtcatcacccagagcaagatcctggcccaattgcaatccatcaaccaagcgcgccgcgatttccttttgaaaaagggtcggggggtgtatctggacccccagaccggcgaggaactcaacccgtccacactctccgtcgaagcagcccccccgagacatgccgcccaagggaaccgccaagcagctgatcgctcggcagagagcgaagaagcaagagctgctccagcagcaggtggaggacgaggaagagatgtgggacagccaggcagaggaggtgtcagaggacgaggaggagatggaaagctgggacagcctagacgaggaggaggacgagctttcagaggaagaggcgaccgaagaaaaaccacctgcatccagcgcgccttctctgagccgacagccgaagccccggcccccgacgcccccggccggctcactcaaagccagccgtaggtgggacgccaccgaatctccagcggcagcggcaacggcagcgggtaaggccaaacgcgagcggcgggggtattgctcctggcgggcccacaaaagcagtattgtgaactgcttgcaacactgcgggggaaacatctcctttgcccgacgctacctcctcttccatcacggtgtggccttccctcgcaacgttctctattattaccgtcatctctacagcccctacgaaacgctcggagaaaaaagctaaggcctcctccgccgcgaggaaaaactccgccgccgctgccgccgccaaggatccaccggccaccgaggagctgagaaagcgcatctttcccactctgtatgctatctttcagcaaagccgcgggcagcaccctcagcgcgaactgaaaataaaaaaccgctccttccgctcgctcacccgcagctgtctgtaccacaagagagaagaccagctgcagcgcaccctggacgacgccgaagcactgttcagcaaatactgctcagcgtctcttaaagactaaaagacccgcgctttttccccctcggccgccaaaacccacgtcatcgccagcatgagcaaggagattcccaccccctacatgtggagctatcagccccagatgggcctggccgcgggggccgcccaggactactccagcaagatgaactggctcagcgccggcccccacatgatctcacgagttaacggcatccgagcccaccgaaaccagattctcttagaacaggcggcaatcaccgccacaccccggcgccaactcaacccgcctagttggcccgccgcccaggtgtatcaggaaaatccccgcccgaccacagtcctcctgccacgcgacgcggaggccgaagtcctcatgactaactctggggtacaattagcgggcgggtccaggtacgccaggtacagaggtcgggccgctccttactctcccgggagtataaagagggtgatcattcgaggccgaggtatccagctcaacgacgagacggtgagctcctcaaccggtctcagacctgacggagtcttccagctcggaggagcgggccgctcttccttcaccactcgccaggcctacctgaccctgcagagctcttcctcgcagccgcgctccgggggaatcggcactctccagttcgtggaagagttcgttccctccgtctacttcaaccccttctccggctcgcctggacgctacccggacgccttcattcccaactttgacgcagtgagtgaatccgtggacggctacgactgatgacagatggtgcggccgtgagagctcggctgcgacatctgcatcactgccgtcagcctcgctgctacgctcgggaggcgatcgtcttcagctactttgagctgccggacgagcaccctcagggtccggctcacgggttgaaactcgagatcgagaacgcgctcgagtctcgcctcatcgacaccttcaccgcccgacctctcctggtagaaatcgaacgcgggatcactaccatcaccctgttctgcatctgccccacgcccggattacatgaagatctgtgctgtcatctttgcgctcagtttaataaaaactgaactttttgccgcaccttcaacgccacgcgtcgtttctccaaaagttgtcgacagctcttcagtcagaggtatacgagaaactgtttatttttacaactctactacttttctcacccttaactgctcctgcactaacgaactaattcagtggttcgcgaacggctcactctgccaagtcttttttaattctgctgttcttcctgagtttggctcctttgcgtgtggaaattctacactagtgggagctatcctgtgtcactgtcacgcgcctgattgtatgcccaaactaattagaactctctgtgccttaggtgatatatttaaaatgtaagtcagtatcaataaacttaccttaaatttgacagcagttttttggtaacatcattcagcagcaccactttaccctcttcccaactctcgtatgggacgtgatggtgggcggcaaacttcctccaaaccctaaaacaaatattaatatccacttccttgtccttacccacaattttcatcttttcatagatgaaaagaaccagagttgatgaagacttcaaccccgtctacccttatgactccacatccactcctgcggtcccctttatatcccccccgtttgtaaacagcgatggtcttcaggaaaaccctcctggagtcttaagtttacgaatagctaaacccttgtattttgacatggaaaggaaactagcgctttcacttggaagaggattggcaattacctccaccggacagctagaaagcacacagagcgtgcaaaccacccctccattagttgtcaacaacagcaacacgcttgtcctgcgttattcctccccgttaggcttatcgggtgacaatttaatactaaattgctccgatcctctccgcgtagtaaacaacagcctgacattcagctacctatctccacttcgttttgaaggtggcagtcttacattcaattacacatctccccttaaactgttgaacagcagccttgcgatcggaataaattccaacaaaggtctcggcaatgacagcgatgaactttctgtcaaactaacatcagatctaaagtttaacaacgatggaaaaatagcttttggtatacaaagcctgtgtaccacccccacagccgcctctaactgtaccgtttttaccaacggtgattctttactctgtttatgtttaaccaaatgtggagctcacgtgttaggaagtgtgagtttaaccggaatgcaaggaaccataacagccatgacacagaactacattagtattcaatttctatttgacaacaatggtgcgttgacttcatcaccgctcctcaacaacaacacttggggtatacggcaaaacgacacttcgtccgctaaccccgcctacaatgctcttgcatttatgcctaacagcactgtatatgtaagaggtcaaagtggtgagcccagaaataactattacacccaaacataccttaggggaaacgttaaaaagccaattatccttaccgttacctacaactcggctgcttcaggttattcactaacttttaaatgggatgctgtagtaacagaaaaatttgccactccaacatcttctttttgctatattacagaacaataaattcctattaccccaccaattcgtttttttcagatgaaacgggccagagttgatgaagacttcaacccagtgtacccttatgaccccccatacgctcccgttatgcccttcattactccaccttttacctcctcggatgggttgcaggaaaaaccacttggagtgttaagtttaaactacaaggatcccattactacacaaaatggatctctcacgttgaaaataggaaacggcctcactctagacaaccagggacaattaacatcaactgctggggaagtagagcctccgctcactaatgctaacaacaaacttgcactagcctatagcgaaccattagcagtaaaaagcaaccgcttaactttatcacacaccgccccccttgtcgttgctaataattctttagcgttgcaagtttcagaacctatttttataaatgacgatgacaagctagccctgcagacagccgccccccttgtaactaacgctggcacccttcgcttacagagcgccgcccctttaggattggttgaaaatactcttagactgctgttttctaaacccttgtatttgcaaaatgattttcttgcattaggcattgaacgccccctggctatagcagccgcaggtactctagcactacaactcactcctccattaaagactaacgatgacgggctgacactatccacagtcgagccattaactgtaaaaaacggaaacttaggcttgcaaatatctcgccctttggttgttcaaaacagcagcctttcgcttgctattacccccccgctgcgtctatttaacagcgaccccgttcttggtttgggctttacttttcccctagccgtgacagacaacctactctccttaaacatgggagacggtgttaaactaacctataataaactaacagccaatttgggtagggatttacaatttgaaaacggtgccattgccgtaacgcttactgccgaatcacctttgcaatacactaacaaacttcaactgaatattggagctggccttcgttacaatggagccagcagaaaactagatgtaaacattaaccaaaataagggcttaacttgggacaacgatgcagttattcccaaattaggatcaggtttacaattcgaccctaatggtaacatcgctgttatccctgaaaccgtaaagccgcaaacgttatggacaactgcagatccatcgcctaactgctcagtgtaccaggacttggacgccaggctgtggctcgctcttgttaaaagtggtgacatggttcatggaagcattgctctaaaagccctaaaaggaacgttgctaaatcctacagcaagctacatctccattgtgatatatttttacagcaacggagtcaggcgtaccaactatcccacgtttgacaacgaaggcaccttagctaacagcgctacctggggataccgagaggggcaatctgctaacactaatgtaaccaatgccactgaatttatgcccagctcaaccaggtaccccgtgaataaaggagacaatattcagaatcaatctttttcatacacctgtatcaaaggagatttcgctatgcctgtcccgttccgtgtaacatataatcatgccctggaaggatactcccttaagttcacctggcgcgttgtagccaaccaagcttttgatattccttgctgttccttttcatacatcacagaataaaccactttttaaaatttttctttttattttacacgcacagtaaggcttcctccccccttccatttgacagcatacaccagcctctcccccttcatggcagtaaactgctgcgagccagtccggtatttgggagttaaaatccaaacagtctctttggtgatgaaacgtcgatccgtgatggacacaaatccctggggcaggttttccagcgtttcggtaaaaaactgcacaccgccctacaaaacaaacaggttcaggctctccatgggttatctccccgatcaaactcagacagggtaaaggtgcggtgatgttccactaaaccacgcaggtggcgctgtctgaacctctcggtgcgactcctgtgaggctggtaagaagttagattgtccagtagcctcacagcatggatgatcagtttacgtgtacgtctggcgcaacagcgcatctgaatctcactgagattccggcaagaatcgcacaccatcacaatcaggttgttcatgatcccatagctgaacacgctccagccaaagctcattcgctccaacagcgccaccgcgtgtccgtccaaccttactttaacataaatcaggtgtctgccgcgtacaaacatactacccgcatacagaacttcccggggcaaacccctgttcaccacctgcctgtaccagggaaacctcacatttatcagggagccatagatagccattttaaaccaattagctaacaccgccccaccagctctacactgaagagaaccgggagagttacaatgacagtgaataatccatctctcataacccctgatggtctgatggaaatccagcacaccgccctacaaaacaaacaggttcaggctctccatgggttatctccccgatcaaactcagacagggtaaaggtgcggtgatgttccactaaaccacgcaggtggcgctgtctgaacctctcggtgcgactcctgtgaggctggtaagaagttagattgtccagtagcctcacagcatggatgatcagtttacgtgtacgtctggcgcaacagcgcatctgaatctcactgagattccggcaagaatcgcacaccatcacaatcaggttgttcatgatcccatagctgaacacgctccagccaaagctcattcgctccaacagcgccaccgcgtgtccgtccaaccttactttaacataaatcaggtgtctgccgcgtacaaacatactacccgcatacagaacttcccggggcaaacccctgttcaccacctgcctgtaccagggaaacctcacatttatcagggagccatagatagccattttaaaccaattagctaacaccgccccaccagctctacactgaagagaaccgggagagttacaatgacagtgaataatccatctctcataacccctgatggtctgatggaaatccagatctaacgtggcacagcagatacacactctcatatacattttcatcacatggttttcccaggccgttaaaatacaatcccaatacacgggccactcctgcagtacaataaagctaatacaagatggtatactcctcacctcactaacattgtgcatgttcatattttcacattctaagtaccgagagttctcctctacaacagcactgctgcggtcctcacaaggtggtagctggtgacgatcgtaaggagccagtctgcaacgataccgtctgtcgcgctgcatcgtagaccagagaccgacgcacctcctggtactgccccgtcttaccgcgtaaacagccacgaaaaattcgagctaaaatccacccaacagcctatagctatatatacactccgcccaatgacgctaataccgcaccacccaccgccaaagttcacccacacccacgaaacccgcgaaaatccagcgccgtcagcacttccgcaatttcagtctcacaacgtcacttccgcgcgccttttcacattcccacacccgcccacaaaccccgcgtcaccgcccgtcaccccggccccgcctcgctcctccccgctcattatcatattggcacgtttccagaataaggtatattattgatgatgttaattaattcgaacccataatacccataatagctgtttgccatcgaccaattctcccatattcccggttgaattgtagtacatgagaccaataaagttatttgaagacgaaagggcctcgtgatacgcctatttttataggttaatgtcatgataataatggtttcttagacgtcaggtggcacttttcggggaaatgtgcgcggaacccctatttgtttatttttctaaatacattcaaatatgtatccgctcatgagacaataaccctgataaatgcttcaataatattgaaaaaggaagagtatgagtattcaacatttccgtgtcgcccttattcccttttttgcggcattttgccttcctgtttttgctcacccagaaacgctggtgaaagtaaaagatgctgaagatcagttgggtgcacgagtgggttacatcgaactggatctcaacagcggtaagatccttgagagttttcgccccgaagaacgttttccaatgatgagcacttttaaagttctgctatgtggcgcggtattatcccgtgttgacgccgggcaagagcaactcggtcgccgcatacactattctcagaatgacttggttgagtactcaccagtcacagaaaagcatcttacggatggcatgacagtaagagaattatgcagtgctgccataaccatgagtgataacactgcggccaacttacttctgacaacgatcggaggaccgaaggagctaaccgcttttttgcacaacatgggggatcatgtaactcgccttgatcgttgggaaccggagctgaatgaagccataccaaacgacgagcgtgacaccacgatgcctgcagcaatggcaacaacgttgcgcaaactattaactggcgaactacttactctagcttcccggcaacaattaatagactggatggaggcggataaagttgcaggaccacttctgcgctcggcccttccggctggctggtttattgctgataaatctggagccggtgagcgtgggtctcgcggtatcattgcagcactggggccagatggtaagccctcccgtatcgtagttatctacacgacggggagtcaggcaactatggatgaacgaaatagacagatcgctgagataggtgcctcactgattaagcattggtaactgtcagaccaagtttactcatatatactttagattgatttaaaacttcatttttaatttaaaaggatctaggtgaagatcctttttgataatctcatgaccaaaatcccttaacgtgagttttcgttccactgagcgtcagaccccgtagaaaagatcaaaggatcttcttgagatcctttttttctgcgcgtaatctgctgcttgcaaacaaaaaaaccaccgctaccagcggtggtttgtttgccggatcaagagctaccaactctttttccgaaggtaactggcttcagcagagcgcagataccaaatactgtccttctagtgtagccgtagttaggccaccacttcaagaactctgtagcaccgcctacatacctcgctctgctaatcctgttaccagtggctgctgccagtggcgataagtcgtgtcttaccgggttggactcaagacgatagttaccggataaggcgcagcggtcgggctgaacggggggttcgtgcacacagcccagcttggagcgaacgacctacaccgaactgagatacctacagcgtgagctatgagaaagcgccacgcttcccgaagggagaaaggcggacaggtatccggtaagcggcagggtcggaacaggagagcgcacgagggagcttccagggggaaacgcctggtatctttatagtcctgtcgggtttcgccacctctgacttgagcgtcgatttttgtgatgctcgtcaggggggcggagcctatggaaaaacgccagcaacgcggcctttttacggttcctggccttttgctggccttgaagctgtccctgatggtcgtcatctacctgcctggacagcatggcctgcaacgcgggcatcccgatgccgccggaagcgagaagaatcataatggggaaggccatccagcctcgcgtcgatggcaaacagctattatgggtattatgggttcgaattaat

SEQ ID NO: 39 - DNA, 8764 bp, Artificial Sequence
  Synthetic oligonucleotide sAdApt4287.E1btg.Empty
attaattcgaacccataatacccataatagctgtttgccatcgacgcgaggctggatggccttccccattatgattcttctcgcttccggcggcatcgggatgcccgcgttgcaggccatgctgtccaggcaggtagatgacgaccatcagggacagcttcaaggccagcaaaaggccaggaaccgtaaaaaggccgcgttgctggcgtttttccataggctccgcccccctgacgagcatcacaaaaatcgacgctcaagtcagaggtggcgaaacccgacaggactataaagataccaggcgtttccccctggaagctccctcgtgcgctctcctgttccgaccctgccgcttaccggatacctgtccgcctttctcccttcgggaagcgtggcgctttctcatagctcacgctgtaggtatctcagttcggtgtaggtcgttcgctccaagctgggctgtgtgcacgaaccccccgttcagcccgaccgctgcgccttatccggtaactatcgtcttgagtccaacccggtaagacacgacttatcgccactggcagcagccactggtaacaggattagcagagcgaggtatgtaggcggtgctacagagttcttgaagtggtggcctaactacggctacactagaaggacagtatttggtatctgcgctctgctgaagccagttaccttcggaaaaagagttggtagctcttgatccggcaaacaaaccaccgctggtagcggtggtttttttgtttgcaagcagcagattacgcgcagaaaaaaaggatctcaagaagatcctttgatcttttctacggggtctgacgctcagtggaacgaaaactcacgttaagggattttggtcatgagattatcaaaaaggatcttcacctagatccttttaaattaaaaatgaagttttaaatcaatctaaagtatatatgagtaaacttggtctgacagttaccaatgcttaatcagtgaggcacctatctcagcgatctgtctatttcgttcatccatagttgcctgactccccgtcgtgtagataactacgatacgggagggcttaccatctggccccagtgctgcaatgataccgcgagacccacgctcaccggctccagatttatcagcaataaaccagccagccggaagggccgagcgcagaagtggtcctgcaactttatccgcctccatccagtctattaattgttgccgggaagctagagtaagtagttcgccagttaatagtttgcgcaacgttgttgccattgctgcaggcatcgtggtgtcacgctcgtcgtttggtatggcttcattcagctccggttcccaacgatcaaggcgagttacatgatcccccatgttgtgcaaaaaagcggttagctccttcggtcctccgatcgttgtcagaagtaagttggccgcagtgttatcactcatggttatggcagcactgcataattctcttactgtcatgccatccgtaagatgcttttctgtgactggtgagtactcaaccaagtcattctgagaatagtgtatgcggcgaccgagttgctcttgcccggcgtcaacacgggataataccgcgccacatagcagaactttaaaagtgctcatcattggaaaacgttcttcggggcgaaaactctcaaggatcttaccgctgttgagatccagttcgatgtaacccactcgtgcacccaactgatcttcagcatcttttactttcaccagcgtttctgggtgagcaaaaacaggaaggcaaaatgccgcaaaaaagggaataagggcgacacggaaatgttgaatactcatactcttcctttttcaatattattgaagcatttatcagggttattgtctcatgagcggatacatatttgaatgtatttagaaaaataaacaaataggggttccgcgcacatttccccgaaaagtgccacctgacgtctaagaaaccattattatcatgacattaacctataaaaataggcgtatcacgaggccctttcgtcttcaagaattggtcgatggcaaacagctattatgggtattatgggttcgaattaattaacatcatcaataatataccttattctggaaacgtgccaatatgataatgagcggggaggagcgaggcggggccggggtgacgtgcggtgacgcggggtgacgcggggtggcgcgagggcggggcgggagtggggaggcgcttagtttttacgtatgcggaaggaggttttataccggaagttgggtaatttgggcgtatatttgtaagttttgtgtaatttggcgcgaaaaccgggtaatgaggaagttgaggttaatatgtactttttatgactgggcggaatttctgctgatcagcagtgaactttgggcgctgacggggaggtttcgctacgtggcagtaccacgagaaggctcaaaggtcccatttattgtactcctcagcgttttcgctgggtatttaaacgctgtcagatcatcaagaggccactcttgagtgccggcgagtagagttttctcctccgcgctgccgcgatgaggctggttcccgagatgtacggtgttttctgcagcgagacggcccggaactcagatgagctgcttaatacagatctgctggatgttcccaactcgcctgtggcttcgcctccgtcgcttcatgatcttttcgatgtggaagtggatccaccgcaagatcccaacgaggacgcggtaaacagtatgttccctgaatgtctgtttgaggcggctgaggagggttctcacagcagtgaagagagcagacggggagaggaactggacttgaaatgctacgaggaatgtctgccttctagcgattctgaaacggaacagacagggggagacggctgtgagtcggcaatgaaaaatgaacttgtattagactgtccagaacatcctggtcatggctgccgtgcctgtgcttttcatagaaatgccagcggaaatcctgagactctatgtgctctgtgttatctgcgccttaccagcgattttgtatacagtaagtaaagtgttttcattggcgtacggtaggggattcgttgaagtgctttgtgacttattatgtgtcattatttctaggtgacgtgtccgacgtggaaggggaaggagatagatcaggggctgctaattctccttgcactttgggggctgtggttccagctggcattattaaacccgtggcggtcagagtctcaggcagacggtgcgcagttgaaaaaattgaagacttgctgcaggaagaacagacgcaacctttggacctgtccatgaaacgccctaagctgacttaagtgtgtttattgtatgcaataaaagtgttgatctttgaactgtgtttatgtgttgggtgtgtctgtgggtatataagcaggtggatgggaagtgagagcacagctgcttcagatggatctgctaggagacctaagagaatttggcgtggttcggcgcttgttggagttggcctctgacagaacttccaagttttggaggttttgttttggctcaacgcttagcaacgtgctatatagggtcaagaaggagcaggagacgcagtttgctaggctgttggccgatactcctggagtttttgtggctctggatctaggccatcactctcttttccaagagaaaattatcaaaaacctaacttttacgtctcctggccgcacggttgcttccgctgcctttattacctatattttggatcaatggagcaacagcggcagccacctgtcgtgggagtacatgctggattacatgtcgatggcgctgtggagggccatgctgcggaggagggtttgcatttacttgcgggcgcagcctccgcggctgggccgagtggaggaggaggacgagccgggagagatggagaacctgagggccgggctggaccctccaacggaggactaggtgctgaggatgatcctgaagaggggactagtgggggagctaggaaaaagcaaaaaactgagcctgaacctagaaactttttgaatgagttgactgtaagcctgatgaatcggcagcgtcctgagacggtgttttgggctgagttggaggatgagttcaagaagggggaattgaacctcttgtacaagtatgggtttgagcagttgaaaactcactggttggagccgtgggaggacatggaaatggctctagacacctttgctaaagtggctctgcggccggataaagtttacactattcgccgcactgttaatataaaaaagagtgtttatgttatcggtcatggagctctggtgcaggtgcagaccccagaccgggtggctttcaattgcggcatgcagagtttgggccccggggtgataggtttgaatggagttacatttcaaaatgtcaggtttactggtgatgattttaatggctctgtgtttgtgactagcacccagctaaccctccacggtgtttacttttttaactttaacaatacatgtgtggagtcatggggtagggtgtctctgaggggctgcagttttcatggttgctggaaggcggtggtgggaagaattaaaagtgtcatgtctgtgaagaaatgcatatttgaacgctgtgtgatagctctagcagtagaggggtacggacggatcaggaataacgccgcatctgagaatggatgttttcttttgctgaaaggtacggccagcgttaagcataatatgatttgcggcagcggcctgtgcccctcgcagctcttaacttgcgcagatggaaactgtcacaccttgcgcaccgtgcacatagtgtcccactcgcgccgcacctggccaacatttgagcacaatatgctcatgcgttgcgccgttcacctaggtgctagacgcggcgtgtttatgccttatcaatgtaactttagtcatactaagattttgctggaaactgattccttccctcgagtatgtttcaatggggtgtttgacatgtcaatggaactttttaaagtgataagatatgatgaaaccaagtctcgttgtcgctcatgtgaatgcggagctaatcatttgaggttgtatcctgtaaccctgaacgtcaccgaggagctgaggacggaccaccacatgctgtcttgcctgcgtaccgactatgaatccagtgatgaggagtgaggtgaggggcggagccacaaagggtataaaggggcatgaagggtggacggtcgactggtcaatattggccattagccatattattcattggttatatagcataaatcaatattggctattggccattgcatacgttgtatccatatcataatatgtacatttatattggctcatgtccaacattaccgccatgttgacattgattattgactagttattaatagtaatcaattacggggtcattagttcatagcccatatatggagttccgcgttacataacttacggtaaatggcccgcctggctgaccgcccaacgacccccgcccattgacgtcaataatgacgtatgttcccatagtaacgccaatagggactttccattgacgtcaatgggtggagtatttacggtaaactgcccacttggcagtacatcaagtgtatcatatgccaagtacgccccctattgacgtcaatgacggtaaatggcccgcctggcattatgcccagtacatgaccttatgggactttcctacttggcagtacatctacgtattagtcatcgctattaccatggtgatgcggttttggcagtacatcaatgggcgtggatagcggtttgactcacggggatttccaagtctccaccccattgacgtcaatgggagtttgttttggcaccaaaatcaacgggactttccaaaatgtcgtaacaactccgccccattgacgcaaatgggcggtaggcgtgtacggtgggaggtctatataagcagagctcgtttagtgaaccgtcagatcgcctggagacgccatccacgctgttttgacctccatagaagacaccgggaccgatccagcctccgcggccgggaacggtgcattggaagcttggtaccggtgaattcgctagcgttaacggatcctctagacgagatccgaacttgtttattgcagcttataatggttacaaataaagcaatagcatcacaaatttcacaaataaagcatttttttcactgcattctagttgtggtttgtccaaactcatcaatgtatcttatcatgtctagatccttaaggaatgcggagctaatcatttgaggttgtatcctgtaaccctgaacgtcaccgaggagctgaggacggaccaccacatgctgtcttgcctgcgtaccgactatgaatccagtgatgaggagtgaggtgaggggcggagccacaaagggtataaaggggcatgaagggtggacgcggtgtttcaaaatgagcgggacgacggacggcaatgcgtttgaggggggagtgttcagcccatatctgacatctcgtcttccttcctgggcaggagtgcgtcagaatgtagtgggctccaccgtggacggacggccggtcgcccctgcaaattccgccaccctcacctatgccaccgtgggatcatcgttggacactgccgcggcagctgccgcttctgctgccgcttctactgctcgcggcatggcggctgattttggactatataaccaactggccactgcagctgtggcgtctcggtctctggttcaagaagatgccctgaatgtgatcttgactcgcctggagatcatgtcacgtcgcctggacgaactggctgcgcagatatcccaagctaaccccgataccgcttcagaatcttaaataaagacaaacaaatttgttgaaaagtaaaatggctttatttgttttttttggctcggtaggctcgggtccacctgtctcggtcgttaaggactttgtgtatgttttccaaaacacggtacagatgggcttggatgttcaagtacatgggcatgaggccatctttggggtggagataggaccactgaagagcgtcatgttccggggtggtattgtaaatcacccagtcgtagcagggtttttgagcgtggaactggaatatgtccttcaggagcaggctaatggccaagggcagccccttagtgtaggtgtttacaaagcggttgagctgggagggatgcatgcggggggagatgatatgcatcttggcttggattttgaggttagctatgttaccacccaggtctctgcgggggttcatgttatgaaggaccaccagcacggtgtagccggtgcacttggggaacttgtcatgcagtttggaggggaaggcgtggaagaatttagatacccccttgtgcccccctaggttttccatgcactcatccataataatggcaatgggacccctggcggccgctttagcaaacacgttttgggggttggaaacatcatagttttgctctagagtgagctcatcataggccatctttacaaagcggggtaggagggtgcccgactgggggatgatagttccatctgggcctggagcgtagttgccctcacagatctgcatctcccaggccttaatttccgagggggggatcatgtccacctggggggcgataaagaacacggtttctggcgggggattgatgagctgggtggaaagcaagttacgcaatagctgggatttgccgcaaccggtggggccgtagatgaccccgatgacgggttgcagctggtagttcagagaggaacagctgccgtcggggcgcaggaggggggccacatcgttcatcatgcttctgacatgtttattttcactcactaagttttgcaagagcctctccccacccagggataagagttcttccaggctgttgaagtgtttcagcggtttcaggccgtcggccatgggcatcttttcaagcgactgacgaagcaagtacagtcggtcccagagctcggtgacgtgctctatggaatctcgatccagcagacttcttggttgcgggggttgggccgactttcgctgtagggcaccagccggtgggcgtccagggccgcgagggttctgtccttccagggtctcagcgttcgggtgagggtggtctcggtgacggtgaagggatgagccccgggctgggcgcttgcgagggtgcgcttcaggctcatcctgctggtgctgaagcgggcgtcgtctccctgtgagtcggccagatagcaacgaagcatgaggtcgtagctgagggactcggccgcgtgtcccttggcgcgcagctttcccttggaaacgtgctgacatttggtgcagtgcagacacttgagggcgtagagttttggggccaggaagaccgactcgggcgagtaggcgtcggctccgcactgagcgcagacggtctcgcactccaccagccacgtgagctcgggtttagcgggatcaaaaaccaagttgcctccattttttttgatgcgtttcttaccttgcgtctccatgagtctgtgtcccgcttccgtgacaaaaaggctgtcggtgtccccgtagaccgacttgagggggcgatcttccaaaggtgttccgaggtcttccgcgtacaggaactgggaccactccgagacaaaggctcgggtccaggctaacacgaaggaggcgatctgcgaggggtatctgtcgttttcaatgagggggtccaccttttccagggtgtgcagacacaggtcgtcctcctccgcgtccacgaagttaat

SEQ ID NO: 40 - DNA, 6091 bp, Artificial Sequence
  Synthetic oligonucleotide sAdApt4310A.Empty
catcatcaataatataccttattctggaaacgtgccaatatgataatgagcggggaggagcgaggcggggccggggtgacgtgcggtgacgcggggtgacgcggggtggcgcgagggcggggcgggtgtgcggaggcgcttagtttttacgtatgcggaaggaggttttataccggaagttgggtaatttgggcgtatacttgtaagttttgtgtagtttggcgcgaaaaccgggtaatgaggaagttgaggttaatatgtactttttatgactgggcggaatttctgctgatcagcagtgaactttgggcgctgacggggaggtttcgctacgtggcagtaccacgagaaggctcaaaggtcccatttattgtactcctcagcgttttcgctgggtatttaaacgctgtcagatcatcaagaggccactcttgagtgccggcgagtagagttttctcctcgtcgactggtcaatattggccattagccatattattcattggttatatagcataaatcaatattggctattggccattgcatacgttgtatccatatcataatatgtacatttatattggctcatgtccaacattaccgccatgttgacattgattattgactagttattaatagtaatcaattacggggtcattagttcatagcccatatatggagttccgcgttacataacttacggtaaatggcccgcctggctgaccgcccaacgacccccgcccattgacgtcaataatgacgtatgttcccatagtaacgccaatagggactttccattgacgtcaatgggtggagtatttacggtaaactgcccacttggcagtacatcaagtgtatcatatgccaagtacgccccctattgacgtcaatgacggtaaatggcccgcctggcattatgcccagtacatgaccttatgggactttcctacttggcagtacatctacgtattagtcatcgctattaccatggtgatgcggttttggcagtacatcaatgggcgtggatagcggtttgactcacggggatttccaagtctccaccccattgacgtcaatgggagtttgttttggcaccaaaatcaacgggactttccaaaatgtcgtaacaactccgccccattgacgcaaatgggcggtaggcgtgtacggtgggaggtctatataagcagagctcgtttagtgaaccgtcagatcgcctggagacgccatccacgctgttttgacctccatagaagacaccgggaccgatccagcctccgcggccgggaacggtgcattggaagcttggtaccggtgaattcgctagcgttaacggatcctctagacgagatccgaacttgtttattgcagcttataatggttacaaataaagcaatagcatcacaaatttcacaaataaagcatttttttcactgcattctagttgtggtttgtccaaactcatcaatgtatcttatcatgtctagatccttaaggacatgtcaatggaactgtttaaagtgataagatatgatgaatccaagtctcgttgtcgcccatgtgaatgcggagctaatcatttgaggttgtatcctgtaactctgaacgtcaccgaggagctgagaacggaccaccacatgctgtcttgcctgcgcactgactatgaatccagcgacgaggagtgaggtgaggggcggagccaaacgggtataaaggggcgtgaggggtcggtgcggtgtttcaaaatgagcgggacgacggacggcaatgcgtttgaggggggagtgttcagcccatatctgacatctcgtcttccttcctgggcaggagtgcgtcagaatgtagtgggatccaccgtggacggacgaccggtggctcctgcaaattccgccaccctcacctatgccaccgtgggatcatcgttggacactgccgcggcagctgccgcttctgctgccgcttctactgctcgcggcatggcggctgattttggactgtataaccaactggccactgcagctgtggcgtctcggtccctggttcaagaagatgccctgaatgtgattctgactcgcctggagatcatgtcacgccgcctggacgaactggctgcgcagatatcctcaactaaccccgataccacttcagaaccttaaataaagacaaacaaatttgttgaaaagtaaaatggctttatttgttttttttggctcggtaggctcgggtccacctgtcccggtcgttaaggaccttgtgtatgttttccaagacccggtacagatgggcttggatgttcaagtacatgggcatgaggccatctcgggggtggagataggaccattgcagagcgtcatgctccggggtggtgttgtaaataacccagtcgtagcagggtttctgagcgtggaactggaagatgtcctttaggagcaggctgatggccaagggcagccccttagtgtaggtgttaacaaagcggttaagctgggagggatgcatgcggggggagatgatatgcatcttggcttgaattttgaggttagctatgttaccacctaggtccctgcgggggttcatgttatgaaggaccaccagcacggtgtagccggtgcacttggggaacttgtcatgcagtttggaggggaaggcgtggaagaatttagagacccccttgtggcctcctaggttttccatgcactcatccataatgatggcaatgggacccctggcggccgctttggcaaacacgttttgggggttggaaacatcatagttttgctctagagtgagctcatcataggccatcttaacaaagcggggtaggagggtgcccgactgggggatgatagttccatctgggcctggggcgtagttgccctcacaaatctgcatttcccaggccttaatttccgaggggggtatcatgtccacctggggggcgataaagaacacggtttctggcgggggattgatgagctgggtggaaagcaagttacgcaacagttgggatttgccgcaaccggtgggaccgtagatgaccccgatgacgggttgcagctggtagttgagagaggaacagctgccgtcggggcgcaggaggggggctacatcgttcatcatgcttctgacatgtttattttcactcactaagttttgcaagagcctctccccacccagggataagagttcttccaggctgttgaagtgtttcagcggtttcaggccgtctgccatgggcatcttttcaagcgactgacgaagcaagtacagtcggtcccagagctcggtgacgtgctctatggaatctcgatccagcagacttcttggttgcgggggttgggccgactttcgctgtagggcaccagccggtgggcgtccagggccgcgagggttctgtccttccagggtctcagcgttcgggtgagggtggtctcggtgacggtgaagggatgagccccgggctgggcgcttgcgagggtgcgcttcaggctcatcctgctggtgctgaagcgggcgtcgtctccctgtgagtcggccagatagcaacgaagcatgaggtcgtagctgagggactcggccgcgtgtcccttggcgcgcagctttcccttggaaacgtgctgacatttggtgcagtgcagacacttgagggcgtagagtttgggggccaggaagaccgactcggacgagtaggcgtcggctccgcactgagcgcagacggtctcgcactccaccagccacgtgagctcgggtttagcgggatcaaaaaccaagttgcctccattttttttgatgcgtttcttaccttgcgtctccatgagtctgtgtcccgcttccgtgacaaaaaggctgtcggtgtccccgtagaccgacttgagggggcgatcttccaaaggtgttccgagatcttccgcgtacaggaactgggaccactccgagacaaaggctcgggtccaggctaacacgaaggaggcgatctgcgaggggtatctgtcgttttcaatgaggttaattaattcgaacccataatacccataatagctgtttgccatcgacgcgaggctggatggccttccccattatgattcttctcgcttccggcggcatcgggatgcccgcgttgcaggccatgctgtccaggcaggtagatgacgaccatcagggacagcttcaaggccagcaaaaggccaggaaccgtaaaaaggccgcgttgctggcgtttttccataggctccgcccccctgacgagcatcacaaaaatcgacgctcaagtcagaggtggcgaaacccgacaggactataaagataccaggcgtttccccctggaagctccctcgtgcgctctcctgttccgaccctgccgcttaccggatacctgtccgcctttctcccttcgggaagcgtggcgctttctcatagctcacgctgtaggtatctcagttcggtgtaggtcgttcgctccaagctgggctgtgtgcacgaaccccccgttcagcccgaccgctgcgccttatccggtaactatcgtcttgagtccaacccggtaagacacgacttatcgccactggcagcagccactggtaacaggattagcagagcgaggtatgtaggcggtgctacagagttcttgaagtggtggcctaactacggctacactagaaggacagtatttggtatctgcgctctgctgaagccagttaccttcggaaaaagagttggtagctcttgatccggcaaacaaaccaccgctggtagcggtggtttttttgtttgcaagcagcagattacgcgcagaaaaaaaggatctcaagaagatcctttgatcttttctacggggtctgacgctcagtggaacgaaaactcacgttaagggattttggtcatgagattatcaaaaaggatcttcacctagatccttttaaattaaaaatgaagttttaaatcaatctaaagtatatatgagtaaacttggtctgacagttaccaatgcttaatcagtgaggcacctatctcagcgatctgtctatttcgttcatccatagttgcctgactccccgtcgtgtagataactacgatacgggagggcttaccatctggccccagtgctgcaatgataccgcgagacccacgctcaccggctccagatttatcagcaataaaccagccagccggaagggccgagcgcagaagtggtcctgcaactttatccgcctccatccagtctattaattgttgccgggaagctagagtaagtagttcgccagttaatagtttgcgcaacgttgttgccattgctgcaggcatcgtggtgtcacgctcgtcgtttggtatggcttcattcagctccggttcccaacgatcaaggcgagttacatgatcccccatgttgtgcaaaaaagcggttagctccttcggtcctccgatcgttgtcagaagtaagttggccgcagtgttatcactcatggttatggcagcactgcataattctcttactgtcatgccatccgtaagatgcttttctgtgactggtgagtactcaaccaagtcattctgagaatagtgtatgcggcgaccgagttgctcttgcccggcgtcaacacgggataataccgcgccacatagcagaactttaaaagtgctcatcattggaaaacgttcttcggggcgaaaactctcaaggatcttaccgctgttgagatccagttcgatgtaacccactcgtgcacccaactgatcttcagcatcttttactttcaccagcgtttctgggtgagcaaaaacaggaaggcaaaatgccgcaaaaaagggaataagggcgacacggaaatgttgaatactcatactcttcctttttcaatattattgaagcatttatcagggttattgtctcatgagcggatacatatttgaatgtatttagaaaaataaacaaataggggttccgcgcacatttccccgaaaagtgccacctgacgtctaagaaaccattattatcatgacattaacctataaaaataggcgtatcacgaggccctttcgtcttcaagaattggtcgatggcaaacagctattatgggtattatgggttcgaattaat

SEQ ID NO: 41 - DNA, 16580 bp, Artificial Sequence
  Synthetic oligonucleotide pBr/sAd4310A.pIX-pV
attaagacatgtcaatggaactgtttaaagtgataagatatgatgaatccaagtctcgttgtcgcccatgtgaatgcggagctaatcatttgaggttgtatcctgtaactctgaacgtcaccgaggagctgagaacggaccaccacatgctgtcttgcctgcgcactgactatgaatccagcgacgaggagtgaggtgaggggcggagccaaacgggtataaaggggcgtgaggggtcggtgcggtgtttcaaaatgagcgggacgacggacggcaatgcgtttgaggggggagtgttcagcccatatctgacatctcgtcttccttcctgggcaggagtgcgtcagaatgtagtgggatccaccgtggacggacgaccggtggctcctgcaaattccgccaccctcacctatgccaccgtgggatcatcgttggacactgccgcggcagctgccgcttctgctgccgcttctactgctcgcggcatggcggctgattttggactgtataaccaactggccactgcagctgtggcgtctcggtccctggttcaagaagatgccctgaatgtgattctgactcgcctggagatcatgtcacgccgcctggacgaactggctgcgcagatatcctcaactaaccccgataccacttcagaaccttaaataaagacaaacaaatttgttgaaaagtaaaatggctttatttgttttttttggctcggtaggctcgggtccacctgtcccggtcgttaaggaccttgtgtatgttttccaagacccggtacagatgggcttggatgttcaagtacatgggcatgaggccatctcgggggtggagataggaccattgcagagcgtcatgctccggggtggtgttgtaaataacccagtcgtagcagggtttctgagcgtggaactggaagatgtcctttaggagcaggctgatggccaagggcagccccttagtgtaggtgttaacaaagcggttaagctgggagggatgcatgcggggggagatgatatgcatcttggcttgaattttgaggttagctatgttaccacctaggtccctgcgggggttcatgttatgaaggaccaccagcacggtgtagccggtgcacttggggaacttgtcatgcagtttggaggggaaggcgtggaagaatttagagacccccttgtggcctcctaggttttccatgcactcatccataatgatggcaatgggacccctggcggccgctttggcaaacacgttttgggggttggaaacatcatagttttgctctagagtgagctcatcataggccatcttaacaaagcggggtaggagggtgcccgactgggggatgatagttccatctgggcctggggcgtagttgccctcacaaatctgcatttcccaggccttaatttccgaggggggtatcatgtccacctggggggcgataaagaacacggtttctggcgggggattgatgagctgggtggaaagcaagttacgcaacagttgggatttgccgcaaccggtgggaccgtagatgaccccgatgacgggttgcagctggtagttgagagaggaacagctgccgtcggggcgcaggaggggggctacatcgttcatcatgcttctgacatgtttattttcactcactaagttttgcaagagcctctccccacccagggataagagttcttccaggctgttgaagtgtttcagcggtttcaggccgtctgccatgggcatcttttcaagcgactgacgaagcaagtacagtcggtcccagagctcggtgacgtgctctatggaatctcgatccagcagacttcttggttgcgggggttgggccgactttcgctgtagggcaccagccggtgggcgtccagggccgcgagggttctgtccttccagggtctcagcgttcgggtgagggtggtctcggtgacggtgaagggatgagccccgggctgggcgcttgcgagggtgcgcttcaggctcatcctgctggtgctgaagcgggcgtcgtctccctgtgagtcggccagatagcaacgaagcatgaggtcgtagctgagggactcggccgcgtgtcccttggcgcgcagctttcccttggaaacgtgctgacatttggtgcagtgcagacacttgagggcgtagagtttgggggccaggaagaccgactcggacgagtaggcgtcggctccgcactgagcgcagacggtctcgcactccaccagccacgtgagctcgggtttagcgggatcaaaaaccaagttgcctccattttttttgatgcgtttcttaccttgcgtctccatgagtctgtgtcccgcttccgtgacaaaaaggctgtcggtgtccccgtagaccgacttgagggggcgatcttccaaaggtgttccgagatcttccgcgtacaggaactgggaccactccgagacaaaggctcgggtccaggctaacacgaaggaggcgatctgcgaggggtatctgtcgttttcaatgagggggtccaccttttccagggtgtgcagacacaggtcgtcctcctccgcgtccacgaaggtgattggcttgtaagtgtaggtcacgtgacccgcacccccccaaggggtataaaagggggcgtgcccactctccccgtcactttcttccgcatcgctgtggaccagagccagctgttcgggtgagtaggccctctcaaaagccggcatgatttcggcgctcaagttgtcagtttctacaaacgaggaggatttgatattcacgtgccccgcggcgatgcttttgatggtggaggggtccatctgatcagaaaacacgatctttttattgtcaagtttggtggcgaaagacccgtagagggcgttggaaagcaacttggcgatggagcgcagggtctgatttttctcccgatcggccctctccttggcggcgatgttgagttgcacgtactcgcgagccacgcaccgccactcggggaacacggcggtgcgctcgtcgggcaggatgcgcacgtgccagccgcggttgtgcagggtgatgaggtccacgctggtggccacctccccgcggaggggctcgttggtccaacacaatcgccccccttttctggagcagaacggaggcaggggatctagcaagttggcgggcggggggtcggcgtcgatggtaaatatgccgggtagcagaattttattaaaataatcgatttcggtgtccgtgtcttgcaacgcgtcttcccacttcttcaccgccagggccctttcgtagggatttaggggcggtccccagggcatggggtgggtcagggccgaggcgtacatgccgcagatgtcgtacacgtacaggggctccctcaacaccccgatgtaagtggggtaacagcgccccccgcggatgctggctcgcacgtagtcgtacatctcgtgagagggagccatgagcccgtctcccaagtgggtcttgtggggtttctcggcccggtagaggatctgcctgaagatggcgtgggagttggaagagatggtggggcgttggaagacgttaaagttggctccgggcagtcccacggagtcttggatgaattgggcgtaggattcccggagcttgtccaccagggctgcggttaccagcacgtcgagagcgcagtagtccaacgtctcgcggaccaggttgtaggccgtctcttgttttttctcccacagttcgcggttgaggaggtattcctcgcggtctttccagtactcttcggcgggaaatcctttttcgtccgctcggtaagaacctaacatgtaaaattcgttcacggctttgtatggacaacagcctttttctaccggcagggcgtacgcttgagcggcctttctgagagaggtgtgggtgagggcgaaggtgtcccgcaccatcactttcaggtactgatgtttgaagtccgtgtcgtcgcaggcaccctgttcccacagcgtgaagtcggtgcgctttttctgcctgggattggggagggcgaaggtgacgtcgttaaagaggattttcccggcgcggggcatgaagttgcgagagatcctgaagggtccgggcacgtccgagcggttgttgatgacttgcgccgccaggacgatctcatcgaagccgttgatgttgtggcccacgatgtaaagttcgataaagcgcggctgtcccttgagggccggcgcttttttcaactcctcgtaggtgagacagtccggcgaggacagacccagctcagcccgggcccagtcggagagttgaggattagccgcgaggaaggaactccatagatccaaggccaggagagtttgcaagcggtcgcggaactcgcggaactttttgcccacggccattttctccggcgttaccacgtaaaaggtgtcggggcggttgttccagacgtcccatcggagctctagggccagctcgcaggcttggcgaacgagggtctcctcgcccgagacgtgcatgaccagcatgaagggtaccaactgtttcccgaacgagcccatccatgtgtaggtttctacgtcgtaggtgacaaagagccgctgggtgcgcgcgtgggagccgatcgggaagaagctgatctcctgccaccagctggaggaatgggtgttgatgtggtgaaagtagaagtcccgccggcgcacagagcattcgtgctgatgtttgtaaaagcgaccgcagtagtcgcagcgttgcacgctctgtatctcctgaatgagatgcgcttttcgcccgcgcaccagaaaccggagggggaagttgagactggggcttggtggggcggcatccccttcgccttggcggtgggagtctgcgtctgcgcccttcttctctgggtggacgacggtggggacgacgacgccccgggtgccgcaagtccagatctccgccacggaggggcgcaggcgctgcaggagggggcgcagctgcccgctgtccagggagtcgagggcggccgcgctgaggtcgacgggaagcgtttgcaagttcactttcagaagaccggtaagagcgtgagccaggtgcagatggtacttgatttccaggggggtgttggaagaggcgtccacggcgtagaggaggccgtgtccgcgcggggtcaccaccgtgccccgaggaggttttatctcactcgtcgagggcgagcgccgggtggtagaggcggctctgcgccggggggcagcggaggcagaggcacgttttcgtgaggattcggcagcggttgatgacgagcccggagactgctggcgtgggcgacgacgcggcggttgaggtcctggatgtgctgtctctgcgtgaagaccaccggtccccgggtcctgaacctgaaagagagttccacagaatcaatgtctgcatcgttaacggcggcctgcctgaggatctcctgtacgtcgcccgagttgtcttgataggcgatctcggccatgaactgctccacttcttcctcgcggaggtcgccgtggcccgctcgctccacggtggcggccaggtcgttggagatgcgacgcatgagttgagagaaggcgttgaggccgttctcgttccacacgcggctgtacaccacgtttccgaaggagtcgcgcgctcgcatgaccacctgggccacgttgagttccacgtggcgggcgaagacggcgtagtttctgaggcgctggaagaggtagttgagcgtggtggcgatgtgctcgcagacgaagaagtacatgatccagcgccgcagggtcatctcgttgatgtctccgatggcttcgagacgctccatggcctcgtagaagtcgacggcgaagttgaaaaattgggagttgcgggcggccaccgtgagttcttcttgcaggaggcggatgagatcggcgaccgtgtcgcgcacctcctgctcgaaagcgccccgaggcgcctctgcttcttcctccggctcctcctcttccaggggcacgggttcctccggcagctctgcgacggggacggggcggcgacgtcgtcgtctgaccggcaggcggtccacgaagcgctcgatcatttcgccgcgccggcgacgcatggtctcggtgacggcgcgtccgttttcgcgaggtcgcagttcgaagacgccgccgcgcagagcgcccccgtgcagggagggtaagtggttagggccgtcgggcagggacacggcgctgacgatgcattttatcaattgctgcgtaggcactccgtgcagggatctgagaacgtcgaggtcgacgggatccgagaacttctctaggaaagcgtctatccaatcgcaatcgcaaggtaagctgaggacggtgggccgctggggggcgtccgcgggcagttgggaggtgatgctgctgatgatgtaattaaagtaggcggtcttcaggcggcggatggtggcgaggaggaccacgtctttgggcccggcctgttgaatgcgcaggcgctcggccatgccccaggcctcgctctgacagcgacgcaggtctttgtagtagtcttgcatcagtctctccaccggaacctctgcttctcccctgtctgccatgcgagtcgagccgaagccccgcaggggctgcagcaacgctaggtcggccacgaccctctcggccagcacggcctgttgaatctgcgtgagggtggtctggaagtcgtccaggtccacgaagcggtgataggcccccgtgttgatggtgtaggtgcagttggccataacggaccagttgacgacttgcatgccgggttgggtgatctccgtgtacttgaggcgcgagtaggcgcgggactcgaacacgtagtcgttgcatgtgcgcaccagatactggtagccgaccaggaagtgaggaggcggttctcggtacaggggccagccgacggtggcgggggcgccgggggacaggtcgtccagcatgaggcggtggtagtggtagatgtagcgggagagccaggtgatgccggccgaggtggtcgcggccctggtgaattcgcggacgcggttccagatgttgcgcagggggcgaaagcgctccatggtgggcacgctctgccccgtgaggcgggcgcaatcttgtacgctctagatggaaaaaagacagggcggtcatcgactcccttccgtagctcggggggtaaagtcgcaagggtgcggcggcggggaaccccggttcgagaccggccggatccgccgctcccgatgcgcctggccccgcatccacgacgtccgcgccgagacccagccgcgacgctccgccccaatacggaggggagtcttttggtgttttttcgtagatgcatccggtgctgcggcagatgcgacctcagacgcccaccaccaccgccgcggcggcagtaaacctgagcggaggcggtgacagggaggaggaggagctggctttagacctggaagagggagaggggttggcccggctgggagcgccgtccccagagagacaccctagggttcagctcgtgagggacgccaggcaggcttttgtgccgaagcagaacctgtttagggaccgcagcggtcaggaggcggaggagatgcgcgattgcaggtttcgcgcgggcagagagctgagggcgggcttcgatcgcgagcggctcctgagggcggaggatttcgagcccgacgagcgttctggggtgagcccggcccgcgctcacgtctcggcggccaacctggtgagcgcgtacgagcagacggtgaacgaggagcgcaacttccaaaagagctttaacaatcacgtgaggaccctgatcgcgagggaggaggtgaccatcgggctgatgcatctgtgggacttcgtggaggcctacgtgcagaacccggccagcaaacctctgacggcccagctgttcctgatcgtgcagcacagccgcgacaacgagacgttccgcgacgccatgttgaacatcgcggagcccgagggtcgctggctcttggatctgattaacatcctgcagagcatcgtggtgcaggagagggggctgagtttagcggacaaggtggcggccattaactattcgatgcagagcctggggaagttctacgctcgcaagatctacaagagcccttacgtgcccatagacaaggaggtgaagatagacagcttttacatgcgcatggcgctgaaggtgctgacgctgagcgacgatctcggcgtgtaccgtaacgacaagatccacaaggcggtgagcgccagccgccggcgggagctgagcgacagggagctgatgcacagcctgcagagggcgctggcgggcgccggggacgaggagcgcgaggcttacttcgacatgggagccgatctgcagtggcgtcccagcgcgcgcgccttggaggcggcgggctaccccgacgaggaggaccgggatgatttggaggaggcaggcgagtacgaggacgaagcctgaccgggcaggtgttgttttagatgcagcggccggcggacggggccaccgcggatcccgcacttttggcatccatgcagagtcaaccttcgggcgtgaccgcctccgatgactgggcggcggccatggaccgcatcatggcgctgaccacccgcaaccccgaggcttttaggcagcaaccccaggccaaccgtttttcggccatattggaagcggtggtaccgtcgcgcaccaaccccacacacgagaaagtcctgactatcgtgaacgccctggtagacagcaaagctatccgccgcgacgaggcggggctgatctacaacgctctgttggaacgggtggcgcgctacaacagcactaacttgcagaccaatctggatcgcctcaccacggacgtgaaggaggcgctggctcagaaggagcggtttctgagggatagcaatctgggttctctggtggcactgaacgcctttctgagcacgcagccggccaacgtgccccgcgggcaggaggattacgtgagcttcatcagcgctctgagactgctggtgtccgaggtgccccagagcgaggtgtaccagtctgggccggattacttttttcagacgtcccgacagggcttgcaaacggtgaacctgactcaggcctttaaaaacttgcaaggtatgtggggcgtcaaggccccggtgggcgatcgcgccactatctccagtctgctgacccccaacactcgcctgctgctgctcttgatcgcaccgttcaccaacagtagcactatcagccgtgactcgtacctgggtcatctcatcactctgtaccgcgaggccatcggccaggctcagatcgacgagcatacgtatcaggagatcactaacgtgagccgggccctgggtcaggaagataccggcagcctggaagccacgttgaactttttgctaaccaaccggaggcaaaaaataccctcccagttcacgttaagcgccgaggaggagaggattctgcgatacgtgcagcagtccgtgagcctgtacttgatgcgcgagggcgccaccgcttccacggctttagacatgacggctcggaacatggaaccgtccttttactccgcccaccggccgttcattaaccgtctgatggactacttccatcgtgcggccgccatgaacggggagtacttcaccaatgccatcctgaatccgcattggatgcccccgtccggcttctacaccggggagtttgacctgcccgaagccgacgacggctttctgtgggacgacgtgtccgatagcattttcacgccggggaatcgccgattccagaagaaggagggcggagacgagctccccctctccagcgtggaggctgcctctaggggagagagcccctttcccagtctgtcttccgccagtagcggtcgggtaacgcgcccgcggttgccgggggagagcgactacctgaacgaccccttgctgcgaccggctagaaagaaaaatttccccaacaacggggtggaaagcttggtggataaaatgaatcgttggaagacctacgcccaggagcagcgggagtgggaggacagtcagccgcgaccgctggttccgccgcactggcgtcgccagagagaagacccggacgactccgcagacgatagtagcgtgttggacctgggagggagcggagccaacccctttgctcacttgcaacccaaggggcgttcgagtcgcctctactaataaaaaagacgcggaaacttaccagagccatggccacagcgtgtgtcctttcttcctctctttcttcctcggcgcggcagaatgagaagagcggtgagagtcacgccggcggcgtatgagggtccgcccccttcttacgaaagcgtgatgggatcagcgaacgtgccggccacgctggaggcgccttacgttcctcccagatacctgggacctaccgagggcagaaacagcatccgttactccgagctggcgcccctgtacgataccaccaaggtgtacctggtggacaacaagtcggcggacatcgcctccctgaattaccaaaacgaccacagcaactttctgaccaccgtggtgcagaacaatgacttcaccccgacggaggcgggcacgcagaccattaactttgacgagcgttcccgctggggcggtcagctgaaaaccatcctgcacaccaacatgcccaacatcaacgagttcatgtccaccaacaagttcagggccaggctgatggttaaaaaggtagaaaaccagcctcccgagtacgaatggtttgagttcaccatccccgagggcaactattccgagactatgactatcgatctgatgaacaatgcgatcgtggacaattacctgcaagtggggaggcagaacggggtattggaaagcgatatcggtgtgaaatttgataccagaaacttccgactggggtgggatcccgtgaccaagctggtaatgccaggcgtgtacaccaacgaggcttttcaccccgacatcgtgctgctgccggggtgcggcgtggatttcactcagagccgcttgagtaacctgttaggaatcaggaagcgccgtcccttccaggagggctttcagatcatgtatgaggacctggagggaggtaacattcccgctctactagatgtgacaaagtacgaacaaagtgtacagcgagccaaggcggaagggcgagagattcgcggagacacttttgccgtgtctccccaggatttggttatagagccgttagagcatgacagcaaaaatcgtagttacaatcttttgcccaacaaaaccgacacggcctatcgcagctggtttttggcttacaactacggagaccccgagaaaggagtgagatcatggaccatactcaccaccacggacgtgacctgcggctcgcagcaagtgtactggtccctgccggatatgatgcaagacccggtcaccttccgcccctccacccaagtcagcaacttcccggtggtgggcaccgagctgctgcccgtccatgccaagagcttctacaacgagcaggccgtctactcgcaactcattcgccagtccaccgcgcttacccacgtgttcaatcgttttcccgagaaccagattctggtgcgccctcccgctcctaccattaccaccgtcagtgaaaacgttcccgccctcacagatcacggaaccctaccgctgcgcagcagtatcagtggagttcagcgcgtgaccatcaccgacgccagacgtcgaacctgcccctacgtttacaaagcgctcggcgtggtggcccctaaagttctctctagtcgcaccttttaaacatgtccattctcatctctcccgataacaacaccggctggggattgggctccggcaagatgtacggcggggctaagcgacgctccagtcagcatcccgttcgcgttcggggtcacttccgcgctccctggggagcttacaagcgaggactctctggccgaacggctgtagacgataccatagatgccgtgattgccgacgcccgccggtacaaccccggaccggtcgctagcgccgcctccaccgtggattccgtgatcgacagcgtggtggccagcgccagggcctatgctcgccgcaagaggcggctgcatcggaaacgtcgccccaccgccgccatgctagcagccagggccgtgctgaggcgggcccggagggtaggcaggagggctatgcgccgcgctgccgccaacgccgccgggagggcccgcagacaagccgcccgccaggccgccgctgccatcgctagcatggccagacccaggagagggaacgtgtactgggtgcgcgattctgtaacgggagtccgagtgccggtgcgcagccgacctccccgaagttagaagatccaagctgcgaagacggcggtactgagtctccctgttgttattagcccaacatgagcaagcgcaagtttaaagaagaactgctgcagacgctggtgcctgagatctatggccctccggacgtgaagcctgacattaagccccgcgatatcaagcgtgttaaaaagcgggaaaaaaaagaggaacttgcggcggtagacgatggcggtgtagaatttattaggagtttcgccccacggcgcagggttcaatggaaagggcggcgtgtacaacgcgttctgaggccgggcaccgcggtagtttttaccccgggagagcggtcggccgttaggggtttcaagcggcagtacgatgaggtgtacggcgacgaagacatactggaacaggcggctcagcagattggagaattcgcttatggcaaacgttctcggcgcgaagacctggccatcgccttggacagcggcaatcccacacccagcctcaaacccgtgacgctgcaacaggtgcttcccgtgagcgccagtactgacagcaaaagggggattaaaagagagatggaagagctgcaacccaccatccaacttatggtccctaaacgacagaggttggaagaggtcctggagaagatgaaagtggaccccagcatagagccggatgtgaaagtgaggcctattaaggaagtggcccccggtcttggggtgcaaacggtggacattcaaatccccgtcacgtccgcttcaacagcggtggaagccatggaaacgcaaacggaagcccccgccgtcacggtcggtaccagggaagtggcgttgcaaacggaaccctggtacgaatacgccacccctaggcgtcagaggcggtccgcccgttacggacccgtcaacgccatcatgcccgagtacgcgctacatccgtctatccggcccactcccggctaccggggagtgacgtatcgcccgtcaggaactcgccgccgttaccgtcgccgccgtcgctctcgccgcgctctggccccagtgtcggtgcggcgcgtgacccgccaggggaaaacagtcaccatccccaacccgcgctaccaccctagcattctttaatgactctgccgttttgcagatggctctgacttgccgcgtgcgccttcccgttctgcactatcgaggaagatctcgtcgtaggagaggcatggcgggcagtggtcgccggcgggctttgcgcaggcgcatgaaaggcggaattttacccgccctaatacctataatcgccgccgccataggcgccatacccggcgtcgcttcagtggccttgcaagcagctcgtaataaataaacgaaggcttttgcacttatgtcctggtcctgactattttatgcagaaaaagcatggaagacatcaattttacgtcgctggctccgcggcaaggctcgcggccgctcatgggcacctggaacgacatcggcaccagtcagctcaacgggggcgctttcaattgggggagcctttggagcggcattaaaaactttggctccacgattaaatcctacggcagcaaagcctggaacagtagtgctggtcaaatgctccgagataaactgaaggacaccaacttccaagagaaagtggtcaacggggtggtgaccggcatacacggcgcggtagatcttgccaaccaagcggtgcagaaagagattgacaggcgattggaaaactcgcgggtgccgccgcagagaggggatgaggtggaggtcgaggaagtagaagtagaggaaaagctgccccccttggagaaagttcccggtgcgattccaaggccgcagaagcggccaaggccagaactagaagaaactctggtgacggagagcaaggagcctccctcgtacgagcaagccttaaaagagggcgcttcaccctacccgatgaccaaaccgatcgcgcctatggctcggccggtgtacgggaaggactacaaacctgtcacgctagaacttcctccgccactcccttcgcgtcctacggtgcctcccatgccagcgccgtcggccggtcccgtgtctgcaccttccgcagcgcctctgccagccgcccgcccagtggccgtggccactgccagaaaccccagaggccagagaggagccaactggcaaaacacgctgaacagcatcttaattaattcgaacccataatacccataatagctgtttgccatcgacgcgaggctggatggccttccccattatgattcttctcgcttccggcggcatcgggatgcccgcgttgcaggccatgctgtccaggcaggtagatgacgaccatcagggacagcttcaaggatcgctcgcggctcttaccagcccagcaaaaggccaggaaccgtaaaaaggccgcgttgctggcgtttttccataggctccgcccccctgacgagcatcacaaaaatcgacgctcaagtcagaggtggcgaaacccgacaggactataaagataccaggcgtttccccctggaagctccctcgtgcgctctcctgttccgaccctgccgcttaccggatacctgtccgcctttctcccttcgggaagcgtggcgctttctcatagctcacgctgtaggtatctcagttcggtgtaggtcgttcgctccaagctgggctgtgtgcacgaaccccccgttcagcccgaccgctgcgccttatccggtaactatcgtcttgagtccaacccggtaagacacgacttatcgccactggcagcagccactggtaacaggattagcagagcgaggtatgtaggcggtgctacagagttcttgaagtggtggcctaactacggctacactagaaggacagtatttggtatctgcgctctgctgaagccagttaccttcggaaaaagagttggtagctcttgatccggcaaacaaaccaccgctggtagcggtggtttttttgtttgcaagcagcagattacgcgcagaaaaaaaggatctcaagaagatcctttgatcttttctacggggtctgacgctcagtggaacgaaaactcacgttaagggattttggtcatgagattatcaaaaaggatcttcacctagatccttttaaattaaaaatgaagttttaaatcaatctaaagtatatatgagtaaacttggtctgacagttaccaatgcttaatcagtgaggcacctatctcagcgatctgtctatttcgttcatccatagttgcctgactccccgtcgtgtagataactacgatacgggagggcttaccatctggccccagtgctgcaatgataccgcgagacccacgctcaccggctccagatttatcagcaataaaccagccagccggaagggccgagcgcagaagtggtcctgcaactttatccgcctccatccagtctattaattgttgccgggaagctagagtaagtagttcgccagttaatagtttgcgcaacgttgttgccattgctgcaggcatcgtggtgtcacgctcgtcgtttggtatggcttcattcagctccggttcccaacgatcaaggcgagttacatgatcccccatgttgtgcaaaaaagcggttagctccttcggtcctccgatcgttgtcagaagtaagttggccgcagtgttatcactcatggttatggcagcactgcataattctcttactgtcatgccatccgtaagatgcttttctgtgactggtgagtactcaaccaagtcattctgagaatagtgtatgcggcgaccgagttgctcttgcccggcgtcaacacgggataataccgcgccacatagcagaactttaaaagtgctcatcattggaaaacgttcttcggggcgaaaactctcaaggatcttaccgctgttgagatccagttcgatgtaacccactcgtgcacccaactgatcttcagcatcttttactttcaccagcgtttctgggtgagcaaaaacaggaaggcaaaatgccgcaaaaaagggaataagggcgacacggaaatgttgaatactcatactcttcctttttcaatattattgaagcatttatcagggttattgtctcatgagcggatacatatttgaatgtatttagaaaaataaacaaataggggttccgcgcacatttccccgaaaagtgccacctgacgtctaagaaaccattattatcatgacattaacctataaaaataggcgtatcacgaggccctttcgtcttcaagaattggtcgatggcaaacagctattatgggtattatgggttcgaattaat

SEQ ID NO: 42 - DNA, 21626 bp, Artificial Sequence
  Synthetic oligonucleotide pBr/sAd4310A.RsrII-rITR
attaacaccgtggattccgtgatcgacagcgtggtggccagcgccagggcctatgctcgccgcaagaggcggctgcatcggaaacgtcgccccaccgccgccatgctagcagccagggccgtgctgaggcgggcccggagggtaggcaggagggctatgcgccgcgctgccgccaacgccgccgggagggcccgcagacaagccgcccgccaggccgccgctgccatcgctagcatggccagacccaggagagggaacgtgtactgggtgcgcgattctgtaacgggagtccgagtgccggtgcgcagccgacctccccgaagttagaagatccaagctgcgaagacggcggtactgagtctccctgttgttattagcccaacatgagcaagcgcaagtttaaagaagaactgctgcagacgctggtgcctgagatctatggccctccggacgtgaagcctgacattaagccccgcgatatcaagcgtgttaaaaagcgggaaaaaaaagaggaacttgcggcggtagacgatggcggtgtagaatttattaggagtttcgccccacggcgcagggttcaatggaaagggcggcgtgtacaacgcgttctgaggccgggcaccgcggtagtttttaccccgggagagcggtcggccgttaggggtttcaagcggcagtacgatgaggtgtacggcgacgaagacatactggaacaggcggctcagcagattggagaattcgcttatggcaaacgttctcggcgcgaagacctggccatcgccttggacagcggcaatcccacacccagcctcaaacccgtgacgctgcaacaggtgcttcccgtgagcgccagtactgacagcaaaagggggattaaaagagagatggaagagctgcaacccaccatccaacttatggtccctaaacgacagaggttggaagaggtcctggagaagatgaaagtggaccccagcatagagccggatgtgaaagtgaggcctattaaggaagtggcccccggtcttggggtgcaaacggtggacattcaaatccccgtcacgtccgcttcaacagcggtggaagccatggaaacgcaaacggaagcccccgccgtcacggtcggtaccagggaagtggcgttgcaaacggaaccctggtacgaatacgccacccctaggcgtcagaggcggtccgcccgttacggacccgtcaacgccatcatgcccgagtacgcgctacatccgtctatccggcccactcccggctaccggggagtgacgtatcgcccgtcaggaactcgccgccgttaccgtcgccgccgtcgctctcgccgcgctctggccccagtgtcggtgcggcgcgtgacccgccaggggaaaacagtcaccatccccaacccgcgctaccaccctagcattctttaatgactctgccgttttgcagatggctctgacttgccgcgtgcgccttcccgttctgcactatcgaggaagatctcgtcgtaggagaggcatggcgggcagtggtcgccggcgggctttgcgcaggcgcatgaaaggcggaattttacccgccctaatacctataatcgccgccgccataggcgccatacccggcgtcgcttcagtggccttgcaagcagctcgtaataaataaacgaaggcttttgcacttatgtcctggtcctgactattttatgcagaaaaagcatggaagacatcaattttacgtcgctggctccgcggcaaggctcgcggccgctcatgggcacctggaacgacatcggcaccagtcagctcaacgggggcgctttcaattgggggagcctttggagcggcattaaaaactttggctccacgattaaatcctacggcagcaaagcctggaacagtagtgctggtcaaatgctccgagataaactgaaggacaccaacttccaagagaaagtggtcaacggggtggtgaccggcatacacggcgcggtagatcttgccaaccaagcggtgcagaaagagattgacaggcgattggaaaactcgcgggtgccgccgcagagaggggatgaggtggaggtcgaggaagtagaagtagaggaaaagctgccccccttggagaaagttcccggtgcgattccaaggccgcagaagcggccaaggccagaactagaagaaactctggtgacggagagcaaggagcctccctcgtacgagcaagccttaaaagagggcgcttcaccctacccgatgaccaaaccgatcgcgcctatggctcggccggtgtacgggaaggactacaaacctgtcacgctagaacttcctccgccactcccttcgcgtcctacggtgcctcccatgccagcgccgtcggccggtcccgtgtctgcaccttccgcagcgcctctgccagccgcccgcccagtggccgtggccactgccagaaaccccagaggccagagaggagccaactggcaaaacacgctgaacagcatcgtgggcctgggagttaaaagcctgaaacgccgccgttgctattattaaaaaagtgtagctaaaaaatctcccgttgtatacgcctcctatgttaccgccagagacgtgtgactgtcgtcgcgagcagcgctttcaagatggccaccccatcgatgatgccgcagtggtcttacatgcacatcgccgggcaggacgcctcggagtatctgagccccggtcttgtgcagtttgcccgcgccaccgacacctacttcagcttgggaaacaagtttagaaatcccaccgtggcccccacgcacgatgtgaccacggatcgttcgcagaggctgactctgcgctttgtaccggtagaccgtgaggatactgcctattcttacaaagttcggtatacgttagccgtaggagacaacagggtgctggacatggccagtacttactttgacatccgcggtgttcttgaccgcggtccaagctttaaaccgtataccggaacggcatacaatgccttggctccaaagggcgctccaaatgcttgccagtggacaacgaccaacgggggcaataaaacgaacacttttgcccaagcccctttaataggcacggctattgacggaaccaacggactgcagattgggcaagataatggacaagctgtttatgctgacaaaacctttcaacccgaaccacaagtgggagaatctcagtggaatactaatccaaccacaaacgcagcaggacgcgtgttaaaaacaactactcgcatgctgccttgctatggttcttttgcaaggcccaccaatgagaaagggggtcaagcttcaggagacgttaccttccaatttttcgacactgcctcggacaatggcaacaaccctaaggtggtgctatatggagaagacgtcaacattgaatcgcctgacacacacttaatctacaaacccaccgctgacaacacaaactctgaaaaccttttgggtcaacaggccgctccaaacagagccaattacattgcctttcgggacaacttcattggactaatgtactataattcaacaggaaacatgggagtgttggcagggcaggcttcccaactaaatgctgtggtagacttgcaagacagaaacactgagctttcctaccaactcatgttagatgcaataggagaccggagtcgttacttttcaatgtggaaccaagcagtggacagctatgatccagatgtgcgaattattgaaaatcatggcgttgaggacgaactgccaaattactgcttccctcttaacgctcaaggaattgctaacacctataaaggcgttaagaaaaacaacggcaattgggcgaaagacgacgcagtagtagaaactaacgaaattggcataggaaatgtttttgccatggagataaatttaactgctaacttgtggcgaaactttctgtattccaatattgctttgtacctgccagactcctacaagtattcaccgggaaacataaccttacccgaaaacaaaaacagttacaattacattaatggtcgagtaacagctcctggtctggtagacacctttgtaaacattggcgcgcgatggtctcccgaccccatggacaacgtgaatccttttaatcaccatcgcaatgctggtctgcgttatcgctccatgcttctaggcaacggccgctacgtgcccttccacattcaggtgcctcaaaaattctttgccattaagaacctgcttctgctgcctgggtcctacacctacgagtggaacttcagaaaagatgtaaacatgatcttgcagagcacgctgggcaacgacctccgtgtcgacggggccagcgtcagattcgacagcattaacctctacgctaatttcttccccatggcacataacaccgcttccaccctggaggctatgttacgcaacgacaccaacgaccagtcctttaatgactacctctgcgcggccaacatgctataccccattcctgccaatgccaccagtgtgcccatctccatcccctctcgcaactgggcagctttcagagggtggagtttcacccgcctcaaaacaaaagaaaccccctcgctgggttccggatttgatccatactttgtttactcaggctccattccctacctggatggtaccttctacctgaaccacaccttcaaaaaggtgtctattatgttcgactcttctgtgagctggcccggcaacgaccgcctgctgacccctaatgagtttgaaattaagcgctcggtggacggagaaggatacaatgtagcccagagcaacatgaccaaagactggttcttaattcaaatgctcagccactacaacattggttaccaagggttttacgtgcccgaggcttacaaagacagaatgtactccttttttagaaacttccaacctatgagtagacaggtagtggatgcagatcggtatgaacaatacaaaaaagtcaccgttgagtatcaacataataattctggttttgtgggatacatgggacccaccatgagggaagggcaggcttatccagcgaattacccttatcctcttattggagacaccgccgtgcccagcctgacccagaaaaagttcctctgtgaccgcaccatgtggagaatccccttctctagcaacttcatgtctatgggggccctcaccgacctggggcagaacatgctgtacgccaattccgctcacgccttggatatgacctttgaggtggaccccatggatgagcccacgcttctctatgttctgtttgaagtcttcgacgtggtgcgcatccaccagccgcaccgcggcgtcatcgaggccgtctacctgcgcacacctttctctgccggtaacgccaccacataagaagcaaatgggctccagcgaacaggagctgcgggccattattcgcgacctgggctgcggaccctactttttgggcaccttcgacaagcgtttccccggattcatgtccccccagaagccggcctgtgccatagtcaacacggccgggcgggagaccgggggggttcactggctcgccttcgcctggaacccgcgcaaccgcacctgctacctgttcgacccttttggtttttccgacgaaaggctgaagcaaatctaccagttcgaatacgaaggactcctcaagcgcagcgctctggcctccacgcccgaccactgcgtcaccctggaaaaatccacccaaacggtgcaggggcccctctcggccgcctgcgggcttttctgttgcatgtttttgcacgccttcgtgcactggcctcacaaccccatggagcgcaaccccaccatggatctgctcaccggagtgcccaacagcatgcttcacagcccccaggtcgcccccaccctgcgccgtaaccaggaacacctgtatcgctttctggggaaacactctgcctatttccgccgccaccggcagcgcatcgagcaggccacggcctttgaaagcatgagccaaagagtgtaatcaataaaaaccatttttatttaacatgatacgcgcttctggcgtttttattaaaaatcgaacggttcgagggaggggtcctcgtgcccgctgggaagggacacgttgcggtactggaaacgggcgctccaacgaaactcggggatcaccagccgcggcaggggcacgtcttctaggttctgcttccagaactgccgcaccagctgcagggctcccatgacgtcgggcgccgagatcttgaagtcgcagttagggccggagcccccgcggctgttgcggaacacggggttggcacactggaacaccagcacgctggggttgtaaatactggccagggccgttgggtcggtcacctccgacgcatccagatcctcggcattgctcagggcgaacggagtcagcttgcacatctgccgtccgatctggggcaccaggtcgggtttgttgaggcaatcgcagcgcagagggattaggatgcgacgctgcccgcgttgcatgatagggtaactcgccgccaggaactcctccatctgacggaaggccatctgggccttggtaccctcggtgaaaaatagcccacaggacttgctagaaaatacgttattgccgcagttgatgtcttccgcgcagcagcgtgcatcttcgttcttcagctgaaccacgttacgcccccagcggttctggaccaccttggctttcgtaggatgctccttcaacgcccgctgaccgttctcgctggtcacatccatttccaccacgtgctccttgcagaccatctccactccgtggaagcagaacaggacgccctcctgctgggtattgcgatgctcccaaacggcacatccggtgggctcccagctcttgcgtttcacccccgcgtatgcttccatgtaagccatgaggaatctgcccatcagctcggtgaaggtcttctggttggtgaaggttagcggcaggccgcggtgctcctcgttcaaccaagtttgacagattttgcggtacacggctccctggtcgggcagaaacttaaaagccgctctgctctcgttgtccacgtggaacttctccatcaacatcgtcatgacttccatgcccttctcccacgccgtcaccaacggttcggtcccggggttcttcaccaacacggcggtggaggggccctcgccggccccgacgtccttcatggtcattctttggaactccacggtgccgtccgcgcggcgtactctgcgcatcggagggtagctgaagcccacctccaccacggtgccttcgccctcgctgtcggaaacgatctccggggatggcggcggcgcgggtgtcgccttgcgagccttcttcttgggagggagcggaggcacctcctgctcgcgctcggggctcatctcccgcaagtagggggtaatggagcttccgggttggttctgacggttggccattgtatcctaggcagaaagacatggatcttatgcgcgaggaaactttaaccgccccgtcccccgtcagcgacgaagaggtcatcgtcgaacaggacccgggctacgttacgccgcccgaggatctggagtcccccttagacgaccgacgcgacgctagtgagcggcaggaaaatgagaaagaggaggaggagggctgctacctcctggaaggcgacgtcttgctaaagcatttcgccaggcagagcaccatactcaaggaggccttgcaagaccgctccgaggtgcccttggacgtcgccgcgctctcccaggcctacgaggcgaaccttttctcgccccgagtgcctccgaagagacagcccaacggcacctgcgagcccaacccgcgactcaacttctaccccgtgttcgccgtgcccgaggcgctggccacctaccacatctttttcaaaaaccagcgcattcccctttcctgccgggccaaccgcaccgcagccgataggaagctaacactcagaaacggagccagcatacctgatatcacgtcactggaggaagtgcctaagatcttcgagggtctgggtcgagatgagaagcgggcggcgaacgctctgcagaaagaacagaaagagagtcagaacgtgctggtggagctggagggggacaacgcgcgtctggccgtcctcaaacgctgcatagaagtctcccacttcgcctaccccgccctcaacttgccacccaaagttatgaaatcggtcatggatcagctgctcatcaagagagctgagcccctggatcccgaccaccccgaggcggaaaactcagaggacggaaagcccgtcgtcagcgacgaggagctcgagcggtggctggaaaccggggacccccaacagttgcaagagaggcgcaagatgatgatggcggccgtgctggtcaccgtggagctggaatgcctgcaacggtttttcagcgacgtggagacgctacgcaaaatcggggagtccctgcactacaccttccgccagggctacgtccgccaggcctgcaagatctccaacgtggagctcagcaacctggtctcctacatgggcatcctccacgagaaccggctggggcagagcgtgctgcactgcaccttgcaaggcgaggcgcggcgggactacgtccgcgactgcatctacctcttcctcaccctcacctggcagaccgccatgggcgtctggcagcagtgcttggaagagagaaacctcaaagagctagacaaactcctctgccgccagcggcgggccctctggaccggtttcagcgagcgcacggtcgcctgcgccctggcagacattatcttcccggagcgcctgatgaaaaccttgcagaacggcctgccggattttatcagtcaaagtattttgcaaaacttccgctccttcgttctggagcgctccgggatcttgcccgccatgagctgcgcgctgccttctgactttgtccccctttcctaccgcgagtgtcctccccccctgtggagccactgctacctcttccaactggccaactttctggcctaccactccgacctcatggaagacgtgagcggagaggggctgctcgagtgccactgccgctgcaacctctgcaccccccacagatcgctggcctgcaacaccgagctgctcagcgaaacccaggtcataggtaccttcgagatccaggggccccagcagcaagagggtgcttccggcttgaagctcactccggcgctgtggacctcggcttacttacgcaaatttgtagccgaggactaccacgcccacaaaattcagttctatgaagaccaatctcgaccacccaaagcccccctcacggcctgcgtcatcactcagagcaaaatcctggcccaattgcaatccatcaaccaagcgcgccgagatttccttttgaaaaagggtcggggggtgtacctagacccccagaccggcgaggaactcaacccgtccacactctccgtcgaagcagcccccccgagacatgccgcccaagggaaccgccaagcagctgatcgctcggcagagagcgaagaagcaagagctgctccagcagcagcagcaggtggaggacgaggaagagctgtgggacagccaggcagaggaggtgtcagaggacgaggaggagatggaaagctgggacagcctagacgaggaggaggacgagctttcagaggaagaggcgaccgaagaaaaaccacctgcatccagcgcgccttctctgagccgacagccgaagccccggcccccgacgcccccggccggctcactcaaagccagccgtaggtgggacgccaccggatctccagcggcagcggcaacggcagcgggtaaggccaaacgcgagcggcgggggtattgctcctggcgggcccacaaaagcagtatcgtgaactgcttgcaacactgcgggggaaacatctcctttgcccgacgctacctcctcttccatcacggtgtggccttccctcgcaacgttctctattattaccgtcatctctacagcccctacgaaacgctcggagaaaaaagctaaggcctcctctgccgcgaggaaaaactccgccgccgctgccgccgccaaggatccgccggccaccgaggagctgagaaagcgcatctttcccactctgtatgctatctttcagcaaagccgcgggcagcaccctcagcgcgaactgaaaataaaaaaccgctccttccgctcactcacccgcagctgtctgtaccacaagagagaagaccagctgcagcgcaccctggacgacgccgaagcactgttcagcaaatactgctcagcgtctcttaaagactaaaagacccgcgctttttccccctcgggcgccaaaacccacgtcattgccagcatgagcaaggagattcccaccccttacatgtggagctatcagccccagatgggcctggccgcgggggccgcccaggactactccagcaagatgaactggctcagcgccggcccccacatgatctcacgagttaacggcatccgagcccaccgaaaccagatcctcttagaacaggcggcaatcaccgccacaccccggcgccaactcaacccgcccagttggcccgccgcccaggtgtatcaggaaactccccgcccgaccacagtcctcctgccacgcgacgcggaggccgaagtcctcatgactaactctggggtacaattagcgggcgggtccaggtacgccaggtacagaggtcgggccgctccttactctcccgggagtataaagagggtgatcattcgaggccgaggtatccagctcaacgacgaggcggtgagctcctcaaccggtctcagacctgacggagtcttccagctcggaggagcgggccgctcttccttcaccactcgccaggcctacctgaccctgcagagctcttcctcgcagccgcgctccgggggaatcggcactctccagttcgtggaagagttcgtcccctccgtctacttcaacccgttttccggctcacctggacgctacccggacgccttcattcccaactttgacgcagtgagtgaatccgtggacggctacgactgatgacagatggtgcggccgtgagagctcggctgcgacatctgcatcactgccgccagcctcgctgctacgctcgggaggcgatcgtgttcagctactttgagctgccggacgagcaccctcaggggccggctcacgggttgaaactcgagatcgagaacgcgctcgagtctcgcctcatcgacgccttcaccgcccggcctctcctggtagaaaccgaacgcgggatcactaccatcaccctgttctgcatctgccccacgcccggattacatgaagatctgtgttgtcatctttgcgctcagtttaataaaaactgaactgtttgccgcaccttcaacgccatctgtgatttctacaacaaaaagttcttctggcaaaggtacacaaactgtattttattctaattctacctcatctattgtgctgaactgcgcctgcactaacgaacttatccagtggattgcaaacggtagtgtgtgcaagtacttttgggggaacgagatagttagtagaaataacagcctttgcaagcactgcaactcctccacactaatcctttatcccccatttgttactggatggtatatgtgcgttggctccggtttaaatcctagttgctttcataagtggtttctacaaaaagagacccttcccaacaattctgtttcttttttcaccctgtcctactgctgttctccctctggttactctttcaaacctctaattggtattttagctttgatactgataatctttattaactttataataattaacaacttacagtaaacatgcttgttatcctcctgctcgccacatttttcgctctctctcacgccagaacaagtattgttggcgcaggttacaatgcaactcttcaatctgcttacatgccagattccgaccagataccccatattacgtggtacttacaaacctccaaacctaattcttcattttatgaaggaaacaaactctgcgatgactccgacaacaggacgcacacatttccccacccttcactacaattcgaatgcgtaaacaaaagcttgaagctttacaacttaaagccttcagattctggcttgtatcatgctgtagttgaaaaaagtaatttagaagtccacagtgattacattgaattgatggttgtggacctgccacctccaaaatgtgaggtttcctcctcttaccttgaagttcaaggcgtggatgcctactgcctcatacacattaactgcagcaactctaaatatccagctagaatttactataatggacaggaaagtaatcttttttattatttaacaacaagcgctggtaacggtaaacagttacctgattattttactgctgttgttgaattttccacctacagagaaacgtatgccaagcggccttacaatttctcatacccgtttaacgacctttgcaatgaaatacaagcgctcgaaactggaactgattttactccaattttcattgctgccattgttgtgagcttaattaccattattgtcagcctagcattttactgcttttgcaagcccaaaaaacctaagtttgaaaaacttaaactaaaacctgtcattcaacaagtgtgattttgttttccagcatggtagctgcatttctacttctcctctgtctacccatcattttcgtctcttcaactttcgccgcagtttcccacctggaaccagagtgcctaccgccttttgacgtgtatctgattctcacctttgtttgttgtatatccatttgcagtatagcctgcttttttataacaatctttcaagccgccgactatctttacgtgcgaattgcttactttagacaccatcctgaatacagaaatcaaaacgttgcctccttactttgtttggcatgattaagctattgctaatacttaattatttacccctaatcaactgtaattgtccattcaccaaaccctggtcattctacacctgttatgataaaatccccgacactcctgttgcttggctttacgcagccaccgccgctttggtatttgtatctacttgccttggagtaaaattgtattttattctacacactgggtggctacatcccagagaagatttacctagacatcctcttgtaaacgcttttcaattacagcctctgcctcctcctgatcttcttcctcgagctccctctattgtgagctactttcaactcaccggtggagatgactgactctcaggacattaatattagtgtggaaagaatagctgctcagcgtcagcgagaaacgcgagtgttggaatacctggaactacaacagcttaaggagtcccactggtgtgagaaaggagtgctgtgtcatgttaagcaggcagccctttcctacgatgtcagcgttcagggacatgaactgtcttacactttgcctttgcagaaacaaaccttctgcaccatgatgggctctacctccatcacaatcacccaacaagccgggcctgtagagggggctatcctctgtcactgtcacgcacctgattgcatgtccaaactaatcaaaactctctgtgctttaggtgatatttttaaaatgtaaatcataataaacttaccttaaatttgacaacaattttctggtgacatcattcagcagcaccactttaccctcttcccagctctcgtatgggatgcgatagtgggtggcaaacttcctccaaaccctaaaagaaatattggtatccacttccttgtcctcacccacaattttcatcttttcatagatgaaaagaaccagagttgatgaagacttcaaccccgtctacccctatgacaccacaaccactcctgcagttccctttatatcacccccctttgtaaacagcgatggtcttcaggaaaaccccccaggtgttttaagtctgcgaatagctaaacccctatatttcgacatggagagaaaactagccctttcacttggaagagggttgacaattaccgccgccggacaattagaaagtacgcagagcgtacaaaccaacccaccgttgataattaccaacaacaacacactgaccctacgtcattctccccccttaaacctaactgacaatagcttagtgctaggctactcgagtccgctccgcgtcacagacaacaaacttacatttaacttcacatcaccactccgttatgaaaatgaaaaccttacttttaactatacagagcctcttaaacttataaataacagccttgccattgacatcaattcctcaaaaggccttagtagcgtcggaggctcactagctgtaaacctgagttcagacttaaagtttgacagcaacggatccatagcttttggcatacaaaccctgtggaccgctccgacctcgactggcaactgcaccgtctacagcgagggcgattccctacttagtctctgtttaaccaaatgcggagctcacgtcttaggaagtgtaagtttaaccggtttaacaggaaccataacccaaatgactgatatttctgtcaccattcaatttacatttgacaacaatggtaagctactaagctctccgcttataaacaacgcctttagtattcgacagaatgacagtacggcctcaaaccctacctacaacgccctggcgtttatgcctaacagtaccatatatgcaagagggggaggtggtgaaccacgaaacaactactacgtccaaacgtatcttaggggaaatgttcaaaaaccaatcattcttactgtaacctacaactcagccgccacaggatattccttatcttttaagtggactgctcttgcacgtgaaaagtttgcaaccccaacaacttcgttttgctacattacagaacaataaaaccgtgtaccccaccgtttcgtttttttcagatgaaacgggcgagagttgatgaagacttcaacccagtgtacccttatgaccccccacatgctcccgttatgcccttcattactccaccttttacctcctcggatgggttgcaggaaaaaccacttggagtgttaagtttaaactacagagatcccattactacgcaaaatgggtctcttacagttaaactaggaaacggcctcactctagacaaccagggacaactaacatcaaccgctggggaagtagaacctccactcactaacgctaacaacaaacttgcactggtctatagcgatcctttagcagtaaagcgcaacagcctaaccttatcgcacaccgctccccttgttattgctgataactctttagcattgcaagtttcagagcctatttttataaatgacaaggacaaactagccctgcaaacagccgcgccccttgtaactaacgctggcacccttcgcttacaaagcgccgcccctttaggcattgcagaccaaaccctaaaactcctgtttaccaaccctttgtacttgcagaataactttctcacgttagccattgaacgaccccttgccattaccaatagtggaaagctggctctacagctctccccaccgctacaaacagcagacacaggcttgactttgcaaaccaacgtgccattaactgtaagcaacgggaccctaggcttagccataaagcgcccacttattgttcaggacaacaacttgtttttggacttcagagctcccctgcgtcttttcaacagcgaccccgtactagggcttaacttttacacccctcttgcagtgcgcgatgaggcgctcactgttaacacaggccgcggcctcacagtgagttacgatggtttaattttaaatcttggtaaggatcttcgctttgacaacaacaccgtttctgtcgctcttagtgctgctttgcctttacaatacactgatcagcttcgccttaacgtgggcgctgggctgcgttacaatccagtgagtaaaaaattggacgtgaaccccaatcaaaacaagggtttaacctgggaaaatgactacctcattgtaaagctaggaaatggattaggttttgatggcaatggaaacatagctgtttctcctcaagttacatcgcctgacaccttatggaccactgccgatccatcccccaattgttccatctacactgatttagatgccaaaatgtggctctcgttggtaaaacaagggggtgtggttcacggttctgttgctttaaaagcattgaaaggaaccctattgagtcctacggaaagtgccattgttattatactacattttgacaattatggagtgcgaattctcaattatcccactttgggcactcaaggcacgttgggaaataatgcaacttggggttataggcagggagaatctgcagacactaatgtactcaatgcactagcatttatgcccagttcaaaaaggtacccaagagggcgtggaagcgaagttcagaatcaaactgtgggctacacttgtatacagggtgacctttctatgcccgtaccgtaccaaatacagtacaactatggaccaactggctactcctttaaatttatttggagaactgtttcaagacaaccatttgacatcccatgctgttttttctcttacattacggaagaataaaacaacttttcctttttattttctttttattttacacgcacagtaaggcttcctccacccttccatttgacagcatacaccagcctctcccccttcatggcagtaaactgctgcgagccagtccggtatttgggagttaagatccaaacagtctctttggtaatcagatgtcgatccgtgatggacacaaatccctggggcaggttctccaacgtttcggtgaaaaactgcatgccgccctacaaaacaaacaggttcaggctctccacgggttatctccccgatcaaactcagacagggtaaaggtgcgatgatgttccactaaaccacgcaggtggcgctgtctgaacctctcggtgcgactcctgtgaggctggtaagaagttagattgtccagcagcctcacagcatggatcatcagtctacgagtgcgtctggcgcagcagcgcatctgaatctcactgagattccggcaagaatcgcacaccatcacaatcaggttgttcatgatcccatagctgaacacgctccagccaaagctcattcgctccaacagcgccaccgcgtgtccgtccaaccttactttaacataaatcaggtgtctgccgcgtacaaacatgctacccgcatacagaacctcccggggcagtcccctgttcaccacctgcctgtaccagggaaacctcacatttatcagggagccatagatagccatcttaaaccaattagctaacaccgccccaccagctctacactgaagagaaccgggagagttacaatgacagtgaataatccatctctcataacccctaatggtctgatggaaatccagatctaacgtggcacagcagatacacactttcatatacattttcatcacatgtttttcccaggccgttaaaatacaatcccaatacacgggccactcctgcagtacaataaagctaatacaagatggtatactcctcacctcactaacattgtgcatgttcatattttcacattctaagtaccgagagctctcctctacaacagcactgccgcggtcctcacaaggtggtagctggtgacaattgtagggagccagtctgcagcgataccgtctgtcgcgttgcatcgtagaccagggaccgacgcacttcctcgtacttgtagtagcagaaccacgtccgctgccagcacgtctccaagtaacgccggtccctgcgtcgctcacgctccctcctcaacgcaaagtgcaaccactcttgtaatccacacagatccctctcggcctccggggcgatgcacacctcaaacctacagatgtctcggtacagttccaaacacgtagtgagggcgagttccaaccaagacagacagcctgatctatcccgacacactggaggtggaggaagacacggaagaggcatgttattccaagcgattcaccaacgggtcgaaatgaagatcccgaagatgacaacggtcgcctccggagccctgatggaatttaacagccagatcaaacattatgcgattttccaggctatcaatcgcggcctccaaaagagcctggacccgcacttccacaaacaccagcaaagcaaaagcgttattatcaaactcttcgatcatcaagctgcaggactgtacaatgcccaagtaattttcatttctccactcgcgaatgatgtcgcggcaaatagtctgaaggttcatgccgtgcatattaaaaagctccgaaagggcgccctctatagccatgcgtagacacaccatcatgactgcaagatatcgggctcctgagacacctgcagcagatttaacagacccaggtcaggttgctctccgcgatcgcgaatctccatccgcaaggtcatttgcaaataattaaatagatctgcgccgactaaatctgttaactccgcgctaggaactaaatcaggtgtggctatgcagcacaaaagttccagggatggcgccaaactcactagaaccgctcccgagtagcaaaactgatgaatgggagtaacacagtgtaaaatgttcagccaaaaatcactaagctgctcctttaaaaagtccagtacttctatattcagtccgtgcaagtactgaagcaactgtgcgggaatatgcacagcaaaaaaaatagggcggctcagatacatgttgacctaaaataaaaataaacattaaactaaagaagcttggcgaacggtgggatatatgacacgctccagcagcaggcaagcaaccggctgtccccgggaaccgcggtaaaattcatccgaatgattaaaaagaacaacagaaacttcccaccatgtactcggttggatctcctgagcacacagcaatacccccctcacattcatatccgccacagaaaaaaaacgtcccagatacccagtgggaatatccaacgacagctgcaaagacagcaaaataatccctctgggagcaagcacaaaatcctccggtgaaaaaagaacatacatattagaataaccctgttgctggggcaaaaaggcccgacgtcccagcaaatgcacatatatgtgttgatcagccattgccccgtcttaccgcgtataaagccacgaaaaagtcgagctaaaatccacccaacagcctatagctatatatacactccgcccaatgacgctaacaccgtaccacccacgaccaaagttcacccacacccacaaaacccgcgaaaatccagcgccgtcagcacttccgcaatttcagtctcacaacgtcacttccgcgcgccttttttcactattcccacacccgccctcgcgccaccccgcgtcaccccgcgtcaccgcacgtcaccccggccccgcctcgctcctccccgctcattatcatattggcacgtttccagaataaggtatattattgatgatgttaattaattcgaacccataatacccataatagctgtttgccatcgacgcgaggctggatggccttccccattatgattcttctcgcttccggcggcatcgggatgcccgcgttgcaggccatgctgtccaggcaggtagatgacgaccatcagggacagcttcaaggatcgctcgcggctcttaccagcccagcaaaaggccaggaaccgtaaaaaggccgcgttgctggcgtttttccataggctccgcccccctgacgagcatcacaaaaatcgacgctcaagtcagaggtggcgaaacccgacaggactataaagataccaggcgtttccccctggaagctccctcgtgcgctctcctgttccgaccctgccgcttaccggatacctgtccgcctttctcccttcgggaagcgtggcgctttctcatagctcacgctgtaggtatctcagttcggtgtaggtcgttcgctccaagctgggctgtgtgcacgaaccccccgttcagcccgaccgctgcgccttatccggtaactatcgtcttgagtccaacccggtaagacacgacttatcgccactggcagcagccactggtaacaggattagcagagcgaggtatgtaggcggtgctacagagttcttgaagtggtggcctaactacggctacactagaaggacagtatttggtatctgcgctctgctgaagccagttaccttcggaaaaagagttggtagctcttgatccggcaaacaaaccaccgctggtagcggtggtttttttgtttgcaagcagcagattacgcgcagaaaaaaaggatctcaagaagatcctttgatcttttctacggggtctgacgctcagtggaacgaaaactcacgttaagggattttggtcatgagattatcaaaaaggatcttcacctagatccttttaaattaaaaatgaagttttaaatcaatctaaagtatatatgagtaaacttggtctgacagttaccaatgcttaatcagtgaggcacctatctcagcgatctgtctatttcgttcatccatagttgcctgactccccgtcgtgtagataactacgatacgggagggcttaccatctggccccagtgctgcaatgataccgcgagacccacgctcaccggctccagatttatcagcaataaaccagccagccggaagggccgagcgcagaagtggtcctgcaactttatccgcctccatccagtctattaattgttgccgggaagctagagtaagtagttcgccagttaatagtttgcgcaacgttgttgccattgctgcaggcatcgtggtgtcacgctcgtcgtttggtatggcttcattcagctccggttcccaacgatcaaggcgagttacatgatcccccatgttgtgcaaaaaagcggttagctccttcggtcctccgatcgttgtcagaagtaagttggccgcagtgttatcactcatggttatggcagcactgcataattctcttactgtcatgccatccgtaagatgcttttctgtgactggtgagtactcaaccaagtcattctgagaatagtgtatgcggcgaccgagttgctcttgcccggcgtcaacacgggataataccgcgccacatagcagaactttaaaagtgctcatcattggaaaacgttcttcggggcgaaaactctcaaggatcttaccgctgttgagatccagttcgatgtaacccactcgtgcacccaactgatcttcagcatcttttactttcaccagcgtttctgggtgagcaaaaacaggaaggcaaaatgccgcaaaaaagggaataagggcgacacggaaatgttgaatactcatactcttcctttttcaatattattgaagcatttatcagggttattgtctcatgagcggatacatatttgaatgtatttagaaaaataaacaaataggggttccgcgcacatttccccgaaaagtgccacctgacgtctaagaaaccattattatcatgacattaacctataaaaataggcgtatcacgaggccctttcgtcttcaagaattggtcgatggcaaacagctattatgggtattatgggttcgaattaat

SEQ ID NO: 43 - DNA, 19593 bp, Artificial Sequence
  Synthetic oligonucleotide pBr/sAd4310A.RsrII-rITR.dE3
attaacaccgtggattccgtgatcgacagcgtggtggccagcgccagggcctatgctcgccgcaagaggcggctgcatcggaaacgtcgccccaccgccgccatgctagcagccagggccgtgctgaggcgggcccggagggtaggcaggagggctatgcgccgcgctgccgccaacgccgccgggagggcccgcagacaagccgcccgccaggccgccgctgccatcgctagcatggccagacccaggagagggaacgtgtactgggtgcgcgattctgtaacgggagtccgagtgccggtgcgcagccgacctccccgaagttagaagatccaagctgcgaagacggcggtactgagtctccctgttgttattagcccaacatgagcaagcgcaagtttaaagaagaactgctgcagacgctggtgcctgagatctatggccctccggacgtgaagcctgacattaagccccgcgatatcaagcgtgttaaaaagcgggaaaaaaaagaggaacttgcggcggtagacgatggcggtgtagaatttattaggagtttcgccccacggcgcagggttcaatggaaagggcggcgtgtacaacgcgttctgaggccgggcaccgcggtagtttttaccccgggagagcggtcggccgttaggggtttcaagcggcagtacgatgaggtgtacggcgacgaagacatactggaacaggcggctcagcagattggagaattcgcttatggcaaacgttctcggcgcgaagacctggccatcgccttggacagcggcaatcccacacccagcctcaaacccgtgacgctgcaacaggtgcttcccgtgagcgccagtactgacagcaaaagggggattaaaagagagatggaagagctgcaacccaccatccaacttatggtccctaaacgacagaggttggaagaggtcctggagaagatgaaagtggaccccagcatagagccggatgtgaaagtgaggcctattaaggaagtggcccccggtcttggggtgcaaacggtggacattcaaatccccgtcacgtccgcttcaacagcggtggaagccatggaaacgcaaacggaagcccccgccgtcacggtcggtaccagggaagtggcgttgcaaacggaaccctggtacgaatacgccacccctaggcgtcagaggcggtccgcccgttacggacccgtcaacgccatcatgcccgagtacgcgctacatccgtctatccggcccactcccggctaccggggagtgacgtatcgcccgtcaggaactcgccgccgttaccgtcgccgccgtcgctctcgccgcgctctggccccagtgtcggtgcggcgcgtgacccgccaggggaaaacagtcaccatccccaacccgcgctaccaccctagcattctttaatgactctgccgttttgcagatggctctgacttgccgcgtgcgccttcccgttctgcactatcgaggaagatctcgtcgtaggagaggcatggcgggcagtggtcgccggcgggctttgcgcaggcgcatgaaaggcggaattttacccgccctaatacctataatcgccgccgccataggcgccatacccggcgtcgcttcagtggccttgcaagcagctcgtaataaataaacgaaggcttttgcacttatgtcctggtcctgactattttatgcagaaaaagcatggaagacatcaattttacgtcgctggctccgcggcaaggctcgcggccgctcatgggcacctggaacgacatcggcaccagtcagctcaacgggggcgctttcaattgggggagcctttggagcggcattaaaaactttggctccacgattaaatcctacggcagcaaagcctggaacagtagtgctggtcaaatgctccgagataaactgaaggacaccaacttccaagagaaagtggtcaacggggtggtgaccggcatacacggcgcggtagatcttgccaaccaagcggtgcagaaagagattgacaggcgattggaaaactcgcgggtgccgccgcagagaggggatgaggtggaggtcgaggaagtagaagtagaggaaaagctgccccccttggagaaagttcccggtgcgattccaaggccgcagaagcggccaaggccagaactagaagaaactctggtgacggagagcaaggagcctccctcgtacgagcaagccttaaaagagggcgcttcaccctacccgatgaccaaaccgatcgcgcctatggctcggccggtgtacgggaaggactacaaacctgtcacgctagaacttcctccgccactcccttcgcgtcctacggtgcctcccatgccagcgccgtcggccggtcccgtgtctgcaccttccgcagcgcctctgccagccgcccgcccagtggccgtggccactgccagaaaccccagaggccagagaggagccaactggcaaaacacgctgaacagcatcgtgggcctgggagttaaaagcctgaaacgccgccgttgctattattaaaaaagtgtagctaaaaaatctcccgttgtatacgcctcctatgttaccgccagagacgtgtgactgtcgtcgcgagcagcgctttcaagatggccaccccatcgatgatgccgcagtggtcttacatgcacatcgccgggcaggacgcctcggagtatctgagccccggtcttgtgcagtttgcccgcgccaccgacacctacttcagcttgggaaacaagtttagaaatcccaccgtggcccccacgcacgatgtgaccacggatcgttcgcagaggctgactctgcgctttgtaccggtagaccgtgaggatactgcctattcttacaaagttcggtatacgttagccgtaggagacaacagggtgctggacatggccagtacttactttgacatccgcggtgttcttgaccgcggtccaagctttaaaccgtataccggaacggcatacaatgccttggctccaaagggcgctccaaatgcttgccagtggacaacgaccaacgggggcaataaaacgaacacttttgcccaagcccctttaataggcacggctattgacggaaccaacggactgcagattgggcaagataatggacaagctgtttatgctgacaaaacctttcaacccgaaccacaagtgggagaatctcagtggaatactaatccaaccacaaacgcagcaggacgcgtgttaaaaacaactactcgcatgctgccttgctatggttcttttgcaaggcccaccaatgagaaagggggtcaagcttcaggagacgttaccttccaatttttcgacactgcctcggacaatggcaacaaccctaaggtggtgctatatggagaagacgtcaacattgaatcgcctgacacacacttaatctacaaacccaccgctgacaacacaaactctgaaaaccttttgggtcaacaggccgctccaaacagagccaattacattgcctttcgggacaacttcattggactaatgtactataattcaacaggaaacatgggagtgttggcagggcaggcttcccaactaaatgctgtggtagacttgcaagacagaaacactgagctttcctaccaactcatgttagatgcaataggagaccggagtcgttacttttcaatgtggaaccaagcagtggacagctatgatccagatgtgcgaattattgaaaatcatggcgttgaggacgaactgccaaattactgcttccctcttaacgctcaaggaattgctaacacctataaaggcgttaagaaaaacaacggcaattgggcgaaagacgacgcagtagtagaaactaacgaaattggcataggaaatgtttttgccatggagataaatttaactgctaacttgtggcgaaactttctgtattccaatattgctttgtacctgccagactcctacaagtattcaccgggaaacataaccttacccgaaaacaaaaacagttacaattacattaatggtcgagtaacagctcctggtctggtagacacctttgtaaacattggcgcgcgatggtctcccgaccccatggacaacgtgaatccttttaatcaccatcgcaatgctggtctgcgttatcgctccatgcttctaggcaacggccgctacgtgcccttccacattcaggtgcctcaaaaattctttgccattaagaacctgcttctgctgcctgggtcctacacctacgagtggaacttcagaaaagatgtaaacatgatcttgcagagcacgctgggcaacgacctccgtgtcgacggggccagcgtcagattcgacagcattaacctctacgctaatttcttccccatggcacataacaccgcttccaccctggaggctatgttacgcaacgacaccaacgaccagtcctttaatgactacctctgcgcggccaacatgctataccccattcctgccaatgccaccagtgtgcccatctccatcccctctcgcaactgggcagctttcagagggtggagtttcacccgcctcaaaacaaaagaaaccccctcgctgggttccggatttgatccatactttgtttactcaggctccattccctacctggatggtaccttctacctgaaccacaccttcaaaaaggtgtctattatgttcgactcttctgtgagctggcccggcaacgaccgcctgctgacccctaatgagtttgaaattaagcgctcggtggacggagaaggatacaatgtagcccagagcaacatgaccaaagactggttcttaattcaaatgctcagccactacaacattggttaccaagggttttacgtgcccgaggcttacaaagacagaatgtactccttttttagaaacttccaacctatgagtagacaggtagtggatgcagatcggtatgaacaatacaaaaaagtcaccgttgagtatcaacataataattctggttttgtgggatacatgggacccaccatgagggaagggcaggcttatccagcgaattacccttatcctcttattggagacaccgccgtgcccagcctgacccagaaaaagttcctctgtgaccgcaccatgtggagaatccccttctctagcaacttcatgtctatgggggccctcaccgacctggggcagaacatgctgtacgccaattccgctcacgccttggatatgacctttgaggtggaccccatggatgagcccacgcttctctatgttctgtttgaagtcttcgacgtggtgcgcatccaccagccgcaccgcggcgtcatcgaggccgtctacctgcgcacacctttctctgccggtaacgccaccacataagaagcaaatgggctccagcgaacaggagctgcgggccattattcgcgacctgggctgcggaccctactttttgggcaccttcgacaagcgtttccccggattcatgtccccccagaagccggcctgtgccatagtcaacacggccgggcgggagaccgggggggttcactggctcgccttcgcctggaacccgcgcaaccgcacctgctacctgttcgacccttttggtttttccgacgaaaggctgaagcaaatctaccagttcgaatacgaaggactcctcaagcgcagcgctctggcctccacgcccgaccactgcgtcaccctggaaaaatccacccaaacggtgcaggggcccctctcggccgcctgcgggcttttctgttgcatgtttttgcacgccttcgtgcactggcctcacaaccccatggagcgcaaccccaccatggatctgctcaccggagtgcccaacagcatgcttcacagcccccaggtcgcccccaccctgcgccgtaaccaggaacacctgtatcgctttctggggaaacactctgcctatttccgccgccaccggcagcgcatcgagcaggccacggcctttgaaagcatgagccaaagagtgtaatcaataaaaaccatttttatttaacatgatacgcgcttctggcgtttttattaaaaatcgaacggttcgagggaggggtcctcgtgcccgctgggaagggacacgttgcggtactggaaacgggcgctccaacgaaactcggggatcaccagccgcggcaggggcacgtcttctaggttctgcttccagaactgccgcaccagctgcagggctcccatgacgtcgggcgccgagatcttgaagtcgcagttagggccggagcccccgcggctgttgcggaacacggggttggcacactggaacaccagcacgctggggttgtaaatactggccagggccgttgggtcggtcacctccgacgcatccagatcctcggcattgctcagggcgaacggagtcagcttgcacatctgccgtccgatctggggcaccaggtcgggtttgttgaggcaatcgcagcgcagagggattaggatgcgacgctgcccgcgttgcatgatagggtaactcgccgccaggaactcctccatctgacggaaggccatctgggccttggtaccctcggtgaaaaatagcccacaggacttgctagaaaatacgttattgccgcagttgatgtcttccgcgcagcagcgtgcatcttcgttcttcagctgaaccacgttacgcccccagcggttctggaccaccttggctttcgtaggatgctccttcaacgcccgctgaccgttctcgctggtcacatccatttccaccacgtgctccttgcagaccatctccactccgtggaagcagaacaggacgccctcctgctgggtattgcgatgctcccaaacggcacatccggtgggctcccagctcttgcgtttcacccccgcgtatgcttccatgtaagccatgaggaatctgcccatcagctcggtgaaggtcttctggttggtgaaggttagcggcaggccgcggtgctcctcgttcaaccaagtttgacagattttgcggtacacggctccctggtcgggcagaaacttaaaagccgctctgctctcgttgtccacgtggaacttctccatcaacatcgtcatgacttccatgcccttctcccacgccgtcaccaacggttcggtcccggggttcttcaccaacacggcggtggaggggccctcgccggccccgacgtccttcatggtcattctttggaactccacggtgccgtccgcgcggcgtactctgcgcatcggagggtagctgaagcccacctccaccacggtgccttcgccctcgctgtcggaaacgatctccggggatggcggcggcgcgggtgtcgccttgcgagccttcttcttgggagggagcggaggcacctcctgctcgcgctcggggctcatctcccgcaagtagggggtaatggagcttccgggttggttctgacggttggccattgtatcctaggcagaaagacatggatcttatgcgcgaggaaactttaaccgccccgtcccccgtcagcgacgaagaggtcatcgtcgaacaggacccgggctacgttacgccgcccgaggatctggagtcccccttagacgaccgacgcgacgctagtgagcggcaggaaaatgagaaagaggaggaggagggctgctacctcctggaaggcgacgtcttgctaaagcatttcgccaggcagagcaccatactcaaggaggccttgcaagaccgctccgaggtgcccttggacgtcgccgcgctctcccaggcctacgaggcgaaccttttctcgccccgagtgcctccgaagagacagcccaacggcacctgcgagcccaacccgcgactcaacttctaccccgtgttcgccgtgcccgaggcgctggccacctaccacatctttttcaaaaaccagcgcattcccctttcctgccgggccaaccgcaccgcagccgataggaagctaacactcagaaacggagccagcatacctgatatcacgtcactggaggaagtgcctaagatcttcgagggtctgggtcgagatgagaagcgggcggcgaacgctctgcagaaagaacagaaagagagtcagaacgtgctggtggagctggagggggacaacgcgcgtctggccgtcctcaaacgctgcatagaagtctcccacttcgcctaccccgccctcaacttgccacccaaagttatgaaatcggtcatggatcagctgctcatcaagagagctgagcccctggatcccgaccaccccgaggcggaaaactcagaggacggaaagcccgtcgtcagcgacgaggagctcgagcggtggctggaaaccggggacccccaacagttgcaagagaggcgcaagatgatgatggcggccgtgctggtcaccgtggagctggaatgcctgcaacggtttttcagcgacgtggagacgctacgcaaaatcggggagtccctgcactacaccttccgccagggctacgtccgccaggcctgcaagatctccaacgtggagctcagcaacctggtctcctacatgggcatcctccacgagaaccggctggggcagagcgtgctgcactgcaccttgcaaggcgaggcgcggcgggactacgtccgcgactgcatctacctcttcctcaccctcacctggcagaccgccatgggcgtctggcagcagtgcttggaagagagaaacctcaaagagctagacaaactcctctgccgccagcggcgggccctctggaccggtttcagcgagcgcacggtcgcctgcgccctggcagacattatcttcccggagcgcctgatgaaaaccttgcagaacggcctgccggattttatcagtcaaagtattttgcaaaacttccgctccttcgttctggagcgctccgggatcttgcccgccatgagctgcgcgctgccttctgactttgtccccctttcctaccgcgagtgtcctccccccctgtggagccactgctacctcttccaactggccaactttctggcctaccactccgacctcatggaagacgtgagcggagaggggctgctcgagtgccactgccgctgcaacctctgcaccccccacagatcgctggcctgcaacaccgagctgctcagcgaaacccaggtcataggtaccttcgagatccaggggccccagcagcaagagggtgcttccggcttgaagctcactccggcgctgtggacctcggcttacttacgcaaatttgtagccgaggactaccacgcccacaaaattcagttctatgaagaccaatctcgaccacccaaagcccccctcacggcctgcgtcatcactcagagcaaaatcctggcccaattgcaatccatcaaccaagcgcgccgagatttccttttgaaaaagggtcggggggtgtacctagacccccagaccggcgaggaactcaacccgtccacactctccgtcgaagcagcccccccgagacatgccgcccaagggaaccgccaagcagctgatcgctcggcagagagcgaagaagcaagagctgctccagcagcagcagcaggtggaggacgaggaagagctgtgggacagccaggcagaggaggtgtcagaggacgaggaggagatggaaagctgggacagcctagacgaggaggaggacgagctttcagaggaagaggcgaccgaagaaaaaccacctgcatccagcgcgccttctctgagccgacagccgaagccccggcccccgacgcccccggccggctcactcaaagccagccgtaggtgggacgccaccggatctccagcggcagcggcaacggcagcgggtaaggccaaacgcgagcggcgggggtattgctcctggcgggcccacaaaagcagtatcgtgaactgcttgcaacactgcgggggaaacatctcctttgcccgacgctacctcctcttccatcacggtgtggccttccctcgcaacgttctctattattaccgtcatctctacagcccctacgaaacgctcggagaaaaaagctaaggcctcctctgccgcgaggaaaaactccgccgccgctgccgccgccaaggatccgccggccaccgaggagctgagaaagcgcatctttcccactctgtatgctatctttcagcaaagccgcgggcagcaccctcagcgcgaactgaaaataaaaaaccgctccttccgctcactcacccgcagctgtctgtaccacaagagagaagaccagctgcagcgcaccctggacgacgccgaagcactgttcagcaaatactgctcagcgtctcttaaagactaaaagacccgcgctttttccccctcgggcgccaaaacccacgtcattgccagcatgagcaaggagattcccaccccttacatgtggagctatcagccccagatgggcctggccgcgggggccgcccaggactactccagcaagatgaactggctcagcgccggcccccacatgatctcacgagttaacggcatccgagcccaccgaaaccagatcctcttagaacaggcggcaatcaccgccacaccccggcgccaactcaacccgcccagttggcccgccgcccaggtgtatcaggaaactccccgcccgaccacagtcctcctgccacgcgacgcggaggccgaagtcctcatgactaactctggggtacaattagcgggcgggtccaggtacgccaggtacagaggtcgggccgctccttactctcccgggagtataaagagggtgatcattcgaggccgaggtatccagctcaacgacgaggcggtgagctcctcaaccggtctcagacctgacggagtcttccagctcggaggagcgggccgctcttccttcaccactcgccaggcctacctgaccctgcagagctcttcctcgcagccgcgctccgggggaatcggcactctccagttcgtggaagagttcgtcccctccgtctacttcaacccgttttccggctcacctggacgctacccggacgccttcattcccaactttgacgcagtgagtgaatccgtggacggctacgactgatgacagatggtgcggccgtgagagctcggctgcgacatctgcatcactgccgccagcctcgctgctacgctcgggaggcgatcgtgttcagctactttgagctgccggacgagcaccctcaggggccggctcacgggttgaaactcgagatcgagaacgcgctcgagtctcgcctcatcgacgccttcaccgcccggcctctcctggtagaaaccgaacgcgggatcactaccatcaccctgttctgcatctgccccacgcccggattacatgaagatctgtgttgtcatctttgcgctcagtttaataaaaactgaactgtttgccgcaccttcaacgccatctgtgatttctacaacaaaaagttcttctggcaaaggtacacaaactgtattttattctaattctacctcatctattgtgctgaactgcgcctgcactaacgaacttatcctgtagagggggctatcctctgtcactgtcacgcacctgattgcatgtccaaactaatcaaaactctctgtgctttaggtgatatttttaaaatgtaaatcataataaacttaccttaaatttgacaacaattttctggtgacatcattcagcagcaccactttaccctcttcccagctctcgtatgggatgcgatagtgggtggcaaacttcctccaaaccctaaaagaaatattggtatccacttccttgtcctcacccacaattttcatcttttcatagatgaaaagaaccagagttgatgaagacttcaaccccgtctacccctatgacaccacaaccactcctgcagttccctttatatcacccccctttgtaaacagcgatggtcttcaggaaaaccccccaggtgttttaagtctgcgaatagctaaacccctatatttcgacatggagagaaaactagccctttcacttggaagagggttgacaattaccgccgccggacaattagaaagtacgcagagcgtacaaaccaacccaccgttgataattaccaacaacaacacactgaccctacgtcattctccccccttaaacctaactgacaatagcttagtgctaggctactcgagtccgctccgcgtcacagacaacaaacttacatttaacttcacatcaccactccgttatgaaaatgaaaaccttacttttaactatacagagcctcttaaacttataaataacagccttgccattgacatcaattcctcaaaaggccttagtagcgtcggaggctcactagctgtaaacctgagttcagacttaaagtttgacagcaacggatccatagcttttggcatacaaaccctgtggaccgctccgacctcgactggcaactgcaccgtctacagcgagggcgattccctacttagtctctgtttaaccaaatgcggagctcacgtcttaggaagtgtaagtttaaccggtttaacaggaaccataacccaaatgactgatatttctgtcaccattcaatttacatttgacaacaatggtaagctactaagctctccgcttataaacaacgcctttagtattcgacagaatgacagtacggcctcaaaccctacctacaacgccctggcgtttatgcctaacagtaccatatatgcaagagggggaggtggtgaaccacgaaacaactactacgtccaaacgtatcttaggggaaatgttcaaaaaccaatcattcttactgtaacctacaactcagccgccacaggatattccttatcttttaagtggactgctcttgcacgtgaaaagtttgcaaccccaacaacttcgttttgctacattacagaacaataaaaccgtgtaccccaccgtttcgtttttttcagatgaaacgggcgagagttgatgaagacttcaacccagtgtacccttatgaccccccacatgctcccgttatgcccttcattactccaccttttacctcctcggatgggttgcaggaaaaaccacttggagtgttaagtttaaactacagagatcccattactacgcaaaatgggtctcttacagttaaactaggaaacggcctcactctagacaaccagggacaactaacatcaaccgctggggaagtagaacctccactcactaacgctaacaacaaacttgcactggtctatagcgatcctttagcagtaaagcgcaacagcctaaccttatcgcacaccgctccccttgttattgctgataactctttagcattgcaagtttcagagcctatttttataaatgacaaggacaaactagccctgcaaacagccgcgccccttgtaactaacgctggcacccttcgcttacaaagcgccgcccctttaggcattgcagaccaaaccctaaaactcctgtttaccaaccctttgtacttgcagaataactttctcacgttagccattgaacgaccccttgccattaccaatagtggaaagctggctctacagctctccccaccgctacaaacagcagacacaggcttgactttgcaaaccaacgtgccattaactgtaagcaacgggaccctaggcttagccataaagcgcccacttattgttcaggacaacaacttgtttttggacttcagagctcccctgcgtcttttcaacagcgaccccgtactagggcttaacttttacacccctcttgcagtgcgcgatgaggcgctcactgttaacacaggccgcggcctcacagtgagttacgatggtttaattttaaatcttggtaaggatcttcgctttgacaacaacaccgtttctgtcgctcttagtgctgctttgcctttacaatacactgatcagcttcgccttaacgtgggcgctgggctgcgttacaatccagtgagtaaaaaattggacgtgaaccccaatcaaaacaagggtttaacctgggaaaatgactacctcattgtaaagctaggaaatggattaggttttgatggcaatggaaacatagctgtttctcctcaagttacatcgcctgacaccttatggaccactgccgatccatcccccaattgttccatctacactgatttagatgccaaaatgtggctctcgttggtaaaacaagggggtgtggttcacggttctgttgctttaaaagcattgaaaggaaccctattgagtcctacggaaagtgccattgttattatactacattttgacaattatggagtgcgaattctcaattatcccactttgggcactcaaggcacgttgggaaataatgcaacttggggttataggcagggagaatctgcagacactaatgtactcaatgcactagcatttatgcccagttcaaaaaggtacccaagagggcgtggaagcgaagttcagaatcaaactgtgggctacacttgtatacagggtgacctttctatgcccgtaccgtaccaaatacagtacaactatggaccaactggctactcctttaaatttatttggagaactgtttcaagacaaccatttgacatcccatgctgttttttctcttacattacggaagaataaaacaacttttcctttttattttctttttattttacacgcacagtaaggcttcctccacccttccatttgacagcatacaccagcctctcccccttcatggcagtaaactgctgcgagccagtccggtatttgggagttaagatccaaacagtctctttggtaatcagatgtcgatccgtgatggacacaaatccctggggcaggttctccaacgtttcggtgaaaaactgcatgccgccctacaaaacaaacaggttcaggctctccacgggttatctccccgatcaaactcagacagggtaaaggtgcgatgatgttccactaaaccacgcaggtggcgctgtctgaacctctcggtgcgactcctgtgaggctggtaagaagttagattgtccagcagcctcacagcatggatcatcagtctacgagtgcgtctggcgcagcagcgcatctgaatctcactgagattccggcaagaatcgcacaccatcacaatcaggttgttcatgatcccatagctgaacacgctccagccaaagctcattcgctccaacagcgccaccgcgtgtccgtccaaccttactttaacataaatcaggtgtctgccgcgtacaaacatgctacccgcatacagaacctcccggggcagtcccctgttcaccacctgcctgtaccagggaaacctcacatttatcagggagccatagatagccatcttaaaccaattagctaacaccgccccaccagctctacactgaagagaaccgggagagttacaatgacagtgaataatccatctctcataacccctaatggtctgatggaaatccagatctaacgtggcacagcagatacacactttcatatacattttcatcacatgtttttcccaggccgttaaaatacaatcccaatacacgggccactcctgcagtacaataaagctaatacaagatggtatactcctcacctcactaacattgtgcatgttcatattttcacattctaagtaccgagagctctcctctacaacagcactgccgcggtcctcacaaggtggtagctggtgacaattgtagggagccagtctgcagcgataccgtctgtcgcgttgcatcgtagaccagggaccgacgcacttcctcgtacttgtagtagcagaaccacgtccgctgccagcacgtctccaagtaacgccggtccctgcgtcgctcacgctccctcctcaacgcaaagtgcaaccactcttgtaatccacacagatccctctcggcctccggggcgatgcacacctcaaacctacagatgtctcggtacagttccaaacacgtagtgagggcgagttccaaccaagacagacagcctgatctatcccgacacactggaggtggaggaagacacggaagaggcatgttattccaagcgattcaccaacgggtcgaaatgaagatcccgaagatgacaacggtcgcctccggagccctgatggaatttaacagccagatcaaacattatgcgattttccaggctatcaatcgcggcctccaaaagagcctggacccgcacttccacaaacaccagcaaagcaaaagcgttattatcaaactcttcgatcatcaagctgcaggactgtacaatgcccaagtaattttcatttctccactcgcgaatgatgtcgcggcaaatagtctgaaggttcatgccgtgcatattaaaaagctccgaaagggcgccctctatagccatgcgtagacacaccatcatgactgcaagatatcgggctcctgagacacctgcagcagatttaacagacccaggtcaggttgctctccgcgatcgcgaatctccatccgcaaggtcatttgcaaataattaaatagatctgcgccgactaaatctgttaactccgcgctaggaactaaatcaggtgtggctatgcagcacaaaagttccagggatggcgccaaactcactagaaccgctcccgagtagcaaaactgatgaatgggagtaacacagtgtaaaatgttcagccaaaaatcactaagctgctcctttaaaaagtccagtacttctatattcagtccgtgcaagtactgaagcaactgtgcgggaatatgcacagcaaaaaaaatagggcggctcagatacatgttgacctaaaataaaaataaacattaaactaaagaagcttggcgaacggtgggatatatgacacgctccagcagcaggcaagcaaccggctgtccccgggaaccgcggtaaaattcatccgaatgattaaaaagaacaacagaaacttcccaccatgtactcggttggatctcctgagcacacagcaatacccccctcacattcatatccgccacagaaaaaaaacgtcccagatacccagtgggaatatccaacgacagctgcaaagacagcaaaataatccctctgggagcaagcacaaaatcctccggtgaaaaaagaacatacatattagaataaccctgttgctggggcaaaaaggcccgacgtcccagcaaatgcacatatatgtgttgatcagccattgccccgtcttaccgcgtataaagccacgaaaaagtcgagctaaaatccacccaacagcctatagctatatatacactccgcccaatgacgctaacaccgtaccacccacgaccaaagttcacccacacccacaaaacccgcgaaaatccagcgccgtcagcacttccgcaatttcagtctcacaacgtcacttccgcgcgccttttttcactattcccacacccgccctcgcgccaccccgcgtcaccccgcgtcaccgcacgtcaccccggccccgcctcgctcctccccgctcattatcatattggcacgtttccagaataaggtatattattgatgatgttaattaattcgaacccataatacccataatagctgtttgccatcgacgcgaggctggatggccttccccattatgattcttctcgcttccggcggcatcgggatgcccgcgttgcaggccatgctgtccaggcaggtagatgacgaccatcagggacagcttcaaggatcgctcgcggctcttaccagcccagcaaaaggccaggaaccgtaaaaaggccgcgttgctggcgtttttccataggctccgcccccctgacgagcatcacaaaaatcgacgctcaagtcagaggtggcgaaacccgacaggactataaagataccaggcgtttccccctggaagctccctcgtgcgctctcctgttccgaccctgccgcttaccggatacctgtccgcctttctcccttcgggaagcgtggcgctttctcatagctcacgctgtaggtatctcagttcggtgtaggtcgttcgctccaagctgggctgtgtgcacgaaccccccgttcagcccgaccgctgcgccttatccggtaactatcgtcttgagtccaacccggtaagacacgacttatcgccactggcagcagccactggtaacaggattagcagagcgaggtatgtaggcggtgctacagagttcttgaagtggtggcctaactacggctacactagaaggacagtatttggtatctgcgctctgctgaagccagttaccttcggaaaaagagttggtagctcttgatccggcaaacaaaccaccgctggtagcggtggtttttttgtttgcaagcagcagattacgcgcagaaaaaaaggatctcaagaagatcctttgatcttttctacggggtctgacgctcagtggaacgaaaactcacgttaagggattttggtcatgagattatcaaaaaggatcttcacctagatccttttaaattaaaaatgaagttttaaatcaatctaaagtatatatgagtaaacttggtctgacagttaccaatgcttaatcagtgaggcacctatctcagcgatctgtctatttcgttcatccatagttgcctgactccccgtcgtgtagataactacgatacgggagggcttaccatctggccccagtgctgcaatgataccgcgagacccacgctcaccggctccagatttatcagcaataaaccagccagccggaagggccgagcgcagaagtggtcctgcaactttatccgcctccatccagtctattaattgttgccgggaagctagagtaagtagttcgccagttaatagtttgcgcaacgttgttgccattgctgcaggcatcgtggtgtcacgctcgtcgtttggtatggcttcattcagctccggttcccaacgatcaaggcgagttacatgatcccccatgttgtgcaaaaaagcggttagctccttcggtcctccgatcgttgtcagaagtaagttggccgcagtgttatcactcatggttatggcagcactgcataattctcttactgtcatgccatccgtaagatgcttttctgtgactggtgagtactcaaccaagtcattctgagaatagtgtatgcggcgaccgagttgctcttgcccggcgtcaacacgggataataccgcgccacatagcagaactttaaaagtgctcatcattggaaaacgttcttcggggcgaaaactctcaaggatcttaccgctgttgagatccagttcgatgtaacccactcgtgcacccaactgatcttcagcatcttttactttcaccagcgtttctgggtgagcaaaaacaggaaggcaaaatgccgcaaaaaagggaataagggcgacacggaaatgttgaatactcatactcttcctttttcaatattattgaagcatttatcagggttattgtctcatgagcggatacatatttgaatgtatttagaaaaataaacaaataggggttccgcgcacatttccccgaaaagtgccacctgacgtctaagaaaccattattatcatgacattaacctataaaaataggcgtatcacgaggccctttcgtcttcaagaattggtcgatggcaaacagctattatgggtattatgggttcgaattaat

SEQ ID NO: 44 - DNA, 18199 bp, Artificial Sequence
  Synthetic oligonucleotide pBr/sAd4310A.RsrII-rITR.dE3.dE4
attaacaccgtggattccgtgatcgacagcgtggtggccagcgccagggcctatgctcgccgcaagaggcggctgcatcggaaacgtcgccccaccgccgccatgctagcagccagggccgtgctgaggcgggcccggagggtaggcaggagggctatgcgccgcgctgccgccaacgccgccgggagggcccgcagacaagccgcccgccaggccgccgctgccatcgctagcatggccagacccaggagagggaacgtgtactgggtgcgcgattctgtaacgggagtccgagtgccggtgcgcagccgacctccccgaagttagaagatccaagctgcgaagacggcggtactgagtctccctgttgttattagcccaacatgagcaagcgcaagtttaaagaagaactgctgcagacgctggtgcctgagatctatggccctccggacgtgaagcctgacattaagccccgcgatatcaagcgtgttaaaaagcgggaaaaaaaagaggaacttgcggcggtagacgatggcggtgtagaatttattaggagtttcgccccacggcgcagggttcaatggaaagggcggcgtgtacaacgcgttctgaggccgggcaccgcggtagtttttaccccgggagagcggtcggccgttaggggtttcaagcggcagtacgatgaggtgtacggcgacgaagacatactggaacaggcggctcagcagattggagaattcgcttatggcaaacgttctcggcgcgaagacctggccatcgccttggacagcggcaatcccacacccagcctcaaacccgtgacgctgcaacaggtgcttcccgtgagcgccagtactgacagcaaaagggggattaaaagagagatggaagagctgcaacccaccatccaacttatggtccctaaacgacagaggttggaagaggtcctggagaagatgaaagtggaccccagcatagagccggatgtgaaagtgaggcctattaaggaagtggcccccggtcttggggtgcaaacggtggacattcaaatccccgtcacgtccgcttcaacagcggtggaagccatggaaacgcaaacggaagcccccgccgtcacggtcggtaccagggaagtggcgttgcaaacggaaccctggtacgaatacgccacccctaggcgtcagaggcggtccgcccgttacggacccgtcaacgccatcatgcccgagtacgcgctacatccgtctatccggcccactcccggctaccggggagtgacgtatcgcccgtcaggaactcgccgccgttaccgtcgccgccgtcgctctcgccgcgctctggccccagtgtcggtgcggcgcgtgacccgccaggggaaaacagtcaccatccccaacccgcgctaccaccctagcattctttaatgactctgccgttttgcagatggctctgacttgccgcgtgcgccttcccgttctgcactatcgaggaagatctcgtcgtaggagaggcatggcgggcagtggtcgccggcgggctttgcgcaggcgcatgaaaggcggaattttacccgccctaatacctataatcgccgccgccataggcgccatacccggcgtcgcttcagtggccttgcaagcagctcgtaataaataaacgaaggcttttgcacttatgtcctggtcctgactattttatgcagaaaaagcatggaagacatcaattttacgtcgctggctccgcggcaaggctcgcggccgctcatgggcacctggaacgacatcggcaccagtcagctcaacgggggcgctttcaattgggggagcctttggagcggcattaaaaactttggctccacgattaaatcctacggcagcaaagcctggaacagtagtgctggtcaaatgctccgagataaactgaaggacaccaacttccaagagaaagtggtcaacggggtggtgaccggcatacacggcgcggtagatcttgccaaccaagcggtgcagaaagagattgacaggcgattggaaaactcgcgggtgccgccgcagagaggggatgaggtggaggtcgaggaagtagaagtagaggaaaagctgccccccttggagaaagttcccggtgcgattccaaggccgcagaagcggccaaggccagaactagaagaaactctggtgacggagagcaaggagcctccctcgtacgagcaagccttaaaagagggcgcttcaccctacccgatgaccaaaccgatcgcgcctatggctcggccggtgtacgggaaggactacaaacctgtcacgctagaacttcctccgccactcccttcgcgtcctacggtgcctcccatgccagcgccgtcggccggtcccgtgtctgcaccttccgcagcgcctctgccagccgcccgcccagtggccgtggccactgccagaaaccccagaggccagagaggagccaactggcaaaacacgctgaacagcatcgtgggcctgggagttaaaagcctgaaacgccgccgttgctattattaaaaaagtgtagctaaaaaatctcccgttgtatacgcctcctatgttaccgccagagacgtgtgactgtcgtcgcgagcagcgctttcaagatggccaccccatcgatgatgccgcagtggtcttacatgcacatcgccgggcaggacgcctcggagtatctgagccccggtcttgtgcagtttgcccgcgccaccgacacctacttcagcttgggaaacaagtttagaaatcccaccgtggcccccacgcacgatgtgaccacggatcgttcgcagaggctgactctgcgctttgtaccggtagaccgtgaggatactgcctattcttacaaagttcggtatacgttagccgtaggagacaacagggtgctggacatggccagtacttactttgacatccgcggtgttcttgaccgcggtccaagctttaaaccgtataccggaacggcatacaatgccttggctccaaagggcgctccaaatgcttgccagtggacaacgaccaacgggggcaataaaacgaacacttttgcccaagcccctttaataggcacggctattgacggaaccaacggactgcagattgggcaagataatggacaagctgtttatgctgacaaaacctttcaacccgaaccacaagtgggagaatctcagtggaatactaatccaaccacaaacgcagcaggacgcgtgttaaaaacaactactcgcatgctgccttgctatggttcttttgcaaggcccaccaatgagaaagggggtcaagcttcaggagacgttaccttccaatttttcgacactgcctcggacaatggcaacaaccctaaggtggtgctatatggagaagacgtcaacattgaatcgcctgacacacacttaatctacaaacccaccgctgacaacacaaactctgaaaaccttttgggtcaacaggccgctccaaacagagccaattacattgcctttcgggacaacttcattggactaatgtactataattcaacaggaaacatgggagtgttggcagggcaggcttcccaactaaatgctgtggtagacttgcaagacagaaacactgagctttcctaccaactcatgttagatgcaataggagaccggagtcgttacttttcaatgtggaaccaagcagtggacagctatgatccagatgtgcgaattattgaaaatcatggcgttgaggacgaactgccaaattactgcttccctcttaacgctcaaggaattgctaacacctataaaggcgttaagaaaaacaacggcaattgggcgaaagacgacgcagtagtagaaactaacgaaattggcataggaaatgtttttgccatggagataaatttaactgctaacttgtggcgaaactttctgtattccaatattgctttgtacctgccagactcctacaagtattcaccgggaaacataaccttacccgaaaacaaaaacagttacaattacattaatggtcgagtaacagctcctggtctggtagacacctttgtaaacattggcgcgcgatggtctcccgaccccatggacaacgtgaatccttttaatcaccatcgcaatgctggtctgcgttatcgctccatgcttctaggcaacggccgctacgtgcccttccacattcaggtgcctcaaaaattctttgccattaagaacctgcttctgctgcctgggtcctacacctacgagtggaacttcagaaaagatgtaaacatgatcttgcagagcacgctgggcaacgacctccgtgtcgacggggccagcgtcagattcgacagcattaacctctacgctaatttcttccccatggcacataacaccgcttccaccctggaggctatgttacgcaacgacaccaacgaccagtcctttaatgactacctctgcgcggccaacatgctataccccattcctgccaatgccaccagtgtgcccatctccatcccctctcgcaactgggcagctttcagagggtggagtttcacccgcctcaaaacaaaagaaaccccctcgctgggttccggatttgatccatactttgtttactcaggctccattccctacctggatggtaccttctacctgaaccacaccttcaaaaaggtgtctattatgttcgactcttctgtgagctggcccggcaacgaccgcctgctgacccctaatgagtttgaaattaagcgctcggtggacggagaaggatacaatgtagcccagagcaacatgaccaaagactggttcttaattcaaatgctcagccactacaacattggttaccaagggttttacgtgcccgaggcttacaaagacagaatgtactccttttttagaaacttccaacctatgagtagacaggtagtggatgcagatcggtatgaacaatacaaaaaagtcaccgttgagtatcaacataataattctggttttgtgggatacatgggacccaccatgagggaagggcaggcttatccagcgaattacccttatcctcttattggagacaccgccgtgcccagcctgacccagaaaaagttcctctgtgaccgcaccatgtggagaatccccttctctagcaacttcatgtctatgggggccctcaccgacctggggcagaacatgctgtacgccaattccgctcacgccttggatatgacctttgaggtggaccccatggatgagcccacgcttctctatgttctgtttgaagtcttcgacgtggtgcgcatccaccagccgcaccgcggcgtcatcgaggccgtctacctgcgcacacctttctctgccggtaacgccaccacataagaagcaaatgggctccagcgaacaggagctgcgggccattattcgcgacctgggctgcggaccctactttttgggcaccttcgacaagcgtttccccggattcatgtccccccagaagccggcctgtgccatagtcaacacggccgggcgggagaccgggggggttcactggctcgccttcgcctggaacccgcgcaaccgcacctgctacctgttcgacccttttggtttttccgacgaaaggctgaagcaaatctaccagttcgaatacgaaggactcctcaagcgcagcgctctggcctccacgcccgaccactgcgtcaccctggaaaaatccacccaaacggtgcaggggcccctctcggccgcctgcgggcttttctgttgcatgtttttgcacgccttcgtgcactggcctcacaaccccatggagcgcaaccccaccatggatctgctcaccggagtgcccaacagcatgcttcacagcccccaggtcgcccccaccctgcgccgtaaccaggaacacctgtatcgctttctggggaaacactctgcctatttccgccgccaccggcagcgcatcgagcaggccacggcctttgaaagcatgagccaaagagtgtaatcaataaaaaccatttttatttaacatgatacgcgcttctggcgtttttattaaaaatcgaacggttcgagggaggggtcctcgtgcccgctgggaagggacacgttgcggtactggaaacgggcgctccaacgaaactcggggatcaccagccgcggcaggggcacgtcttctaggttctgcttccagaactgccgcaccagctgcagggctcccatgacgtcgggcgccgagatcttgaagtcgcagttagggccggagcccccgcggctgttgcggaacacggggttggcacactggaacaccagcacgctggggttgtaaatactggccagggccgttgggtcggtcacctccgacgcatccagatcctcggcattgctcagggcgaacggagtcagcttgcacatctgccgtccgatctggggcaccaggtcgggtttgttgaggcaatcgcagcgcagagggattaggatgcgacgctgcccgcgttgcatgatagggtaactcgccgccaggaactcctccatctgacggaaggccatctgggccttggtaccctcggtgaaaaatagcccacaggacttgctagaaaatacgttattgccgcagttgatgtcttccgcgcagcagcgtgcatcttcgttcttcagctgaaccacgttacgcccccagcggttctggaccaccttggctttcgtaggatgctccttcaacgcccgctgaccgttctcgctggtcacatccatttccaccacgtgctccttgcagaccatctccactccgtggaagcagaacaggacgccctcctgctgggtattgcgatgctcccaaacggcacatccggtgggctcccagctcttgcgtttcacccccgcgtatgcttccatgtaagccatgaggaatctgcccatcagctcggtgaaggtcttctggttggtgaaggttagcggcaggccgcggtgctcctcgttcaaccaagtttgacagattttgcggtacacggctccctggtcgggcagaaacttaaaagccgctctgctctcgttgtccacgtggaacttctccatcaacatcgtcatgacttccatgcccttctcccacgccgtcaccaacggttcggtcccggggttcttcaccaacacggcggtggaggggccctcgccggccccgacgtccttcatggtcattctttggaactccacggtgccgtccgcgcggcgtactctgcgcatcggagggtagctgaagcccacctccaccacggtgccttcgccctcgctgtcggaaacgatctccggggatggcggcggcgcgggtgtcgccttgcgagccttcttcttgggagggagcggaggcacctcctgctcgcgctcggggctcatctcccgcaagtagggggtaatggagcttccgggttggttctgacggttggccattgtatcctaggcagaaagacatggatcttatgcgcgaggaaactttaaccgccccgtcccccgtcagcgacgaagaggtcatcgtcgaacaggacccgggctacgttacgccgcccgaggatctggagtcccccttagacgaccgacgcgacgctagtgagcggcaggaaaatgagaaagaggaggaggagggctgctacctcctggaaggcgacgtcttgctaaagcatttcgccaggcagagcaccatactcaaggaggccttgcaagaccgctccgaggtgcccttggacgtcgccgcgctctcccaggcctacgaggcgaaccttttctcgccccgagtgcctccgaagagacagcccaacggcacctgcgagcccaacccgcgactcaacttctaccccgtgttcgccgtgcccgaggcgctggccacctaccacatctttttcaaaaaccagcgcattcccctttcctgccgggccaaccgcaccgcagccgataggaagctaacactcagaaacggagccagcatacctgatatcacgtcactggaggaagtgcctaagatcttcgagggtctgggtcgagatgagaagcgggcggcgaacgctctgcagaaagaacagaaagagagtcagaacgtgctggtggagctggagggggacaacgcgcgtctggccgtcctcaaacgctgcatagaagtctcccacttcgcctaccccgccctcaacttgccacccaaagttatgaaatcggtcatggatcagctgctcatcaagagagctgagcccctggatcccgaccaccccgaggcggaaaactcagaggacggaaagcccgtcgtcagcgacgaggagctcgagcggtggctggaaaccggggacccccaacagttgcaagagaggcgcaagatgatgatggcggccgtgctggtcaccgtggagctggaatgcctgcaacggtttttcagcgacgtggagacgctacgcaaaatcggggagtccctgcactacaccttccgccagggctacgtccgccaggcctgcaagatctccaacgtggagctcagcaacctggtctcctacatgggcatcctccacgagaaccggctggggcagagcgtgctgcactgcaccttgcaaggcgaggcgcggcgggactacgtccgcgactgcatctacctcttcctcaccctcacctggcagaccgccatgggcgtctggcagcagtgcttggaagagagaaacctcaaagagctagacaaactcctctgccgccagcggcgggccctctggaccggtttcagcgagcgcacggtcgcctgcgccctggcagacattatcttcccggagcgcctgatgaaaaccttgcagaacggcctgccggattttatcagtcaaagtattttgcaaaacttccgctccttcgttctggagcgctccgggatcttgcccgccatgagctgcgcgctgccttctgactttgtccccctttcctaccgcgagtgtcctccccccctgtggagccactgctacctcttccaactggccaactttctggcctaccactccgacctcatggaagacgtgagcggagaggggctgctcgagtgccactgccgctgcaacctctgcaccccccacagatcgctggcctgcaacaccgagctgctcagcgaaacccaggtcataggtaccttcgagatccaggggccccagcagcaagagggtgcttccggcttgaagctcactccggcgctgtggacctcggcttacttacgcaaatttgtagccgaggactaccacgcccacaaaattcagttctatgaagaccaatctcgaccacccaaagcccccctcacggcctgcgtcatcactcagagcaaaatcctggcccaattgcaatccatcaaccaagcgcgccgagatttccttttgaaaaagggtcggggggtgtacctagacccccagaccggcgaggaactcaacccgtccacactctccgtcgaagcagcccccccgagacatgccgcccaagggaaccgccaagcagctgatcgctcggcagagagcgaagaagcaagagctgctccagcagcagcagcaggtggaggacgaggaagagctgtgggacagccaggcagaggaggtgtcagaggacgaggaggagatggaaagctgggacagcctagacgaggaggaggacgagctttcagaggaagaggcgaccgaagaaaaaccacctgcatccagcgcgccttctctgagccgacagccgaagccccggcccccgacgcccccggccggctcactcaaagccagccgtaggtgggacgccaccggatctccagcggcagcggcaacggcagcgggtaaggccaaacgcgagcggcgggggtattgctcctggcgggcccacaaaagcagtatcgtgaactgcttgcaacactgcgggggaaacatctcctttgcccgacgctacctcctcttccatcacggtgtggccttccctcgcaacgttctctattattaccgtcatctctacagcccctacgaaacgctcggagaaaaaagctaaggcctcctctgccgcgaggaaaaactccgccgccgctgccgccgccaaggatccgccggccaccgaggagctgagaaagcgcatctttcccactctgtatgctatctttcagcaaagccgcgggcagcaccctcagcgcgaactgaaaataaaaaaccgctccttccgctcactcacccgcagctgtctgtaccacaagagagaagaccagctgcagcgcaccctggacgacgccgaagcactgttcagcaaatactgctcagcgtctcttaaagactaaaagacccgcgctttttccccctcgggcgccaaaacccacgtcattgccagcatgagcaaggagattcccaccccttacatgtggagctatcagccccagatgggcctggccgcgggggccgcccaggactactccagcaagatgaactggctcagcgccggcccccacatgatctcacgagttaacggcatccgagcccaccgaaaccagatcctcttagaacaggcggcaatcaccgccacaccccggcgccaactcaacccgcccagttggcccgccgcccaggtgtatcaggaaactccccgcccgaccacagtcctcctgccacgcgacgcggaggccgaagtcctcatgactaactctggggtacaattagcgggcgggtccaggtacgccaggtacagaggtcgggccgctccttactctcccgggagtataaagagggtgatcattcgaggccgaggtatccagctcaacgacgaggcggtgagctcctcaaccggtctcagacctgacggagtcttccagctcggaggagcgggccgctcttccttcaccactcgccaggcctacctgaccctgcagagctcttcctcgcagccgcgctccgggggaatcggcactctccagttcgtggaagagttcgtcccctccgtctacttcaacccgttttccggctcacctggacgctacccggacgccttcattcccaactttgacgcagtgagtgaatccgtggacggctacgactgatgacagatggtgcggccgtgagagctcggctgcgacatctgcatcactgccgccagcctcgctgctacgctcgggaggcgatcgtgttcagctactttgagctgccggacgagcaccctcaggggccggctcacgggttgaaactcgagatcgagaacgcgctcgagtctcgcctcatcgacgccttcaccgcccggcctctcctggtagaaaccgaacgcgggatcactaccatcaccctgttctgcatctgccccacgcccggattacatgaagatctgtgttgtcatctttgcgctcagtttaataaaaactgaactgtttgccgcaccttcaacgccatctgtgatttctacaacaaaaagttcttctggcaaaggtacacaaactgtattttattctaattctacctcatctattgtgctgaactgcgcctgcactaacgaacttatcctgtagagggggctatcctctgtcactgtcacgcacctgattgcatgtccaaactaatcaaaactctctgtgctttaggtgatatttttaaaatgtaaatcataataaacttaccttaaatttgacaacaattttctggtgacatcattcagcagcaccactttaccctcttcccagctctcgtatgggatgcgatagtgggtggcaaacttcctccaaaccctaaaagaaatattggtatccacttccttgtcctcacccacaattttcatcttttcatagatgaaaagaaccagagttgatgaagacttcaaccccgtctacccctatgacaccacaaccactcctgcagttccctttatatcacccccctttgtaaacagcgatggtcttcaggaaaaccccccaggtgttttaagtctgcgaatagctaaacccctatatttcgacatggagagaaaactagccctttcacttggaagagggttgacaattaccgccgccggacaattagaaagtacgcagagcgtacaaaccaacccaccgttgataattaccaacaacaacacactgaccctacgtcattctccccccttaaacctaactgacaatagcttagtgctaggctactcgagtccgctccgcgtcacagacaacaaacttacatttaacttcacatcaccactccgttatgaaaatgaaaaccttacttttaactatacagagcctcttaaacttataaataacagccttgccattgacatcaattcctcaaaaggccttagtagcgtcggaggctcactagctgtaaacctgagttcagacttaaagtttgacagcaacggatccatagcttttggcatacaaaccctgtggaccgctccgacctcgactggcaactgcaccgtctacagcgagggcgattccctacttagtctctgtttaaccaaatgcggagctcacgtcttaggaagtgtaagtttaaccggtttaacaggaaccataacccaaatgactgatatttctgtcaccattcaatttacatttgacaacaatggtaagctactaagctctccgcttataaacaacgcctttagtattcgacagaatgacagtacggcctcaaaccctacctacaacgccctggcgtttatgcctaacagtaccatatatgcaagagggggaggtggtgaaccacgaaacaactactacgtccaaacgtatcttaggggaaatgttcaaaaaccaatcattcttactgtaacctacaactcagccgccacaggatattccttatcttttaagtggactgctcttgcacgtgaaaagtttgcaaccccaacaacttcgttttgctacattacagaacaataaaaccgtgtaccccaccgtttcgtttttttcagatgaaacgggcgagagttgatgaagacttcaacccagtgtacccttatgaccccccacatgctcccgttatgcccttcattactccaccttttacctcctcggatgggttgcaggaaaaaccacttggagtgttaagtttaaactacagagatcccattactacgcaaaatgggtctcttacagttaaactaggaaacggcctcactctagacaaccagggacaactaacatcaaccgctggggaagtagaacctccactcactaacgctaacaacaaacttgcactggtctatagcgatcctttagcagtaaagcgcaacagcctaaccttatcgcacaccgctccccttgttattgctgataactctttagcattgcaagtttcagagcctatttttataaatgacaaggacaaactagccctgcaaacagccgcgccccttgtaactaacgctggcacccttcgcttacaaagcgccgcccctttaggcattgcagaccaaaccctaaaactcctgtttaccaaccctttgtacttgcagaataactttctcacgttagccattgaacgaccccttgccattaccaatagtggaaagctggctctacagctctccccaccgctacaaacagcagacacaggcttgactttgcaaaccaacgtgccattaactgtaagcaacgggaccctaggcttagccataaagcgcccacttattgttcaggacaacaacttgtttttggacttcagagctcccctgcgtcttttcaacagcgaccccgtactagggcttaacttttacacccctcttgcagtgcgcgatgaggcgctcactgttaacacaggccgcggcctcacagtgagttacgatggtttaattttaaatcttggtaaggatcttcgctttgacaacaacaccgtttctgtcgctcttagtgctgctttgcctttacaatacactgatcagcttcgccttaacgtgggcgctgggctgcgttacaatccagtgagtaaaaaattggacgtgaaccccaatcaaaacaagggtttaacctgggaaaatgactacctcattgtaaagctaggaaatggattaggttttgatggcaatggaaacatagctgtttctcctcaagttacatcgcctgacaccttatggaccactgccgatccatcccccaattgttccatctacactgatttagatgccaaaatgtggctctcgttggtaaaacaagggggtgtggttcacggttctgttgctttaaaagcattgaaaggaaccctattgagtcctacggaaagtgccattgttattatactacattttgacaattatggagtgcgaattctcaattatcccactttgggcactcaaggcacgttgggaaataatgcaacttggggttataggcagggagaatctgcagacactaatgtactcaatgcactagcatttatgcccagttcaaaaaggtacccaagagggcgtggaagcgaagttcagaatcaaactgtgggctacacttgtatacagggtgacctttctatgcccgtaccgtaccaaatacagtacaactatggaccaactggctactcctttaaatttatttggagaactgtttcaagacaaccatttgacatcccatgctgttttttctcttacattacggaagaataaaacaacttttcctttttattttctttttattttacacgcacagtaaggcttcctccacccttccatttgacagcatacaccagcctctcccccttcatggcagtaaactgctgcgagccagtccggtatttgggagttaagatccaaacagtctctttggtaatcagatgtcgatccgtgatggacacaaatccctggggcaggttctccaacgtttcggtgaaaaactgcatgccgccctacaaaacaaacaggttcaggctctccacgggttatctccccgatcaaactcagacagggtaaaggtgcgatgatgttccactaaaccacgcaggtggcgctgtctgaacctctcggtgcgactcctgtgaggctggtaagaagttagattgtccagcagcctcacagcatggatcatcagtctacgagtgcgtctggcgcagcagcgcatctgaatctcactgagattccggcaagaatcgcacaccatcacaatcaggttgttcatgatcccatagctgaacacgctccagccaaagctcattcgctccaacagcgccaccgcgtgtccgtccaaccttactttaacataaatcaggtgtctgccgcgtacaaacatgctacccgcatacagaacctcccggggcagtcccctgttcaccacctgcctgtaccagggaaacctcacatttatcagggagccatagatagccatcttaaaccaattagctaacaccgccccaccagctctacactgaagagaaccgggagagttacaatgacagtgaataatccatctctcataacccctaatggtctgatggaaatccagatctaacgtggcacagcagatacacactttcatatacattttcatcacatgtttttcccaggccgttaaaatacaatcccaatacacgggccactcctgcagtacaataaagctaatacaagatggtatactcctcacctcactaacattgtgcatgttcatattttcacattctaagtaccgagagctctcctctacaacagcactgccgcggtcctcacaaggtggtagctggtgacaattgtagggagccagtctgcagcgataccgtctgtcgcgttgcatcgtagaccagggaccgacgcacttcctcgtacttgtagtagcagaactgccccgtcttaccgcgtataaagccacgaaaaagtcgagctaaaatccacccaacagcctatagctatatatacactccgcccaatgacgctaacaccgtaccacccacgaccaaagttcacccacacccacaaaacccgcgaaaatccagcgccgtcagcacttccgcaatttcagtctcacaacgtcacttccgcgcgccttttttcactattcccacacccgccctcgcgccaccccgcgtcaccccgcgtcaccgcacgtcaccccggccccgcctcgctcctccccgctcattatcatattggcacgtttccagaataaggtatattattgatgatgttaattaattcgaacccataatacccataatagctgtttgccatcgacgcgaggctggatggccttccccattatgattcttctcgcttccggcggcatcgggatgcccgcgttgcaggccatgctgtccaggcaggtagatgacgaccatcagggacagcttcaaggatcgctcgcggctcttaccagcccagcaaaaggccaggaaccgtaaaaaggccgcgttgctggcgtttttccataggctccgcccccctgacgagcatcacaaaaatcgacgctcaagtcagaggtggcgaaacccgacaggactataaagataccaggcgtttccccctggaagctccctcgtgcgctctcctgttccgaccctgccgcttaccggatacctgtccgcctttctcccttcgggaagcgtggcgctttctcatagctcacgctgtaggtatctcagttcggtgtaggtcgttcgctccaagctgggctgtgtgcacgaaccccccgttcagcccgaccgctgcgccttatccggtaactatcgtcttgagtccaacccggtaagacacgacttatcgccactggcagcagccactggtaacaggattagcagagcgaggtatgtaggcggtgctacagagttcttgaagtggtggcctaactacggctacactagaaggacagtatttggtatctgcgctctgctgaagccagttaccttcggaaaaagagttggtagctcttgatccggcaaacaaaccaccgctggtagcggtggtttttttgtttgcaagcagcagattacgcgcagaaaaaaaggatctcaagaagatcctttgatcttttctacggggtctgacgctcagtggaacgaaaactcacgttaagggattttggtcatgagattatcaaaaaggatcttcacctagatccttttaaattaaaaatgaagttttaaatcaatctaaagtatatatgagtaaacttggtctgacagttaccaatgcttaatcagtgaggcacctatctcagcgatctgtctatttcgttcatccatagttgcctgactccccgtcgtgtagataactacgatacgggagggcttaccatctggccccagtgctgcaatgataccgcgagacccacgctcaccggctccagatttatcagcaataaaccagccagccggaagggccgagcgcagaagtggtcctgcaactttatccgcctccatccagtctattaattgttgccgggaagctagagtaagtagttcgccagttaatagtttgcgcaacgttgttgccattgctgcaggcatcgtggtgtcacgctcgtcgtttggtatggcttcattcagctccggttcccaacgatcaaggcgagttacatgatcccccatgttgtgcaaaaaagcggttagctccttcggtcctccgatcgttgtcagaagtaagttggccgcagtgttatcactcatggttatggcagcactgcataattctcttactgtcatgccatccgtaagatgcttttctgtgactggtgagtactcaaccaagtcattctgagaatagtgtatgcggcgaccgagttgctcttgcccggcgtcaacacgggataataccgcgccacatagcagaactttaaaagtgctcatcattggaaaacgttcttcggggcgaaaactctcaaggatcttaccgctgttgagatccagttcgatgtaacccactcgtgcacccaactgatcttcagcatcttttactttcaccagcgtttctgggtgagcaaaaacaggaaggcaaaatgccgcaaaaaagggaataagggcgacacggaaatgttgaatactcatactcttcctttttcaatattattgaagcatttatcagggttattgtctcatgagcggatacatatttgaatgtatttagaaaaataaacaaataggggttccgcgcacatttccccgaaaagtgccacctgacgtctaagaaaccattattatcatgacattaacctataaaaataggcgtatcacgaggccctttcgtcttcaagaattggtcgatggcaaacagctattatgggtattatgggttcgaattaat

SEQ ID NO: 45 - DNA, 8765 bp, Artificial Sequence
  Synthetic oligonucleotide sAdApt4310A.E1btg.Empty
attaacatcatcaataatataccttattctggaaacgtgccaatatgataatgagcggggaggagcgaggcggggccggggtgacgtgcggtgacgcggggtgacgcggggtggcgcgagggcggggcgggtgtgcggaggcgcttagtttttacgtatgcggaaggaggttttataccggaagttgggtaatttgggcgtatacttgtaagttttgtgtagtttggcgcgaaaaccgggtaatgaggaagttgaggttaatatgtactttttatgactgggcggaatttctgctgatcagcagtgaactttgggcgctgacggggaggtttcgctacgtggcagtaccacgagaaggctcaaaggtcccatttattgtactcctcagcgttttcgctgggtatttaaacgctgtcagatcatcaagaggccactcttgagtgccggcgagtagagttttctcctccgcgctgccgcgatgaggctggttcccgagatgtacggtgttttctgcagcgagacggcccggaactcagatgagctgctgaattcagacctgctggaaatttcgaattcgcctgtgcttttgccgccgtcacttcacgacctgtttgatgtggaagtggaccctccggaagatcccaacgaggacgcggtaaatactatgtttccagaatgtctgtttgaggcggctgaggagggttcttacagcggtgaagacggcgggcagggagaggaagtggacctgaagtgctacgaggaatgtctaccttctagcgattctgaaacggaacagacagggggagatggctgtgctgaacctgttgtgaaaaatgaacttgtattagactgtcctgataatcctggtcacggttgccgcgcctgtgattttcatagaaatgccagtggaaatcctgagactctatgtgctctgtgttacctgcgccttaccagccattgtgtatacagtaagtagaaactttttcgctttgtgcatgctggtgggatttttaaagtgcgttgggcttattgttgcgtaatgttttacaggcgacgtgtctgacgcggaaggggatggagatagatcaggctctgctggttctccttgcactttgggggctgtggttccagatggcattattaaacccgtggcggtaagagtttcaggcagacggtgtgcggtcgaaaaaattgaagacttgctgcaggaggaacagatgcaacctttggacctgtccctgaaacgccctaagctgacctaagagtgtttattgtatgcaataaaaagtgttgatctttgaactgtgtttatgtgttgggtgtgtctgtgggtatataagcaggtggatgggaagtgagagcacagctgcttcagatggatctgctaggagacctgagggaatttggcgtggttcggcgcttgctggagttggcctctgacagaacttccaagttttggaggttttgttttggctcaacgcttagcaacgtgctatatagggtcaagaaggagcaggagacgcagtttgctaggctgttggccgatactcctggagtttttgtggctctggatctaggccatcactctcttttccaagagaaaattatcaaaaacttaacttttacgtctcctggtcgcacggttgcttccgctgcctttattacctatattttggatcaatggagcaacagcggcagtcacctgtcgtgggagtacatgctggattacatgtcgatggcgctgtggagggccatgctgcggaggagggtttgcatttacttgcgggcgcagcctccgcggctggaccgagtggaggaggaggacgagccgggggagaccgagaacctgagggccgggctggaccctccaacggaggactaggtgctgaggatgatcccgaagaggggactagtggggctaggaagaagcaaaagactgagtctgaacctcgaaactttttgaatgagttgactgtgagtttgatgaatcgtcagcgtccggagacaattttctggtctgaattggaggaggaattcaggaggggggaactgaacctgctatacaagtatgggtttgaacagttgaaaactcactggttggagccgtgggaggattttgaaaccgccttggacacttttgctaaagtggctctgcgaccggataaggtttacactatccgccgcactgttaacataaagaagagtgtttatgttataggccatggagctctggtgcaggtgcaaaccgccgaccgggtggcctttagttgcggcatgcaaaatctgggccccggggtgataggcttaaatggtgtaacatttcacaatgtaaggtttactggtgaaagttttaacggctctgtgtttgcaaataacacacagctgacgctccacggcgtttacttttttaactttaataacacatgtgtggagtcgtggggcagggtgtctttgaggggctgctgttttcacggctgctggaaggcggtggtgggaagacttaaaagtgtaacatctgtaaaaaaatgcgtgtttgagcgctgtgtgttggctttaaccgtggagggctgtggacgcattaggaataatgcagcgtctgagaatggatgtttccttttgctaaaaggcacggctagcgttaagcataacatgatatgcggcagcggtttgtacccttcgcagctgttaacttgcgcggatggaaactgtcagaccctgcgcaccgtgcacatagcgtcccaccagcgacgcgcctggccaacattcgagcacaatatgcttatgcgctgtgccgttcacctgggccctaggcgaggcgtgtttgtgccttaccagtgtaactttagccataccaagtttttactagaacctgacaccttctctcgagtgtgtttcaacggggtttttgacatgtcaatggaactgtttaaagtgataagatatgatgaatccaagtctcgttgtcgcccatgtgaatgcggagctaatcatttgaggttgtatcctgtaactctgaacgtcaccgaggagctgagaacggaccaccacatgctgtcttgcctgcgcactgactatgaatccagcgacgaggagtgaggtgaggggcggagccaaacgggtataaaggggcgtgaggtcgactggtcaatattggccattagccatattattcattggttatatagcataaatcaatattggctattggccattgcatacgttgtatccatatcataatatgtacatttatattggctcatgtccaacattaccgccatgttgacattgattattgactagttattaatagtaatcaattacggggtcattagttcatagcccatatatggagttccgcgttacataacttacggtaaatggcccgcctggctgaccgcccaacgacccccgcccattgacgtcaataatgacgtatgttcccatagtaacgccaatagggactttccattgacgtcaatgggtggagtatttacggtaaactgcccacttggcagtacatcaagtgtatcatatgccaagtacgccccctattgacgtcaatgacggtaaatggcccgcctggcattatgcccagtacatgaccttatgggactttcctacttggcagtacatctacgtattagtcatcgctattaccatggtgatgcggttttggcagtacatcaatgggcgtggatagcggtttgactcacggggatttccaagtctccaccccattgacgtcaatgggagtttgttttggcaccaaaatcaacgggactttccaaaatgtcgtaacaactccgccccattgacgcaaatgggcggtaggcgtgtacggtgggaggtctatataagcagagctcgtttagtgaaccgtcagatcgcctggagacgccatccacgctgttttgacctccatagaagacaccgggaccgatccagcctccgcggccgggaacggtgcattggaagcttggtaccggtgaattcgctagcgttaacggatcctctagacgagatccgaacttgtttattgcagcttataatggttacaaataaagcaatagcatcacaaatttcacaaataaagcatttttttcactgcattctagttgtggtttgtccaaactcatcaatgtatcttatcatgtctagatccttaaggacatgtcaatggaactgtttaaagtgataagatatgatgaatccaagtctcgttgtcgcccatgtgaatgcggagctaatcatttgaggttgtatcctgtaactctgaacgtcaccgaggagctgagaacggaccaccacatgctgtcttgcctgcgcactgactatgaatccagcgacgaggagtgaggtgaggggcggagccaaacgggtataaaggggcgtgaggggtcggtgcggtgtttcaaaatgagcgggacgacggacggcaatgcgtttgaggggggagtgttcagcccatatctgacatctcgtcttccttcctgggcaggagtgcgtcagaatgtagtgggatccaccgtggacggacgaccggtggctcctgcaaattccgccaccctcacctatgccaccgtgggatcatcgttggacactgccgcggcagctgccgcttctgctgccgcttctactgctcgcggcatggcggctgattttggactgtataaccaactggccactgcagctgtggcgtctcggtccctggttcaagaagatgccctgaatgtgattctgactcgcctggagatcatgtcacgccgcctggacgaactggctgcgcagatatcctcaactaaccccgataccacttcagaaccttaaataaagacaaacaaatttgttgaaaagtaaaatggctttatttgttttttttggctcggtaggctcgggtccacctgtcccggtcgttaaggaccttgtgtatgttttccaagacccggtacagatgggcttggatgttcaagtacatgggcatgaggccatctcgggggtggagataggaccattgcagagcgtcatgctccggggtggtgttgtaaataacccagtcgtagcagggtttctgagcgtggaactggaagatgtcctttaggagcaggctgatggccaagggcagccccttagtgtaggtgttaacaaagcggttaagctgggagggatgcatgcggggggagatgatatgcatcttggcttgaattttgaggttagctatgttaccacctaggtccctgcgggggttcatgttatgaaggaccaccagcacggtgtagccggtgcacttggggaacttgtcatgcagtttggaggggaaggcgtggaagaatttagagacccccttgtggcctcctaggttttccatgcactcatccataatgatggcaatgggacccctggcggccgctttggcaaacacgttttgggggttggaaacatcatagttttgctctagagtgagctcatcataggccatcttaacaaagcggggtaggagggtgcccgactgggggatgatagttccatctgggcctggggcgtagttgccctcacaaatctgcatttcccaggccttaatttccgaggggggtatcatgtccacctggggggcgataaagaacacggtttctggcgggggattgatgagctgggtggaaagcaagttacgcaacagttgggatttgccgcaaccggtgggaccgtagatgaccccgatgacgggttgcagctggtagttgagagaggaacagctgccgtcggggcgcaggaggggggctacatcgttcatcatgcttctgacatgtttattttcactcactaagttttgcaagagcctctccccacccagggataagagttcttccaggctgttgaagtgtttcagcggtttcaggccgtctgccatgggcatcttttcaagcgactgacgaagcaagtacagtcggtcccagagctcggtgacgtgctctatggaatctcgatccagcagacttcttggttgcgggggttgggccgactttcgctgtagggcaccagccggtgggcgtccagggccgcgagggttctgtccttccagggtctcagcgttcgggtgagggtggtctcggtgacggtgaagggatgagccccgggctgggcgcttgcgagggtgcgcttcaggctcatcctgctggtgctgaagcgggcgtcgtctccctgtgagtcggccagatagcaacgaagcatgaggtcgtagctgagggactcggccgcgtgtcccttggcgcgcagctttcccttggaaacgtgctgacatttggtgcagtgcagacacttgagggcgtagagtttgggggccaggaagaccgactcggacgagtaggcgtcggctccgcactgagcgcagacggtctcgcactccaccagccacgtgagctcgggtttagcgggatcaaaaaccaagttgcctccattttttttgatgcgtttcttaccttgcgtctccatgagtctgtgtcccgcttccgtgacaaaaaggctgtcggtgtccccgtagaccgacttgagggggcgatcttccaaaggtgttccgagatcttccgcgtacaggaactgggaccactccgagacaaaggctcgggtccaggctaacacgaaggaggcgatctgcgaggggtatctgtcgttttcaatgaggttaattaattcgaacccataatacccataatagctgtttgccatcgacgcgaggctggatggccttccccattatgattcttctcgcttccggcggcatcgggatgcccgcgttgcaggccatgctgtccaggcaggtagatgacgaccatcagggacagcttcaaggccagcaaaaggccaggaaccgtaaaaaggccgcgttgctggcgtttttccataggctccgcccccctgacgagcatcacaaaaatcgacgctcaagtcagaggtggcgaaacccgacaggactataaagataccaggcgtttccccctggaagctccctcgtgcgctctcctgttccgaccctgccgcttaccggatacctgtccgcctttctcccttcgggaagcgtggcgctttctcatagctcacgctgtaggtatctcagttcggtgtaggtcgttcgctccaagctgggctgtgtgcacgaaccccccgttcagcccgaccgctgcgccttatccggtaactatcgtcttgagtccaacccggtaagacacgacttatcgccactggcagcagccactggtaacaggattagcagagcgaggtatgtaggcggtgctacagagttcttgaagtggtggcctaactacggctacactagaaggacagtatttggtatctgcgctctgctgaagccagttaccttcggaaaaagagttggtagctcttgatccggcaaacaaaccaccgctggtagcggtggtttttttgtttgcaagcagcagattacgcgcagaaaaaaaggatctcaagaagatcctttgatcttttctacggggtctgacgctcagtggaacgaaaactcacgttaagggattttggtcatgagattatcaaaaaggatcttcacctagatccttttaaattaaaaatgaagttttaaatcaatctaaagtatatatgagtaaacttggtctgacagttaccaatgcttaatcagtgaggcacctatctcagcgatctgtctatttcgttcatccatagttgcctgactccccgtcgtgtagataactacgatacgggagggcttaccatctggccccagtgctgcaatgataccgcgagacccacgctcaccggctccagatttatcagcaataaaccagccagccggaagggccgagcgcagaagtggtcctgcaactttatccgcctccatccagtctattaattgttgccgggaagctagagtaagtagttcgccagttaatagtttgcgcaacgttgttgccattgctgcaggcatcgtggtgtcacgctcgtcgtttggtatggcttcattcagctccggttcccaacgatcaaggcgagttacatgatcccccatgttgtgcaaaaaagcggttagctccttcggtcctccgatcgttgtcagaagtaagttggccgcagtgttatcactcatggttatggcagcactgcataattctcttactgtcatgccatccgtaagatgcttttctgtgactggtgagtactcaaccaagtcattctgagaatagtgtatgcggcgaccgagttgctcttgcccggcgtcaacacgggataataccgcgccacatagcagaactttaaaagtgctcatcattggaaaacgttcttcggggcgaaaactctcaaggatcttaccgctgttgagatccagttcgatgtaacccactcgtgcacccaactgatcttcagcatcttttactttcaccagcgtttctgggtgagcaaaaacaggaaggcaaaatgccgcaaaaaagggaataagggcgacacggaaatgttgaatactcatactcttcctttttcaatattattgaagcatttatcagggttattgtctcatgagcggatacatatttgaatgtatttagaaaaataaacaaataggggttccgcgcacatttccccgaaaagtgccacctgacgtctaagaaaccattattatcatgacattaacctataaaaataggcgtatcacgaggccctttcgtcttcaagaattggtcgatggcaaacagctattatgggtattatgggttcgaattaat

SEQ ID NO: 46 - DNA, 6174 bp, Artificial Sequence
  Synthetic oligonucleotide sAdApt4312.Empty
attaacatcatcaataatataccttattctggaaacgtgccaatatgataatgagtggggaggagcgaggcggggccggggtggggtgaggcggggccggggtggggtgagggtgacgtcggggcgggcggggcggccgacgtgtgtggggaggcgcgtagtgtttacgtatgcggaaggaggttttataccggaagatgggtaatttgggcgtatacttgtaagttttgtgtaatttggcgcgaaaactgggtaatgaggaagttgaggttaatatgtactttttatgactgggcggaatttctgctgttcagcagtgaactttgggcgctgacggggaggtttcgctacgtggcagtaccacgagaaggctcaaaggtcccatttattgtactcctcagcgttttcgccgggtatttaaacgctgtcagatcatcaagaggccactcttgagtgctggcgagtagagttttctcctccggtcgactggtcaatattggccattagccatattattcattggttatatagcataaatcaatattggctattggccattgcatacgttgtatccatatcataatatgtacatttatattggctcatgtccaacattaccgccatgttgacattgattattgactagttattaatagtaatcaattacggggtcattagttcatagcccatatatggagttccgcgttacataacttacggtaaatggcccgcctggctgaccgcccaacgacccccgcccattgacgtcaataatgacgtatgttcccatagtaacgccaatagggactttccattgacgtcaatgggtggagtatttacggtaaactgcccacttggcagtacatcaagtgtatcatatgccaagtacgccccctattgacgtcaatgacggtaaatggcccgcctggcattatgcccagtacatgaccttatgggactttcctacttggcagtacatctacgtattagtcatcgctattaccatggtgatgcggttttggcagtacatcaatgggcgtggatagcggtttgactcacggggatttccaagtctccaccccattgacgtcaatgggagtttgttttggcaccaaaatcaacgggactttccaaaatgtcgtaacaactccgccccattgacgcaaatgggcggtaggcgtgtacggtgggaggtctatataagcagagctcgtttagtgaaccgtcagatcgcctggagacgccatccacgctgttttgacctccatagaagacaccgggaccgatccagcctccgcggccgggaacggtgcattggaagcttggtaccggtgaattcgctagcgttaacggatcctctagacgagatccgaacttgtttattgcagcttataatggttacaaataaagcaatagcatcacaaatttcacaaataaagcatttttttcactgcattctagttgtggtttgtccaaactcatcaatgtatcttatcatgtctagatccttaaggtgataagatatgatgaatccaagtctcgttgtcgcccctgtgaatgcggagctaatcatttgaggttgtatcccgcgaccctgaacgtaaccgaggagctgagggccgaccaccacatgttgtcctgcttgcgcaccgactatgagtccagcgacgaagagtgaggtgaggggcggagccacaaagggtataaagggtcaggatgggtgggcacaggtattcaaaatgagcgggacgacggacggcaacgcgtttgaggggggagtgttcagcccatatctgacatctcgtcttccttcctgggcaggagtgcgtcagaatgtagtgggctccaccgtggacggacggccggtcgcccctgcgaattccgccacccttacctatgccaccgtgggatcaccgttggacactgccgcggcagccgcagcttctgctgccgcttctactgctcgcggtatggcggctgactttggactttataaccaactggctaccgcggctgtggcatctcgcactctggttcaagaagatgccctgagcgtggttctgcttcgactggaagatctgtctcgtcgcttggatcagctggctgcgcagatatccccacctaaccccgatactactcaagaatcttaaataaagacaaacagatttgttgaaaataaatggctttatttgttttttttggctcgataggctcgggtccacctgtcccggtcgttaaggactttgtgtatgctttccaagacccggtacagatgggcttggatgtttagatacatgggcatgaggccatcccgggggtggagataggaccattgcagagcgtcatgctccggggtggtgttgtagatgacccagtcgtagcagggtttttgggcgtggaactgaaaaatgtccttgagaagcaggctgatggccaggggcagacccttagtgtaggtgttcacaaagcggttgagctgggagggatgcatgcggggagagatgatatgcatcttagcctggattttcaggttagctatgttgccccccaggtcccttcgagggttcatattgtggaggaccaccagaacggtgtagccggtacacttgggaaacttatcgtgcagtttggaggggaaggcgtgaaagaatttggaaacccctttgtgaccacctaagttttccatgcactcgtccatgataatggcgatgggccccttggcggcagctttagcgaacacgttgtgggggttggaaacatcatagttttgctctagagttagctcgtcataggccatttttacgaagcggggtaggagggtgccagactgagggacgatagttccatctggccccggtgcgtaattaccctcgcagatctgcatctcccaagctttaatttccgagggagggatcatgtccacctggggggcgataaagaacacggtttctggcgggggattaatgagctgggtggaaagcaggttgcgcaagagctgagacttgccgcaaccggtgggaccgtagatgaccccgatgacgggctgcagctggtagttgagagaggagcagctgccgtcggggcgtaggaggggagccacctcgttcatcatgcttcttacatgtttattttcactgactaagctttgcaagagcctctccccacccagggacaagagttcttccaggctgttgaagtgtttcagcggtttcaggccgtcggccatgggcatcttttcaagcgactgacgaagcaagtacagccggtcccagagctcggtgacgtgctctatggaatctcgatccagcagacttcttggttgcgggggttgggccgactttcgctgtagggtacgagccggtgggcgtccagggccgcgagggttttgtccttccagggtctcagcgtccgggtgagggtggtctcggtgacggtgaacggatgagccccgggctgggcgcttgccagggtgcgcttcaggctcatccggctggtgctgaagcgggcgtcgtctccctgggaatcggccagatagcaacggagcatgaggtcgtagctaagggattcggccgcgtgtcccttggcgcgcagttttcccttggaaacatgctggcatctggtgcagtgtaaacacttgagggcgtacagcttgggggcgaggaagacggactcgggcgagtaggcgtcggccccgcactcggcgcagacggtttcacactccaccagccacgtgagctcgggtttgtcggggtcaaaaaccaggttgcctccattttttttgatgcgtttcttaccttgcgtctccatgagcctgtgacccgcttcggtgacaaaaaggctgtctgtgtctccgtagaccgacttgagggggcgttcttccaagggcgtgccgcggtcttctgcgtacaaaaactgggaccactccgaaacgaaggccctggtccacgctaacacgaaggatgcgatctgcgaggggtatctgtcgttctcaatgaggggatccaccttttccagggtatgcagacacaggtcgtcctcctccgcgtccacaaaggtgattggcttgtaagtgtaggtcacgtgacttaattaattcgaacccataatacccataatagctgtttgccatcgacgcgaggctggatggccttccccattatgattcttctcgcttccggcggcatcgggatgcccgcgttgcaggccatgctgtccaggcaggtagatgacgaccatcagggacagcttcaaggccagcaaaaggccaggaaccgtaaaaaggccgcgttgctggcgtttttccataggctccgcccccctgacgagcatcacaaaaatcgacgctcaagtcagaggtggcgaaacccgacaggactataaagataccaggcgtttccccctggaagctccctcgtgcgctctcctgttccgaccctgccgcttaccggatacctgtccgcctttctcccttcgggaagcgtggcgctttctcatagctcacgctgtaggtatctcagttcggtgtaggtcgttcgctccaagctgggctgtgtgcacgaaccccccgttcagcccgaccgctgcgccttatccggtaactatcgtcttgagtccaacccggtaagacacgacttatcgccactggcagcagccactggtaacaggattagcagagcgaggtatgtaggcggtgctacagagttcttgaagtggtggcctaactacggctacactagaaggacagtatttggtatctgcgctctgctgaagccagttaccttcggaaaaagagttggtagctcttgatccggcaaacaaaccaccgctggtagcggtggtttttttgtttgcaagcagcagattacgcgcagaaaaaaaggatctcaagaagatcctttgatcttttctacggggtctgacgctcagtggaacgaaaactcacgttaagggattttggtcatgagattatcaaaaaggatcttcacctagatccttttaaattaaaaatgaagttttaaatcaatctaaagtatatatgagtaaacttggtctgacagttaccaatgcttaatcagtgaggcacctatctcagcgatctgtctatttcgttcatccatagttgcctgactccccgtcgtgtagataactacgatacgggagggcttaccatctggccccagtgctgcaatgataccgcgagacccacgctcaccggctccagatttatcagcaataaaccagccagccggaagggccgagcgcagaagtggtcctgcaactttatccgcctccatccagtctattaattgttgccgggaagctagagtaagtagttcgccagttaatagtttgcgcaacgttgttgccattgctgcaggcatcgtggtgtcacgctcgtcgtttggtatggcttcattcagctccggttcccaacgatcaaggcgagttacatgatcccccatgttgtgcaaaaaagcggttagctccttcggtcctccgatcgttgtcagaagtaagttggccgcagtgttatcactcatggttatggcagcactgcataattctcttactgtcatgccatccgtaagatgcttttctgtgactggtgagtactcaaccaagtcattctgagaatagtgtatgcggcgaccgagttgctcttgcccggcgtcaacacgggataataccgcgccacatagcagaactttaaaagtgctcatcattggaaaacgttcttcggggcgaaaactctcaaggatcttaccgctgttgagatccagttcgatgtaacccactcgtgcacccaactgatcttcagcatcttttactttcaccagcgtttctgggtgagcaaaaacaggaaggcaaaatgccgcaaaaaagggaataagggcgacacggaaatgttgaatactcatactcttcctttttcaatattattgaagcatttatcagggttattgtctcatgagcggatacatatttgaatgtatttagaaaaataaacaaataggggttccgcgcacatttccccgaaaagtgccacctgacgtctaagaaaccattattatcatgacattaacctataaaaataggcgtatcacgaggccctttcgtcttcaagaattggtcgatggcaaacagctattatgggtattatgggttcgaattaat

SEQ ID NO: 47 - DNA, 16854 bp, Artificial Sequence
  Synthetic oligonucleotide pBr/sAd4312.pIX-pV
attaagtgataagatatgatgaatccaagtctcgttgtcgcccctgtgaatgcggagctaatcatttgaggttgtatcccgcgaccctgaacgtaaccgaggagctgagggccgaccaccacatgttgtcctgcttgcgcaccgactatgagtccagcgacgaagagtgaggtgaggggcggagccacaaagggtataaagggtcaggatgggtgggcacaggtattcaaaatgagcgggacgacggacggcaacgcgtttgaggggggagtgttcagcccatatctgacatctcgtcttccttcctgggcaggagtgcgtcagaatgtagtgggctccaccgtggacggacggccggtcgcccctgcgaattccgccacccttacctatgccaccgtgggatcaccgttggacactgccgcggcagccgcagcttctgctgccgcttctactgctcgcggtatggcggctgactttggactttataaccaactggctaccgcggctgtggcatctcgcactctggttcaagaagatgccctgagcgtggttctgcttcgactggaagatctgtctcgtcgcttggatcagctggctgcgcagatatccccacctaaccccgatactactcaagaatcttaaataaagacaaacagatttgttgaaaataaatggctttatttgttttttttggctcgataggctcgggtccacctgtcccggtcgttaaggactttgtgtatgctttccaagacccggtacagatgggcttggatgtttagatacatgggcatgaggccatcccgggggtggagataggaccattgcagagcgtcatgctccggggtggtgttgtagatgacccagtcgtagcagggtttttgggcgtggaactgaaaaatgtccttgagaagcaggctgatggccaggggcagacccttagtgtaggtgttcacaaagcggttgagctgggagggatgcatgcggggagagatgatatgcatcttagcctggattttcaggttagctatgttgccccccaggtcccttcgagggttcatattgtggaggaccaccagaacggtgtagccggtacacttgggaaacttatcgtgcagtttggaggggaaggcgtgaaagaatttggaaacccctttgtgaccacctaagttttccatgcactcgtccatgataatggcgatgggccccttggcggcagctttagcgaacacgttgtgggggttggaaacatcatagttttgctctagagttagctcgtcataggccatttttacgaagcggggtaggagggtgccagactgagggacgatagttccatctggccccggtgcgtaattaccctcgcagatctgcatctcccaagctttaatttccgagggagggatcatgtccacctggggggcgataaagaacacggtttctggcgggggattaatgagctgggtggaaagcaggttgcgcaagagctgagacttgccgcaaccggtgggaccgtagatgaccccgatgacgggctgcagctggtagttgagagaggagcagctgccgtcggggcgtaggaggggagccacctcgttcatcatgcttcttacatgtttattttcactgactaagctttgcaagagcctctccccacccagggacaagagttcttccaggctgttgaagtgtttcagcggtttcaggccgtcggccatgggcatcttttcaagcgactgacgaagcaagtacagccggtcccagagctcggtgacgtgctctatggaatctcgatccagcagacttcttggttgcgggggttgggccgactttcgctgtagggtacgagccggtgggcgtccagggccgcgagggttttgtccttccagggtctcagcgtccgggtgagggtggtctcggtgacggtgaacggatgagccccgggctgggcgcttgccagggtgcgcttcaggctcatccggctggtgctgaagcgggcgtcgtctccctgggaatcggccagatagcaacggagcatgaggtcgtagctaagggattcggccgcgtgtcccttggcgcgcagttttcccttggaaacatgctggcatctggtgcagtgtaaacacttgagggcgtacagcttgggggcgaggaagacggactcgggcgagtaggcgtcggccccgcactcggcgcagacggtttcacactccaccagccacgtgagctcgggtttgtcggggtcaaaaaccaggttgcctccattttttttgatgcgtttcttaccttgcgtctccatgagcctgtgacccgcttcggtgacaaaaaggctgtctgtgtctccgtagaccgacttgagggggcgttcttccaagggcgtgccgcggtcttctgcgtacaaaaactgggaccactccgaaacgaaggccctggtccacgctaacacgaaggatgcgatctgcgaggggtatctgtcgttctcaatgaggggatccaccttttccagggtatgcagacacaggtcgtcctcctccgcgtccacaaaggtgattggcttgtaagtgtaggtcacgtgaccggcgccccccggaggggtataaaagggggcgtgcccaccctccccgtcactttcttccgcatcgctgtggaccagagccagctgttcgggtgagtaggccctctcaaaggccggcatgacttcggcactcaagttgtcagtttctacaaacgaggaggatttgatgttcacgtgccccgcggcgatgcttttgatggtggagtggtccatctggtcagaaaacacgatctttttgttgtcaagtttggtggcaaaagacccatagagggcgttggaaagcaacttggcgatggagcgcagggtctgatttttttcccgatcggccctttccttcgcggcgatgtttaattgcacgtactcgcgggccacgcatcgccattccgggaacacggcggtgcgctcgtcgggcaggatgcgcacgcgccagccgcgattgtgcagggtgatcatgtccacgctggtggccacctccccccggaggggctcgttggtccaacacaatctccctccttttctggagcagaacggagggaggggatctaggaggttggcgtgcggggggtcggcgtcgatggtgaagatgccaggcaggagaactttattaaagtaatcgatctcggtttccacgtcttgcaacgcctcctcccatctctttaccgccagggccctctcgtaggggttcaggggcgccccccagggcatggggtgggtgagagccgaggcgtacatgccacagatgtcatagacgtagaggggctcccgtaggaccccgatgtaagtgggataacagcgccccccgcggatgctggcccgcacgtagtcgtacatctcgtgagatggggccaggagaccctctcccaagtgggtcttgtggggcttctccgcccggtagaggatctgcctgaagatggcgtgggagttggaagagatggtgggccgttggaagacgttaaagttggcccgcggcagccccaccgagtcttcgatgaactgggcgtaggattcctggagtttgttcacgagggcggcggtgaccagcacgtccagggcgcagtaatccagggtctcgcggaccaggttgtaggagctctcttgttttttctcccacagttcgcggttgaggaggtattcctcgcggtctttccagtactcttcggcgggaaatcctttttcgtccgctcggtaagaacctaacatgtaaaactcgttcaccgctttgtatggacaacagcctttctctaccggcagggcgtacgcctgagcggcctttctgagagaagtgtgggtgagggcgaaggtgtcccgcaccatgactttcaggtactgatgtttgaagtccgtgtcgtcgcagcttccttgttcccacaggctgaagtcggtgcgctttttctgcctcgggttggggagggcgaaagtgacatcgttaaacaagattttcccggcgcggggcataaagttgcgagagattctgaagggccctggcacgtccgagcggttgttgatgacctgcgccgccaggacgatctcgtcgaagccgttgatgttatgccccacgatgtacagttctatgaagcgcggctgtcccttgagggcgggcgcttttttcagttcctcgtaggtgagggactcgggagaggcgagccccagctccgcgcgggcccagtcggccagttgagggttagccgcgaggaaggaattccagagctccgaggccagaagagtttgcaagcgatcgcgaaactcgcggaactttttccccacggccattttttctggcgtgaccacgtagaaagtggcggagcgatcgttccagacgtcccacttgagctcccgggccagctcgcaggcctgacgcacgagagtttcctcgcccgagacgtgcatgaccaacatgaaaggcactaactgttttccgaacgcgcccatccacgtgtaggtctctacatcgtaggtgacaaagagccgttgggtgcgtgcgtgggagccgatcggaaagaagctgatctcctgccaccagctggaggaatgggtgttgatgtggtgaaagtagaagtcccgccggcgcacagagcattcgtgctggtgtttgtaaaagcgaccgcagtagtcgcagcgctgcacgctctgtatttcttgaatgagatgcacttttcgcccgcgaaccagaaatcggaggggaaagttgagcccgggggatggtggagtcgcgtccccttcgccttggcggtgggcgtctgcgtctgcgtcctgtttttctgggtggacgacggtggggacgacgacgccccgggttccgcaagtccagatttcagcgacggaggggcgcagacgcagaaggagggggcgcagttgcccgctgtccagagagtcgaggaaagcgacgctgaggtcagcggggagcgtttgcaaattcactttcaagagaccggtaagagcgtgagccaggtggagatgatacttgatttccaggggggtgttggaagaggcgtccacgccgtacaagaggccgtgtccgcgcggagccaccacggttccccgcggaggttttatctcactcgccgagggcgagcgccggggggtagaggcggctctgcgccgggtggtagcggaggcagaggcacgttttcgtgaggattcggcagcggctgatgacgcgctcggagactgctggcgtgggcgacgacgcggcggttgaggtcctggatgtgctgcctctgcgtgaagaccaccggtcccctggtcctgaacctgaaagagagttccacagagtcaatgtctgcatcgttaacggccgcctgcctgaggatctcctgcacgtcgcccgagttgtcttggtaggcgatctcggccatgaactgttcgacttcttcttcgcggaggtcgccgtggcccgcgcgttctacggtggcggccaggtcgttagagatgcgacgcatgagctgggagaaggcgttgaggccgttctcgttccacacgcggctgtacaccacgttaccgaaggagtcgcgcgctcgcatgaccacctgcgccacgttgagttccacgtggcgggcgaagacggcgtagtttctgaggcgctggaagaggtagttgagcgtggtggcgatgtgctcgcagacgaagaagtacatgatccagcgcctcagagtctgctcgttgatgtctccgatggcttcgaggcgttccatggcctcgtagaagtcgacggcgaagttgaaaaattgggagttgcgggcggccaccgtgagttcttcttgcaggaggcggatgagatcggcgacggtgtcgcgcacctcctgttcgaaagcgccccgaggcgcctctgcttcttcctccagctcctcctcttccaggggcacaggttcctccggcacctctgcggcggggacggggcggcgacgtcgtcgtctgaccggcagtcggtccacgaagcgttcgatcatttcaccgcgccggcgacgcatggtctcggtgacggcgcgtccgttttcgcggggacgcagttcgaagacgccgccgcgcagagcgcccccgtgcagggagggtaagtggttagggccgtcgggcagagacacggcgctgacgatgcattttatcaattgttgcgtaggcactccgtgcagggatctgagaacgtcgaggtcgacgggatccgaaaacttctctaggaaagcgtctatccaatcgcaatcgcaaggtaagctgaggacggtgggccgctggggggcgtccgcgggtagttgggaggtgatgctgctgatgatgtaattaaagtaggcggttttcaggcggcggatggtggcgaggaggaccacgtctttgggcccggcctgttgaatgcgcaggcgctcggccatcccccaggcctcgctctgacagcgacgcaggtctttgtagtagtcttgcatcagtctctccaccggaatctctgcttctcccctgtctgccatgcgagtcgagccgtacccccgcaagggctgcagcaacgctaggtctgccactactctttcggccagcacggcctgttgaatctgcgtgagggtggcctggaagtcgtccaggtccacgaagcggtggtaggctcccgtgttgatggtgtaggtgcagttggccatgacggaccagttgacgacttggatgccgggttgggtgatctccgtgtacttgaggcgcgagtaggccctggactcgaacacgtagtcgttgcatgcgcgcaccagatactggtagccgacgagaaagtgcggaggcggttcccgatacaggggccagcccacggtggcgggggctccgggggccaggtcttccagcatgaggcggtggtagtggtacacgtatcgagagagccaggtgatgccggctgaggtggtggcggccctggtgaactcgcggacgcggttccagatgttgcgcagggggcggaagcgttccatggtgggcacgctctgtcccgtcaggcgcgcgcaatcctgtacgctctagatggagaaaagacagggcggtcatcgactcccgtccgtagctgggaggtaaagtcgcaagggtgcggcggcggggaaccccggttcgagaccggctggatccgccgttcccgatgcgcctggccccgcatccacgacgttcgcgccgagacccagccgcggcacaccgccccaatacggaggggagtcttttggtgttttttcatagatgcatccggtgctgcgacagatgcgaccccagacgcccactgctactaccgccgcggcggcagtaaacctgagcggaggcggtgacagggaggacgaagagctggctttagacctggaagagggagagggtctggcgcgactgggcgccccctcccccgagagacaccccagggtccagctcgtgagggatgcgagacaggcttttgtaccgcggcagaacctgtttagggaccgcagcggccaggaggcggaggagatgcgcgattgtcggtttcgggcgggcagagagctgagggcggggttcgaccgggagcggttgctgcgggcggaggatttcgaacccgacgagcggtcgggggtgagtccggcccgagcccacgtgtcggccgccaacctggtgagtgcgtatgagcagacggtgaacgaggagcgtaactttcaaaagagctttaataatcacgttcggaccctcatcgcgagggaggaggtggccatcgggctgatgcatctgtgggacttcgtggaggcctacgtgcagaacccggcgagcaagcccctgacggctcagctgttcctgatcgtgcagcacagccgcgacaacgagacgtttcgcgacgccatgctcaacatcgccgagcccgagggccgctggctcttggatcttatcaacatcttgcagagcatcgtggttcaggagaggggtctcagcttagcggacaaggtggcggccattaactactccatgcagagtctgggaaaattctacgctcgcaagatctacaagagcccctacgtgcccatagacaaggaggtgaagatagacagcttttacatgcgcatggcgctgaaggtgctgacgctgagcgacgatctcggcgtgtaccgtaacgacaagatccacaaggcggtgagcgccagccgccggcgggagctgagcgatagggagctgatgcacagcctgcagagggcgctggcgggtgccggggacgaggagcgcgagacttacttcgatatgggagcggacttacagtggaaacccagcgcccgagcgttggaggcggcgggctaccgtggcgacgaggatcgggatgactttgaggaggcaggcgagtacgaggacgaagcctgaccgggcaggtgttgttttagatgcagcgtccggcggacggggccaccgtggatcccgcgcttttggcatccatgcagagtcaacctacgggcgtgaccgcctccgatgactgggcggcggccatggaccgcatcatggcactgaccacccgcaaccccgaggcttttaggcagcaaccccaggccaaccgtttttcggccatcttggaagcggtagtgccgtctcgcactaatccgacccacgaaaaggttttaactatcgtgaacgcgctggtagacagcaaggccatccgccgcgacgaggcggggctgatttacaacgctctgctggaacgcgtggcgcgctacaacagcactaacgtgcagaccaatctggaccgcctcaccacggacgtgaaggaagcgttggctcagaaggagcggttcttaagggacagcaatctgggttctctggtggcgctgaacgcttttctgagcacgcagccggcgaacgtaccccgcgggcaggaggactacgtgagcttcatcagcgctctgagactgctcgtttccgaggtgccgcagagcgaggtgtaccagtcgggacctgactacttcttccagacgtcccgacagggcttgcaaacggtgaacctgactcaggcttttaaaaacttgcaaggcatgtggggcgtgaaggcgccggttggcgatcgcgcgaccatttccagcctgctgacccccaacacgagactgctgttgcttttaatcgccccgttcaccaacagcagcaccatcagccgcgactcgtacctgggccatctcatcactctgtaccgagaggccataggtcaggctcagattgacgagcatacgtatcaagagatcaccaatgtgagccgagccctgggtcaggaagacaccggcagtttggaagccacgctaaactttctgctgaccaatcggagacaaaagattccctcgcagtacacgttaagcgccgaggaggagaggattctgcgctacgtgcagcagtccgtgagcctgtacttgatgcgggagggtgctaccgcttccacggccttggacatgacggctcgaaacatggaaccgtctttttactcagcccaccgtccgttcatcaatcgcctgatggactacttccatcgcgcggccgccatgaacggggagtatttcaccaatgccatcttgaatccgcattggatgcctccgtccggtttctacaccggggagttcgacctgcccgaggccgacgacggctttctgtgggacgatgtgtccgacagcatttttacgccaggtaacagtcgtttccataaaaaggaagggggagacgaacttcccctttcgagtgtggaggcggcctccaggggggagagccccttttccagcttgtcttccgtgagtagcggtcgggtgacgcgcccacgcttgccgggggagagcgactacctaaacgaccctttgctgcgaccggctaaaaagaaaaattttcccaacaacggggtggaaagcttggtggataaaatgaatcgttggaagacctacgctcaggagcagcgggagtgggaggacagtcagccccgaccgctggtcccgccgcactggcgccgccagagagaagacccggacgactccgcagacgatagtagcgtgttggacttgggagggagcggagccaacccctttgctcacttgcaacccaaggggcgcttgagtcgcctgtactaataaaaagaaagcggaaacgtaccagagccatggccacagcgtgtgtcctttcttcctctctttcctcctcggcgcggcagaatgagaagagcggtgagagtcacgccggcggtgtatgccgagggtccgcccccttcttacgaaagcgtgatgggatcagcgaacgtgccggccacgctggaggcgccttacgttcctcccagatacctgggacctaccgagggcagaaacagcatccgttactccgagctggcccccctgtacgataccaccaaggtgtacctggtggacaacaagtcggcggacatcgcctccctgaattaccaaaacgaccacagcaacttcctgaccaccgtggtgcagaacaatgacttcaccccgacggaggcgggcacgcaaaccattaactttgacgagcgttcccgctggggcggtcagctgaaaaccatcctgcacaccaacatgcccaacatcaacgagtttatgtccaccaacaagtttagggccaggttgatggtagagaagactagcggccagccgcccaaatacgagtggttcgagttcaccattcccgagggtaactactccgagaccatgactatcgatctcatgaataacgcgatcgtggacaattacctgcaagttggaaggcaaaacggggtattggagagcgacataggagtaaaatttgataccaggaacttccgactggggtgggatccggtgaccaagctggtgatgcctggcgtgtacaccaacgaggcttttcaccccgatatcgtgctgcttccggggtgcggagtggactttacgcagagccgcttgagtaacctgttaggaatcaggaagcgccgtccctttcaggagggctttcagattatgtatgaggacttggagggaggtaatattccaggcctgctagacgtgccggcctatgaacaaagcttacaacaggcccaagaggagggaagagtcactcgcggagacacctttgccacggctcccaacgaggtagtgattaagcccttattgaaagacagtaaggatagaagttataatattataaccgacaccacggacactttgtaccggagttggtttctggcttacaactacggggaccccgaaaacggagtgagatcatggaccatactcaccaccacggacgtgacctgcggctcgcagcaagtgtactggtccctgccggatatgatgcaagacccagtcaccttccgcccctccacccaagtcagcaactttccggtggtgggcactgagctgttgcccgttcacgccaagagcttctacaacgagcaggctgtttattcgcaactcattcgccagtctaccgcgcttacccacgtattcaaccgtttccccgagaaccagattctcgtgcgccctcccgctcctaccattaccaccgtgagtgaaaacgttcccgccctcacagatcacggaaccctgccgctgcgcagcagtatcagtggagttcagcgcgtgaccatcaccgacgccagacgtcgaacctgcccttacgtttacaaagcgctcggcgtagtggccccaaaagtgctctctagtcgcaccttctaaaacatgtccattctcatctctcccgataacaacaccggctggggactgggctccggcaagatgtatggcggggcgaagcggcgctccagtcagcaccctgttcgcgttcggggtcatttccgcgctccctggggagcttacaaacgaggactctcgggccgaacggcggtagacgacaccattgacgccgtcattgccgatgcccgccggtataaccccggaacggtcgctagcgccgcctccaccgtggattccgtgatcgacagcgtggtggccggcgccagggcctacgctcgccgcaaaaggcggctgcaccgcaggcgtcgacccacggccgccatgctggccgccagggccgtgctgagacgggcccgcagggtaggcaggagggccatgcgccgcgcggccgccaacgctgccgccgggagggcccgcaggcaagccgccagccgggccgccgccgccatcgctaacatggccagacccaggagagggaacgtttactgggtgcgcgattctgtgacgggagtcagagtgccggtgcgcagccgacctccccgaagttagaagaccaaaggtgcgaagacggcgtactgagtctccctgttgttatcagcccaacatgagcaagcgcaagtttaaagaagaactcctgcagaccctggctcctgaaatctatggccctccggacgtgaagcccgacattaagccccgcgatatcaagcgtgttaaaaagcgggaaaaaaaagaggaactcgcggtggtagacgatggcggggtagaatttattagaagtttcgccccgcgacgcagggtgcagtggaaagggcggcgcgtgcaacgcgttctcaggccaggcaccgcggtagtttttactccgggagagcggtcggctgtcaggggtttcaagcggcaatatgacgaggtgtacggcgacgaagacatcctggaacaggcggctcagcagattggagaattcgcctacggaaagcggtctcgccgcgaagacctggccattgccttggacagtggcaaccccacccccagcctcaaacccgtcacgctgcagcaggtgctccccgtgagcgcgagcacggagagcaaaaggggaatcaagagagagatggaagatctgaagcccaccatccaacttatggtccctaaacgacagaagctggaggaggttctggaaaacatgaaagtggaccccagcatagagccggatgtaaaagtgaggcctattaaggaagtggctccgggtctcggggtgcaaacggtggacattcagatcccagtcagatccgcttcgaccgccgtggaagccatggaaacgcaaaccgaaactccggtcgcggccggtaccagagaagtggctttgcaaacggagccctggtacgaatacaccgctcctcggcgccagaggcggcgttacggcccggcaaatgccatcatgccagagtatgcgctgcacccgtctatccgacccacccccggctaccggggggtaacgtatcgcccgtcgccaacccgacgccgttatcgtcgccgccgccgttctcgtcgcgctctggcgcccgtgtccgtgcgacgcgtaacgcgccggggaagaacagtcaccatccctaacccgcgctaccaccctagcattctttaatgactctgccgttttgcagatggctctgacttgccgcgtgcgccttcccgttctgcactatcgaggaagatctcgtcgtaggagaggcatggcggggagcggccgccgtcgggctttacgcaggcgcatgaaaggcggaattttgcccgcactgattcccataattgccgccgccattggggcgatacccggcgttgcttcagtggccttgcaagcagctcgtaataaataaacgaaggcttttcaacttatgacctggtcctgactattttatgcagaaaaagcatggaagacatcaattttacgtcgctggctccgcggcaaggctcacgcccgctcatgggcacctggaacgacatcggcagcagccagctcaacgggggcgctttcaattgggggagcctttggagcggcattaaaaactttggctccgcgattaaatcctacggcagcaaagcctggaacagtagtactggtcagatgctccgggataaactgaaggacacaaactttcaagagaaagtggtcaacggggtggtgaccggcatccacggcgcggtggatctcgctaatcaagcggtgcaaaaagagatagacagacgatgggaaaactcgcgggtgcctccgcagagaggggacgaagtggaggtggaggaagtagaagtcgaggagaaactgcccccgctagagaaagttcccggggcgccgcccaggccacagaagcgtccccggccggatctggaagaaactttagtgacggaaaccatcgaacctccctcgtacgaacaagctttaaaggagggcgcctctccttaccccatgactaagcccatcgcgcccatggcgcgtccggtgtacggaaaagatcacaagccagtaacgttagagctacccccaccacccccttcccgtcctacggtgcctccgttacccgccccgtcggcaggtcccagctctgcaccatccgcagctcctgcaccaaccgctcgcccggtggccgtggcaaccgccagagcccccagaggatccaactggcaaagcacgctgaacagcatcgtgggcttgggagtgaaaaccctaaaacgccgccgctgctattattaaagagtgtagctaaaaatttcccgttgtatacgcctcctatgttaccgccagagacgcgtgactggtcgccgctccgccgctttcaagatggccaccccatcgatgatgccgcagtggtcttacatgcacatcgccggccaggacgcctcggagtacctgagtcccggcctggtgcagtttgcccgcgccaccgaaagctacttcagcttgggaaacaagtttagaaaccccaccgtggcccccacgcacgatgtaaccacggaccgctcgcagaggctgacacttaattaattcgaacccataatacccataatagctgtttgccatcgacgcgaggctggatggccttccccattatgattcttctcgcttccggcggcatcgggatgcccgcgttgcaggccatgctgtccaggcaggtagatgacgaccatcagggacagcttcaaggccagcaaaaggccaggaaccgtaaaaaggccgcgttgctggcgtttttccataggctccgcccccctgacgagcatcacaaaaatcgacgctcaagtcagaggtggcgaaacccgacaggactataaagataccaggcgtttccccctggaagctccctcgtgcgctctcctgttccgaccctgccgcttaccggatacctgtccgcctttctcccttcgggaagcgtggcgctttctcatagctcacgctgtaggtatctcagttcggtgtaggtcgttcgctccaagctgggctgtgtgcacgaaccccccgttcagcccgaccgctgcgccttatccggtaactatcgtcttgagtccaacccggtaagacacgacttatcgccactggcagcagccactggtaacaggattagcagagcgaggtatgtaggcggtgctacagagttcttgaagtggtggcctaactacggctacactagaaggacagtatttggtatctgcgctctgctgaagccagttaccttcggaaaaagagttggtagctcttgatccggcaaacaaaccaccgctggtagcggtggtttttttgtttgcaagcagcagattacgcgcagaaaaaaaggatctcaagaagatcctttgatcttttctacggggtctgacgctcagtggaacgaaaactcacgttaagggattttggtcatgagattatcaaaaaggatcttcacctagatccttttaaattaaaaatgaagttttaaatcaatctaaagtatatatgagtaaacttggtctgacagttaccaatgcttaatcagtgaggcacctatctcagcgatctgtctatttcgttcatccatagttgcctgactccccgtcgtgtagataactacgatacgggagggcttaccatctggccccagtgctgcaatgataccgcgagacccacgctcaccggctccagatttatcagcaataaaccagccagccggaagggccgagcgcagaagtggtcctgcaactttatccgcctccatccagtctattaattgttgccgggaagctagagtaagtagttcgccagttaatagtttgcgcaacgttgttgccattgctgcaggcatcgtggtgtcacgctcgtcgtttggtatggcttcattcagctccggttcccaacgatcaaggcgagttacatgatcccccatgttgtgcaaaaaagcggttagctccttcggtcctccgatcgttgtcagaagtaagttggccgcagtgttatcactcatggttatggcagcactgcataattctcttactgtcatgccatccgtaagatgcttttctgtgactggtgagtactcaaccaagtcattctgagaatagtgtatgcggcgaccgagttgctcttgcccggcgtcaacacgggataataccgcgccacatagcagaactttaaaagtgctcatcattggaaaacgttcttcggggcgaaaactctcaaggatcttaccgctgttgagatccagttcgatgtaacccactcgtgcacccaactgatcttcagcatcttttactttcaccagcgtttctgggtgagcaaaaacaggaaggcaaaatgccgcaaaaaagggaataagggcgacacggaaatgttgaatactcatactcttcctttttcaatattattgaagcatttatcagggttattgtctcatgagcggatacatatttgaatgtatttagaaaaataaacaaataggggttccgcgcacatttccccgaaaagtgccacctgacgtctaagaaaccattattatcatgacattaacctataaaaataggcgtatcacgaggccctttcgtcttcaagaattggtcgatggcaaacagctattatgggtattatgggttcgaattaat

SEQ ID NO: 48 - DNA, 21377 bp, Artificial Sequence
  Synthetic oligonucleotide pBr/sAd4312.pV-rITR
attaaccgaagttagaagaccaaaggtgcgaagacggcgtactgagtctccctgttgttatcagcccaacatgagcaagcgcaagtttaaagaagaactcctgcagaccctggctcctgaaatctatggccctccggacgtgaagcccgacattaagccccgcgatatcaagcgtgttaaaaagcgggaaaaaaaagaggaactcgcggtggtagacgatggcggggtagaatttattagaagtttcgccccgcgacgcagggtgcagtggaaagggcggcgcgtgcaacgcgttctcaggccaggcaccgcggtagtttttactccgggagagcggtcggctgtcaggggtttcaagcggcaatatgacgaggtgtacggcgacgaagacatcctggaacaggcggctcagcagattggagaattcgcctacggaaagcggtctcgccgcgaagacctggccattgccttggacagtggcaaccccacccccagcctcaaacccgtcacgctgcagcaggtgctccccgtgagcgcgagcacggagagcaaaaggggaatcaagagagagatggaagatctgaagcccaccatccaacttatggtccctaaacgacagaagctggaggaggttctggaaaacatgaaagtggaccccagcatagagccggatgtaaaagtgaggcctattaaggaagtggctccgggtctcggggtgcaaacggtggacattcagatcccagtcagatccgcttcgaccgccgtggaagccatggaaacgcaaaccgaaactccggtcgcggccggtaccagagaagtggctttgcaaacggagccctggtacgaatacaccgctcctcggcgccagaggcggcgttacggcccggcaaatgccatcatgccagagtatgcgctgcacccgtctatccgacccacccccggctaccggggggtaacgtatcgcccgtcgccaacccgacgccgttatcgtcgccgccgccgttctcgtcgcgctctggcgcccgtgtccgtgcgacgcgtaacgcgccggggaagaacagtcaccatccctaacccgcgctaccaccctagcattctttaatgactctgccgttttgcagatggctctgacttgccgcgtgcgccttcccgttctgcactatcgaggaagatctcgtcgtaggagaggcatggcggggagcggccgccgtcgggctttacgcaggcgcatgaaaggcggaattttgcccgcactgattcccataattgccgccgccattggggcgatacccggcgttgcttcagtggccttgcaagcagctcgtaataaataaacgaaggcttttcaacttatgacctggtcctgactattttatgcagaaaaagcatggaagacatcaattttacgtcgctggctccgcggcaaggctcacgcccgctcatgggcacctggaacgacatcggcagcagccagctcaacgggggcgctttcaattgggggagcctttggagcggcattaaaaactttggctccgcgattaaatcctacggcagcaaagcctggaacagtagtactggtcagatgctccgggataaactgaaggacacaaactttcaagagaaagtggtcaacggggtggtgaccggcatccacggcgcggtggatctcgctaatcaagcggtgcaaaaagagatagacagacgatgggaaaactcgcgggtgcctccgcagagaggggacgaagtggaggtggaggaagtagaagtcgaggagaaactgcccccgctagagaaagttcccggggcgccgcccaggccacagaagcgtccccggccggatctggaagaaactttagtgacggaaaccatcgaacctccctcgtacgaacaagctttaaaggagggcgcctctccttaccccatgactaagcccatcgcgcccatggcgcgtccggtgtacggaaaagatcacaagccagtaacgttagagctacccccaccacccccttcccgtcctacggtgcctccgttacccgccccgtcggcaggtcccagctctgcaccatccgcagctcctgcaccaaccgctcgcccggtggccgtggcaaccgccagagcccccagaggatccaactggcaaagcacgctgaacagcatcgtgggcttgggagtgaaaaccctaaaacgccgccgctgctattattaaagagtgtagctaaaaatttcccgttgtatacgcctcctatgttaccgccagagacgcgtgactggtcgccgctccgccgctttcaagatggccaccccatcgatgatgccgcagtggtcttacatgcacatcgccggccaggacgcctcggagtacctgagtcccggcctggtgcagtttgcccgcgccaccgaaagctacttcagcttgggaaacaagtttagaaaccccaccgtggcccccacgcacgatgtaaccacggaccgctcgcagaggctgacactgcgcttcgtgcccgtagaccgggaggacaccgcgtactcctacaaagtgcgcttcaccctcgccgtaggggacaacagggtgctggacatggccagcacgtactttgacatccggggaatgctggaccgagggcccagctttaaaccctactcgggaactgcctacaattcgctggcacctaagggcgctcccaaccctagtcaatggactactaccaacggagggaataaaacaaattcatttgcccaagcatcctacataggtcaaagcctgtcgaaagacggggtgcaagtagcagtagatacagccgctgggggggctgcagtatatgctgacaaaacgtttcaaccagaaccccaagtaggaatatcacaatggaatgaaaatcctactacaaatgctgcaggaagaattttaaagcctactaccgcaatgcgtccatgctacggttcatacgcttaccccaccaacgaaaaaggtgggcaggtaaaaatcactgaccctaacaatgacaaaaccggcgctaataacgttagcttaaattttttcaacactgccgctgacaatgggaataacaatccaaaagtagtactctacagcgaagatgtaaatttagaagggccagatacccaccttgtttttaagccagatgtaactggcgacgcaaccagtgcagaaaccctgttaggtcaacaagcagctcccaatcgtccaaactacattgggttcagggacaactttattggcctgatgtactacaattcaactggaaacatgggagtgctagcaggtcaggcttctcagctaaacgccgtagtggatcttcaagacagaaataccgaattgtcatatcagctaatgcttgacgctttgggtgacagaagtcggtacttttctatgtggaatcaagcagtggacagctacgatcctgacgttagaatcatagaaaatcatggagtagaagacgaacttccaaattattgttttccgttaaatggacaggggatttcgaatacatacaaaggtgtgaaatataacacaaacacttggacgcaagacactgatgtagtcacaaccaatgaaatttccattggcaacatttttgccatggaaataaacctggcggctaacttgtggcgcagctttctgtactccaatgtcgccctgtacttgccagattcctacaaatacactcccgacaatattgaacttcctacaaacaagaacagctacggctacattaacggaagggtaaccgcccccactgccatcgacacttacgttaacatcggcgcccggtggtctccggaccccatggacaacgttaaccctttcaaccaccaccgcaacgccggcttgcgataccgctccatgctgctgggcaacggtcgctacgtacccttccacattcaggtgccccagaaattttttgccattaaaaacctgcttctgcttcccgggtcctacacctacgagtggaacttcaggaaagatgtaaacatgatcttgcagagcaccttgggcaacgacctccgcgttgacggagctagcgtgaggtttgacagcattaacctctacgctaacttcttccccatggcccacaacacggcctccaccttggaagccatgctgcgcaacgacaccaacgaccagtcctttaatgattacctgtgcgcggccaacatgctgtaccccatccccgccaatgccaccagcgtgccgatctccattccctcacgcaactgggccgccttcagaggttggagtttcactcgcctgaaaaccaaggagaccccctcgctgggctccggtttcgacccatactttgtttactccgggagcattccctacctggacggaactttctacctgaaccacaccttcaaaaaggtgtctattatgtttgactcctccgtgagctggcccggtaacgaccgcttgctaacccccaacgagttcgaaatcaaacgctcggtggacggagagggttacaatgtagcccagagcaacatgaccaaagactggtttttaattcaaatgctaagccactataacattggctaccaaggattctacgtgcctgaagcctacaaggacagaatgtactccttctttagaaacttccaacccatgagccgccaggtagtagacacggtaaactatgctaactacaaggaagtaacaatgccattccagcacaacaactcaggcttcgtggggtacatgggacctaccatgagagaggggcaggcctacccggctaattatccctaccccctaatcggagccactgccgtgcccagcctgacacagaaaaagtttctctgcgatcgaacaatgtggaggattcccttctctagcaacttcatgtccatgggggctctcaccgacctggggcagaacatgctgtacgctaactccgctcacgccttggacatgacctttgaggtggaccccatggatgagcccacgcttctctatgttctgtttgaagtcttcgacgtggtgcgcattcaccagccgcaccgcggcgtcatcgaggccgtctacctgcgcacacctttctctgccggtaacgccaccacctaagaagctgatgggctccagcgaacaggagctgcgggccattgttcgcgacctgggctgcgggccctactttttgggcaccttcgacaagcgcttccccggcttcatgtccccccacaagccggcctgcgccatcgtcaacacggccggacgcgagaccgggggggttcactggctcgcctttgcctggaacccgcgtaaccacacctgctacctgttcgacccttttggtttttctgacgaaaggcttaaacagatttaccagttcgagtacgaggggctccttaaacgcagcgctctggcctccacgcccgaccactgcgtcaccctggagaagtccacccaaacggttcagggtcccctctcggcggcctgcggactcttttgttgcatgtttttgcatgctttcgtccactggccgaacacccccatggaccgcaaccccactatggatctgctcacgggagtgcctaacagcatgcttcacagccctcaggtcgcacccaccctgcgtcgcaatcaggaacagctgtatgcttttctgggaaaacattctgcctactttcgccgccaccggcagcgcatagaacaggccacggcctttgaaagcatgagtcaaagagtgtaatcaataaaatcaacttttattttacatcacacgcgcttctggcgttttcttaaaaatcaaagggttcgggggaggggtcgtcgtgcccgctgggcagggacacgttgcgatactggaagcgggggctccagcggaactcggggatcgccagccggggcagaggcacttcttccaggttctgcttccaaaactgccgcaccagctggagggctcccattacgtcgggcgccgagatcttgaagtcgcagttggggcccgagcttccgcggctgttgcgaaacacggggttggcacactggaacaccagcacgctcgggtagttgatactggccagggccgttgcgtcggtcaccgccgttacatccagatcctccgcgttggtcagggcgaagggagtcagcttgcacatctgccgcccgatgtggggcacgccgtcatgcttgttgaggcagtcgcaacgcaggggaatcagaatgcgatgctggccgcgttgcatctgagggtagttggcccgcaagaacgcttccatctgacggaaggccgtctgggctttcattccctcggtgtagaaaagaccgcaggacttgctagaaaatacattattgccgcaggtgacgtcttccgcgcagcagcgggcgtcttcgttctttagctgcaccacgttgcgaccccaccggttctgtaccaccttggccctcgtgggctgctccttcagcgcccgctggccgttttcgctggtcacatccatttccaacacgtgctccttacacaccatttccactccgtggaagcagaacaggacgccctcctgctgggtattgcgatgctcccacacggcgcagcctgtggcctcccagctcttatgcttcacccccgcgtagttttccatgtaagccatcaggaatctgcccatcatctcggtaaaggttttctgactggtgaaggtcaaaggcaagccgcggtgctcttcgttcagccacgtttgacagatcttgcggtacgtggcgccctgatccggcagaaacttaaacgcccccttgctctcgttgtccacgtggaacttttccatcagcattagcataacttccatacccttctcccacgccgtcaccagcggtgtgctgtcggggttcttcaccaacatggtagaagggccctcgccggccctgaagtcgctcatactcattttttgaaactccacagtgccgtccgcacgacggacccggcgcatcggagggtagctgaagccaacctccaccagggtgccttcgctctcgctgtcggagacgatctccggggagggcggcggcgcgggtgtcgacttgcgagccttcttcttgggaggaagcggtggcgcctcttggtcgcgctcgggactcatctccctcaagtagggggtgatggagcttcctgcttggttctgacggttggccattgtatcctaggcagaaacacatggagcttatgcgcgaggaaactttaaccgccccgtcccccgtcaacgacgaagaggtcatcatcgaacaggacccgggctacgttactccgcccgaggatctggaggggcctttagacgaccggcgcgacgctagtgagcagcaggaaaatgagaaagaggaagcctgctacctcctggaaggcgacgtgttgctaaaacatttcgccaggcagagcaccatagtgaaggaggctttgcaagaccgctcggaggtgcccttggacgtcgccgcgctctcccaggcctacgaggcgaacctcttctcgccccgagtgcctccgaagagacagcccaacggcacctgcgagcccaacccgcgccttaacttctaccccgtgttcgccgtgcccgaggcgctggccacctaccacatttttttcaagaaccagcgcatcccgctctcgtgccgggccaaccgcaccgcggccgatagaaagctgagactcaaaaacggagctagcatacctgatatcacgtccctggaggaagtgcctaagatcttcgaaggtctgggtcgagacgagaaacgggcggcaaacgctctgcagaaagaacagaaggacagtcagaacgtgctggtggaactggagggggacaatgcgcgtctggccgttctcaagcgctgcatagaagtttcccacttcgcctaccctgccctgaacctgccgcccaaagtcatgcgctcggtcatggaccagctgctcatcaagagagctgagcccctgaaccccgagcaccccgaggcggagaactcggaggacggaaagcccgtcgtcagcgacgaggagctcgagcggtggctggacagcacggaccccgagcagttgcaagagcggcgcaaaatgatgatggcggccgtcctggtcaccgttgagctggagtgcctgcagcggttttttagcgacgtggaaacgctgcgtaaaatcggagagtccctgcactacaccttccgccagggctacgtccgccaggcctgcaagatctccaacgtggagctcagcaacctggtctcctacatgggcatcctccacgagaaccggctgggacagagcgtgctgcactgcaccttgcaaggcgaggcgcggcgggactacgtgcgagactgcgtctacctcttcctcactctcacctggcagaccgccatgggagtgtggcagcagtgcttggaagacagaaacctcaaagagctagacaaactcctctgccgccagcggcgcgccctgtggtccggtttcagcgagcgcacggtcgccagcgctctggcggacatcatcttcccggagcgcctgatgaaaaccttgcaaaacggcctgccggatttcatcagtcaaagcattttgcaaaacttccgctcttttgtcctggaacgctccgggatattgcccgccatgagctgcgcgctaccttctgactttgtccccctctcctaccgcgagtgccctcccccactgtggagccactgctacctcttccaactggccaactttctggcctaccactccgacctcatggaagacgtaagcggagagggtttactggagtgccactgccgctgcaacctgtgcaccccccacagatcgctggcctgcaacaccgagctactcagcgaaacccaggtcataggtaccttcgagatccaggggccccagcagcaagagggtgcttccggcttgaagctcactccggcgctgtggacctcggcttacttacgcaaatttgtagccgaggactaccacgcccacaaaattcagttttacgaagaccaatctcgaccaccgaaagcccccctcacggcctgcgtcatcacccagagcaagatcctggcccaattgcaatccatcaaccaagcgcgccgcgatttccttttgaaaaagggtcggggggtgtacctggacccccagaccggcgaggaactcaacccgtccacactctccgtcgaagcagcccccccgagacatgccgcccaagggaaccgccaagcagctgatcgctcggcagagagcgaagaagcaagagctgctccagcagcaggtggaggacgaggaagagatgtgggacagccaggcagaggaggtgtcagaggacgaggaggagatggaaagctgggacagcctagacgaggaggaggacgagctttcagaggaagaggcgaccgaagaaaaaccacctgcatccagcgcgccttctctgagccgacagccgaagccccggcccccgacgcccccggccggctcactcaaagccagccgtaggtgggacgccaccgaatctccagcggcagcggcaacggcagcgggtaaggccaaacgcgagcggcgggggtattgctcctggcgggcccacaaaagcagtattgtgaactgcttgcaacactgcgggggaaacatctcctttgcccgacgctacctcctcttccatcacggtgtggccttccctcgcaacgttctctattattaccgtcatctctacagcccctacgaaacgctcggagaaaaaagctaaggcctcctccgccgcgaggaaaaactccgccgccgctgccgccgccaaggatccaccggccaccgaagagctgagaaagcgcatctttcccactctgtatgctatctttcagcaaagccgcgggcagcaccctcagcgcgaactgaaaataaaaaaccgctccttccgctcgctcacccgcagctgtctgtaccacaagagagaagaccagctgcagcgcaccctggacgacgccgaagcactgttcagcaaatactgctcagcgtctcttaaagactaaaagacccgcgctttttccccctcggccgccaaaacccacgtcatcgccagcatgagcaaggagattcccaccccctacatgtggagctatcagccccagatgggcctggccgcgggggccgcccaggactactccagcaagatgaactggctcagcgccggcccccacatgatctcacgagttaacggcatccgagcccaccgaaaccagattctcttagaacaggcggcaatcaccgccacaccccggcgccaactcaacccgcctagttggcccgccgcccaggtgtatcaggaaaatccccgcccgaccacagtcctcctgccacgcgacgcggaggccgaagtcctcatgactaactctggggtacaattagcgggcgggtccaggtacgccaggtacagaggtcgggccgctccttactctcccgggagtataaagagggtgatcattcgaggccgaggtatccagctcaacgacgagacggtgagctcctcaaccggtctcagacctgacggagtcttccagctcggaggagcaggccgctcttccttcaccactcgccaggcctacctgaccctgcagagctcttcctcgcagccgcgctccgggggaatcggcactctccagttcgtggaagagttcgttccctccgtctacttcaaccccttctccggctcgcctggacgctacccggacgccttcattcccaactttgacgcagtgagtgaatccgtggacggctacgactgatgacagatggtgcggccgtgagagctcggctgcgacatctgcatcactgccgtcagcctcgctgctacgctcgggaggcgatcgtgttcagctactttgagctgccggacgagcaccctcagggtccggctcacgggttgaaactcgagatcgagaacgcgctcgagtctcgcctcatcgacaccttcaccgcccgacctctcctggtagaaatccaacgggggatcactaccatcaccctgttctgcatctgccccacgcccggattacatgaagatctgtgttgtcatctttgcgctcagtttaataaaaactgaactttttgccgcaccttcaacgccacgcgttgtttctccaacagtcgacgatagctcttcaattaaaggtacccgagaaactgtttattttgacaattctactacttctcttatccttaactgttcttgcactaacgaactaattcagtggttcgccaacggttcactctgcaaagttttccttgactctgcgatacttcccggatttagcagctctgcgtgtgataattctaccccctccaccttaaccatcacaaagccattttcagaagtccagtatttttgtattggagcggggggtaaaccgggctgtattcaccgcttctttctggagacatttgttgcttcgattcccattaacacttcactttcctctaatacatacttaactaccttacattctactcacccctcctggaaacctcttattggcctcacagcttttatttccgttgttttactaaactttataattcttaacaaactttcttaaacatgcttgccattttgcttctgctcgttactttaacctccgcagattaccacaatgcaattgtacgagaaaacagtttacaaaacccatcacaggtatatgttaaagcaggttctaacttaactctacaatccttctattcgccttaccctgaggacatgccacgtgtcacctggtacttagaagtttttgattcgctatttgaaagacatacaattcctccattttttacaggcgttatactttgtgacatttctggtgacatacagcatgtgtggaaccattggcctttacaatttaattgcataaataaaagcttacatattatcaatctcaaaccaagtgatgaaggcctttacaatgtgaaggttttaaagggcagcattcagcataatacatactttcgtgtgcatgtagtaagttttccaaaacctgaatgtaacatcaccactacatatctttcagatgactactgccttattaacattgattgctctcaattaccataccctgctaaggtctattataatggcaatgaaagtaagctgcattactacttatctgaacgcggtggccaaccaaaccttccaaattactttactgttgggtatcgatatagagatctccgacagaattatacagttgaatatccatttaatgaactctgtacagatataattgctcttgaaacagggtctgattttacgccaatttttatagttaccctagtggtgagcattatagttattgtgatgggcatcacatatcttatttatcactgtaggactttaaaaaccaaaaccaaaaccaagcctcctgaaatccgtctgctttaattttttccagaatggtagctgctttcttcattctcctctgtataccaatcatctgcgcctccacaacttttgccgctgtttcccacctggaaccagactgtctaccaccttttgttgtatacctaatactgacttttgtggtctgtacagccattaccagtatagcctgcttttttgtaacaattttccaagccgccgattacctctacgtacggtttgcttactttagacatcaccccgagtatcggaatcaaaacgtagcctctctgctttgtttagcatgattcgcatttttatactttgtaagctctttaccaccacaatatgtcaatgcccttttaccaaaccctggtccttttacacttgttataatgtattacccgaaacccccattgcctggctttacgtagccacagcggctttagtttttgtagcaacctgcattggcgttaaactgtacttttacttaaaaattggatggcttcatcccccagaagatttaccccgatatcctcttgttaataactttcaacagcctctaccgcctcctgatcttccgcgagctccctccgttgttagctactttcaactcaccggtggagatgactgacactcaggacattaacattactgtggaaagaatagctgctcagcgtcagcgagagacgcgggtgatggagtacgtggaactacagcagcttaaagagtcccactggtgtgaaaaaggagtgctttgccatgttaagcaagcagccctttcttacgatgtcagcactcagggacatgaactgtcctacactttgcctttacagaaacaaaccttctgcaccatgatgggctctacctccattacaatcagccaacaaaccggacctgtcgagggggctatcctgtgtcactgtcacgcgcctgattgtatgcccaaactaatcagaactctttgtgctttaggtgatatatttaaaatatagatagtatcaataaacttaccttaaatttgacagcaattttttggtatcatcattcagcagcaccactttaccctcttcccaactctcatatgggatatgatggtgggcggcaaacttcctccaaaccctgaaagaaatatcggtatccacttccttgtcctcacccacaattttcatcttttcatagatgaaaagaacccgagttgatgaagacttcaaccccgtctacccttatgacaccacaaccactccagccgttcctttcatatcacccccgtttgtaaacagtgacggtcttcaggaaaacccccccggagttttaagcctgcgaatagctaaacccctgtattttgacatggagagaaaactagccctttcacttggaagagggttaacaattaccgcgaacggacaattagaaagcacccagagcgtgcagactaacccgccgttaactgtcaccaataacaacacacttatcctacgccactcctcccctttaatcctaactgacaataatttaaccgtaggcttctcaagtcctctccgtgttatagacaacaaactgacattcacttttacctcacctctccgttatgaaaacgaaacccttaccttcaattacacagagccccttacacttatgaacagcaaccttgcgcttaacgtaaactcctctaaaggccttagggttgacgggggctcactaggtacaaacttaagtccggacttaaggtttaacagcagtggagccatagcttttggtatacaaaccctatggacacccccgacctcaaatcctaactgcaccgtttacaccgaaagcgattccttacttagtctctgcttaactaaatgcggagctcacgttttaggaagtgtaagcttaaccggggtagcaggtaccatgataaacatggctgaaacttcgcttgctattgaatttacgtttgacgacactggaaaactacttcactcaccacttgttaacaccacttttagcattcgtcagggcgacagccccgcctcaaatcctacctacaatgctctagcatttatgccaaacagtaccctctacgctagaggaggaagtggtgaaccccgaaacaattactacgtccaaacatacctcaggggaaatgttcagagaccgattaccctcactgttactttcaactcagccgccacgggatattccttatcttttaagtggactgctgttgcacgtgaaaaatttgcagctcctgcaacttcattttgctacattaccgaacaataaaaccctgtgttcccaccgtttcgttttttccagatgaaacgggccagagttgatgaagacttcaatcccgtgtacccttacgatcccccttacgcccccattatgccgtttattaccccgccgtttacatcttcagatgggttacaggaaaaaccacttggtgttttaagtttaaaatacaaggatcctatcactacacaaaatggttctctaacccttaaattaggaaacgggctgaacattaacaaccagggccaacttacatcatctgctggggaagtcgagcctcccctcaccaatgctgacaacaagctggccttagcctacagcgaccctctgacattaaaaaacagccgtctaacactgtctcacaatgccccacttgcaattaacaataattctctaagtttggaagtatcagagcctatatttataaataacgacaacaaactgtctctgaaagctgacgcccccctgacaaccagcgctggaaccctccgcctgcaaagcgctgctccattaggacttgctgaacagacactaaagctgctgttttctaaccctttgtacttgcgaggtgacttccttacattagccattgaacgcccattggctgtaacagcagacgggctattatcacttgccctcaaccctccgctcacaacaactaacacaggcttagctctctctaccgcggttccattaactgttaccaacgggaaccttagcctaaacgtaaaacggccgtttattatacaggacggcagcctttacatggattttagacccccactatatctgtttaacagcgagccacaacttggtgttaattttaatgcccctctaactgttagagataacggcctagctataaacaccggagacgggctaacagtaacgtataataaactaacattaaacctcggtagagacttgcaatatgaaaatggagctgcagctgttaagctaagtaccgcccctcctctacagtatactactcaactgcagctgaatttgggagcgggcttacgtctaggtcctactaggaacttagacgtggccattaaccacaataaagggttagcgtgggaaaacaatgaagtggttactaaattaggacaaggcctttactttgattcctccggaagcatagctttatcgcctacaaaccccagaccagatactttatggaccacggccgatccttcgccaaactgcactgtatatgaatcacttgactctagactgtggctagcgcttgttaaatgtgggggaatggtacacggcagcatagccctacaagctgaaaaaggccaattgctgcgtcctactgctagttttatctccatcgtaatttacttctacagtgatggggtccgtcgcaccaactaccctacaattggcaatgatgagggtactctggccaacagcgctacttggggctacagacaagggcaatctgcagacaccaacgtcaccaatgctgttgaattcatgcctagtttacacagatatcctataaatcagggagacaatattaaaaaccaaatgataacttacacttgcatacaaggcaacgtgaacatgccagtacccttgaaaatcacgttcaatcatgctcttgaaggctactccttaaagtttacatggcgtgtggtggctaatgaaaagtttgatattccttgctgttcgttttcttacattacagaacaataaaacaacttttttatttttcatttcttttattttacacgcacagtaagacttcctccccccttccatttaacagcgtacaccagcctttcccccttcatggcggtaaacttctgtgagttagtccggtatttgggagttaaaatccaaacaggctctttggtgattaaacgttgatccgtgatggacacaaatccctgagacaggtcctccaacgttgcggtaaaaaactgaacgccgccctacaaaacaaacagttcaggctctccacgggttatcaccccgatcaaactcagacagagtaaaggtgcggtgatgttccacaagaccgcgcaagtggcgctgtctaaagctctcagtgcgacttctatgcggctggtaggatgttacattatccaacagcctcacagcgcggattattagtctacgagtgcgcctggcgcagcagcgcatctgaatttcagtcaagtcttgacaagaagcgcataccataacaatcaggttgttcatgatcccatagctaaacgcgctccagccaaaactcattcgctccaacagcaccaccgcgtgtccgtcaagtcttacttttacataaacaaggtgtctgccacgtacatacatgctacccgcatacaaaacttcccggggcaaacctctattcaccacctgtctgtaccagggaaacctgatgtttatcagggaaccatagatggccattttaaaccagttagccagcaccaccccgccagctctacactgaagggaaccgggagagttacaatgacagtggatcatccacctctcgtaacccctaattacctgattaaaatccaaatctaacgtggcacaacagatacacactctcataaacattttcatgacatgtttttcccaggatgttaaaatacaatcccaatacacgggccactcctgtaatacaataaagctaatgcatgatggaacgctcctcacctcactaacattgtgcatgtttacattttcacactctaagtaccgagtcctctcctcaacagccgcagtgtcgcgctcctcacacggtggtagctgatgacaattgtaaggggccagtctgcagcgatatcgtctgtcgcgctgcatcgtaaaacagggaccgtctcacttcctcgtacttccaatagcagaaccacgtccgctgccagcaggtttccacgaaccgccgatcccttcgtcgttcacgctccctcctcaacgcaaaatgcagccactcctgcaatccacacaaatccctctcggcctccggagtcatgcacacctcatacctatatatgtctcggtacagttccaaacacgaagtaagggcgagctccaaccaacacaaacaggctgatttatcccgacacactggaggtggaggaagacacggaagaggcatgttattccaagcgatccggcaaaggatcaaagtgcagatcccgaagatggcaacgctcgcctccggagccctggtgaaatttaacggccaaatcaaacattatgcggttttccaaactatcaatcgccgcctccaaaagggcctgaacccgcacttccacaatcaccagcaaagcaaaagcgtgattatcaaagtcttcaatcatcagatggcatgactgtacaatgcccaaataattctcatttctccactcgcgaatagtgtcgcggcagatcgtctgaaggtccatgccatgcatgttaaaaagctcccagagggcgccctctaccgacatgcgtagacacaccatcatgactgcaaaatatcaggctcctgagacacctgcagcagatttaacagatcaaagtcaggttgctgtccgcggtcacgaatctccatgcgcaaagccatttgcaaaaaattatataggtctgtgccaactagctctgttaattccgcgttaggaagcaaatcaggtgaggctatgcagcacaaaagttgcagggaaggcgccaaactcagtaaaaccgctccagaataacaaaattgatgaagcggagtcacacagtgtaaaatgtgcaaccaaaaatcattcagctgctcttttaaatagtccagtacttctatattcaatccgtgcaagtactgaagcaactgcgcgggaacagtcacattaaaaaaaatggggcggctcaaatacatgtcgacctaaaataaaaataatcattaaaccagagaagcttgacgaatggaaggataaaatacacgctccagcaaaaggcaggcaaccggctgtccccgagaaccgtaaaaaaattcatccgaatgattaaaaagaaccacagaaatttcccaccatgtactcggttgtaactcctgagcacacagcaacacccccctaacgttcatgtccgccactgaaaaaagacgtcccaaatacccaggtggaatgtcaagagacaactgcagagacagcaaaacaacccctctgggagcgatcataaactcctccggtgagaaaagcgcatacaaattagaataaccctgttgctggggcaaaatagcccggcggcccagcaaatggacataaatatgttcagcagccatcgccccgtcttaccgcgtaaaaagccagaaaaatccagctaactacactctacagcctattactatatatactctcctcccactgacgctataccaccccgcccacgtccaaagttcacccacgcccaaaaaacccgcgaaaatccagcgccgtcagcacttccgcaattgtagtctctcaacgtcacttccgcgcgccttttccctattcccacacacgcccgcggacttcgccccgcccgccctcgcgccaccccgcgtcaccccgcgtcaccgcacgtcaccccggccccgcctcgctcctccccactcattatcatattggcacgtttccagaataaggtatattattgatgatgttaattaattcgaacccataatacccataatagctgtttgccatcgacgcgaggctggatggccttccccattatgattcttctcgcttccggcggcatcgggatgcccgcgttgcaggccatgctgtccaggcaggtagatgacgaccatcagggacagcttcaaggatcgctcgcggctcttaccagcccagcaaaaggccaggaaccgtaaaaaggccgcgttgctggcgtttttccataggctccgcccccctgacgagcatcacaaaaatcgacgctcaagtcagaggtggcgaaacccgacaggactataaagataccaggcgtttccccctggaagctccctcgtgcgctctcctgttccgaccctgccgcttaccggatacctgtccgcctttctcccttcgggaagcgtggcgctttctcatagctcacgctgtaggtatctcagttcggtgtaggtcgttcgctccaagctgggctgtgtgcacgaaccccccgttcagcccgaccgctgcgccttatccggtaactatcgtcttgagtccaacccggtaagacacgacttatcgccactggcagcagccactggtaacaggattagcagagcgaggtatgtaggcggtgctacagagttcttgaagtggtggcctaactacggctacactagaaggacagtatttggtatctgcgctctgctgaagccagttaccttcggaaaaagagttggtagctcttgatccggcaaacaaaccaccgctggtagcggtggtttttttgtttgcaagcagcagattacgcgcagaaaaaaaggatctcaagaagatcctttgatcttttctacggggtctgacgctcagtggaacgaaaactcacgttaagggattttggtcatgagattatcaaaaaggatcttcacctagatccttttaaattaaaaatgaagttttaaatcaatctaaagtatatatgagtaaacttggtctgacagttaccaatgcttaatcagtgaggcacctatctcagcgatctgtctatttcgttcatccatagttgcctgactccccgtcgtgtagataactacgatacgggagggcttaccatctggccccagtgctgcaatgataccgcgagacccacgctcaccggctccagatttatcagcaataaaccagccagccggaagggccgagcgcagaagtggtcctgcaactttatccgcctccatccagtctattaattgttgccgggaagctagagtaagtagttcgccagttaatagtttgcgcaacgttgttgccattgctgcaggcatcgtggtgtcacgctcgtcgtttggtatggcttcattcagctccggttcccaacgatcaaggcgagttacatgatcccccatgttgtgcaaaaaagcggttagctccttcggtcctccgatcgttgtcagaagtaagttggccgcagtgttatcactcatggttatggcagcactgcataattctcttactgtcatgccatccgtaagatgcttttctgtgactggtgagtactcaaccaagtcattctgagaatagtgtatgcggcgaccgagttgctcttgcccggcgtcaacacgggataataccgcgccacatagcagaactttaaaagtgctcatcattggaaaacgttcttcggggcgaaaactctcaaggatcttaccgctgttgagatccagttcgatgtaacccactcgtgcacccaactgatcttcagcatcttttactttcaccagcgtttctgggtgagcaaaaacaggaaggcaaaatgccgcaaaaaagggaataagggcgacacggaaatgttgaatactcatactcttcctttttcaatattattgaagcatttatcagggttattgtctcatgagcggatacatatttgaatgtatttagaaaaataaacaaataggggttccgcgcacatttccccgaaaagtgccacctgacgtctaagaaaccattattatcatgacattaacctataaaaataggcgtatcacgaggccctttcgtcttcaagaattggtcgatggcaaacagctattatgggtattatgggttcgaattaat

SEQ ID NO: 49 - DNA, 19308 bp, Artificial Sequence
  Synthetic oligonucleotide pBr/sAd4312.pV-rITR.dE3
attaaccgaagttagaagaccaaaggtgcgaagacggcgtactgagtctccctgttgttatcagcccaacatgagcaagcgcaagtttaaagaagaactcctgcagaccctggctcctgaaatctatggccctccggacgtgaagcccgacattaagccccgcgatatcaagcgtgttaaaaagcgggaaaaaaaagaggaactcgcggtggtagacgatggcggggtagaatttattagaagtttcgccccgcgacgcagggtgcagtggaaagggcggcgcgtgcaacgcgttctcaggccaggcaccgcggtagtttttactccgggagagcggtcggctgtcaggggtttcaagcggcaatatgacgaggtgtacggcgacgaagacatcctggaacaggcggctcagcagattggagaattcgcctacggaaagcggtctcgccgcgaagacctggccattgccttggacagtggcaaccccacccccagcctcaaacccgtcacgctgcagcaggtgctccccgtgagcgcgagcacggagagcaaaaggggaatcaagagagagatggaagatctgaagcccaccatccaacttatggtccctaaacgacagaagctggaggaggttctggaaaacatgaaagtggaccccagcatagagccggatgtaaaagtgaggcctattaaggaagtggctccgggtctcggggtgcaaacggtggacattcagatcccagtcagatccgcttcgaccgccgtggaagccatggaaacgcaaaccgaaactccggtcgcggccggtaccagagaagtggctttgcaaacggagccctggtacgaatacaccgctcctcggcgccagaggcggcgttacggcccggcaaatgccatcatgccagagtatgcgctgcacccgtctatccgacccacccccggctaccggggggtaacgtatcgcccgtcgccaacccgacgccgttatcgtcgccgccgccgttctcgtcgcgctctggcgcccgtgtccgtgcgacgcgtaacgcgccggggaagaacagtcaccatccctaacccgcgctaccaccctagcattctttaatgactctgccgttttgcagatggctctgacttgccgcgtgcgccttcccgttctgcactatcgaggaagatctcgtcgtaggagaggcatggcggggagcggccgccgtcgggctttacgcaggcgcatgaaaggcggaattttgcccgcactgattcccataattgccgccgccattggggcgatacccggcgttgcttcagtggccttgcaagcagctcgtaataaataaacgaaggcttttcaacttatgacctggtcctgactattttatgcagaaaaagcatggaagacatcaattttacgtcgctggctccgcggcaaggctcacgcccgctcatgggcacctggaacgacatcggcagcagccagctcaacgggggcgctttcaattgggggagcctttggagcggcattaaaaactttggctccgcgattaaatcctacggcagcaaagcctggaacagtagtactggtcagatgctccgggataaactgaaggacacaaactttcaagagaaagtggtcaacggggtggtgaccggcatccacggcgcggtggatctcgctaatcaagcggtgcaaaaagagatagacagacgatgggaaaactcgcgggtgcctccgcagagaggggacgaagtggaggtggaggaagtagaagtcgaggagaaactgcccccgctagagaaagttcccggggcgccgcccaggccacagaagcgtccccggccggatctggaagaaactttagtgacggaaaccatcgaacctccctcgtacgaacaagctttaaaggagggcgcctctccttaccccatgactaagcccatcgcgcccatggcgcgtccggtgtacggaaaagatcacaagccagtaacgttagagctacccccaccacccccttcccgtcctacggtgcctccgttacccgccccgtcggcaggtcccagctctgcaccatccgcagctcctgcaccaaccgctcgcccggtggccgtggcaaccgccagagcccccagaggatccaactggcaaagcacgctgaacagcatcgtgggcttgggagtgaaaaccctaaaacgccgccgctgctattattaaagagtgtagctaaaaatttcccgttgtatacgcctcctatgttaccgccagagacgcgtgactggtcgccgctccgccgctttcaagatggccaccccatcgatgatgccgcagtggtcttacatgcacatcgccggccaggacgcctcggagtacctgagtcccggcctggtgcagtttgcccgcgccaccgaaagctacttcagcttgggaaacaagtttagaaaccccaccgtggcccccacgcacgatgtaaccacggaccgctcgcagaggctgacactgcgcttcgtgcccgtagaccgggaggacaccgcgtactcctacaaagtgcgcttcaccctcgccgtaggggacaacagggtgctggacatggccagcacgtactttgacatccggggaatgctggaccgagggcccagctttaaaccctactcgggaactgcctacaattcgctggcacctaagggcgctcccaaccctagtcaatggactactaccaacggagggaataaaacaaattcatttgcccaagcatcctacataggtcaaagcctgtcgaaagacggggtgcaagtagcagtagatacagccgctgggggggctgcagtatatgctgacaaaacgtttcaaccagaaccccaagtaggaatatcacaatggaatgaaaatcctactacaaatgctgcaggaagaattttaaagcctactaccgcaatgcgtccatgctacggttcatacgcttaccccaccaacgaaaaaggtgggcaggtaaaaatcactgaccctaacaatgacaaaaccggcgctaataacgttagcttaaattttttcaacactgccgctgacaatgggaataacaatccaaaagtagtactctacagcgaagatgtaaatttagaagggccagatacccaccttgtttttaagccagatgtaactggcgacgcaaccagtgcagaaaccctgttaggtcaacaagcagctcccaatcgtccaaactacattgggttcagggacaactttattggcctgatgtactacaattcaactggaaacatgggagtgctagcaggtcaggcttctcagctaaacgccgtagtggatcttcaagacagaaataccgaattgtcatatcagctaatgcttgacgctttgggtgacagaagtcggtacttttctatgtggaatcaagcagtggacagctacgatcctgacgttagaatcatagaaaatcatggagtagaagacgaacttccaaattattgttttccgttaaatggacaggggatttcgaatacatacaaaggtgtgaaatataacacaaacacttggacgcaagacactgatgtagtcacaaccaatgaaatttccattggcaacatttttgccatggaaataaacctggcggctaacttgtggcgcagctttctgtactccaatgtcgccctgtacttgccagattcctacaaatacactcccgacaatattgaacttcctacaaacaagaacagctacggctacattaacggaagggtaaccgcccccactgccatcgacacttacgttaacatcggcgcccggtggtctccggaccccatggacaacgttaaccctttcaaccaccaccgcaacgccggcttgcgataccgctccatgctgctgggcaacggtcgctacgtacccttccacattcaggtgccccagaaattttttgccattaaaaacctgcttctgcttcccgggtcctacacctacgagtggaacttcaggaaagatgtaaacatgatcttgcagagcaccttgggcaacgacctccgcgttgacggagctagcgtgaggtttgacagcattaacctctacgctaacttcttccccatggcccacaacacggcctccaccttggaagccatgctgcgcaacgacaccaacgaccagtcctttaatgattacctgtgcgcggccaacatgctgtaccccatccccgccaatgccaccagcgtgccgatctccattccctcacgcaactgggccgccttcagaggttggagtttcactcgcctgaaaaccaaggagaccccctcgctgggctccggtttcgacccatactttgtttactccgggagcattccctacctggacggaactttctacctgaaccacaccttcaaaaaggtgtctattatgtttgactcctccgtgagctggcccggtaacgaccgcttgctaacccccaacgagttcgaaatcaaacgctcggtggacggagagggttacaatgtagcccagagcaacatgaccaaagactggtttttaattcaaatgctaagccactataacattggctaccaaggattctacgtgcctgaagcctacaaggacagaatgtactccttctttagaaacttccaacccatgagccgccaggtagtagacacggtaaactatgctaactacaaggaagtaacaatgccattccagcacaacaactcaggcttcgtggggtacatgggacctaccatgagagaggggcaggcctacccggctaattatccctaccccctaatcggagccactgccgtgcccagcctgacacagaaaaagtttctctgcgatcgaacaatgtggaggattcccttctctagcaacttcatgtccatgggggctctcaccgacctggggcagaacatgctgtacgctaactccgctcacgccttggacatgacctttgaggtggaccccatggatgagcccacgcttctctatgttctgtttgaagtcttcgacgtggtgcgcattcaccagccgcaccgcggcgtcatcgaggccgtctacctgcgcacacctttctctgccggtaacgccaccacctaagaagctgatgggctccagcgaacaggagctgcgggccattgttcgcgacctgggctgcgggccctactttttgggcaccttcgacaagcgcttccccggcttcatgtccccccacaagccggcctgcgccatcgtcaacacggccggacgcgagaccgggggggttcactggctcgcctttgcctggaacccgcgtaaccacacctgctacctgttcgacccttttggtttttctgacgaaaggcttaaacagatttaccagttcgagtacgaggggctccttaaacgcagcgctctggcctccacgcccgaccactgcgtcaccctggagaagtccacccaaacggttcagggtcccctctcggcggcctgcggactcttttgttgcatgtttttgcatgctttcgtccactggccgaacacccccatggaccgcaaccccactatggatctgctcacgggagtgcctaacagcatgcttcacagccctcaggtcgcacccaccctgcgtcgcaatcaggaacagctgtatgcttttctgggaaaacattctgcctactttcgccgccaccggcagcgcatagaacaggccacggcctttgaaagcatgagtcaaagagtgtaatcaataaaatcaacttttattttacatcacacgcgcttctggcgttttcttaaaaatcaaagggttcgggggaggggtcgtcgtgcccgctgggcagggacacgttgcgatactggaagcgggggctccagcggaactcggggatcgccagccggggcagaggcacttcttccaggttctgcttccaaaactgccgcaccagctggagggctcccattacgtcgggcgccgagatcttgaagtcgcagttggggcccgagcttccgcggctgttgcgaaacacggggttggcacactggaacaccagcacgctcgggtagttgatactggccagggccgttgcgtcggtcaccgccgttacatccagatcctccgcgttggtcagggcgaagggagtcagcttgcacatctgccgcccgatgtggggcacgccgtcatgcttgttgaggcagtcgcaacgcaggggaatcagaatgcgatgctggccgcgttgcatctgagggtagttggcccgcaagaacgcttccatctgacggaaggccgtctgggctttcattccctcggtgtagaaaagaccgcaggacttgctagaaaatacattattgccgcaggtgacgtcttccgcgcagcagcgggcgtcttcgttctttagctgcaccacgttgcgaccccaccggttctgtaccaccttggccctcgtgggctgctccttcagcgcccgctggccgttttcgctggtcacatccatttccaacacgtgctccttacacaccatttccactccgtggaagcagaacaggacgccctcctgctgggtattgcgatgctcccacacggcgcagcctgtggcctcccagctcttatgcttcacccccgcgtagttttccatgtaagccatcaggaatctgcccatcatctcggtaaaggttttctgactggtgaaggtcaaaggcaagccgcggtgctcttcgttcagccacgtttgacagatcttgcggtacgtggcgccctgatccggcagaaacttaaacgcccccttgctctcgttgtccacgtggaacttttccatcagcattagcataacttccatacccttctcccacgccgtcaccagcggtgtgctgtcggggttcttcaccaacatggtagaagggccctcgccggccctgaagtcgctcatactcattttttgaaactccacagtgccgtccgcacgacggacccggcgcatcggagggtagctgaagccaacctccaccagggtgccttcgctctcgctgtcggagacgatctccggggagggcggcggcgcgggtgtcgacttgcgagccttcttcttgggaggaagcggtggcgcctcttggtcgcgctcgggactcatctccctcaagtagggggtgatggagcttcctgcttggttctgacggttggccattgtatcctaggcagaaacacatggagcttatgcgcgaggaaactttaaccgccccgtcccccgtcaacgacgaagaggtcatcatcgaacaggacccgggctacgttactccgcccgaggatctggaggggcctttagacgaccggcgcgacgctagtgagcagcaggaaaatgagaaagaggaagcctgctacctcctggaaggcgacgtgttgctaaaacatttcgccaggcagagcaccatagtgaaggaggctttgcaagaccgctcggaggtgcccttggacgtcgccgcgctctcccaggcctacgaggcgaacctcttctcgccccgagtgcctccgaagagacagcccaacggcacctgcgagcccaacccgcgccttaacttctaccccgtgttcgccgtgcccgaggcgctggccacctaccacatttttttcaagaaccagcgcatcccgctctcgtgccgggccaaccgcaccgcggccgatagaaagctgagactcaaaaacggagctagcatacctgatatcacgtccctggaggaagtgcctaagatcttcgaaggtctgggtcgagacgagaaacgggcggcaaacgctctgcagaaagaacagaaggacagtcagaacgtgctggtggaactggagggggacaatgcgcgtctggccgttctcaagcgctgcatagaagtttcccacttcgcctaccctgccctgaacctgccgcccaaagtcatgcgctcggtcatggaccagctgctcatcaagagagctgagcccctgaaccccgagcaccccgaggcggagaactcggaggacggaaagcccgtcgtcagcgacgaggagctcgagcggtggctggacagcacggaccccgagcagttgcaagagcggcgcaaaatgatgatggcggccgtcctggtcaccgttgagctggagtgcctgcagcggttttttagcgacgtggaaacgctgcgtaaaatcggagagtccctgcactacaccttccgccagggctacgtccgccaggcctgcaagatctccaacgtggagctcagcaacctggtctcctacatgggcatcctccacgagaaccggctgggacagagcgtgctgcactgcaccttgcaaggcgaggcgcggcgggactacgtgcgagactgcgtctacctcttcctcactctcacctggcagaccgccatgggagtgtggcagcagtgcttggaagacagaaacctcaaagagctagacaaactcctctgccgccagcggcgcgccctgtggtccggtttcagcgagcgcacggtcgccagcgctctggcggacatcatcttcccggagcgcctgatgaaaaccttgcaaaacggcctgccggatttcatcagtcaaagcattttgcaaaacttccgctcttttgtcctggaacgctccgggatattgcccgccatgagctgcgcgctaccttctgactttgtccccctctcctaccgcgagtgccctcccccactgtggagccactgctacctcttccaactggccaactttctggcctaccactccgacctcatggaagacgtaagcggagagggtttactggagtgccactgccgctgcaacctgtgcaccccccacagatcgctggcctgcaacaccgagctactcagcgaaacccaggtcataggtaccttcgagatccaggggccccagcagcaagagggtgcttccggcttgaagctcactccggcgctgtggacctcggcttacttacgcaaatttgtagccgaggactaccacgcccacaaaattcagttttacgaagaccaatctcgaccaccgaaagcccccctcacggcctgcgtcatcacccagagcaagatcctggcccaattgcaatccatcaaccaagcgcgccgcgatttccttttgaaaaagggtcggggggtgtacctggacccccagaccggcgaggaactcaacccgtccacactctccgtcgaagcagcccccccgagacatgccgcccaagggaaccgccaagcagctgatcgctcggcagagagcgaagaagcaagagctgctccagcagcaggtggaggacgaggaagagatgtgggacagccaggcagaggaggtgtcagaggacgaggaggagatggaaagctgggacagcctagacgaggaggaggacgagctttcagaggaagaggcgaccgaagaaaaaccacctgcatccagcgcgccttctctgagccgacagccgaagccccggcccccgacgcccccggccggctcactcaaagccagccgtaggtgggacgccaccgaatctccagcggcagcggcaacggcagcgggtaaggccaaacgcgagcggcgggggtattgctcctggcgggcccacaaaagcagtattgtgaactgcttgcaacactgcgggggaaacatctcctttgcccgacgctacctcctcttccatcacggtgtggccttccctcgcaacgttctctattattaccgtcatctctacagcccctacgaaacgctcggagaaaaaagctaaggcctcctccgccgcgaggaaaaactccgccgccgctgccgccgccaaggatccaccggccaccgaagagctgagaaagcgcatctttcccactctgtatgctatctttcagcaaagccgcgggcagcaccctcagcgcgaactgaaaataaaaaaccgctccttccgctcgctcacccgcagctgtctgtaccacaagagagaagaccagctgcagcgcaccctggacgacgccgaagcactgttcagcaaatactgctcagcgtctcttaaagactaaaagacccgcgctttttccccctcggccgccaaaacccacgtcatcgccagcatgagcaaggagattcccaccccctacatgtggagctatcagccccagatgggcctggccgcgggggccgcccaggactactccagcaagatgaactggctcagcgccggcccccacatgatctcacgagttaacggcatccgagcccaccgaaaccagattctcttagaacaggcggcaatcaccgccacaccccggcgccaactcaacccgcctagttggcccgccgcccaggtgtatcaggaaaatccccgcccgaccacagtcctcctgccacgcgacgcggaggccgaagtcctcatgactaactctggggtacaattagcgggcgggtccaggtacgccaggtacagaggtcgggccgctccttactctcccgggagtataaagagggtgatcattcgaggccgaggtatccagctcaacgacgagacggtgagctcctcaaccggtctcagacctgacggagtcttccagctcggaggagcaggccgctcttccttcaccactcgccaggcctacctgaccctgcagagctcttcctcgcagccgcgctccgggggaatcggcactctccagttcgtggaagagttcgttccctccgtctacttcaaccccttctccggctcgcctggacgctacccggacgccttcattcccaactttgacgcagtgagtgaatccgtggacggctacgactgatgacagatggtgcggccgtgagagctcggctgcgacatctgcatcactgccgtcagcctcgctgctacgctcgggaggcgatcgtgttcagctactttgagctgccggacgagcaccctcagggtccggctcacgggttgaaactcgagatcgagaacgcgctcgagtctcgcctcatcgacaccttcaccgcccgacctctcctggtagaaatccaacgggggatcactaccatcaccctgttctgcatctgccccacgcccggattacatgaagatctgtgttgtcatctttgcgctcagtttaataaaaactgaactttttgccgcaccttcaacgccacgcgttgtttctccaacagtcgacgatagctcttcaattaaaggtacccgagaaactgtttattttgacaattctactacttctcttatccttaactgttcttgcacactagtgagggggctatcctgtgtcactgtcacgcgcctgattgtatgcccaaactaatcagaactctttgtgctttaggtgatatatttaaaatatagatagtatcaataaacttaccttaaatttgacagcaattttttggtatcatcattcagcagcaccactttaccctcttcccaactctcatatgggatatgatggtgggcggcaaacttcctccaaaccctgaaagaaatatcggtatccacttccttgtcctcacccacaattttcatcttttcatagatgaaaagaacccgagttgatgaagacttcaaccccgtctacccttatgacaccacaaccactccagccgttcctttcatatcacccccgtttgtaaacagtgacggtcttcaggaaaacccccccggagttttaagcctgcgaatagctaaacccctgtattttgacatggagagaaaactagccctttcacttggaagagggttaacaattaccgcgaacggacaattagaaagcacccagagcgtgcagactaacccgccgttaactgtcaccaataacaacacacttatcctacgccactcctcccctttaatcctaactgacaataatttaaccgtaggcttctcaagtcctctccgtgttatagacaacaaactgacattcacttttacctcacctctccgttatgaaaacgaaacccttaccttcaattacacagagccccttacacttatgaacagcaaccttgcgcttaacgtaaactcctctaaaggccttagggttgacgggggctcactaggtacaaacttaagtccggacttaaggtttaacagcagtggagccatagcttttggtatacaaaccctatggacacccccgacctcaaatcctaactgcaccgtttacaccgaaagcgattccttacttagtctctgcttaactaaatgcggagctcacgttttaggaagtgtaagcttaaccggggtagcaggtaccatgataaacatggctgaaacttcgcttgctattgaatttacgtttgacgacactggaaaactacttcactcaccacttgttaacaccacttttagcattcgtcagggcgacagccccgcctcaaatcctacctacaatgctctagcatttatgccaaacagtaccctctacgctagaggaggaagtggtgaaccccgaaacaattactacgtccaaacatacctcaggggaaatgttcagagaccgattaccctcactgttactttcaactcagccgccacgggatattccttatcttttaagtggactgctgttgcacgtgaaaaatttgcagctcctgcaacttcattttgctacattaccgaacaataaaaccctgtgttcccaccgtttcgttttttccagatgaaacgggccagagttgatgaagacttcaatcccgtgtacccttacgatcccccttacgcccccattatgccgtttattaccccgccgtttacatcttcagatgggttacaggaaaaaccacttggtgttttaagtttaaaatacaaggatcctatcactacacaaaatggttctctaacccttaaattaggaaacgggctgaacattaacaaccagggccaacttacatcatctgctggggaagtcgagcctcccctcaccaatgctgacaacaagctggccttagcctacagcgaccctctgacattaaaaaacagccgtctaacactgtctcacaatgccccacttgcaattaacaataattctctaagtttggaagtatcagagcctatatttataaataacgacaacaaactgtctctgaaagctgacgcccccctgacaaccagcgctggaaccctccgcctgcaaagcgctgctccattaggacttgctgaacagacactaaagctgctgttttctaaccctttgtacttgcgaggtgacttccttacattagccattgaacgcccattggctgtaacagcagacgggctattatcacttgccctcaaccctccgctcacaacaactaacacaggcttagctctctctaccgcggttccattaactgttaccaacgggaaccttagcctaaacgtaaaacggccgtttattatacaggacggcagcctttacatggattttagacccccactatatctgtttaacagcgagccacaacttggtgttaattttaatgcccctctaactgttagagataacggcctagctataaacaccggagacgggctaacagtaacgtataataaactaacattaaacctcggtagagacttgcaatatgaaaatggagctgcagctgttaagctaagtaccgcccctcctctacagtatactactcaactgcagctgaatttgggagcgggcttacgtctaggtcctactaggaacttagacgtggccattaaccacaataaagggttagcgtgggaaaacaatgaagtggttactaaattaggacaaggcctttactttgattcctccggaagcatagctttatcgcctacaaaccccagaccagatactttatggaccacggccgatccttcgccaaactgcactgtatatgaatcacttgactctagactgtggctagcgcttgttaaatgtgggggaatggtacacggcagcatagccctacaagctgaaaaaggccaattgctgcgtcctactgctagttttatctccatcgtaatttacttctacagtgatggggtccgtcgcaccaactaccctacaattggcaatgatgagggtactctggccaacagcgctacttggggctacagacaagggcaatctgcagacaccaacgtcaccaatgctgttgaattcatgcctagtttacacagatatcctataaatcagggagacaatattaaaaaccaaatgataacttacacttgcatacaaggcaacgtgaacatgccagtacccttgaaaatcacgttcaatcatgctcttgaaggctactccttaaagtttacatggcgtgtggtggctaatgaaaagtttgatattccttgctgttcgttttcttacattacagaacaataaaacaacttttttatttttcatttcttttattttacacgcacagtaagacttcctccccccttccatttaacagcgtacaccagcctttcccccttcatggcggtaaacttctgtgagttagtccggtatttgggagttaaaatccaaacaggctctttggtgattaaacgttgatccgtgatggacacaaatccctgagacaggtcctccaacgttgcggtaaaaaactgaacgccgccctacaaaacaaacagttcaggctctccacgggttatcaccccgatcaaactcagacagagtaaaggtgcggtgatgttccacaagaccgcgcaagtggcgctgtctaaagctctcagtgcgacttctatgcggctggtaggatgttacattatccaacagcctcacagcgcggattattagtctacgagtgcgcctggcgcagcagcgcatctgaatttcagtcaagtcttgacaagaagcgcataccataacaatcaggttgttcatgatcccatagctaaacgcgctccagccaaaactcattcgctccaacagcaccaccgcgtgtccgtcaagtcttacttttacataaacaaggtgtctgccacgtacatacatgctacccgcatacaaaacttcccggggcaaacctctattcaccacctgtctgtaccagggaaacctgatgtttatcagggaaccatagatggccattttaaaccagttagccagcaccaccccgccagctctacactgaagggaaccgggagagttacaatgacagtggatcatccacctctcgtaacccctaattacctgattaaaatccaaatctaacgtggcacaacagatacacactctcataaacattttcatgacatgtttttcccaggatgttaaaatacaatcccaatacacgggccactcctgtaatacaataaagctaatgcatgatggaacgctcctcacctcactaacattgtgcatgtttacattttcacactctaagtaccgagtcctctcctcaacagccgcagtgtcgcgctcctcacacggtggtagctgatgacaattgtaaggggccagtctgcagcgatatcgtctgtcgcgctgcatcgtaaaacagggaccgtctcacttcctcgtacttccaatagcagaaccacgtccgctgccagcaggtttccacgaaccgccgatcccttcgtcgttcacgctccctcctcaacgcaaaatgcagccactcctgcaatccacacaaatccctctcggcctccggagtcatgcacacctcatacctatatatgtctcggtacagttccaaacacgaagtaagggcgagctccaaccaacacaaacaggctgatttatcccgacacactggaggtggaggaagacacggaagaggcatgttattccaagcgatccggcaaaggatcaaagtgcagatcccgaagatggcaacgctcgcctccggagccctggtgaaatttaacggccaaatcaaacattatgcggttttccaaactatcaatcgccgcctccaaaagggcctgaacccgcacttccacaatcaccagcaaagcaaaagcgtgattatcaaagtcttcaatcatcagatggcatgactgtacaatgcccaaataattctcatttctccactcgcgaatagtgtcgcggcagatcgtctgaaggtccatgccatgcatgttaaaaagctcccagagggcgccctctaccgacatgcgtagacacaccatcatgactgcaaaatatcaggctcctgagacacctgcagcagatttaacagatcaaagtcaggttgctgtccgcggtcacgaatctccatgcgcaaagccatttgcaaaaaattatataggtctgtgccaactagctctgttaattccgcgttaggaagcaaatcaggtgaggctatgcagcacaaaagttgcagggaaggcgccaaactcagtaaaaccgctccagaataacaaaattgatgaagcggagtcacacagtgtaaaatgtgcaaccaaaaatcattcagctgctcttttaaatagtccagtacttctatattcaatccgtgcaagtactgaagcaactgcgcgggaacagtcacattaaaaaaaatggggcggctcaaatacatgtcgacctaaaataaaaataatcattaaaccagagaagcttgacgaatggaaggataaaatacacgctccagcaaaaggcaggcaaccggctgtccccgagaaccgtaaaaaaattcatccgaatgattaaaaagaaccacagaaatttcccaccatgtactcggttgtaactcctgagcacacagcaacacccccctaacgttcatgtccgccactgaaaaaagacgtcccaaatacccaggtggaatgtcaagagacaactgcagagacagcaaaacaacccctctgggagcgatcataaactcctccggtgagaaaagcgcatacaaattagaataaccctgttgctggggcaaaatagcccggcggcccagcaaatggacataaatatgttcagcagccatcgccccgtcttaccgcgtaaaaagccagaaaaatccagctaactacactctacagcctattactatatatactctcctcccactgacgctataccaccccgcccacgtccaaagttcacccacgcccaaaaaacccgcgaaaatccagcgccgtcagcacttccgcaattgtagtctctcaacgtcacttccgcgcgccttttccctattcccacacacgcccgcggacttcgccccgcccgccctcgcgccaccccgcgtcaccccgcgtcaccgcacgtcaccccggccccgcctcgctcctccccactcattatcatattggcacgtttccagaataaggtatattattgatgatgttaattaattcgaacccataatacccataatagctgtttgccatcgacgcgaggctggatggccttccccattatgattcttctcgcttccggcggcatcgggatgcccgcgttgcaggccatgctgtccaggcaggtagatgacgaccatcagggacagcttcaaggatcgctcgcggctcttaccagcccagcaaaaggccaggaaccgtaaaaaggccgcgttgctggcgtttttccataggctccgcccccctgacgagcatcacaaaaatcgacgctcaagtcagaggtggcgaaacccgacaggactataaagataccaggcgtttccccctggaagctccctcgtgcgctctcctgttccgaccctgccgcttaccggatacctgtccgcctttctcccttcgggaagcgtggcgctttctcatagctcacgctgtaggtatctcagttcggtgtaggtcgttcgctccaagctgggctgtgtgcacgaaccccccgttcagcccgaccgctgcgccttatccggtaactatcgtcttgagtccaacccggtaagacacgacttatcgccactggcagcagccactggtaacaggattagcagagcgaggtatgtaggcggtgctacagagttcttgaagtggtggcctaactacggctacactagaaggacagtatttggtatctgcgctctgctgaagccagttaccttcggaaaaagagttggtagctcttgatccggcaaacaaaccaccgctggtagcggtggtttttttgtttgcaagcagcagattacgcgcagaaaaaaaggatctcaagaagatcctttgatcttttctacggggtctgacgctcagtggaacgaaaactcacgttaagggattttggtcatgagattatcaaaaaggatcttcacctagatccttttaaattaaaaatgaagttttaaatcaatctaaagtatatatgagtaaacttggtctgacagttaccaatgcttaatcagtgaggcacctatctcagcgatctgtctatttcgttcatccatagttgcctgactccccgtcgtgtagataactacgatacgggagggcttaccatctggccccagtgctgcaatgataccgcgagacccacgctcaccggctccagatttatcagcaataaaccagccagccggaagggccgagcgcagaagtggtcctgcaactttatccgcctccatccagtctattaattgttgccgggaagctagagtaagtagttcgccagttaatagtttgcgcaacgttgttgccattgctgcaggcatcgtggtgtcacgctcgtcgtttggtatggcttcattcagctccggttcccaacgatcaaggcgagttacatgatcccccatgttgtgcaaaaaagcggttagctccttcggtcctccgatcgttgtcagaagtaagttggccgcagtgttatcactcatggttatggcagcactgcataattctcttactgtcatgccatccgtaagatgcttttctgtgactggtgagtactcaaccaagtcattctgagaatagtgtatgcggcgaccgagttgctcttgcccggcgtcaacacgggataataccgcgccacatagcagaactttaaaagtgctcatcattggaaaacgttcttcggggcgaaaactctcaaggatcttaccgctgttgagatccagttcgatgtaacccactcgtgcacccaactgatcttcagcatcttttactttcaccagcgtttctgggtgagcaaaaacaggaaggcaaaatgccgcaaaaaagggaataagggcgacacggaaatgttgaatactcatactcttcctttttcaatattattgaagcatttatcagggttattgtctcatgagcggatacatatttgaatgtatttagaaaaataaacaaataggggttccgcgcacatttccccgaaaagtgccacctgacgtctaagaaaccattattatcatgacattaacctataaaaataggcgtatcacgaggccctttcgtcttcaagaattggtcgatggcaaacagctattatgggtattatgggttcgaattaat

SEQ ID NO: 50 - DNA, 17915 bp, Artificial Sequence
  Synthetic oligonucleotide pBr/sAd4312.pV-rITR.dE3.dE4
attaaccgaagttagaagaccaaaggtgcgaagacggcgtactgagtctccctgttgttatcagcccaacatgagcaagcgcaagtttaaagaagaactcctgcagaccctggctcctgaaatctatggccctccggacgtgaagcccgacattaagccccgcgatatcaagcgtgttaaaaagcgggaaaaaaaagaggaactcgcggtggtagacgatggcggggtagaatttattagaagtttcgccccgcgacgcagggtgcagtggaaagggcggcgcgtgcaacgcgttctcaggccaggcaccgcggtagtttttactccgggagagcggtcggctgtcaggggtttcaagcggcaatatgacgaggtgtacggcgacgaagacatcctggaacaggcggctcagcagattggagaattcgcctacggaaagcggtctcgccgcgaagacctggccattgccttggacagtggcaaccccacccccagcctcaaacccgtcacgctgcagcaggtgctccccgtgagcgcgagcacggagagcaaaaggggaatcaagagagagatggaagatctgaagcccaccatccaacttatggtccctaaacgacagaagctggaggaggttctggaaaacatgaaagtggaccccagcatagagccggatgtaaaagtgaggcctattaaggaagtggctccgggtctcggggtgcaaacggtggacattcagatcccagtcagatccgcttcgaccgccgtggaagccatggaaacgcaaaccgaaactccggtcgcggccggtaccagagaagtggctttgcaaacggagccctggtacgaatacaccgctcctcggcgccagaggcggcgttacggcccggcaaatgccatcatgccagagtatgcgctgcacccgtctatccgacccacccccggctaccggggggtaacgtatcgcccgtcgccaacccgacgccgttatcgtcgccgccgccgttctcgtcgcgctctggcgcccgtgtccgtgcgacgcgtaacgcgccggggaagaacagtcaccatccctaacccgcgctaccaccctagcattctttaatgactctgccgttttgcagatggctctgacttgccgcgtgcgccttcccgttctgcactatcgaggaagatctcgtcgtaggagaggcatggcggggagcggccgccgtcgggctttacgcaggcgcatgaaaggcggaattttgcccgcactgattcccataattgccgccgccattggggcgatacccggcgttgcttcagtggccttgcaagcagctcgtaataaataaacgaaggcttttcaacttatgacctggtcctgactattttatgcagaaaaagcatggaagacatcaattttacgtcgctggctccgcggcaaggctcacgcccgctcatgggcacctggaacgacatcggcagcagccagctcaacgggggcgctttcaattgggggagcctttggagcggcattaaaaactttggctccgcgattaaatcctacggcagcaaagcctggaacagtagtactggtcagatgctccgggataaactgaaggacacaaactttcaagagaaagtggtcaacggggtggtgaccggcatccacggcgcggtggatctcgctaatcaagcggtgcaaaaagagatagacagacgatgggaaaactcgcgggtgcctccgcagagaggggacgaagtggaggtggaggaagtagaagtcgaggagaaactgcccccgctagagaaagttcccggggcgccgcccaggccacagaagcgtccccggccggatctggaagaaactttagtgacggaaaccatcgaacctccctcgtacgaacaagctttaaaggagggcgcctctccttaccccatgactaagcccatcgcgcccatggcgcgtccggtgtacggaaaagatcacaagccagtaacgttagagctacccccaccacccccttcccgtcctacggtgcctccgttacccgccccgtcggcaggtcccagctctgcaccatccgcagctcctgcaccaaccgctcgcccggtggccgtggcaaccgccagagcccccagaggatccaactggcaaagcacgctgaacagcatcgtgggcttgggagtgaaaaccctaaaacgccgccgctgctattattaaagagtgtagctaaaaatttcccgttgtatacgcctcctatgttaccgccagagacgcgtgactggtcgccgctccgccgctttcaagatggccaccccatcgatgatgccgcagtggtcttacatgcacatcgccggccaggacgcctcggagtacctgagtcccggcctggtgcagtttgcccgcgccaccgaaagctacttcagcttgggaaacaagtttagaaaccccaccgtggcccccacgcacgatgtaaccacggaccgctcgcagaggctgacactgcgcttcgtgcccgtagaccgggaggacaccgcgtactcctacaaagtgcgcttcaccctcgccgtaggggacaacagggtgctggacatggccagcacgtactttgacatccggggaatgctggaccgagggcccagctttaaaccctactcgggaactgcctacaattcgctggcacctaagggcgctcccaaccctagtcaatggactactaccaacggagggaataaaacaaattcatttgcccaagcatcctacataggtcaaagcctgtcgaaagacggggtgcaagtagcagtagatacagccgctgggggggctgcagtatatgctgacaaaacgtttcaaccagaaccccaagtaggaatatcacaatggaatgaaaatcctactacaaatgctgcaggaagaattttaaagcctactaccgcaatgcgtccatgctacggttcatacgcttaccccaccaacgaaaaaggtgggcaggtaaaaatcactgaccctaacaatgacaaaaccggcgctaataacgttagcttaaattttttcaacactgccgctgacaatgggaataacaatccaaaagtagtactctacagcgaagatgtaaatttagaagggccagatacccaccttgtttttaagccagatgtaactggcgacgcaaccagtgcagaaaccctgttaggtcaacaagcagctcccaatcgtccaaactacattgggttcagggacaactttattggcctgatgtactacaattcaactggaaacatgggagtgctagcaggtcaggcttctcagctaaacgccgtagtggatcttcaagacagaaataccgaattgtcatatcagctaatgcttgacgctttgggtgacagaagtcggtacttttctatgtggaatcaagcagtggacagctacgatcctgacgttagaatcatagaaaatcatggagtagaagacgaacttccaaattattgttttccgttaaatggacaggggatttcgaatacatacaaaggtgtgaaatataacacaaacacttggacgcaagacactgatgtagtcacaaccaatgaaatttccattggcaacatttttgccatggaaataaacctggcggctaacttgtggcgcagctttctgtactccaatgtcgccctgtacttgccagattcctacaaatacactcccgacaatattgaacttcctacaaacaagaacagctacggctacattaacggaagggtaaccgcccccactgccatcgacacttacgttaacatcggcgcccggtggtctccggaccccatggacaacgttaaccctttcaaccaccaccgcaacgccggcttgcgataccgctccatgctgctgggcaacggtcgctacgtacccttccacattcaggtgccccagaaattttttgccattaaaaacctgcttctgcttcccgggtcctacacctacgagtggaacttcaggaaagatgtaaacatgatcttgcagagcaccttgggcaacgacctccgcgttgacggagctagcgtgaggtttgacagcattaacctctacgctaacttcttccccatggcccacaacacggcctccaccttggaagccatgctgcgcaacgacaccaacgaccagtcctttaatgattacctgtgcgcggccaacatgctgtaccccatccccgccaatgccaccagcgtgccgatctccattccctcacgcaactgggccgccttcagaggttggagtttcactcgcctgaaaaccaaggagaccccctcgctgggctccggtttcgacccatactttgtttactccgggagcattccctacctggacggaactttctacctgaaccacaccttcaaaaaggtgtctattatgtttgactcctccgtgagctggcccggtaacgaccgcttgctaacccccaacgagttcgaaatcaaacgctcggtggacggagagggttacaatgtagcccagagcaacatgaccaaagactggtttttaattcaaatgctaagccactataacattggctaccaaggattctacgtgcctgaagcctacaaggacagaatgtactccttctttagaaacttccaacccatgagccgccaggtagtagacacggtaaactatgctaactacaaggaagtaacaatgccattccagcacaacaactcaggcttcgtggggtacatgggacctaccatgagagaggggcaggcctacccggctaattatccctaccccctaatcggagccactgccgtgcccagcctgacacagaaaaagtttctctgcgatcgaacaatgtggaggattcccttctctagcaacttcatgtccatgggggctctcaccgacctggggcagaacatgctgtacgctaactccgctcacgccttggacatgacctttgaggtggaccccatggatgagcccacgcttctctatgttctgtttgaagtcttcgacgtggtgcgcattcaccagccgcaccgcggcgtcatcgaggccgtctacctgcgcacacctttctctgccggtaacgccaccacctaagaagctgatgggctccagcgaacaggagctgcgggccattgttcgcgacctgggctgcgggccctactttttgggcaccttcgacaagcgcttccccggcttcatgtccccccacaagccggcctgcgccatcgtcaacacggccggacgcgagaccgggggggttcactggctcgcctttgcctggaacccgcgtaaccacacctgctacctgttcgacccttttggtttttctgacgaaaggcttaaacagatttaccagttcgagtacgaggggctccttaaacgcagcgctctggcctccacgcccgaccactgcgtcaccctggagaagtccacccaaacggttcagggtcccctctcggcggcctgcggactcttttgttgcatgtttttgcatgctttcgtccactggccgaacacccccatggaccgcaaccccactatggatctgctcacgggagtgcctaacagcatgcttcacagccctcaggtcgcacccaccctgcgtcgcaatcaggaacagctgtatgcttttctgggaaaacattctgcctactttcgccgccaccggcagcgcatagaacaggccacggcctttgaaagcatgagtcaaagagtgtaatcaataaaatcaacttttattttacatcacacgcgcttctggcgttttcttaaaaatcaaagggttcgggggaggggtcgtcgtgcccgctgggcagggacacgttgcgatactggaagcgggggctccagcggaactcggggatcgccagccggggcagaggcacttcttccaggttctgcttccaaaactgccgcaccagctggagggctcccattacgtcgggcgccgagatcttgaagtcgcagttggggcccgagcttccgcggctgttgcgaaacacggggttggcacactggaacaccagcacgctcgggtagttgatactggccagggccgttgcgtcggtcaccgccgttacatccagatcctccgcgttggtcagggcgaagggagtcagcttgcacatctgccgcccgatgtggggcacgccgtcatgcttgttgaggcagtcgcaacgcaggggaatcagaatgcgatgctggccgcgttgcatctgagggtagttggcccgcaagaacgcttccatctgacggaaggccgtctgggctttcattccctcggtgtagaaaagaccgcaggacttgctagaaaatacattattgccgcaggtgacgtcttccgcgcagcagcgggcgtcttcgttctttagctgcaccacgttgcgaccccaccggttctgtaccaccttggccctcgtgggctgctccttcagcgcccgctggccgttttcgctggtcacatccatttccaacacgtgctccttacacaccatttccactccgtggaagcagaacaggacgccctcctgctgggtattgcgatgctcccacacggcgcagcctgtggcctcccagctcttatgcttcacccccgcgtagttttccatgtaagccatcaggaatctgcccatcatctcggtaaaggttttctgactggtgaaggtcaaaggcaagccgcggtgctcttcgttcagccacgtttgacagatcttgcggtacgtggcgccctgatccggcagaaacttaaacgcccccttgctctcgttgtccacgtggaacttttccatcagcattagcataacttccatacccttctcccacgccgtcaccagcggtgtgctgtcggggttcttcaccaacatggtagaagggccctcgccggccctgaagtcgctcatactcattttttgaaactccacagtgccgtccgcacgacggacccggcgcatcggagggtagctgaagccaacctccaccagggtgccttcgctctcgctgtcggagacgatctccggggagggcggcggcgcgggtgtcgacttgcgagccttcttcttgggaggaagcggtggcgcctcttggtcgcgctcgggactcatctccctcaagtagggggtgatggagcttcctgcttggttctgacggttggccattgtatcctaggcagaaacacatggagcttatgcgcgaggaaactttaaccgccccgtcccccgtcaacgacgaagaggtcatcatcgaacaggacccgggctacgttactccgcccgaggatctggaggggcctttagacgaccggcgcgacgctagtgagcagcaggaaaatgagaaagaggaagcctgctacctcctggaaggcgacgtgttgctaaaacatttcgccaggcagagcaccatagtgaaggaggctttgcaagaccgctcggaggtgcccttggacgtcgccgcgctctcccaggcctacgaggcgaacctcttctcgccccgagtgcctccgaagagacagcccaacggcacctgcgagcccaacccgcgccttaacttctaccccgtgttcgccgtgcccgaggcgctggccacctaccacatttttttcaagaaccagcgcatcccgctctcgtgccgggccaaccgcaccgcggccgatagaaagctgagactcaaaaacggagctagcatacctgatatcacgtccctggaggaagtgcctaagatcttcgaaggtctgggtcgagacgagaaacgggcggcaaacgctctgcagaaagaacagaaggacagtcagaacgtgctggtggaactggagggggacaatgcgcgtctggccgttctcaagcgctgcatagaagtttcccacttcgcctaccctgccctgaacctgccgcccaaagtcatgcgctcggtcatggaccagctgctcatcaagagagctgagcccctgaaccccgagcaccccgaggcggagaactcggaggacggaaagcccgtcgtcagcgacgaggagctcgagcggtggctggacagcacggaccccgagcagttgcaagagcggcgcaaaatgatgatggcggccgtcctggtcaccgttgagctggagtgcctgcagcggttttttagcgacgtggaaacgctgcgtaaaatcggagagtccctgcactacaccttccgccagggctacgtccgccaggcctgcaagatctccaacgtggagctcagcaacctggtctcctacatgggcatcctccacgagaaccggctgggacagagcgtgctgcactgcaccttgcaaggcgaggcgcggcgggactacgtgcgagactgcgtctacctcttcctcactctcacctggcagaccgccatgggagtgtggcagcagtgcttggaagacagaaacctcaaagagctagacaaactcctctgccgccagcggcgcgccctgtggtccggtttcagcgagcgcacggtcgccagcgctctggcggacatcatcttcccggagcgcctgatgaaaaccttgcaaaacggcctgccggatttcatcagtcaaagcattttgcaaaacttccgctcttttgtcctggaacgctccgggatattgcccgccatgagctgcgcgctaccttctgactttgtccccctctcctaccgcgagtgccctcccccactgtggagccactgctacctcttccaactggccaactttctggcctaccactccgacctcatggaagacgtaagcggagagggtttactggagtgccactgccgctgcaacctgtgcaccccccacagatcgctggcctgcaacaccgagctactcagcgaaacccaggtcataggtaccttcgagatccaggggccccagcagcaagagggtgcttccggcttgaagctcactccggcgctgtggacctcggcttacttacgcaaatttgtagccgaggactaccacgcccacaaaattcagttttacgaagaccaatctcgaccaccgaaagcccccctcacggcctgcgtcatcacccagagcaagatcctggcccaattgcaatccatcaaccaagcgcgccgcgatttccttttgaaaaagggtcggggggtgtacctggacccccagaccggcgaggaactcaacccgtccacactctccgtcgaagcagcccccccgagacatgccgcccaagggaaccgccaagcagctgatcgctcggcagagagcgaagaagcaagagctgctccagcagcaggtggaggacgaggaagagatgtgggacagccaggcagaggaggtgtcagaggacgaggaggagatggaaagctgggacagcctagacgaggaggaggacgagctttcagaggaagaggcgaccgaagaaaaaccacctgcatccagcgcgccttctctgagccgacagccgaagccccggcccccgacgcccccggccggctcactcaaagccagccgtaggtgggacgccaccgaatctccagcggcagcggcaacggcagcgggtaaggccaaacgcgagcggcgggggtattgctcctggcgggcccacaaaagcagtattgtgaactgcttgcaacactgcgggggaaacatctcctttgcccgacgctacctcctcttccatcacggtgtggccttccctcgcaacgttctctattattaccgtcatctctacagcccctacgaaacgctcggagaaaaaagctaaggcctcctccgccgcgaggaaaaactccgccgccgctgccgccgccaaggatccaccggccaccgaagagctgagaaagcgcatctttcccactctgtatgctatctttcagcaaagccgcgggcagcaccctcagcgcgaactgaaaataaaaaaccgctccttccgctcgctcacccgcagctgtctgtaccacaagagagaagaccagctgcagcgcaccctggacgacgccgaagcactgttcagcaaatactgctcagcgtctcttaaagactaaaagacccgcgctttttccccctcggccgccaaaacccacgtcatcgccagcatgagcaaggagattcccaccccctacatgtggagctatcagccccagatgggcctggccgcgggggccgcccaggactactccagcaagatgaactggctcagcgccggcccccacatgatctcacgagttaacggcatccgagcccaccgaaaccagattctcttagaacaggcggcaatcaccgccacaccccggcgccaactcaacccgcctagttggcccgccgcccaggtgtatcaggaaaatccccgcccgaccacagtcctcctgccacgcgacgcggaggccgaagtcctcatgactaactctggggtacaattagcgggcgggtccaggtacgccaggtacagaggtcgggccgctccttactctcccgggagtataaagagggtgatcattcgaggccgaggtatccagctcaacgacgagacggtgagctcctcaaccggtctcagacctgacggagtcttccagctcggaggagcaggccgctcttccttcaccactcgccaggcctacctgaccctgcagagctcttcctcgcagccgcgctccgggggaatcggcactctccagttcgtggaagagttcgttccctccgtctacttcaaccccttctccggctcgcctggacgctacccggacgccttcattcccaactttgacgcagtgagtgaatccgtggacggctacgactgatgacagatggtgcggccgtgagagctcggctgcgacatctgcatcactgccgtcagcctcgctgctacgctcgggaggcgatcgtgttcagctactttgagctgccggacgagcaccctcagggtccggctcacgggttgaaactcgagatcgagaacgcgctcgagtctcgcctcatcgacaccttcaccgcccgacctctcctggtagaaatccaacgggggatcactaccatcaccctgttctgcatctgccccacgcccggattacatgaagatctgtgttgtcatctttgcgctcagtttaataaaaactgaactttttgccgcaccttcaacgccacgcgttgtttctccaacagtcgacgatagctcttcaattaaaggtacccgagaaactgtttattttgacaattctactacttctcttatccttaactgttcttgcacactagtgagggggctatcctgtgtcactgtcacgcgcctgattgtatgcccaaactaatcagaactctttgtgctttaggtgatatatttaaaatatagatagtatcaataaacttaccttaaatttgacagcaattttttggtatcatcattcagcagcaccactttaccctcttcccaactctcatatgggatatgatggtgggcggcaaacttcctccaaaccctgaaagaaatatcggtatccacttccttgtcctcacccacaattttcatcttttcatagatgaaaagaacccgagttgatgaagacttcaaccccgtctacccttatgacaccacaaccactccagccgttcctttcatatcacccccgtttgtaaacagtgacggtcttcaggaaaacccccccggagttttaagcctgcgaatagctaaacccctgtattttgacatggagagaaaactagccctttcacttggaagagggttaacaattaccgcgaacggacaattagaaagcacccagagcgtgcagactaacccgccgttaactgtcaccaataacaacacacttatcctacgccactcctcccctttaatcctaactgacaataatttaaccgtaggcttctcaagtcctctccgtgttatagacaacaaactgacattcacttttacctcacctctccgttatgaaaacgaaacccttaccttcaattacacagagccccttacacttatgaacagcaaccttgcgcttaacgtaaactcctctaaaggccttagggttgacgggggctcactaggtacaaacttaagtccggacttaaggtttaacagcagtggagccatagcttttggtatacaaaccctatggacacccccgacctcaaatcctaactgcaccgtttacaccgaaagcgattccttacttagtctctgcttaactaaatgcggagctcacgttttaggaagtgtaagcttaaccggggtagcaggtaccatgataaacatggctgaaacttcgcttgctattgaatttacgtttgacgacactggaaaactacttcactcaccacttgttaacaccacttttagcattcgtcagggcgacagccccgcctcaaatcctacctacaatgctctagcatttatgccaaacagtaccctctacgctagaggaggaagtggtgaaccccgaaacaattactacgtccaaacatacctcaggggaaatgttcagagaccgattaccctcactgttactttcaactcagccgccacgggatattccttatcttttaagtggactgctgttgcacgtgaaaaatttgcagctcctgcaacttcattttgctacattaccgaacaataaaaccctgtgttcccaccgtttcgttttttccagatgaaacgggccagagttgatgaagacttcaatcccgtgtacccttacgatcccccttacgcccccattatgccgtttattaccccgccgtttacatcttcagatgggttacaggaaaaaccacttggtgttttaagtttaaaatacaaggatcctatcactacacaaaatggttctctaacccttaaattaggaaacgggctgaacattaacaaccagggccaacttacatcatctgctggggaagtcgagcctcccctcaccaatgctgacaacaagctggccttagcctacagcgaccctctgacattaaaaaacagccgtctaacactgtctcacaatgccccacttgcaattaacaataattctctaagtttggaagtatcagagcctatatttataaataacgacaacaaactgtctctgaaagctgacgcccccctgacaaccagcgctggaaccctccgcctgcaaagcgctgctccattaggacttgctgaacagacactaaagctgctgttttctaaccctttgtacttgcgaggtgacttccttacattagccattgaacgcccattggctgtaacagcagacgggctattatcacttgccctcaaccctccgctcacaacaactaacacaggcttagctctctctaccgcggttccattaactgttaccaacgggaaccttagcctaaacgtaaaacggccgtttattatacaggacggcagcctttacatggattttagacccccactatatctgtttaacagcgagccacaacttggtgttaattttaatgcccctctaactgttagagataacggcctagctataaacaccggagacgggctaacagtaacgtataataaactaacattaaacctcggtagagacttgcaatatgaaaatggagctgcagctgttaagctaagtaccgcccctcctctacagtatactactcaactgcagctgaatttgggagcgggcttacgtctaggtcctactaggaacttagacgtggccattaaccacaataaagggttagcgtgggaaaacaatgaagtggttactaaattaggacaaggcctttactttgattcctccggaagcatagctttatcgcctacaaaccccagaccagatactttatggaccacggccgatccttcgccaaactgcactgtatatgaatcacttgactctagactgtggctagcgcttgttaaatgtgggggaatggtacacggcagcatagccctacaagctgaaaaaggccaattgctgcgtcctactgctagttttatctccatcgtaatttacttctacagtgatggggtccgtcgcaccaactaccctacaattggcaatgatgagggtactctggccaacagcgctacttggggctacagacaagggcaatctgcagacaccaacgtcaccaatgctgttgaattcatgcctagtttacacagatatcctataaatcagggagacaatattaaaaaccaaatgataacttacacttgcatacaaggcaacgtgaacatgccagtacccttgaaaatcacgttcaatcatgctcttgaaggctactccttaaagtttacatggcgtgtggtggctaatgaaaagtttgatattccttgctgttcgttttcttacattacagaacaataaaacaacttttttatttttcatttcttttattttacacgcacagtaagacttcctccccccttccatttaacagcgtacaccagcctttcccccttcatggcggtaaacttctgtgagttagtccggtatttgggagttaaaatccaaacaggctctttggtgattaaacgttgatccgtgatggacacaaatccctgagacaggtcctccaacgttgcggtaaaaaactgaacgccgccctacaaaacaaacagttcaggctctccacgggttatcaccccgatcaaactcagacagagtaaaggtgcggtgatgttccacaagaccgcgcaagtggcgctgtctaaagctctcagtgcgacttctatgcggctggtaggatgttacattatccaacagcctcacagcgcggattattagtctacgagtgcgcctggcgcagcagcgcatctgaatttcagtcaagtcttgacaagaagcgcataccataacaatcaggttgttcatgatcccatagctaaacgcgctccagccaaaactcattcgctccaacagcaccaccgcgtgtccgtcaagtcttacttttacataaacaaggtgtctgccacgtacatacatgctacccgcatacaaaacttcccggggcaaacctctattcaccacctgtctgtaccagggaaacctgatgtttatcagggaaccatagatggccattttaaaccagttagccagcaccaccccgccagctctacactgaagggaaccgggagagttacaatgacagtggatcatccacctctcgtaacccctaattacctgattaaaatccaaatctaacgtggcacaacagatacacactctcataaacattttcatgacatgtttttcccaggatgttaaaatacaatcccaatacacgggccactcctgtaatacaataaagctaatgcatgatggaacgctcctcacctcactaacattgtgcatgtttacattttcacactctaagtaccgagtcctctcctcaacagccgcagtgtcgcgctcctcacacggtggtagctgatgacaattgtaaggggccagtctgcagcgatatcgtctgtcgcgctgcatcgtaaaacagggaccgtctcacttcctcgtacttccaatagcagaacccgccccgtcttaccgcgtaaaaagccagaaaaatccagctaactacactctacagcctattactatatatactctcctcccactgacgctataccaccccgcccacgtccaaagttcacccacgcccaaaaaacccgcgaaaatccagcgccgtcagcacttccgcaattgtagtctctcaacgtcacttccgcgcgccttttccctattcccacacacgcccgcggacttcgccccgcccgccctcgcgccaccccgcgtcaccccgcgtcaccgcacgtcaccccggccccgcctcgctcctccccactcattatcatattggcacgtttccagaataaggtatattattgatgatgttaattaattcgaacccataatacccataatagctgtttgccatcgacgcgaggctggatggccttccccattatgattcttctcgcttccggcggcatcgggatgcccgcgttgcaggccatgctgtccaggcaggtagatgacgaccatcagggacagcttcaaggatcgctcgcggctcttaccagcccagcaaaaggccaggaaccgtaaaaaggccgcgttgctggcgtttttccataggctccgcccccctgacgagcatcacaaaaatcgacgctcaagtcagaggtggcgaaacccgacaggactataaagataccaggcgtttccccctggaagctccctcgtgcgctctcctgttccgaccctgccgcttaccggatacctgtccgcctttctcccttcgggaagcgtggcgctttctcatagctcacgctgtaggtatctcagttcggtgtaggtcgttcgctccaagctgggctgtgtgcacgaaccccccgttcagcccgaccgctgcgccttatccggtaactatcgtcttgagtccaacccggtaagacacgacttatcgccactggcagcagccactggtaacaggattagcagagcgaggtatgtaggcggtgctacagagttcttgaagtggtggcctaactacggctacactagaaggacagtatttggtatctgcgctctgctgaagccagttaccttcggaaaaagagttggtagctcttgatccggcaaacaaaccaccgctggtagcggtggtttttttgtttgcaagcagcagattacgcgcagaaaaaaaggatctcaagaagatcctttgatcttttctacggggtctgacgctcagtggaacgaaaactcacgttaagggattttggtcatgagattatcaaaaaggatcttcacctagatccttttaaattaaaaatgaagttttaaatcaatctaaagtatatatgagtaaacttggtctgacagttaccaatgcttaatcagtgaggcacctatctcagcgatctgtctatttcgttcatccatagttgcctgactccccgtcgtgtagataactacgatacgggagggcttaccatctggccccagtgctgcaatgataccgcgagacccacgctcaccggctccagatttatcagcaataaaccagccagccggaagggccgagcgcagaagtggtcctgcaactttatccgcctccatccagtctattaattgttgccgggaagctagagtaagtagttcgccagttaatagtttgcgcaacgttgttgccattgctgcaggcatcgtggtgtcacgctcgtcgtttggtatggcttcattcagctccggttcccaacgatcaaggcgagttacatgatcccccatgttgtgcaaaaaagcggttagctccttcggtcctccgatcgttgtcagaagtaagttggccgcagtgttatcactcatggttatggcagcactgcataattctcttactgtcatgccatccgtaagatgcttttctgtgactggtgagtactcaaccaagtcattctgagaatagtgtatgcggcgaccgagttgctcttgcccggcgtcaacacgggataataccgcgccacatagcagaactttaaaagtgctcatcattggaaaacgttcttcggggcgaaaactctcaaggatcttaccgctgttgagatccagttcgatgtaacccactcgtgcacccaactgatcttcagcatcttttactttcaccagcgtttctgggtgagcaaaaacaggaaggcaaaatgccgcaaaaaagggaataagggcgacacggaaatgttgaatactcatactcttcctttttcaatattattgaagcatttatcagggttattgtctcatgagcggatacatatttgaatgtatttagaaaaataaacaaataggggttccgcgcacatttccccgaaaagtgccacctgacgtctaagaaaccattattatcatgacattaacctataaaaataggcgtatcacgaggccctttcgtcttcaagaattggtcgatggcaaacagctattatgggtattatgggttcgaattaat

SEQ ID NO: 51 - DNA, 8865 bp, Artificial Sequence
  Synthetic oligonucleotide sAdApt4312.E1btg.Empty
attaacatcatcaataaagggtcaggatgggtgggcacaggtattgtcgactggtcaatattggccattgagcgaggcggggccggggtggggtgaggcggggccggggtggggtgagggtgacgtcggggcgggcggggcggccgacgtgtgtggggaggcgcgtagtgtttacgtatgcggaaggaggttttataccggaagatgggtaatttgggcgtatacttgtaagttttgtgtaatttggcgcgaaaactgggtaatgaggaagttgaggttaatatgtactttttatgactgggcggaatttctgctgttcagcagtgaactttgggcgctgacggggaggtttcgctacgtggcagtaccacgagaaggctcaaaggtcccatttattgtactcctcagcgttttcgccgggtatttaaacgctgtcagatcatcaagaggccactcttgagtgctggcgagtagagttttctcctccgcgctgccacaatgaggctggtccccgagatgtttggtgttttttgcgacgaggcggcgcggaactcagatgacctgctgaattcagatttgctggaaattcccaattcgcctgtggcttcgcctccgtcacttcacgaccttttcgatgtggaagtggatcctccggcagatcccaacgaggacgcggtaaatagtatgtttcccgaatgtctgttcgaggcggctgacgagggtagcgacagcggtggagagagtggacagggtgaggaactggacttaaaatgctacgaggaatgcataccgtctagcgattctgaaacggaacaaacagggggagatggctgcgctgagccaactgagaaaaatgaacttatattagactgtcctgaacatcctggtcatggctgccgtgcctgtgcttttcatagagatgccagtggaaatcctgaaactctatgtgctctgtgttacctgcgtcttaccggcaattttgtatacagtaagtaggttttttactttgtgtacggtagggaagtttttgtaaagtgtgttatgacttattgcttgtgtaatgttttacaggtgacgtgtctgatgtggaggagggagataagtcagtccatactagttctccttgcactttgggggctgtggttccagataatgttattaaacccgtggcggtcagagtatcaggcaggcggtgtgcagtcgaaaaaattgaagacttgctgcaggaagagcagatgcaacctttggacctgtccctcaaacgccctaagatgacctaagcctgtttattgagtgcaataaaactgttgatctttgaactgtgtttatgtgttgggtgtgtctgtggatatataagcaggtggatgggaagtgagagcacatctgccttgatggatctgttggggaacttgcgggaatttgacgtggttcgtcgcttgctggagttggcctccgacaaaacttccaggctttggaggttttggtttggctcaacgcttagcagcgtagtgtacagggtcaagaaggagcaggaggggcaattttctaggctgttggctgatattcctggagtttttgtggctctggatttaggccatcacagtctttttcaagagaaaattgtcaaaagcttaactttctcgtctcctggccgcacggttgtttcagcagcctttattacctatattttggatcaatggagcagcagcggcagccacctgtcgtgggattacatgctggattacctggcaatggccctgtggagggccatgctgcggaggagggtttgcatttactcgcgggcgcagcctccgcggctggatcgagtggtggaggaggacgagccggacgagaccgagaacctgagagccggcctggaccctccaatggaagactaggtgcagaggataatcctgaagagggaactagtgggggtgctagaaaaaagcaaaaaaccgagactgagcctagaaactttttgaatgagctgactgtgagtttgatgaatcgccatcgtcccgagacaattttctggtctgagttggaggaagagtttaggaagggggatttgaacctgctgtacaagtatgggttcgaacagttgaagactcactggttggagccgtgggaggattttgaaaccgctctggacacttttgctaaagtggctttgcggccggataaagtttatactatccgctgcactgttaatataaggaaaagtgtttatgttataggccatggagcactggtgcaggtggagaccgccgatcgggtggctttcaactgcggcatgcagaatctgggccctggggtgataggtgttaatggtgtcacgtttcagaacgtgaggttcgcgggtgaaagctttagcggctccgtgtttgcaaataacacacagctcactctccacggcgtttacttttttaactttaacaatacatgtgtggagtcgtggggcagggcgtccttgaggggctgcacttttcacggttgctggaaggcggtggtgggaagactgaaaagtgtaacgtctgtgaaaaaatgcatattcgagcggtgtgtgctagctgtaaccgtggaagggcatggacgcattagaaacaacgcagcgtctgagaatgggtgttttcttttactgaaaggcacggccagcgttaagcataacatgatctgtggcagtgggctgtacccgtcgcagttgttaacctgcgcggatggaaactgccagacattgcgcaccgtgcacatagtgtctcacccgcgtcgccactggccaacgtttgagcacaacttgcttatgcgttgtacggtccatctggggcctagacggggcatgtttgtgccttttcagtgtaactttagccacactaagatcttactagaagcagatgccttcactcgagtgtgtttcaatggggtgtttgacatgtcggtggaaatttttaaagtgataagatatgatgaatccaagtctcgttgtcgcccctgtgaatgcggagctaatcatttgaggttgtatcccgcgaccctgaacgtaaccgaggagctgagggccgaccaccacatgttgtcctgcttgcgcaccgactatgagtccagcgacgaagagtgaggtgaggggcggagccacaaagggtataaagggtcaggatgggtgggcacaggtattgtcgactggtcaatattggccattagccatattattcattggttatatagcataaatcaatattggctattggccattgcatacgttgtatccatatcataatatgtacatttatattggctcatgtccaacattaccgccatgttgacattgattattgactagttattaatagtaatcaattacggggtcattagttcatagcccatatatggagttccgcgttacataacttacggtaaatggcccgcctggctgaccgcccaacgacccccgcccattgacgtcaataatgacgtatgttcccatagtaacgccaatagggactttccattgacgtcaatgggtggagtatttacggtaaactgcccacttggcagtacatcaagtgtatcatatgccaagtacgccccctattgacgtcaatgacggtaaatggcccgcctggcattatgcccagtacatgaccttatgggactttcctacttggcagtacatctacgtattagtcatcgctattaccatggtgatgcggttttggcagtacatcaatgggcgtggatagcggtttgactcacggggatttccaagtctccaccccattgacgtcaatgggagtttgttttggcaccaaaatcaacgggactttccaaaatgtcgtaacaactccgccccattgacgcaaatgggcggtaggcgtgtacggtgggaggtctatataagcagagctcgtttagtgaaccgtcagatcgcctggagacgccatccacgctgttttgacctccatagaagacaccgggaccgatccagcctccgcggccgggaacggtgcattggaagcttggtaccggtgaattcgctagcgttaacggatcctctagacgagatccgaacttgtttattgcagcttataatggttacaaataaagcaatagcatcacaaatttcacaaataaagcatttttttcactgcattctagttgtggtttgtccaaactcatcaatgtatcttatcatgtctagatccttaaggtgataagatatgatgaatccaagtctcgttgtcgcccctgtgaatgcggagctaatcatttgaggttgtatcccgcgaccctgaacgtaaccgaggagctgagggccgaccaccacatgttgtcctgcttgcgcaccgactatgagtccagcgacgaagagtgaggtgaggggcggagccacaaagggtataaagggtcaggatgggtgggcacaggtattcaaaatgagcgggacgacggacggcaacgcgtttgaggggggagtgttcagcccatatctgacatctcgtcttccttcctgggcaggagtgcgtcagaatgtagtgggctccaccgtggacggacggccggtcgcccctgcgaattccgccacccttacctatgccaccgtgggatcaccgttggacactgccgcggcagccgcagcttctgctgccgcttctactgctcgcggtatggcggctgactttggactttataaccaactggctaccgcggctgtggcatctcgcactctggttcaagaagatgccctgagcgtggttctgcttcgactggaagatctgtctcgtcgcttggatcagctggctgcgcagatatccccacctaaccccgatactactcaagaatcttaaataaagacaaacagatttgttgaaaataaatggctttatttgttttttttggctcgataggctcgggtccacctgtcccggtcgttaaggactttgtgtatgctttccaagacccggtacagatgggcttggatgtttagatacatgggcatgaggccatcccgggggtggagataggaccattgcagagcgtcatgctccggggtggtgttgtagatgacccagtcgtagcagggtttttgggcgtggaactgaaaaatgtccttgagaagcaggctgatggccaggggcagacccttagtgtaggtgttcacaaagcggttgagctgggagggatgcatgcggggagagatgatatgcatcttagcctggattttcaggttagctatgttgccccccaggtcccttcgagggttcatattgtggaggaccaccagaacggtgtagccggtacacttgggaaacttatcgtgcagtttggaggggaaggcgtgaaagaatttggaaacccctttgtgaccacctaagttttccatgcactcgtccatgataatggcgatgggccccttggcggcagctttagcgaacacgttgtgggggttggaaacatcatagttttgctctagagttagctcgtcataggccatttttacgaagcggggtaggagggtgccagactgagggacgatagttccatctggccccggtgcgtaattaccctcgcagatctgcatctcccaagctttaatttccgagggagggatcatgtccacctggggggcgataaagaacacggtttctggcgggggattaatgagctgggtggaaagcaggttgcgcaagagctgagacttgccgcaaccggtgggaccgtagatgaccccgatgacgggctgcagctggtagttgagagaggagcagctgccgtcggggcgtaggaggggagccacctcgttcatcatgcttcttacatgtttattttcactgactaagctttgcaagagcctctccccacccagggacaagagttcttccaggctgttgaagtgtttcagcggtttcaggccgtcggccatgggcatcttttcaagcgactgacgaagcaagtacagccggtcccagagctcggtgacgtgctctatggaatctcgatccagcagacttcttggttgcgggggttgggccgactttcgctgtagggtacgagccggtgggcgtccagggccgcgagggttttgtccttccagggtctcagcgtccgggtgagggtggtctcggtgacggtgaacggatgagccccgggctgggcgcttgccagggtgcgcttcaggctcatccggctggtgctgaagcgggcgtcgtctccctgggaatcggccagatagcaacggagcatgaggtcgtagctaagggattcggccgcgtgtcccttggcgcgcagttttcccttggaaacatgctggcatctggtgcagtgtaaacacttgagggcgtacagcttgggggcgaggaagacggactcgggcgagtaggcgtcggccccgcactcggcgcagacggtttcacactccaccagccacgtgagctcgggtttgtcggggtcaaaaaccaggttgcctccattttttttgatgcgtttcttaccttgcgtctccatgagcctgtgacccgcttcggtgacaaaaaggctgtctgtgtctccgtagaccgacttgagggggcgttcttccaagggcgtgccgcggtcttctgcgtacaaaaactgggaccactccgaaacgaaggccctggtccacgctaacacgaaggatgcgatctgcgaggggtatctgtcgttctcaatgaggggatccaccttttccagggtatgcagacacaggtcgtcctcctccgcgtccacaaaggtgattggcttgtaagtgtaggtcacgtgacttaattaattcgaacccataatacccataatagctgtttgccatcgacgcgaggctggatggccttccccattatgattcttctcgcttccggcggcatcgggatgcccgcgttgcaggccatgctgtccaggcaggtagatgacgaccatcagggacagcttcaaggccagcaaaaggccaggaaccgtaaaaaggccgcgttgctggcgtttttccataggctccgcccccctgacgagcatcacaaaaatcgacgctcaagtcagaggtggcgaaacccgacaggactataaagataccaggcgtttccccctggaagctccctcgtgcgctctcctgttccgaccctgccgcttaccggatacctgtccgcctttctcccttcgggaagcgtggcgctttctcatagctcacgctgtaggtatctcagttcggtgtaggtcgttcgctccaagctgggctgtgtgcacgaaccccccgttcagcccgaccgctgcgccttatccggtaactatcgtcttgagtccaacccggtaagacacgacttatcgccactggcagcagccactggtaacaggattagcagagcgaggtatgtaggcggtgctacagagttcttgaagtggtggcctaactacggctacactagaaggacagtatttggtatctgcgctctgctgaagccagttaccttcggaaaaagagttggtagctcttgatccggcaaacaaaccaccgctggtagcggtggtttttttgtttgcaagcagcagattacgcgcagaaaaaaaggatctcaagaagatcctttgatcttttctacggggtctgacgctcagtggaacgaaaactcacgttaagggattttggtcatgagattatcaaaaaggatcttcacctagatccttttaaattaaaaatgaagttttaaatcaatctaaagtatatatgagtaaacttggtctgacagttaccaatgcttaatcagtgaggcacctatctcagcgatctgtctatttcgttcatccatagttgcctgactccccgtcgtgtagataactacgatacgggagggcttaccatctggccccagtgctgcaatgataccgcgagacccacgctcaccggctccagatttatcagcaataaaccagccagccggaagggccgagcgcagaagtggtcctgcaactttatccgcctccatccagtctattaattgttgccgggaagctagagtaagtagttcgccagttaatagtttgcgcaacgttgttgccattgctgcaggcatcgtggtgtcacgctcgtcgtttggtatggcttcattcagctccggttcccaacgatcaaggcgagttacatgatcccccatgttgtgcaaaaaagcggttagctccttcggtcctccgatcgttgtcagaagtaagttggccgcagtgttatcactcatggttatggcagcactgcataattctcttactgtcatgccatccgtaagatgcttttctgtgactggtgagtactcaaccaagtcattctgagaatagtgtatgcggcgaccgagttgctcttgcccggcgtcaacacgggataataccgcgccacatagcagaactttaaaagtgctcatcattggaaaacgttcttcggggcgaaaactctcaaggatcttaccgctgttgagatccagttcgatgtaacccactcgtgcacccaactgatcttcagcatcttttactttcaccagcgtttctgggtgagcaaaaacaggaaggcaaaatgccgcaaaaaagggaataagggcgacacggaaatgttgaatactcatactcttcctttttcaatattattgaagcatttatcagggttattgtctcatgagcggatacatatttgaatgtatttagaaaaataaacaaataggggttccgcgcacatttccccgaaaagtgccacctgacgtctaagaaaccattattatcatgacattaacctataaaaataggcgtatcacgaggccctttcgtcttcaagaattggtcgatggcaaacagctattatgggtattatgggttcgaattaat

SEQ ID NO: 52 - DNA, 40 bp, Artificial Sequence
  Synthetic oligonucleotide sAd4287.1A.fwd
tctcacttaattaacatcatcaataatataccttattctg

SEQ ID NO: 53 - DNA, 35 bp, Artificial Sequence
  Synthetic oligonucleotide sAd4287.1A.rev
ttatgagtcgacaggagaaaactctactcgccggc

SEQ ID NO: 54 - DNA, 36 bp, Artificial Sequence
  Synthetic oligonucleotide sAd4287.1B.fwd
tatactcttaaggaatgcggagctaatcatttgagg

SEQ ID NO: 55 - DNA, 36 bp, Artificial Sequence
  Synthetic oligonucleotide sAd4287.1B.rev
tctcacttaattaacttcgtggacgcggaggaggac

SEQ ID NO: 56 - DNA, 36 bp, Artificial Sequence
  Synthetic oligonucleotide sAd4287.TGC.fwd
ttatgagtcgactggtcaatattggccattagccat

SEQ ID NO: 57 - DNA, 37 bp, Artificial Sequence
  Synthetic oligonucleotide sAd4287.TGC.rev
tatactcttaaggatctagacatgataagatacattg

SEQ ID NO: 58 - DNA, 36 bp, Artificial Sequence
  Synthetic oligonucleotide sAd4287.2A.rev
tctcaccctgcaggcaggagatcctcaggcaggccg

SEQ ID NO: 59 - DNA, 37 bp, Artificial Sequence
  Synthetic oligonucleotide sAd4287.2A.fwd
tctcaccctgcaggcgactacctgaacgaccccttgc

SEQ ID NO: 60 - DNA, 35 bp, Artificial Sequence
  Synthetic oligonucleotide sAd4287.2B.fwd
tctcacattaatcgactacctgaacgaccccttgc

SEQ ID NO: 61 - DNA, 37 bp, Artificial Sequence
  Synthetic oligonucleotide sAd4287.2B.rev
tctcacttaattaactgactggtgccgatgtcgttcc

SEQ ID NO: 62 - DNA, 37 bp, Artificial Sequence
  Synthetic oligonucleotide sAd4287.3A.fwd
tctcacttaattaacccaggacctggaaatagtgcct

SEQ ID NO: 63 - DNA, 37 bp, Artificial Sequence
  Synthetic oligonucleotide sAd4287.3A.rev
tctcaccctgcaggggtgggctgtattgcttgtccgc

SEQ ID NO: 64 - DNA, 38 bp, Artificial Sequence
  Synthetic oligonucleotide sAd4287.3B.fwd
tctcaccctgcaggggttgcaggaaaaaccacttggag

SEQ ID NO: 65 - DNA, 40 bp, Artificial Sequence; identical to SEQ ID NO: 52
  Synthetic oligonucleotide sAd4287.3B.rev

SEQ ID NO: 66 - DNA, 23 bp, Artificial Sequence
  Synthetic oligonucleotide sAd4287.dE3A.fwd
gagctagacaaactcctctgccg

SEQ ID NO: 67 - DNA, 36 bp, Artificial Sequence
  Synthetic oligonucleotide sAd4287.dE3A.rev
ttcctaactagtgtagaatttccacacgcaaaggag

SEQ ID NO: 68 - DNA, 35 bp, Artificial Sequence
  Synthetic oligonucleotide sAd4287.dE3B.fwd
ttcctaactagtgggagctatcctgtgtcactgtc

SEQ ID NO: 69 - DNA, 24 bp, Artificial Sequence
  Synthetic oligonucleotide sAd4287.dE3B.rev
cagcagttgatgttaattgtccct

SEQ ID NO: 70 - DNA, 24 bp, Artificial Sequence
  Synthetic oligonucleotide sAd4287.E1.fwd
cgctgtcagatcatcaagaggcca

SEQ ID NO: 71 - DNA, 54 bp, Artificial Sequence
  Synthetic oligonucleotide sAd4287.E1.rev
atggctaatggccaatattgaccagtcgaccgtccacccttcatgcccctttat

SEQ ID NO: 72 - DNA, 55 bp, Artificial Sequence
  Synthetic oligonucleotide sAd4287.dE4A.fwd
ctcacgttgaaaataggaaacggcctcactctagacaaccagggacaattaacat

SEQ ID NO: 73 - DNA, 38 bp, Artificial Sequence
  Synthetic oligonucleotide sAd4287.dE4A.rev
cggtaagacggggcagtaccaggaggtgcgtcggtctc

SEQ ID NO: 74 - DNA, 38 bp, Artificial Sequence
  Synthetic oligonucleotide sAd4287.dE4B.fwd
cgcacctcctggtactgccccgtcttaccgcgtaaaca

SEQ ID NO: 75 - DNA, 53 bp, Artificial Sequence
  Synthetic oligonucleotide sAd4287.dE4B.rev
tgccgatgtcgttccaggtgcccatgagcggccgcgagccgtgccgcggagcc

SEQ ID NO: 76 - DNA, 40 bp, Artificial Sequence; identical to SEQ ID NO: 52
  Synthetic oligonucleotide sAd4310A.1A.fwd

SEQ ID NO: 77 - DNA, 35 bp, Artificial Sequence
  Synthetic oligonucleotide sAd4310A.1A.rev
ttatgagtcgacgaggagaaaactctactcgccgg

SEQ ID NO: 78 - DNA, 37 bp, Artificial Sequence
  Synthetic oligonucleotide sAd4310A.1B.fwd
tatactcttaaggacatgtcaatggaactgtttaaag

SEQ ID NO: 79 - DNA, 38 bp, Artificial Sequence
  Synthetic oligonucleotide sAd4310A.1B.rev
tctcacttaattaacctcattgaaaacgacagataccc

SEQ ID NO: 80 - DNA, 36 bp, Artificial Sequence; identical to SEQ ID NO: 56
  Synthetic oligonucleotide sAd4310A.TGC.fwd

SEQ ID NO: 81 - DNA, 37 bp, Artificial Sequence; identical to SEQ ID NO: 57
  Synthetic oligonucleotide sAd4310A.TGC.rev

SEQ ID NO: 82 - DNA, 39 bp, Artificial Sequence
  Synthetic oligonucleotide sAd4310A.2A.fwd
tctcacttaattaagacatgtcaatggaactgtttaaag

SEQ ID NO: 83 - DNA, 38 bp, Artificial Sequence
  Synthetic oligonucleotide sAd4310A.2A.rev
tctcaccctgcaggcaaactctcctggccttggatcta

SEQ ID NO: 84 - DNA, 37 bp, Artificial Sequence
  Synthetic oligonucleotide sAd4310A.2B.fwd
tctcaccctgcagggtgactcgtacctgggtcatctc

SEQ ID NO: 85 - DNA, 38 bp, Artificial Sequence
  Synthetic oligonucleotide sAd4310A.2B.rev
tctcacttaattaagatgctgttcagcgtgttttgcca

SEQ ID NO: 86 - DNA, 37 bp, Artificial Sequence
  Synthetic oligonucleotide sAd4310A.3A.fwd
tctcacttaattaacaccgtggattccgtgatcgaca

SEQ ID NO: 87 - DNA, 38 bp, Artificial Sequence
  Synthetic oligonucleotide sAd4310A.3A.rev
tctcaccctgcagggttaatgctgtcgaatctgacgct

SEQ ID NO: 88 - DNA, 38 bp, Artificial Sequence
  Synthetic oligonucleotide sAd4310A.3B.fwd
tctcaccctgcagggaagacttcaacccagtgtaccct

SEQ ID NO: 89 - DNA, 40 bp, Artificial Sequence; identical to SEQ ID NO: 52
  Synthetic oligonucleotide sAd4310A.3B.rev

SEQ ID NO: 90 - DNA, 23 bp, Artificial Sequence
  Synthetic oligonucleotide sAd4310A.dE3A.fwd.G
gttgcatgatagggtaactcgcc

SEQ ID NO: 91 - DNA, 47 bp, Artificial Sequence
  Synthetic oligonucleotide sAd4310A.dE3A.rev.G
agagaggatagccccctctacaggataagttcgttagtgcaggcgca

SEQ ID NO: 92 - DNA, 47 bp, Artificial Sequence
  Synthetic oligonucleotide sAd4310A.dE3B.fwd.G
tgcgcctgcactaacgaacttatcctgtagagggggctatcctctgt

SEQ ID NO: 93 - DNA, 23 bp, Artificial Sequence
  Synthetic oligonucleotide sAd4310A.dE3B.rev.G
gttctacttccccagcggttgat

SEQ ID NO: 94 - DNA, 24 bp, Artificial Sequence
  Synthetic oligonucleotide sAd4310A.E1.fwd
cgtatgcggaaggaggttttatac

SEQ ID NO: 95 - DNA, 54 bp, Artificial Sequence
  Synthetic oligonucleotide sAd4310A.E1.rev
atggctaatggccaatattgaccagtcgacctcacgcccctttatacccgtttg

SEQ ID NO: 96 - DNA, 53 bp, Artificial Sequence
  Synthetic oligonucleotide sAd4310A.dE4A.fwd
ttacagttaaactaggaaacggcctcactctagacaaccagggacaactaaca

SEQ ID NO: 97 - DNA, 43 bp, Artificial Sequence
  Synthetic oligonucleotide sAd4310A.dE4A.rev
gcggtaagacggggcagttctgctactacaagtacgaggaagt

SEQ ID NO: 98 - DNA, 39 bp, Artificial Sequence
  Synthetic oligonucleotide sAd4310A.dE4B.fwd
ttgtagtagcagaactgccccgtcttaccgcgtataaag

SEQ ID NO: 99 - DNA, 51 bp, Artificial Sequence
  Synthetic oligonucleotide sAd4310A.dE4B.rev
gtgccgatgtcgttccaggtgcccatgagcggccgcgagccttgccgcgga

SEQ ID NO: 100 - DNA, 40 bp, Artificial Sequence; identical to SEQ ID NO: 52
  Synthetic oligonucleotide sAd4312.1A.fwd

SEQ ID NO: 101 - DNA, 35 bp, Artificial Sequence
  Synthetic oligonucleotide sAd4312.1A.rev
ttatgagtcgaccggaggagaaaactctactcgcc

SEQ ID NO: 102 - DNA, 38 bp, Artificial Sequence
  Synthetic oligonucleotide sAd4312.1B.fwd
tatactcttaaggtgataagatatgatgaatccaagtc

SEQ ID NO: 103 - DNA, 38 bp, Artificial Sequence
  Synthetic oligonucleotide sAd4312.1B.rev
tctcacttaattaagtcacgtgacctacacttacaagc

SEQ ID NO: 104 - DNA, 36 bp, Artificial Sequence; identical to SEQ ID NO: 56
  Synthetic oligonucleotide sAd4312.TGC.fwd

SEQ ID NO: 105 - DNA, 37 bp, Artificial Sequence; identical to SEQ ID NO: 57
  Synthetic oligonucleotide sAd4312.TGC.rev

SEQ ID NO: 106 - DNA, 40 bp, Artificial Sequence
  Synthetic oligonucleotide sAd4312.2A.fwd
tctcacttaattaagtgataagatatgatgaatccaagtc

SEQ ID NO: 107 - DNA, 35 bp, Artificial Sequence
  Synthetic oligonucleotide sAd4312.2A.rev
tctcaccatatgcttctctcagaaaggccgctcag

SEQ ID NO: 108 - DNA, 36 bp, Artificial Sequence
  Synthetic oligonucleotide sAd4312.2B.fwd
tctcaccatatgcaagcggcaatatgacgaggtgta

SEQ ID NO: 109 - DNA, 36 bp, Artificial Sequence
  Synthetic oligonucleotide sAd4312.2B.rev
tctcacttaattaagtgtcagcctctgcgagcggtc

SEQ ID NO: 110 - DNA, 38 bp, Artificial Sequence
  Synthetic oligonucleotide sAd4312.3A.fwd
tctcacttaattaaccgaagttagaagaccaaaggtgc

SEQ ID NO: 111 - DNA, 36 bp, Artificial Sequence
  Synthetic oligonucleotide sAd4312.3A.rev
tctcaccctgcagggtgtcagcctctgcgagcggtc

SEQ ID NO: 112 - DNA, 38 bp, Artificial Sequence
  Synthetic oligonucleotide sAd4312.3B.fwd
tctcaccctgcaggccagaccagatactttatggacca

SEQ ID NO: 113 - DNA, 40 bp, Artificial Sequence; identical to SEQ ID NO: 52
  Synthetic oligonucleotide sAd4312.3B.rev

SEQ ID NO: 114 - DNA, 24 bp, Artificial Sequence
  Synthetic oligonucleotide sAd4312.dE3A.fwd
ggaagacagaaacctcaaagagct

SEQ ID NO: 115 - DNA, 37 bp, Artificial Sequence
  Synthetic oligonucleotide sAd4312.dE3A.rev
ttcctaactagtgtgcaagaacagttaaggataagag

SEQ ID NO: 116 - DNA, 35 bp, Artificial Sequence
  Synthetic oligonucleotide sAd4312.dE3B.fwd
ttcctaactagtgagggggctatcctgtgtcactg

SEQ ID NO: 117 - DNA, 24 bp, Artificial Sequence
  Synthetic oligonucleotide sAd4312.dE3B.rev
ccacatttaacaagcgctagccac

SEQ ID NO: 118 - DNA, 24 bp, Artificial Sequence
  Synthetic oligonucleotide sAd4312.E1.fwd
gaaggaggttttataccggaagat

SEQ ID NO: 119 - DNA, 53 bp, Artificial Sequence
  Synthetic oligonucleotide sAd4312.E1.rev
atggctaatggccaatattgaccagtcgacaatacctgtgcccacccatcctg

SEQ ID NO: 120 - DNA, 53 bp, Artificial Sequence
  Synthetic oligonucleotide sAd4312.dE4A.fwd
agcaccactttaccctcttcccaactctcatatgggatatgatggtgggcggc

SEQ ID NO: 121 - DNA, 40 bp, Artificial Sequence
  Synthetic oligonucleotide sAd4312.dE4A.rev
gcggtaagacggggcgggttctgctattggaagtacgagg

SEQ ID NO: 122 - DNA, 38 bp, Artificial Sequence
  Synthetic oligonucleotide sAd4312.dE4B.fwd
tccaatagcagaacccgccccgtcttaccgcgtaaaaa

SEQ ID NO: 123 - DNA, 50 bp, Artificial Sequence
  Synthetic oligonucleotide sAd4312.dE4B.rev
ctttcatgcgcctgcgtaaagcccgacggcggccgctccccgccatgcct